European Patent Application EP 4 450 617 A1, published October 23, 2024. Title: Mutated Hydroxyphenylpyruvate Dioxygenase Polypeptide, and Coding Gene and Use thereof. Applicant: BEIJING DABEINONG BIOTECHNOLOGY CO., LTD. The sequence listing filed with the application follows.

SEQUENCE LISTING (234 sequences)

SEQ ID NO: 1 - protein, 440 aa, Avena sativa
  The amino acid sequence of Avena sativa wild-type HPPD (AsHPPD)
MPPTPATATGAAAAAVTPEHAARSFPRVVRVNPRSDRFPVLSFHHVELWCADAASAAGRFSFALGAPLAARSDLSTGNSAHASLLLRSGALAFLFTAPYAPPPQEAATAAATASIPSFSADAARTFAAAHGLAVRSVGVRVADAAEAFRVSVAGGARPAFAPADLGHGFGLAEVELYGDVVLRFVSYPDETDLPFLPGFERVSSPGAVDYGLTRFDHVVGNVPEMAPVIDYMKGFLGFHEFAEFTAEDVGTTESGLNSVVLANNSEAVLLPLNEPVHGTKRRSQIQTYLEYHGGPGVQHIALASNDVLRTLREMRARTPMGGFEFMAPPQAKYYEGVRRIAGDVLSEEQIKECQELGVLVDRDDQGVLLQIFTKPVGDRPTFFLEMIQRIGCMEKDEVGQEYQKGGCGGFGKGNFSELFKSIEDYEKSLEVKQSVVAQKS

SEQ ID NO: 2 - DNA, 1323 bp, Avena sativa
  AsHPPD-01 Nucleotide Sequence
atgccgcccacccccgccaccgccaccggcgccgccgcggccgccgtgactccagagcacgcggcccggagctttccccgagtggtccgcgtcaacccgcgcagcgaccgcttccccgtgctctccttccaccacgtcgagctctggtgcgccgacgccgcctcagcggccggacgcttctccttcgcgctcggcgcgccgctcgccgcccggtccgacctctccacggggaactccgcgcacgcctccctcctgctccgctcgggcgccctcgccttcctcttcacggcgccctacgcgccgccgccgcaggaggccgccacggccgcagccaccgcctccatcccctccttctccgccgacgccgcgcggacgttcgccgccgcccacggcctcgcggtgcgctccgtcggggtccgcgtcgctgacgccgccgaggccttccgcgtcagcgtagccggcggcgctcgcccggccttcgccccagccgacctcggccatggcttcggcctcgccgaggtcgagctctacggcgacgtcgtgctacgcttcgtcagctacccggacgagacagacctgccattcctgccagggttcgagcgcgtgagcagccccggcgccgtggactacggcctcacgcggttcgaccacgtcgtgggcaacgtcccggagatggccccggtcatagactacatgaaaggcttcttggggttccacgagttcgccgagttcaccgccgaggacgtgggcacgaccgagagcgggctcaactcggtggtgctcgccaacaactccgaggccgtgctgctgccgctcaacgagcccgtgcacggcacaaagcgacggagccagatacagacgtacctggagtatcacggcgggcccggcgtgcagcacatcgcgctcgccagcaacgacgtgctcaggacgctcagggagatgcgggcgcgcacgcccatgggcggcttcgagttcatggcgccaccgcaggcgaaatactatgaaggcgtgcggcgcatcgcaggtgacgtgctctcggaagagcagatcaaggaatgccaggagctgggggtgctagtcgacagggatgatcaaggggtgttgctccaaatcttcaccaagccagtaggggacaggccaacgtttttcctggagatgatccaaagaatcgggtgcatggagaaggacgaggtcgggcaagagtaccagaagggtggctgcggcgggtttggcaagggcaatttctccgagctgttcaagtccattgaggactatgagaaatcccttgaggtcaagcaatctgttgtagctcagaaatcctag

SEQ ID NO: 3 - DNA, 1323 bp, Artificial Sequence
  AsHPPD-02 Nucleotide Sequence
atgccacctactccagctacagctactggtgctgctgctgctgccgttactcctgagcacgctgccaggtcattccccagggtggttcgcgtgaaccccagatctgataggttcccagttctgagcttccaccatgttgagctgtggtgcgctgatgctgcttctgctgctggcaggttctctttcgctcttggtgctccactcgctgctagatctgatctgtctacaggaaatagcgctcatgcctcactcctgcttcgctcaggtgctttggccttcctcttcaccgctccatatgctcccccacctcaggaggctgctactgctgctgctacagcctccattccaagcttctcagctgatgccgctagaaccttcgctgctgctcatggacttgccgtgaggtctgttggtgttcgcgtggctgatgctgctgaggctttcagagtttccgttgccggcggagctaggccagctttcgctcctgctgatttgggacatggtttcggcctggctgaggttgagctttacggtgacgtggttctccgcttcgtgtcttacccagatgagactgacctgcctttccttcccggcttcgagagagtttcctctcctggtgccgtggattacggcctgacaaggttcgaccacgtggttggaaacgttcccgagatggctccagtgatcgattacatgaagggcttccttggattccatgagttcgccgagttcactgctgaggacgtgggaaccactgagtccggtttgaactctgtggttctcgccaacaattctgaggctgttttgctccctctgaatgagcctgtgcatggaaccaagaggagaagccagattcaaacttacctggagtaccacggtggccctggagttcagcatatcgcccttgcttctaatgatgtgttgcgcacactcagagagatgcgcgccagaacccccatgggaggtttcgagttcatggccccaccacaggctaagtactacgagggcgttagaaggattgctggagacgtgttgagcgaggagcagatcaaggagtgccaagagctgggtgttcttgtggatagggatgaccagggcgttctgcttcaaattttcactaagccagtgggcgaccgccctacattcttccttgagatgattcaaagaatcggctgcatggagaaggatgaggttggacaggagtaccaaaagggcggatgcggtggcttcggaaagggtaacttcagcgagttgttcaagtcaatcgaggactacgagaagagcctcgaggtgaagcagtcagtggttgcccaaaagtcctga

SEQ ID NO: 4 - protein, 440 aa, Artificial Sequence
  AsHPPDm-F372A Amino Acid Sequence
MPPTPATATGAAAAAVTPEHAARSFPRVVRVNPRSDRFPVLSFHHVELWCADAASAAGRFSFALGAPLAARSDLSTGNSAHASLLLRSGALAFLFTAPYAPPPQEAATAAATASIPSFSADAARTFAAAHGLAVRSVGVRVADAAEAFRVSVAGGARPAFAPADLGHGFGLAEVELYGDVVLRFVSYPDETDLPFLPGFERVSSPGAVDYGLTRFDHVVGNVPEMAPVIDYMKGFLGFHEFAEFTAEDVGTTESGLNSVVLANNSEAVLLPLNEPVHGTKRRSQIQTYLEYHGGPGVQHIALASNDVLRTLREMRARTPMGGFEFMAPPQAKYYEGVRRIAGDVLSEEQIKECQELGVLVDRDDQGVLLQIATKPVGDRPTFFLEMIQRIGCMEKDEVGQEYQKGGCGGFGKGNFSELFKSIEDYEKSLEVKQSVVAQKS

SEQ ID NO: 5 - DNA, 1323 bp, Artificial Sequence
  AsHPPDm-F372A-01 Nucleotide Sequence
atgccgcccacccccgccaccgccaccggcgccgccgcggccgccgtgactccagagcacgcggcccggagctttccccgagtggtccgcgtcaacccgcgcagcgaccgcttccccgtgctctccttccaccacgtcgagctctggtgcgccgacgccgcctcagcggccggacgcttctccttcgcgctcggcgcgccgctcgccgcccggtccgacctctccacggggaactccgcgcacgcctccctcctgctccgctcgggcgccctcgccttcctcttcacggcgccctacgcgccgccgccgcaggaggccgccacggccgcagccaccgcctccatcccctccttctccgccgacgccgcgcggacgttcgccgccgcccacggcctcgcggtgcgctccgtcggggtccgcgtcgctgacgccgccgaggccttccgcgtcagcgtagccggcggcgctcgcccggccttcgccccagccgacctcggccatggcttcggcctcgccgaggtcgagctctacggcgacgtcgtgctacgcttcgtcagctacccggacgagacagacctgccattcctgccagggttcgagcgcgtgagcagccccggcgccgtggactacggcctcacgcggttcgaccacgtcgtgggcaacgtcccggagatggccccggtcatagactacatgaaaggcttcttggggttccacgagttcgccgagttcaccgccgaggacgtgggcacgaccgagagcgggctcaactcggtggtgctcgccaacaactccgaggccgtgctgctgccgctcaacgagcccgtgcacggcacaaagcgacggagccagatacagacgtacctggagtatcacggcgggcccggcgtgcagcacatcgcgctcgccagcaacgacgtgctcaggacgctcagggagatgcgggcgcgcacgcccatgggcggcttcgagttcatggcgccaccgcaggcgaaatactatgaaggcgtgcggcgcatcgcaggtgacgtgctctcggaagagcagatcaaggaatgccaggagctgggggtgctagtcgacagggatgatcaaggggtgttgctccaaatcgctaccaagccagtaggggacaggccaacgtttttcctggagatgatccaaagaatcgggtgcatggagaaggacgaggtcgggcaagagtaccagaagggtggctgcggcgggtttggcaagggcaatttctccgagctgttcaagtccattgaggactatgagaaatcccttgaggtcaagcaatctgttgtagctcagaaatcctag

SEQ ID NO: 6 - DNA, 1323 bp, Artificial Sequence
  AsHPPDm-F372A-02 Nucleotide Sequence
atgccacctactccagctacagctactggtgctgctgctgctgccgttactcctgagcacgctgccaggtcattccccagggtggttcgcgtgaaccccagatctgataggttcccagttctgagcttccaccatgttgagctgtggtgcgctgatgctgcttctgctgctggcaggttctctttcgctcttggtgctccactcgctgctagatctgatctgtctacaggaaatagcgctcatgcctcactcctgcttcgctcaggtgctttggccttcctcttcaccgctccatatgctcccccacctcaggaggctgctactgctgctgctacagcctccattccaagcttctcagctgatgccgctagaaccttcgctgctgctcatggacttgccgtgaggtctgttggtgttcgcgtggctgatgctgctgaggctttcagagtttccgttgccggcggagctaggccagctttcgctcctgctgatttgggacatggtttcggcctggctgaggttgagctttacggtgacgtggttctccgcttcgtgtcttacccagatgagactgacctgcctttccttcccggcttcgagagagtttcctctcctggtgccgtggattacggcctgacaaggttcgaccacgtggttggaaacgttcccgagatggctccagtgatcgattacatgaagggcttccttggattccatgagttcgccgagttcactgctgaggacgtgggaaccactgagtccggtttgaactctgtggttctcgccaacaattctgaggctgttttgctccctctgaatgagcctgtgcatggaaccaagaggagaagccagattcaaacttacctggagtaccacggtggccctggagttcagcatatcgcccttgcttctaatgatgtgttgcgcacactcagagagatgcgcgccagaacccccatgggaggtttcgagttcatggccccaccacaggctaagtactacgagggcgttagaaggattgctggagacgtgttgagcgaggagcagatcaaggagtgccaagagctgggtgttcttgtggatagggatgaccagggcgttctgcttcaaattgccactaagccagtgggcgaccgccctacattcttccttgagatgattcaaagaatcggctgcatggagaaggatgaggttggacaggagtaccaaaagggcggatgcggtggcttcggaaagggtaacttcagcgagttgttcaagtcaatcgaggactacgagaagagcctcgaggtgaagcagtcagtggttgcccaaaagtcctga

SEQ ID NO: 7 - protein, 440 aa, Artificial Sequence
  AsHPPDm-F383W Amino Acid Sequence
MPPTPATATGAAAAAVTPEHAARSFPRVVRVNPRSDRFPVLSFHHVELWCADAASAAGRFSFALGAPLAARSDLSTGNSAHASLLLRSGALAFLFTAPYAPPPQEAATAAATASIPSFSADAARTFAAAHGLAVRSVGVRVADAAEAFRVSVAGGARPAFAPADLGHGFGLAEVELYGDVVLRFVSYPDETDLPFLPGFERVSSPGAVDYGLTRFDHVVGNVPEMAPVIDYMKGFLGFHEFAEFTAEDVGTTESGLNSVVLANNSEAVLLPLNEPVHGTKRRSQIQTYLEYHGGPGVQHIALASNDVLRTLREMRARTPMGGFEFMAPPQAKYYEGVRRIAGDVLSEEQIKECQELGVLVDRDDQGVLLQIFTKPVGDRPTFWLEMIQRIGCMEKDEVGQEYQKGGCGGFGKGNFSELFKSIEDYEKSLEVKQSVVAQKS

SEQ ID NO: 8 - DNA, 1323 bp, Artificial Sequence
  AsHPPDm-F383W-01 Nucleotide Sequence
atgccgcccacccccgccaccgccaccggcgccgccgcggccgccgtgactccagagcacgcggcccggagctttccccgagtggtccgcgtcaacccgcgcagcgaccgcttccccgtgctctccttccaccacgtcgagctctggtgcgccgacgccgcctcagcggccggacgcttctccttcgcgctcggcgcgccgctcgccgcccggtccgacctctccacggggaactccgcgcacgcctccctcctgctccgctcgggcgccctcgccttcctcttcacggcgccctacgcgccgccgccgcaggaggccgccacggccgcagccaccgcctccatcccctccttctccgccgacgccgcgcggacgttcgccgccgcccacggcctcgcggtgcgctccgtcggggtccgcgtcgctgacgccgccgaggccttccgcgtcagcgtagccggcggcgctcgcccggccttcgccccagccgacctcggccatggcttcggcctcgccgaggtcgagctctacggcgacgtcgtgctacgcttcgtcagctacccggacgagacagacctgccattcctgccagggttcgagcgcgtgagcagccccggcgccgtggactacggcctcacgcggttcgaccacgtcgtgggcaacgtcccggagatggccccggtcatagactacatgaaaggcttcttggggttccacgagttcgccgagttcaccgccgaggacgtgggcacgaccgagagcgggctcaactcggtggtgctcgccaacaactccgaggccgtgctgctgccgctcaacgagcccgtgcacggcacaaagcgacggagccagatacagacgtacctggagtatcacggcgggcccggcgtgcagcacatcgcgctcgccagcaacgacgtgctcaggacgctcagggagatgcgggcgcgcacgcccatgggcggcttcgagttcatggcgccaccgcaggcgaaatactatgaaggcgtgcggcgcatcgcaggtgacgtgctctcggaagagcagatcaaggaatgccaggagctgggggtgctagtcgacagggatgatcaaggggtgttgctccaaatcttcaccaagccagtaggggacaggccaacgttttggctggagatgatccaaagaatcgggtgcatggagaaggacgaggtcgggcaagagtaccagaagggtggctgcggcgggtttggcaagggcaatttctccgagctgttcaagtccattgaggactatgagaaatcccttgaggtcaagcaatctgttgtagctcagaaatcctag

SEQ ID NO: 9 - DNA, 1323 bp, Artificial Sequence
  AsHPPDm-F383W-02 Nucleotide Sequence
atgccacctactccagctacagctactggtgctgctgctgctgccgttactcctgagcacgctgccaggtcattccccagggtggttcgcgtgaaccccagatctgataggttcccagttctgagcttccaccatgttgagctgtggtgcgctgatgctgcttctgctgctggcaggttctctttcgctcttggtgctccactcgctgctagatctgatctgtctacaggaaatagcgctcatgcctcactcctgcttcgctcaggtgctttggccttcctcttcaccgctccatatgctcccccacctcaggaggctgctactgctgctgctacagcctccattccaagcttctcagctgatgccgctagaaccttcgctgctgctcatggacttgccgtgaggtctgttggtgttcgcgtggctgatgctgctgaggctttcagagtttccgttgccggcggagctaggccagctttcgctcctgctgatttgggacatggtttcggcctggctgaggttgagctttacggtgacgtggttctccgcttcgtgtcttacccagatgagactgacctgcctttccttcccggcttcgagagagtttcctctcctggtgccgtggattacggcctgacaaggttcgaccacgtggttggaaacgttcccgagatggctccagtgatcgattacatgaagggcttccttggattccatgagttcgccgagttcactgctgaggacgtgggaaccactgagtccggtttgaactctgtggttctcgccaacaattctgaggctgttttgctccctctgaatgagcctgtgcatggaaccaagaggagaagccagattcaaacttacctggagtaccacggtggccctggagttcagcatatcgcccttgcttctaatgatgtgttgcgcacactcagagagatgcgcgccagaacccccatgggaggtttcgagttcatggccccaccacaggctaagtactacgagggcgttagaaggattgctggagacgtgttgagcgaggagcagatcaaggagtgccaagagctgggtgttcttgtggatagggatgaccagggcgttctgcttcaaattttcactaagccagtgggcgaccgccctacattctggcttgagatgattcaaagaatcggctgcatggagaaggatgaggttggacaggagtaccaaaagggcggatgcggtggcttcggaaagggtaacttcagcgagttgttcaagtcaatcgaggactacgagaagagcctcgaggtgaagcagtcagtggttgcccaaaagtcctga

SEQ ID NO: 10 - protein, 440 aa, Artificial Sequence
  AsHPPDm-F372A-F383W Amino Acid Sequence
MPPTPATATGAAAAAVTPEHAARSFPRVVRVNPRSDRFPVLSFHHVELWCADAASAAGRFSFALGAPLAARSDLSTGNSAHASLLLRSGALAFLFTAPYAPPPQEAATAAATASIPSFSADAARTFAAAHGLAVRSVGVRVADAAEAFRVSVAGGARPAFAPADLGHGFGLAEVELYGDVVLRFVSYPDETDLPFLPGFERVSSPGAVDYGLTRFDHVVGNVPEMAPVIDYMKGFLGFHEFAEFTAEDVGTTESGLNSVVLANNSEAVLLPLNEPVHGTKRRSQIQTYLEYHGGPGVQHIALASNDVLRTLREMRARTPMGGFEFMAPPQAKYYEGVRRIAGDVLSEEQIKECQELGVLVDRDDQGVLLQIATKPVGDRPTFWLEMIQRIGCMEKDEVGQEYQKGGCGGFGKGNFSELFKSIEDYEKSLEVKQSVVAQKS

SEQ ID NO: 11 - DNA, 1323 bp, Artificial Sequence
  AsHPPDm-F372A-F383W-01 Nucleotide Sequence
atgccgcccacccccgccaccgccaccggcgccgccgcggccgccgtgactccagagcacgcggcccggagctttccccgagtggtccgcgtcaacccgcgcagcgaccgcttccccgtgctctccttccaccacgtcgagctctggtgcgccgacgccgcctcagcggccggacgcttctccttcgcgctcggcgcgccgctcgccgcccggtccgacctctccacggggaactccgcgcacgcctccctcctgctccgctcgggcgccctcgccttcctcttcacggcgccctacgcgccgccgccgcaggaggccgccacggccgcagccaccgcctccatcccctccttctccgccgacgccgcgcggacgttcgccgccgcccacggcctcgcggtgcgctccgtcggggtccgcgtcgctgacgccgccgaggccttccgcgtcagcgtagccggcggcgctcgcccggccttcgccccagccgacctcggccatggcttcggcctcgccgaggtcgagctctacggcgacgtcgtgctacgcttcgtcagctacccggacgagacagacctgccattcctgccagggttcgagcgcgtgagcagccccggcgccgtggactacggcctcacgcggttcgaccacgtcgtgggcaacgtcccggagatggccccggtcatagactacatgaaaggcttcttggggttccacgagttcgccgagttcaccgccgaggacgtgggcacgaccgagagcgggctcaactcggtggtgctcgccaacaactccgaggccgtgctgctgccgctcaacgagcccgtgcacggcacaaagcgacggagccagatacagacgtacctggagtatcacggcgggcccggcgtgcagcacatcgcgctcgccagcaacgacgtgctcaggacgctcagggagatgcgggcgcgcacgcccatgggcggcttcgagttcatggcgccaccgcaggcgaaatactatgaaggcgtgcggcgcatcgcaggtgacgtgctctcggaagagcagatcaaggaatgccaggagctgggggtgctagtcgacagggatgatcaaggggtgttgctccaaatcgctaccaagccagtaggggacaggccaacgttttggctggagatgatccaaagaatcgggtgcatggagaaggacgaggtcgggcaagagtaccagaagggtggctgcggcgggtttggcaagggcaatttctccgagctgttcaagtccattgaggactatgagaaatcccttgaggtcaagcaatctgttgtagctcagaaatcctag

SEQ ID NO: 12 - DNA, 1323 bp, Artificial Sequence
  AsHPPDm-F372A-F383W-02 Nucleotide Sequence
atgccacctactccagctacagctactggtgctgctgctgctgccgttactcctgagcacgctgccaggtcattccccagggtggttcgcgtgaaccccagatctgataggttcccagttctgagcttccaccatgttgagctgtggtgcgctgatgctgcttctgctgctggcaggttctctttcgctcttggtgctccactcgctgctagatctgatctgtctacaggaaatagcgctcatgcctcactcctgcttcgctcaggtgctttggccttcctcttcaccgctccatatgctcccccacctcaggaggctgctactgctgctgctacagcctccattccaagcttctcagctgatgccgctagaaccttcgctgctgctcatggacttgccgtgaggtctgttggtgttcgcgtggctgatgctgctgaggctttcagagtttccgttgccggcggagctaggccagctttcgctcctgctgatttgggacatggtttcggcctggctgaggttgagctttacggtgacgtggttctccgcttcgtgtcttacccagatgagactgacctgcctttccttcccggcttcgagagagtttcctctcctggtgccgtggattacggcctgacaaggttcgaccacgtggttggaaacgttcccgagatggctccagtgatcgattacatgaagggcttccttggattccatgagttcgccgagttcactgctgaggacgtgggaaccactgagtccggtttgaactctgtggttctcgccaacaattctgaggctgttttgctccctctgaatgagcctgtgcatggaaccaagaggagaagccagattcaaacttacctggagtaccacggtggccctggagttcagcatatcgcccttgcttctaatgatgtgttgcgcacactcagagagatgcgcgccagaacccccatgggaggtttcgagttcatggccccaccacaggctaagtactacgagggcgttagaaggattgctggagacgtgttgagcgaggagcagatcaaggagtgccaagagctgggtgttcttgtggatagggatgaccagggcgttctgcttcaaattgccactaagccagtgggcgaccgccctacattctggcttgagatgattcaaagaatcggctgcatggagaaggatgaggttggacaggagtaccaaaagggcggatgcggtggcttcggaaagggtaacttcagcgagttgttcaagtcaatcgaggactacgagaagagcctcgaggtgaagcagtcagtggttgcccaaaagtcctga

SEQ ID NO: 13 - DNA, 542 bp, Figwort mosaic virus
  Figwort mosaic virus 34S enhancer
aattctcagtccaaagcctcaacaaggtcagggtacagagtctccaaaccattagccaaaagctacaggagatcaatgaagaatcttcaatcaaagtaaactactgttccagcacatgcatcatggtcagtaagtttcagaaaaagacatccaccgaagacttaaagttagtgggcatctttgaaagtaatcttgtcaacatcgagcagctggcttgtggggaccagacaaaaaaggaatggtgcagaattgttaggcgcacctaccaaaagcatctttgcctttattgcaaagataaagcagattcctctagtacaagtggggaacaaaataacgtggaaaagagctgtcctgacagcccactcactaatgcgtatgacgaacgcagtgacgaccacaaaagaattagcttgagctcaggatttagcagcattccagattgggttcaatcaacaaggtacgagccatatcactttattcaaattggtatcgccaaaaccaagaaggaactcccatcctcaaaggtttgtaaggaagaattc

SEQ ID NO: 14 - DNA, 1534 bp, Brassica napus
  Promoter of oilseed rape eukaryotic elongation factor gene 1a (Tsf1)
gattatgacattgctcgtggaatgggacagttatggtatttttttgtaataaattgtttccattgtcatgagattttgaggttaatctatgagacattgaatcacttagcattagggattaagtagtcacaaatcgcattcaagaagctgaagaacacgttatggtctaatggttgtgtctctttattagaaaatgttggtcagtagctatatgcactgtttctgtaaaaccatgttggtgttgtgtttatttcaagacacatgttgagtccgttgattcagagcttttgtcttcgaacacaatctagagagcaaatttgggttcaatttggatatcaatatgggttcgattcagatagaacaataccctttgatgtcgggtttcgatttggttgagattcatttttatcgggtttggttcgattttcgaattcggtttattcgccccctcatagcatctacattctgcagattaatgtacaagttatggaaaaaaaaatgtggttttcgaattcggtttagtagctaaacgttgcttgcagtgtagttatgggaattatgaaacacgaccgaaggtatcaattagaagaacgggtcaacgggtaagtattgagaaattaccggagggtaaaaataaacagtattctttttttttcttaacgaccgaccaaggttaaaaaaagaaaggaggacgagatacaggggcatgactgtaattgtacataagatctgatctttaaaccctaggtttccttcgcatcagcaactataaataattctgagtgccactcttcttcattcctagatctttcgccttatcgctttagctgaggtaagcctttctatacgcatagacgctctcttttctcttctctcgatcttcgttgaaacggtcctcgatacgcataggatcggttagaatcgttaatctatcgtcttagatcttcttgattgttgaattgagcttctaggatgtattgtatcatgtgatggatagttgattggatctctttgagtgaactagctagctttcgatgcgtgtgatttcagtataacaggatccgatgaattatagctcgcttacaattaatctctgcagatttattgtttaatcttggatttgatgctcgttgttgatagaggatcgtttatagaacttattgattctggaattgagcttgtgtgatgtattgtatcatgtgatcgatagctgatggatctatttgagtgaactagcgtacgatcttaagatgagtgtgtattgtgaactgatgattcgagatcagcaaaacaagatctgatgatatcttcgtcttgtatgcatcttgaatttcatgattttttattaattatagctcgcttagctcaaaggatagagcaccacaaaattttattgtggtagaaatcggttcgattccgatagcagcttactgtgatgaatgattttgagatttggtatttgatatatgtctactgtgttgaatgatcgtttatgcattgtttaatcgctgcagatttgcattgacaagtagcc

SEQ ID NO: 15 - DNA, 228 bp, Arabidopsis thaliana
  Arabidopsis thaliana chloroplast transit peptide
atggcgcaagttagcagaatctgcaatggtgtgcagaacccatctcttatctccaatctctcgaaatccagtcaacgcaaatctcccttatcggtttctctgaagacgcagcagcatccacgagcttatccgatttcgtcgtcgtggggattgaagaagagtgggatgacgttaattggctctgagcttcgtcctcttaaggtcatgtcttctgtttccacggcgtgc

SEQ ID NO: 16 - DNA, 1368 bp, Artificial Sequence
  5-enolpyruvylshikimate-3-phosphate synthase gene
atgcttcacggtgcaagcagccgtccagcaactgctcgtaagtcctctggtctttctggaaccgtccgtattccaggtgacaagtctatctcccacaggtccttcatgtttggaggtctcgctagcggtgaaactcgtatcaccggtcttttggaaggtgaagatgttatcaacactggtaaggctatgcaagctatgggtgccagaatccgtaaggaaggtgatacttggatcattgatggtgttggtaacggtggactccttgctcctgaggctcctctcgatttcggtaacgctgcaactggttgccgtttgactatgggtcttgttggtgtttacgatttcgatagcactttcattggtgacgcttctctcactaagcgtccaatgggtcgtgtgttgaacccacttcgcgaaatgggtgtgcaggtgaagtctgaagacggtgatcgtcttccagttaccttgcgtggaccaaagactccaacgccaatcacctacagggtacctatggcttccgctcaagtgaagtccgctgttctgcttgctggtctcaacaccccaggtatcaccactgttatcgagccaatcatgactcgtgaccacactgaaaagatgcttcaaggttttggtgctaaccttaccgttgagactgatgctgacggtgtgcgtaccatccgtcttgaaggtcgtggtaagctcaccggtcaagtgattgatgttccaggtgatccatcctctactgctttcccattggttgctgccttgcttgttccaggttccgacgtcaccatccttaacgttttgatgaacccaacccgtactggtctcatcttgactctgcaggaaatgggtgccgacatcgaagtgatcaacccacgtcttgctggtggagaagacgtggctgacttgcgtgttcgttcttctactttgaagggtgttactgttccagaagaccgtgctccttctatgatcgacgagtatccaattctcgctgttgcagctgcattcgctgaaggtgctaccgttatgaacggtttggaagaactccgtgttaaggaaagcgaccgtctttctgctgtcgcaaacggtctcaagctcaacggtgttgattgcgatgaaggtgagacttctctcgtcgtgcgtggtcgtcctgacggtaagggtctcggtaacgcttctggagcagctgtcgctacccacctcgatcaccgtatcgctatgagcttcctcgttatgggtctcgtttctgaaaaccctgttactgttgatgatgctactatgatcgctactagcttcccagagttcatggatttgatggctggtcttggagctaagatcgaactctccgacactaaggctgcttga

SEQ ID NO: 17 - DNA, 643 bp, Pisum sativum
  Terminator of pea RbcS gene (Pisum sativum)
agctttcgttcgtatcatcggtttcgacaacgttcgtcaagttcaatgcatcagtttcattgcgcacacaccagaatcctactgagtttgagtattatggcattgggaaaactgtttttcttgtaccatttgttgtgcttgtaatttactgtgttttttattcggttttcgctatcgaactgtgaaatggaaatggatggagaagagttaatgaatgatatggtccttttgttcattctcaaattaatattatttgttttttctcttatttgttgtgtgttgaatttgaaattataagagatatgcaaacattttgttttgagtaaaaatgtgtcaaatcgtggcctctaatgaccgaagttaatatgaggagtaaaacacttgtagttgtaccattatgcttattcactaggcaacaaatatattttcagacctagaaaagctgcaaatgttactgaatacaagtatgtcctcttgtgttttagacatttatgaactttcctttatgtaattttccagaatccttgtcagattctaatcattgctttataattatagttatactcatggatttgtagttgagtatgaaaatattttttaatgcattttatgacttgccaattgattgacaacatgcatcaat

SEQ ID NO: 18 - DNA, 1322 bp, Arabidopsis thaliana
  Promoter of Arabidopsis thaliana Ubiquitin 10 gene
gtcgacctgcaggtcaacggatcaggatattcttgtttaagatgttgaactctatggaggtttgtatgaactgatgatctaggaccggataagttcccttcttcatagcgaacttattcaaagaatgttttgtgtatcattcttgttacattgttattaatgaaaaaatattattggtcattggactgaacacgagtgttaaatatggaccaggccccaaataagatccattgatatatgaattaaataacaagaataaatcgagtcaccaaaccacttgccttttttaacgagacttgttcaccaacttgatacaaaagtcattatcctatgcaaatcaataatcatacaaaaatatccaataacactaaaaaattaaaagaaatggataatttcacaatatgttatacgataaagaagttacttttccaagaaattcactgattttataagcccacttgcattagataaatggcaaaaaaaaacaaaaaggaaaagaaataaagcacgaagaattctagaaaatacgaaatacgcttcaatgcagtgggacccacggttcaattattgccaattttcagctccaccgtatatttaaaaaataaaacgataatgctaaaaaaatataaatcgtaacgatcgttaaatctcaacggctggatcttatgacgaccgttagaaattgtggttgtcgacgagtcagtaataaacggcgtcaaagtggttgcagccggcacacacgagtcgtgtttatcaactcaaagcacaaatacttttcctcaacctaaaaataaggcaattagccaaaaacaactttgcgtgtaaacaacgctcaatacacgtgtcattttattattagctattgcttcaccgccttagctttctcgtgacctagtcgtcctcgtcttttcttcttcttcttctataaaacaatacccaaagcttcttcttcacaattcagatttcaatttctcaaaatcttaaaaactttctctcaattctctctaccgtgatcaaggtaaatttctgtgttccttattctctcaaaatcttcgattttgttttcgttcgatcccaatttcgtatatgttctttggtttagattctgttaatcttagatcgaagacgattttctgggtttgatcgttagatatcatcttaattctcgattagggtttcataaatatcatccgatttgttcaaataatttgagttttgtcgaataattactcttcgatttgtgatttctatctagatctggtgttagtttctagtttgtgcgatcgaatttgtcgattaatctgagtttttctgattaacag

SEQ ID NO: 19 - DNA, 253 bp, Agrobacterium tumefaciens
  Terminator of nopaline synthetase gene (Agrobacterium tumefaciens)
gatcgttcaaacatttggcaataaagtttcttaagattgaatcctgttgccggtcttgcgatgattatcatataatttctgttgaattacgttaagcatgtaataattaacatgtaatgcatgacgttatttatgagatgggtttttatgattagagtcccgcaattatacatttaatacgcgatagaaaacaaaatatagcgcgcaaactaggataaattatcgcgcgcggtgtcatctatgttactagatc

SEQ ID NO: 20 - DNA, 530 bp, cauliflower mosaic virus
  Promoter of cauliflower mosaic virus 35S
ccatggagtcaaagattcaaatagaggacctaacagaactcgccgtaaagactggcgaacagttcatacagagtctcttacgactcaatgacaagaagaaaatcttcgtcaacatggtggagcacgacacgcttgtctactccaaaaatatcaaagatacagtctcagaagaccaaagggcaattgagacttttcaacaaagggtaatatccggaaacctcctcggattccattgcccagctatctgtcactttattgtgaagatagtggaaaaggaaggtggctcctacaaatgccatcattgcgataaaggaaaggccatcgttgaagatgcctctgccgacagtggtcccaaagatggacccccacccacgaggagcatcgtggaaaaagaagacgttccaaccacgtcttcaaagcaagtggattgatgtgatatctccactgacgtaagggatgacgcacaatcccactatccttcgcaagacccttcctctatataaggaagttcatttcatttggagaggaca

SEQ ID NO: 21 - DNA, 552 bp, Streptomyces viridochromogenes
  Phosphinothricin-N-acetyl-transferase gene
atgtctccggagaggagaccagttgagattaggccagctacagcagctgatatggccgcggtttgtgatatcgttaaccattacattgagacgtctacagtgaactttaggacagagccacaaacaccacaagagtggattgatgatctagagaggttgcaagatagatacccttggttggttgctgaggttgagggtgttgtggctggtattgcttacgctgggccctggaaggctaggaacgcttacgattggacagttgagagtactgtttacgtgtcacataggcatcaaaggttgggcctaggatccacattgtacacacatttgcttaagtctatggaggcgcaaggttttaagtctgtggttgctgttataggccttccaaacgatccatctgttaggttgcatgaggctttgggatacacagcccggggtacattgcgcgcagctggatacaagcatggtggatggcatgatgttggtttttggcaaagggattttgagttgccagctcctccaaggccagttaggccagttacccagatctga

SEQ ID NO: 22 - DNA, 195 bp, cauliflower mosaic virus
  Terminator of the cauliflower mosaic virus 35S
ctgaaatcaccagtctctctctacaaatctatctctctctataataatgtgtgagtagttcccagataagggaattagggttcttatagggtttcgctcatgtgttgagcatataagaaacccttagtatgtatttgtatttgtaaaatacttctatcaataaaatttctaattcctaaaaccaaaatccagtgg

SEQ ID NO: 23 - protein, 445 aa, Arabidopsis thaliana
  The amino acid sequence of Arabidopsis thaliana wild-type HPPD (AtHPPD)
MGHQNAAVSENQNHDDGAASSPGFKLVGFSKFVRKNPKSDKFKVKRFHHIEFWCGDATNVARRFSWGLGMRFSAKSDLSTGNMVHASYLLTSGDLRFLFTAPYSPSLSAGEIKPTTTASIPSFDHGSCRSFFSSHGLGVRAVAIEVEDAESAFSISVANGAIPSSPPIVLNEAVTIAEVKLYGDVVLRYVSYKAEDTEKSEFLPGFERVEDASSFPLDYGIRRLDHAVGNVPELGPALTYVAGFTGFHQFAEFTADDVGTAESGLNSAVLASNDEMVLLPINEPVHGTKRKSQIQTYLEHNEGAGLQHLALMSEDIFRTLREMRKRSSIGGFDFMPSPPPTYYQNLKKRVGDVLSDDQIKECEELGILVDRDDQGTLLQIFTKPLGDRPTIFIEIIQRVGCMMKDEEGKAYQSGGCGGFGKGNFSELFKSIEEYEKTLEAKQLVG

SEQ ID NO: 24 - DNA, 1338 bp, Arabidopsis thaliana
  AtHPPD-01 Nucleotide Sequence
atgggccaccaaaacgccgccgtttcagagaatcaaaaccatgatgacggcgctgcgtcgtcgccgggattcaagctcgtcggattttccaagttcgtaagaaagaatccaaagtctgataaattcaaggttaagcgcttccatcacatcgagttctggtgcggcgacgcaaccaacgtcgctcgtcgcttctcctggggtctggggatgagattctccgccaaatccgatctttccaccggaaacatggttcacgcctcttacctactcacctccggtgacctccgattccttttcactgctccttactctccgtctctctccgccggagagattaaaccgacaaccacagcttctatcccaagtttcgatcacggctcttgtcgttccttcttctcttcacatggtctcggtgttagagccgttgcgattgaagtagaagacgcagagtcagctttctccatcagtgtagctaatggcgctattccttcgtcgcctcctatcgtcctcaatgaagcagttacgatcgctgaggttaaactatacggcgatgttgttctccgatatgttagttacaaagcagaagataccgaaaaatccgaattcttgccagggttcgagcgtgtagaggatgcgtcgtcgttcccattggattatggtatccggcggcttgaccacgccgtgggaaacgttcctgagcttggtccggctttaacttatgtagcggggttcactggttttcaccaattcgcagagttcacagcagacgacgttggaaccgccgagagcggtttaaattcagcggtcctggctagcaatgatgaaatggttcttctaccgattaacgagccagtgcacggaacaaagaggaagagtcagattcagacgtatttggaacataacgaaggcgcagggctacaacatctggctctgatgagtgaagacatattcaggaccctgagagagatgaggaagaggagcagtattggaggattcgacttcatgccttctcctccgcctacttactaccagaatctcaagaaacgggtcggcgacgtgctcagcgatgatcagatcaaggagtgtgaggaattagggattcttgtagacagagatgatcaagggacgttgcttcaaatcttcacaaaaccactaggtgacaggccgacgatatttatagagataatccagagagtaggatgcatgatgaaagatgaggaagggaaggcttaccagagtggaggatgtggtggttttggcaaaggcaatttctctgagctcttcaagtccattgaagaatacgaaaagactcttgaagccaaacagttagtgggatga

SEQ ID NO: 25 - DNA, 1338 bp, Artificial Sequence
  AtHPPD-02 Nucleotide Sequence
atgggacatcagaatgctgctgtatcagaaaatcaaaatcatgatgatggagccgcctcctcaccagggtttaagttggttgggttctccaagtttgtacggaagaacccaaaatccgacaagttcaaggttaaacgcttccaccacattgaattctggtgcggcgacgccaccaatgttgctcggcgtttttcatggggtttaggcatgagattctcagcaaagagtgacctgagcaccggcaacatggttcatgctagctatctcttaacatctggagatttgaggtttcttttcacggcgccgtactcaccatcactctccgccggcgagatcaaacccaccacgactgcaagcataccttcatttgatcatggtagttgcagatccttcttctcgtcgcacggcctaggggtgcgcgcggtcgccatcgaagttgaagatgcagaatcagcgtttagtatcagcgtggcaaatggagctattccttcctcccctccaattgtcctcaatgaggctgtaactattgccgaggtgaagttgtatggagatgttgtgctgagatatgtttcttacaaggcagaggacactgagaaatctgaatttttgcctggttttgaaagggtcgaggatgcttcaagttttcctcttgattacggcatacgacggttggatcacgcggttggaaatgtaccagaacttgggccggcgctcacttatgtggctggtttcactggattccatcaatttgctgagttcacagctgatgatgttgggactgctgaaagtgggttgaactctgcagtcctcgcctctaatgatgaaatggtgctcctcccgatcaacgagcctgtgcatggcaccaaaaggaaatcacaaatacagacatatcttgagcacaatgaaggtgcagggcttcaacatcttgcactgatgtctgaagacattttccgtacgctgagagagatgaggaagagaagtagtattggtggatttgacttcatgccttctcccccaccaacttactaccagaacttgaagaagagggttggtgatgtgctatctgatgaccagatcaaggagtgtgaagaattgggcattcttgttgatcgggacgaccaaggaacattactgcagatatttacaaaaccacttggtgaccgccccactatttttattgagatcatacaaagagtcggctgcatgatgaaggatgaggaaggaaaagcatatcaatctggtggttgtggcggctttgggaaaggaaacttctctgagctgttcaaatccatcgaggagtatgagaagaccttggaggccaagcagctcgtgggttga

SEQ ID NO: 26 - protein, 445 aa, Artificial Sequence
  AtHPPDm-F372A Amino Acid Sequence
MGHQNAAVSENQNHDDGAASSPGFKLVGFSKFVRKNPKSDKFKVKRFHHIEFWCGDATNVARRFSWGLGMRFSAKSDLSTGNMVHASYLLTSGDLRFLFTAPYSPSLSAGEIKPTTTASIPSFDHGSCRSFFSSHGLGVRAVAIEVEDAESAFSISVANGAIPSSPPIVLNEAVTIAEVKLYGDVVLRYVSYKAEDTEKSEFLPGFERVEDASSFPLDYGIRRLDHAVGNVPELGPALTYVAGFTGFHQFAEFTADDVGTAESGLNSAVLASNDEMVLLPINEPVHGTKRKSQIQTYLEHNEGAGLQHLALMSEDIFRTLREMRKRSSIGGFDFMPSPPPTYYQNLKKRVGDVLSDDQIKECEELGILVDRDDQGTLLQIATKPLGDRPTIFIEIIQRVGCMMKDEEGKAYQSGGCGGFGKGNFSELFKSIEEYEKTLEAKQLVG

SEQ ID NO: 27 - DNA, 1338 bp, Artificial Sequence
  AtHPPDm-F372A-01 Nucleotide Sequence
atgggccaccaaaacgccgccgtttcagagaatcaaaaccatgatgacggcgctgcgtcgtcgccgggattcaagctcgtcggattttccaagttcgtaagaaagaatccaaagtctgataaattcaaggttaagcgcttccatcacatcgagttctggtgcggcgacgcaaccaacgtcgctcgtcgcttctcctggggtctggggatgagattctccgccaaatccgatctttccaccggaaacatggttcacgcctcttacctactcacctccggtgacctccgattccttttcactgctccttactctccgtctctctccgccggagagattaaaccgacaaccacagcttctatcccaagtttcgatcacggctcttgtcgttccttcttctcttcacatggtctcggtgttagagccgttgcgattgaagtagaagacgcagagtcagctttctccatcagtgtagctaatggcgctattccttcgtcgcctcctatcgtcctcaatgaagcagttacgatcgctgaggttaaactatacggcgatgttgttctccgatatgttagttacaaagcagaagataccgaaaaatccgaattcttgccagggttcgagcgtgtagaggatgcgtcgtcgttcccattggattatggtatccggcggcttgaccacgccgtgggaaacgttcctgagcttggtccggctttaacttatgtagcggggttcactggttttcaccaattcgcagagttcacagcagacgacgttggaaccgccgagagcggtttaaattcagcggtcctggctagcaatgatgaaatggttcttctaccgattaacgagccagtgcacggaacaaagaggaagagtcagattcagacgtatttggaacataacgaaggcgcagggctacaacatctggctctgatgagtgaagacatattcaggaccctgagagagatgaggaagaggagcagtattggaggattcgacttcatgccttctcctccgcctacttactaccagaatctcaagaaacgggtcggcgacgtgctcagcgatgatcagatcaaggagtgtgaggaattagggattcttgtagacagagatgatcaagggacgttgcttcaaatcgctacaaaaccactaggtgacaggccgacgatatttatagagataatccagagagtaggatgcatgatgaaagatgaggaagggaaggcttaccagagtggaggatgtggtggttttggcaaaggcaatttctctgagctcttcaagtccattgaagaatacgaaaagactcttgaagccaaacagttagtgggatga

SEQ ID NO: 28 - DNA, 1338 bp, Artificial Sequence
  AtHPPDm-F372A-02 Nucleotide Sequence
atgggacatcagaatgctgctgtatcagaaaatcaaaatcatgatgatggagccgcctcctcaccagggtttaagttggttgggttctccaagtttgtacggaagaacccaaaatccgacaagttcaaggttaaacgcttccaccacattgaattctggtgcggcgacgccaccaatgttgctcggcgtttttcatggggtttaggcatgagattctcagcaaagagtgacctgagcaccggcaacatggttcatgctagctatctcttaacatctggagatttgaggtttcttttcacggcgccgtactcaccatcactctccgccggcgagatcaaacccaccacgactgcaagcataccttcatttgatcatggtagttgcagatccttcttctcgtcgcacggcctaggggtgcgcgcggtcgccatcgaagttgaagatgcagaatcagcgtttagtatcagcgtggcaaatggagctattccttcctcccctccaattgtcctcaatgaggctgtaactattgccgaggtgaagttgtatggagatgttgtgctgagatatgtttcttacaaggcagaggacactgagaaatctgaatttttgcctggttttgaaagggtcgaggatgcttcaagttttcctcttgattacggcatacgacggttggatcacgcggttggaaatgtaccagaacttgggccggcgctcacttatgtggctggtttcactggattccatcaatttgctgagttcacagctgatgatgttgggactgctgaaagtgggttgaactctgcagtcctcgcctctaatgatgaaatggtgctcctcccgatcaacgagcctgtgcatggcaccaaaaggaaatcacaaatacagacatatcttgagcacaatgaaggtgcagggcttcaacatcttgcactgatgtctgaagacattttccgtacgctgagagagatgaggaagagaagtagtattggtggatttgacttcatgccttctcccccaccaacttactaccagaacttgaagaagagggttggtgatgtgctatctgatgaccagatcaaggagtgtgaagaattgggcattcttgttgatcgggacgaccaaggaacattactgcagatagccacaaaaccacttggtgaccgccccactatttttattgagatcatacaaagagtcggctgcatgatgaaggatgaggaaggaaaagcatatcaatctggtggttgtggcggctttgggaaaggaaacttctctgagctgttcaaatccatcgaggagtatgagaagaccttggaggccaagcagctcgtgggttga

SEQ ID NO: 29 - protein, 445 aa, Artificial Sequence
  AtHPPDm-F383W Amino Acid Sequence
MGHQNAAVSENQNHDDGAASSPGFKLVGFSKFVRKNPKSDKFKVKRFHHIEFWCGDATNVARRFSWGLGMRFSAKSDLSTGNMVHASYLLTSGDLRFLFTAPYSPSLSAGEIKPTTTASIPSFDHGSCRSFFSSHGLGVRAVAIEVEDAESAFSISVANGAIPSSPPIVLNEAVTIAEVKLYGDVVLRYVSYKAEDTEKSEFLPGFERVEDASSFPLDYGIRRLDHAVGNVPELGPALTYVAGFTGFHQFAEFTADDVGTAESGLNSAVLASNDEMVLLPINEPVHGTKRKSQIQTYLEHNEGAGLQHLALMSEDIFRTLREMRKRSSIGGFDFMPSPPPTYYQNLKKRVGDVLSDDQIKECEELGILVDRDDQGTLLQIFTKPLGDRPTIWIEIIQRVGCMMKDEEGKAYQSGGCGGFGKGNFSELFKSIEEYEKTLEAKQLVG

SEQ ID NO: 30 - DNA, 1338 bp, Artificial Sequence
  AtHPPDm-F383W-01 Nucleotide Sequence
atgggccaccaaaacgccgccgtttcagagaatcaaaaccatgatgacggcgctgcgtcgtcgccgggattcaagctcgtcggattttccaagttcgtaagaaagaatccaaagtctgataaattcaaggttaagcgcttccatcacatcgagttctggtgcggcgacgcaaccaacgtcgctcgtcgcttctcctggggtctggggatgagattctccgccaaatccgatctttccaccggaaacatggttcacgcctcttacctactcacctccggtgacctccgattccttttcactgctccttactctccgtctctctccgccggagagattaaaccgacaaccacagcttctatcccaagtttcgatcacggctcttgtcgttccttcttctcttcacatggtctcggtgttagagccgttgcgattgaagtagaagacgcagagtcagctttctccatcagtgtagctaatggcgctattccttcgtcgcctcctatcgtcctcaatgaagcagttacgatcgctgaggttaaactatacggcgatgttgttctccgatatgttagttacaaagcagaagataccgaaaaatccgaattcttgccagggttcgagcgtgtagaggatgcgtcgtcgttcccattggattatggtatccggcggcttgaccacgccgtgggaaacgttcctgagcttggtccggctttaacttatgtagcggggttcactggttttcaccaattcgcagagttcacagcagacgacgttggaaccgccgagagcggtttaaattcagcggtcctggctagcaatgatgaaatggttcttctaccgattaacgagccagtgcacggaacaaagaggaagagtcagattcagacgtatttggaacataacgaaggcgcagggctacaacatctggctctgatgagtgaagacatattcaggaccctgagagagatgaggaagaggagcagtattggaggattcgacttcatgccttctcctccgcctacttactaccagaatctcaagaaacgggtcggcgacgtgctcagcgatgatcagatcaaggagtgtgaggaattagggattcttgtagacagagatgatcaagggacgttgcttcaaatcttcacaaaaccactaggtgacaggccgacgatatggatagagataatccagagagtaggatgcatgatgaaagatgaggaagggaaggcttaccagagtggaggatgtggtggttttggcaaaggcaatttctctgagctcttcaagtccattgaagaatacgaaaagactcttgaagccaaacagttagtgggatga

SEQ ID NO: 31 - DNA, 1338 bp, Artificial Sequence
  AtHPPDm-F383W-02 Nucleotide Sequence
atgggacatcagaatgctgctgtatcagaaaatcaaaatcatgatgatggagccgcctcctcaccagggtttaagttggttgggttctccaagtttgtacggaagaacccaaaatccgacaagttcaaggttaaacgcttccaccacattgaattctggtgcggcgacgccaccaatgttgctcggcgtttttcatggggtttaggcatgagattctcagcaaagagtgacctgagcaccggcaacatggttcatgctagctatctcttaacatctggagatttgaggtttcttttcacggcgccgtactcaccatcactctccgccggcgagatcaaacccaccacgactgcaagcataccttcatttgatcatggtagttgcagatccttcttctcgtcgcacggcctaggggtgcgcgcggtcgccatcgaagttgaagatgcagaatcagcgtttagtatcagcgtggcaaatggagctattccttcctcccctccaattgtcctcaatgaggctgtaactattgccgaggtgaagttgtatggagatgttgtgctgagatatgtttcttacaaggcagaggacactgagaaatctgaatttttgcctggttttgaaagggtcgaggatgcttcaagttttcctcttgattacggcatacgacggttggatcacgcggttggaaatgtaccagaacttgggccggcgctcacttatgtggctggtttcactggattccatcaatttgctgagttcacagctgatgatgttgggactgctgaaagtgggttgaactctgcagtcctcgcctctaatgatgaaatggtgctcctcccgatcaacgagcctgtgcatggcaccaaaaggaaatcacaaatacagacatatcttgagcacaatgaaggtgcagggcttcaacatcttgcactgatgtctgaagacattttccgtacgctgagagagatgaggaagagaagtagtattggtggatttgacttcatgccttctcccccaccaacttactaccagaacttgaagaagagggttggtgatgtgctatctgatgaccagatcaaggagtgtgaagaattgggcattcttgttgatcgggacgaccaaggaacattactgcagatatttacaaaaccacttggtgaccgccccactatttggattgagatcatacaaagagtcggctgcatgatgaaggatgaggaaggaaaagcatatcaatctggtggttgtggcggctttgggaaaggaaacttctctgagctgttcaaatccatcgaggagtatgagaagaccttggaggccaagcagctcgtgggttga

SEQ ID NO: 32 - protein, 445 aa, Artificial Sequence
  AtHPPDm-F372A-F383W Amino Acid Sequence
MGHQNAAVSENQNHDDGAASSPGFKLVGFSKFVRKNPKSDKFKVKRFHHIEFWCGDATNVARRFSWGLGMRFSAKSDLSTGNMVHASYLLTSGDLRFLFTAPYSPSLSAGEIKPTTTASIPSFDHGSCRSFFSSHGLGVRAVAIEVEDAESAFSISVANGAIPSSPPIVLNEAVTIAEVKLYGDVVLRYVSYKAEDTEKSEFLPGFERVEDASSFPLDYGIRRLDHAVGNVPELGPALTYVAGFTGFHQFAEFTADDVGTAESGLNSAVLASNDEMVLLPINEPVHGTKRKSQIQTYLEHNEGAGLQHLALMSEDIFRTLREMRKRSSIGGFDFMPSPPPTYYQNLKKRVGDVLSDDQIKECEELGILVDRDDQGTLLQIATKPLGDRPTIWIEIIQRVGCMMKDEEGKAYQSGGCGGFGKGNFSELFKSIEEYEKTLEAKQLVG

SEQ ID NO: 33 - DNA, 1338 bp, Artificial Sequence
  AtHPPDm-F372A-F383W-01 Nucleotide Sequence
atgggccaccaaaacgccgccgtttcagagaatcaaaaccatgatgacggcgctgcgtcgtcgccgggattcaagctcgtcggattttccaagttcgtaagaaagaatccaaagtctgataaattcaaggttaagcgcttccatcacatcgagttctggtgcggcgacgcaaccaacgtcgctcgtcgcttctcctggggtctggggatgagattctccgccaaatccgatctttccaccggaaacatggttcacgcctcttacctactcacctccggtgacctccgattccttttcactgctccttactctccgtctctctccgccggagagattaaaccgacaaccacagcttctatcccaagtttcgatcacggctcttgtcgttccttcttctcttcacatggtctcggtgttagagccgttgcgattgaagtagaagacgcagagtcagctttctccatcagtgtagctaatggcgctattccttcgtcgcctcctatcgtcctcaatgaagcagttacgatcgctgaggttaaactatacggcgatgttgttctccgatatgttagttacaaagcagaagataccgaaaaatccgaattcttgccagggttcgagcgtgtagaggatgcgtcgtcgttcccattggattatggtatccggcggcttgaccacgccgtgggaaacgttcctgagcttggtccggctttaacttatgtagcggggttcactggttttcaccaattcgcagagttcacagcagacgacgttggaaccgccgagagcggtttaaattcagcggtcctggctagcaatgatgaaatggttcttctaccgattaacgagccagtgcacggaacaaagaggaagagtcagattcagacgtatttggaacataacgaaggcgcagggctacaacatctggctctgatgagtgaagacatattcaggaccctgagagagatgaggaagaggagcagtattggaggattcgacttcatgccttctcctccgcctacttactaccagaatctcaagaaacgggtcggcgacgtgctcagcgatgatcagatcaaggagtgtgaggaattagggattcttgtagacagagatgatcaagggacgttgcttcaaatcgctacaaaaccactaggtgacaggccgacgatatggatagagataatccagagagtaggatgcatgatgaaagatgaggaagggaaggcttaccagagtggaggatgtggtggttttggcaaaggcaatttctctgagctcttcaagtccattgaagaatacgaaaagactcttgaagccaaacagttagtgggatga

SEQ ID NO: 34 - DNA, 1338 bp, Artificial Sequence
  AtHPPDm-F372A-F383W-02 Nucleotide Sequence
atgggacatcagaatgctgctgtatcagaaaatcaaaatcatgatgatggagccgcctcctcaccagggtttaagttggttgggttctccaagtttgtacggaagaacccaaaatccgacaagttcaaggttaaacgcttccaccacattgaattctggtgcggcgacgccaccaatgttgctcggcgtttttcatggggtttaggcatgagattctcagcaaagagtgacctgagcaccggcaacatggttcatgctagctatctcttaacatctggagatttgaggtttcttttcacggcgccgtactcaccatcactctccgccggcgagatcaaacccaccacgactgcaagcataccttcatttgatcatggtagttgcagatccttcttctcgtcgcacggcctaggggtgcgcgcggtcgccatcgaagttgaagatgcagaatcagcgtttagtatcagcgtggcaaatggagctattccttcctcccctccaattgtcctcaatgaggctgtaactattgccgaggtgaagttgtatggagatgttgtgctgagatatgtttcttacaaggcagaggacactgagaaatctgaatttttgcctggttttgaaagggtcgaggatgcttcaagttttcctcttgattacggcatacgacggttggatcacgcggttggaaatgtaccagaacttgggccggcgctcacttatgtggctggtttcactggattccatcaatttgctgagttcacagctgatgatgttgggactgctgaaagtgggttgaactctgcagtcctcgcctctaatgatgaaatggtgctcctcccgatcaacgagcctgtgcatggcaccaaaaggaaatcacaaatacagacatatcttgagcacaatgaaggtgcagggcttcaacatcttgcactgatgtctgaagacattttccgtacgctgagagagatgaggaagagaagtagtattggtggatttgacttcatgccttctcccccaccaacttactaccagaacttgaagaagagggttggtgatgtgctatctgatgaccagatcaaggagtgtgaagaattgggcattcttgttgatcgggacgaccaaggaacattactgcagatagccacaaaaccacttggtgaccgccccactatttggattgagatcatacaaagagtcggctgcatgatgaaggatgaggaaggaaaagcatatcaatctggtggttgtggcggctttgggaaaggaaacttctctgagctgttcaaatccatcgaggagtatgagaagaccttggaggccaagcagctcgtgggttga

SEQ ID NO: 35 - protein, 435 aa, Medicago Sativa Linn
  The amino acid sequence of Medicago Sativa Linn wild-type HPPD (MsHPPD)
MAIETETQTQTGFKLVGFKNFVRANPKSDRFKVKRFHHVEFWCTDATNTARRFSHGLGMPIVAKSDLSTGNQTHASYLLRSGDLNFLFSAAYSPSISLSSPSSTAAIPTFSASNCFSFSASHGLAVRAVAVEVEDAELAFTTSVNNGAIPSSPPVILENHVKLAEVRLYGDVVLRYVSYNDPNPNQNPNLLFLPGFERVSDESSNSSLDFGIRRLDHAVGNVPELSSAVKYVKDFTGFHEFAEFTAEDVGTSESGLNSVVLANNEETVLLPMNEPVYGTKRKSQIETYLEHNEGAGLQHLALKSEDIFRTLREMRKRSGVGGFEFMPSPPVTYYRNLKNRVGDVLSDEQIKECEELGILVDRDDQGTLLQIFTKPIGDRPTIFIEIIQRVGCMLKDEEGKEYQKGGCGGFGKGNFSELFKSIEEYEKTLETRRTA

SEQ ID NO: 36 - DNA, 1308 bp, Medicago Sativa Linn
  MsHPPD-01 Nucleotide Sequence
atggccatcgaaacagaaactcaaacccaaaccgggttcaaactagttgggttcaagaacttcgtccgagccaatccaaaatcagaccggttcaaagtaaaacgcttccaccatgttgagttctggtgcaccgacgcaacaaacaccgcacgccgtttctctcacggactcggaatgccgattgtcgctaaatcagacctctccaccggaaatcaaactcacgcctcctatctcctccgctccggtgacctcaacttcctcttctccgccgcttattccccttccatttctctctcctcaccttcctcaactgccgcaatccccactttctccgcatccaattgtttctccttctccgcttcccacggcctcgccgtccgtgctgttgctgttgaagtcgaagacgccgaactggctttcaccaccagcgtaaacaacggtgccattccatcgtctcctccagttatcctcgaaaaccacgtcaaactggccgaagttcgtctctacggcgacgttgttctacgttacgtcagttacaacgacccgaacccaaaccagaatccgaacctgctcttcctccctggttttgaacgtgtatcagatgaatcatctaattcatcgttagatttcggaatccggcgactagaccatgccgttggaaatgtaccggagctttcatccgctgtgaaatacgtgaaagatttcaccggatttcatgaatttgctgagtttacagcggaagacgttggaacgagtgagagtggattaaactcagtggtgttagctaacaatgaagaaacagtgttgcttccgatgaatgaaccggtttatggaacaaagaggaagagtcaaatagaaacgtatttggaacataatgaaggtgctgggttacaacatttggcattgaagtctgaggatatatttaggacattgagggaaatgagaaagagaagtggtgttggtgggtttgagtttatgccttctcctccggtcacttattatcgtaatttgaagaatcgcgttggcgatgttttgagtgatgaacagattaaggagtgtgaagagcttgggattttggttgatagagatgatcagggtactctgcttcagatttttaccaagcctattggagataggccaaccatatttatagagataattcagagagttggatgcatgctcaaggacgaagaagggaaggagtatcaaaagggaggatgtgggggctttggaaaaggaaacttctcggagcttttcaaatccattgaagagtatgagaagactttggaaactagaagaactgcatga

SEQ ID NO: 37 - DNA, 1308 bp, Artificial Sequence
  MsHPPD-02 Nucleotide Sequence
atggctattgaaaccgaaacacaaactcagactggatttaaactggtagggttcaagaatttcgttagggctaatcccaagtctgatcgttttaaggtcaagaggttccaccacgtggagttctggtgcactgatgcaaccaacacggcgcggcgtttttcacatggtcttggaatgcctattgttgcaaaatccgacctctccacggggaaccaaacacacgcctcttacctgctacggagtggtgacttgaacttcctcttcagcgccgcctactcaccctccatatcgttgtcttcaccatcctcgaccgcagcaattcctacattttctgcgagcaactgcttctctttctctgccagtcatggcctcgccgtcagagcagtggccgttgaagtagaggatgctgaacttgcttttacaacttcagtgaataatggagcaataccgagcagtccgccggtcatacttgagaatcatgtgaagctagcggaggtgaggctttatggggacgtcgttttaagatatgtcagctacaatgatccaaaccccaatcaaaatccaaatttgttgttccttcctggcttcgagcgtgttagcgatgaatcttcaaactcttcactggattttggaatcagacggttggatcatgctgttggaaatgttcctgaactctcgagcgctgtgaaatatgtgaaggacttcaccggttttcatgaatttgctgagtttactgcagaagatgtgggtacatcagagagtggcttgaattccgtggtgctcgccaacaacgaggagactgtactcttaccaatgaatgagccagtctatggcaccaagcgtaaatctcaaattgagacatatttggagcacaatgaaggagctggacttcagcatctcgcgctgaagagtgaggacatcttccgcaccctacgggagatgaggaaaagaagtggtgttggtgggtttgaattcatgccatcacctcctgtcacctactacaggaacctgaagaacagagttggtgatgtactttcggacgagcagataaaggaatgtgaagagttggggattttggttgatagagatgatcaaggaacactcctgcagatttttacaaaaccaattggcgaccgccccactatcttcatagagatcatccagagggtggggtgcatgctcaaagacgaggaagggaaggagtaccagaagggcggctgtggtggttttgggaaaggaaacttttctgagttattcaaatcaattgaagagtatgagaagacgcttgaaacgcgtcgcactgcttga

SEQ ID NO: 38 - protein, 435 aa, Artificial Sequence
  MsHPPDm-F372A Amino Acid Sequence
MAIETETQTQTGFKLVGFKNFVRANPKSDRFKVKRFHHVEFWCTDATNTARRFSHGLGMPIVAKSDLSTGNQTHASYLLRSGDLNFLFSAAYSPSISLSSPSSTAAIPTFSASNCFSFSASHGLAVRAVAVEVEDAELAFTTSVNNGAIPSSPPVILENHVKLAEVRLYGDVVLRYVSYNDPNPNQNPNLLFLPGFERVSDESSNSSLDFGIRRLDHAVGNVPELSSAVKYVKDFTGFHEFAEFTAEDVGTSESGLNSVVLANNEETVLLPMNEPVYGTKRKSQIETYLEHNEGAGLQHLALKSEDIFRTLREMRKRSGVGGFEFMPSPPVTYYRNLKNRVGDVLSDEQIKECEELGILVDRDDQGTLLQIATKPIGDRPTIFIEIIQRVGCMLKDEEGKEYQKGGCGGFGKGNFSELFKSIEEYEKTLETRRTA

SEQ ID NO: 39 - DNA, 1308 bp, Artificial Sequence
  MsHPPDm-F372A-01 Nucleotide Sequence
atggccatcgaaacagaaactcaaacccaaaccgggttcaaactagttgggttcaagaacttcgtccgagccaatccaaaatcagaccggttcaaagtaaaacgcttccaccatgttgagttctggtgcaccgacgcaacaaacaccgcacgccgtttctctcacggactcggaatgccgattgtcgctaaatcagacctctccaccggaaatcaaactcacgcctcctatctcctccgctccggtgacctcaacttcctcttctccgccgcttattccccttccatttctctctcctcaccttcctcaactgccgcaatccccactttctccgcatccaattgtttctccttctccgcttcccacggcctcgccgtccgtgctgttgctgttgaagtcgaagacgccgaactggctttcaccaccagcgtaaacaacggtgccattccatcgtctcctccagttatcctcgaaaaccacgtcaaactggccgaagttcgtctctacggcgacgttgttctacgttacgtcagttacaacgacccgaacccaaaccagaatccgaacctgctcttcctccctggttttgaacgtgtatcagatgaatcatctaattcatcgttagatttcggaatccggcgactagaccatgccgttggaaatgtaccggagctttcatccgctgtgaaatacgtgaaagatttcaccggatttcatgaatttgctgagtttacagcggaagacgttggaacgagtgagagtggattaaactcagtggtgttagctaacaatgaagaaacagtgttgcttccgatgaatgaaccggtttatggaacaaagaggaagagtcaaatagaaacgtatttggaacataatgaaggtgctgggttacaacatttggcattgaagtctgaggatatatttaggacattgagggaaatgagaaagagaagtggtgttggtgggtttgagtttatgccttctcctccggtcacttattatcgtaatttgaagaatcgcgttggcgatgttttgagtgatgaacagattaaggagtgtgaagagcttgggattttggttgatagagatgatcagggtactctgcttcagattgctaccaagcctattggagataggccaaccatatttatagagataattcagagagttggatgcatgctcaaggacgaagaagggaaggagtatcaaaagggaggatgtgggggctttggaaaaggaaacttctcggagcttttcaaatccattgaagagtatgagaagactttggaaactagaagaactgcatga

SEQ ID NO: 40 - DNA, 1308 bp, Artificial Sequence
  MsHPPDm-F372A-02 Nucleotide Sequence
atggctattgaaaccgaaacacaaactcagactggatttaaactggtagggttcaagaatttcgttagggctaatcccaagtctgatcgttttaaggtcaagaggttccaccacgtggagttctggtgcactgatgcaaccaacacggcgcggcgtttttcacatggtcttggaatgcctattgttgcaaaatccgacctctccacggggaaccaaacacacgcctcttacctgctacggagtggtgacttgaacttcctcttcagcgccgcctactcaccctccatatcgttgtcttcaccatcctcgaccgcagcaattcctacattttctgcgagcaactgcttctctttctctgccagtcatggcctcgccgtcagagcagtggccgttgaagtagaggatgctgaacttgcttttacaacttcagtgaataatggagcaataccgagcagtccgccggtcatacttgagaatcatgtgaagctagcggaggtgaggctttatggggacgtcgttttaagatatgtcagctacaatgatccaaaccccaatcaaaatccaaatttgttgttccttcctggcttcgagcgtgttagcgatgaatcttcaaactcttcactggattttggaatcagacggttggatcatgctgttggaaatgttcctgaactctcgagcgctgtgaaatatgtgaaggacttcaccggttttcatgaatttgctgagtttactgcagaagatgtgggtacatcagagagtggcttgaattccgtggtgctcgccaacaacgaggagactgtactcttaccaatgaatgagccagtctatggcaccaagcgtaaatctcaaattgagacatatttggagcacaatgaaggagctggacttcagcatctcgcgctgaagagtgaggacatcttccgcaccctacgggagatgaggaaaagaagtggtgttggtgggtttgaattcatgccatcacctcctgtcacctactacaggaacctgaagaacagagttggtgatgtactttcggacgagcagataaaggaatgtgaagagttggggattttggttgatagagatgatcaaggaacactcctgcagattgccacaaaaccaattggcgaccgccccactatcttcatagagatcatccagagggtggggtgcatgctcaaagacgaggaagggaaggagtaccagaagggcggctgtggtggttttgggaaaggaaacttttctgagttattcaaatcaattgaagagtatgagaagacgcttgaaacgcgtcgcactgcttga

SEQ ID NO: 41 - protein, 435 aa, Artificial Sequence
  MsHPPDm-F383W Amino Acid Sequence
MAIETETQTQTGFKLVGFKNFVRANPKSDRFKVKRFHHVEFWCTDATNTARRFSHGLGMPIVAKSDLSTGNQTHASYLLRSGDLNFLFSAAYSPSISLSSPSSTAAIPTFSASNCFSFSASHGLAVRAVAVEVEDAELAFTTSVNNGAIPSSPPVILENHVKLAEVRLYGDVVLRYVSYNDPNPNQNPNLLFLPGFERVSDESSNSSLDFGIRRLDHAVGNVPELSSAVKYVKDFTGFHEFAEFTAEDVGTSESGLNSVVLANNEETVLLPMNEPVYGTKRKSQIETYLEHNEGAGLQHLALKSEDIFRTLREMRKRSGVGGFEFMPSPPVTYYRNLKNRVGDVLSDEQIKECEELGILVDRDDQGTLLQIFTKPIGDRPTIWIEIIQRVGCMLKDEEGKEYQKGGCGGFGKGNFSELFKSIEEYEKTLETRRTA

SEQ ID NO: 42 - DNA, 1308 bp, Artificial Sequence
  MsHPPDm-F383W-01 Nucleotide Sequence
atggccatcgaaacagaaactcaaacccaaaccgggttcaaactagttgggttcaagaacttcgtccgagccaatccaaaatcagaccggttcaaagtaaaacgcttccaccatgttgagttctggtgcaccgacgcaacaaacaccgcacgccgtttctctcacggactcggaatgccgattgtcgctaaatcagacctctccaccggaaatcaaactcacgcctcctatctcctccgctccggtgacctcaacttcctcttctccgccgcttattccccttccatttctctctcctcaccttcctcaactgccgcaatccccactttctccgcatccaattgtttctccttctccgcttcccacggcctcgccgtccgtgctgttgctgttgaagtcgaagacgccgaactggctttcaccaccagcgtaaacaacggtgccattccatcgtctcctccagttatcctcgaaaaccacgtcaaactggccgaagttcgtctctacggcgacgttgttctacgttacgtcagttacaacgacccgaacccaaaccagaatccgaacctgctcttcctccctggttttgaacgtgtatcagatgaatcatctaattcatcgttagatttcggaatccggcgactagaccatgccgttggaaatgtaccggagctttcatccgctgtgaaatacgtgaaagatttcaccggatttcatgaatttgctgagtttacagcggaagacgttggaacgagtgagagtggattaaactcagtggtgttagctaacaatgaagaaacagtgttgcttccgatgaatgaaccggtttatggaacaaagaggaagagtcaaatagaaacgtatttggaacataatgaaggtgctgggttacaacatttggcattgaagtctgaggatatatttaggacattgagggaaatgagaaagagaagtggtgttggtgggtttgagtttatgccttctcctccggtcacttattatcgtaatttgaagaatcgcgttggcgatgttttgagtgatgaacagattaaggagtgtgaagagcttgggattttggttgatagagatgatcagggtactctgcttcagatttttaccaagcctattggagataggccaaccatatggatagagataattcagagagttggatgcatgctcaaggacgaagaagggaaggagtatcaaaagggaggatgtgggggctttggaaaaggaaacttctcggagcttttcaaatccattgaagagtatgagaagactttggaaactagaagaactgcatga

SEQ ID NO: 43 - DNA, 1308 bp, Artificial Sequence
  MsHPPDm-F383W-02 Nucleotide Sequence
atggctattgaaaccgaaacacaaactcagactggatttaaactggtagggttcaagaatttcgttagggctaatcccaagtctgatcgttttaaggtcaagaggttccaccacgtggagttctggtgcactgatgcaaccaacacggcgcggcgtttttcacatggtcttggaatgcctattgttgcaaaatccgacctctccacggggaaccaaacacacgcctcttacctgctacggagtggtgacttgaacttcctcttcagcgccgcctactcaccctccatatcgttgtcttcaccatcctcgaccgcagcaattcctacattttctgcgagcaactgcttctctttctctgccagtcatggcctcgccgtcagagcagtggccgttgaagtagaggatgctgaacttgcttttacaacttcagtgaataatggagcaataccgagcagtccgccggtcatacttgagaatcatgtgaagctagcggaggtgaggctttatggggacgtcgttttaagatatgtcagctacaatgatccaaaccccaatcaaaatccaaatttgttgttccttcctggcttcgagcgtgttagcgatgaatcttcaaactcttcactggattttggaatcagacggttggatcatgctgttggaaatgttcctgaactctcgagcgctgtgaaatatgtgaaggacttcaccggttttcatgaatttgctgagtttactgcagaagatgtgggtacatcagagagtggcttgaattccgtggtgctcgccaacaacgaggagactgtactcttaccaatgaatgagccagtctatggcaccaagcgtaaatctcaaattgagacatatttggagcacaatgaaggagctggacttcagcatctcgcgctgaagagtgaggacatcttccgcaccctacgggagatgaggaaaagaagtggtgttggtgggtttgaattcatgccatcacctcctgtcacctactacaggaacctgaagaacagagttggtgatgtactttcggacgagcagataaaggaatgtgaagagttggggattttggttgatagagatgatcaaggaacactcctgcagatttttacaaaaccaattggcgaccgccccactatctggatagagatcatccagagggtggggtgcatgctcaaagacgaggaagggaaggagtaccagaagggcggctgtggtggttttgggaaaggaaacttttctgagttattcaaatcaattgaagagtatgagaagacgcttgaaacgcgtcgcactgcttga

SEQ ID NO: 44 - protein, 435 aa, Artificial Sequence
  MsHPPDm-F372A-F383W Amino Acid Sequence
MAIETETQTQTGFKLVGFKNFVRANPKSDRFKVKRFHHVEFWCTDATNTARRFSHGLGMPIVAKSDLSTGNQTHASYLLRSGDLNFLFSAAYSPSISLSSPSSTAAIPTFSASNCFSFSASHGLAVRAVAVEVEDAELAFTTSVNNGAIPSSPPVILENHVKLAEVRLYGDVVLRYVSYNDPNPNQNPNLLFLPGFERVSDESSNSSLDFGIRRLDHAVGNVPELSSAVKYVKDFTGFHEFAEFTAEDVGTSESGLNSVVLANNEETVLLPMNEPVYGTKRKSQIETYLEHNEGAGLQHLALKSEDIFRTLREMRKRSGVGGFEFMPSPPVTYYRNLKNRVGDVLSDEQIKECEELGILVDRDDQGTLLQIATKPIGDRPTIWIEIIQRVGCMLKDEEGKEYQKGGCGGFGKGNFSELFKSIEEYEKTLETRRTA

SEQ ID NO: 45 - DNA, 1308 bp, Artificial Sequence
  MsHPPDm-F372A-F383W-01 Nucleotide Sequence
atggccatcgaaacagaaactcaaacccaaaccgggttcaaactagttgggttcaagaacttcgtccgagccaatccaaaatcagaccggttcaaagtaaaacgcttccaccatgttgagttctggtgcaccgacgcaacaaacaccgcacgccgtttctctcacggactcggaatgccgattgtcgctaaatcagacctctccaccggaaatcaaactcacgcctcctatctcctccgctccggtgacctcaacttcctcttctccgccgcttattccccttccatttctctctcctcaccttcctcaactgccgcaatccccactttctccgcatccaattgtttctccttctccgcttcccacggcctcgccgtccgtgctgttgctgttgaagtcgaagacgccgaactggctttcaccaccagcgtaaacaacggtgccattccatcgtctcctccagttatcctcgaaaaccacgtcaaactggccgaagttcgtctctacggcgacgttgttctacgttacgtcagttacaacgacccgaacccaaaccagaatccgaacctgctcttcctccctggttttgaacgtgtatcagatgaatcatctaattcatcgttagatttcggaatccggcgactagaccatgccgttggaaatgtaccggagctttcatccgctgtgaaatacgtgaaagatttcaccggatttcatgaatttgctgagtttacagcggaagacgttggaacgagtgagagtggattaaactcagtggtgttagctaacaatgaagaaacagtgttgcttccgatgaatgaaccggtttatggaacaaagaggaagagtcaaatagaaacgtatttggaacataatgaaggtgctgggttacaacatttggcattgaagtctgaggatatatttaggacattgagggaaatgagaaagagaagtggtgttggtgggtttgagtttatgccttctcctccggtcacttattatcgtaatttgaagaatcgcgttggcgatgttttgagtgatgaacagattaaggagtgtgaagagcttgggattttggttgatagagatgatcagggtactctgcttcagattgctaccaagcctattggagataggccaaccatatggatagagataattcagagagttggatgcatgctcaaggacgaagaagggaaggagtatcaaaagggaggatgtgggggctttggaaaaggaaacttctcggagcttttcaaatccattgaagagtatgagaagactttggaaactagaagaactgcatga

SEQ ID NO: 46 - DNA, 1308 bp, Artificial Sequence
  MsHPPDm-F372A-F383W-02 Nucleotide Sequence
atggctattgaaaccgaaacacaaactcagactggatttaaactggtagggttcaagaatttcgttagggctaatcccaagtctgatcgttttaaggtcaagaggttccaccacgtggagttctggtgcactgatgcaaccaacacggcgcggcgtttttcacatggtcttggaatgcctattgttgcaaaatccgacctctccacggggaaccaaacacacgcctcttacctgctacggagtggtgacttgaacttcctcttcagcgccgcctactcaccctccatatcgttgtcttcaccatcctcgaccgcagcaattcctacattttctgcgagcaactgcttctctttctctgccagtcatggcctcgccgtcagagcagtggccgttgaagtagaggatgctgaacttgcttttacaacttcagtgaataatggagcaataccgagcagtccgccggtcatacttgagaatcatgtgaagctagcggaggtgaggctttatggggacgtcgttttaagatatgtcagctacaatgatccaaaccccaatcaaaatccaaatttgttgttccttcctggcttcgagcgtgttagcgatgaatcttcaaactcttcactggattttggaatcagacggttggatcatgctgttggaaatgttcctgaactctcgagcgctgtgaaatatgtgaaggacttcaccggttttcatgaatttgctgagtttactgcagaagatgtgggtacatcagagagtggcttgaattccgtggtgctcgccaacaacgaggagactgtactcttaccaatgaatgagccagtctatggcaccaagcgtaaatctcaaattgagacatatttggagcacaatgaaggagctggacttcagcatctcgcgctgaagagtgaggacatcttccgcaccctacgggagatgaggaaaagaagtggtgttggtgggtttgaattcatgccatcacctcctgtcacctactacaggaacctgaagaacagagttggtgatgtactttcggacgagcagataaaggaatgtgaagagttggggattttggttgatagagatgatcaaggaacactcctgcagattgccacaaaaccaattggcgaccgccccactatctggatagagatcatccagagggtggggtgcatgctcaaagacgaggaagggaaggagtaccagaagggcggctgtggtggttttgggaaaggaaacttttctgagttattcaaatcaattgaagagtatgagaagacgcttgaaacgcgtcgcactgcttga

SEQ ID NO: 47 - protein, 436 aa, Gossypium hirsutum
  The amino acid sequence of Gossypium hirsutum wild-type HPPD (GsHPPD)
MVQTNQSGSGNDFKLVGFSNFVRSNPKSDRFTVKRFHHIEFWCTDATNVARRFSWGLGMQFVAKSDLSTGNLTHASYLLRSRDLNFLFTAPYSPSIAVAQNLSPQSTASIPSFDHSLCRSFAATHGLGVRAIAIEVDDAETAFTTSVTHGALPFCPPTPLGDVATIAEVKLYGDVVLRYVSYTTTINSDHDFLPGFEKIEDTLSYPLDYGLRRLDHAVGNVPELGPAVSYVKSFTGFHEFAEFTAEDVGTSESGLNSVVLANNEEMVLLPMNEPVFGTKRKSQIQTYLEHNEGAGVQHLALVSEDIFKTLREMRKRSFVGGFEFMPSPPPTYYKKLKQRAGDILSDEQIKECEELGILVDRDDQGTLLQIFTKPVGDRPTIFIEIIQRIGCMVKDEEGKQYQKGGCGGFGKGNFSELFKSIEEYEKSLEAKQSQNP

SEQ ID NO: 48 - DNA, 1311 bp, Gossypium hirsutum
  GsHPPD-01 Nucleotide Sequence
atggtccagacaaaccagtctggttccggcaatgatttcaagctcgtcggattctcgaatttcgtccggtcaaatccaaaatccgatcggttcaccgtcaaacgtttccaccacatcgagttttggtgtaccgacgccactaacgtcgctcgccgtttttcatggggtctcggtatgcaatttgtagctaaatcggatttatccaccggaaatttgacccatgcttcttatctcctccgttcccgtgacctgaacttccttttcactgccccctattccccttctattgccgttgctcaaaacctctcccctcaatccaccgcttcgatcccttcttttgatcattcactctgccgctccttcgctgccacccacggcttaggcgttcgcgccatcgccatcgaagttgacgatgccgaaaccgctttcaccaccagtgtcacacatggcgcgttacccttttgccctcctaccccactcggcgacgtcgccactatcgccgaagtcaaactctacggcgacgtcgttttgcgttacgtcagttacaccaccaccataaactccgaccatgatttcttgccgggattcgagaaaatagaagacaccctttcttaccctttagattacggactccgacgactcgaccacgccgtcggcaacgtcccagaactcggtcccgctgtttcgtacgttaaatccttcaccggcttccacgaattcgctgaattcacagctgaagacgtcggaactagcgaaagtggactaaactccgtcgttttagctaacaacgaagaaatggtattacttccgatgaacgaaccggtgttcggaacaaaaaggaaaagccaaatccaaacgtatttagaacacaacgaaggtgccggagttcaacatttggcattggtgagtgaagatatattcaagacgttaagagaaatgaggaagagaagcttcgtcggcggttttgagttcatgccgtcgccgccgccgacttattataaaaaattgaagcaaagggcaggggatattttgagtgatgaacagattaaagagtgtgaagaactggggattctggttgatagagatgatcaagggactttgctgcaaattttcactaagccagttggtgataggccaaccatcttcatagagataatacaaagaattgggtgcatggtgaaggatgaagaaggaaagcaataccaaaaaggtggatgtggtggttttgggaaaggcaacttttctgagctcttcaaatccattgaagaatatgagaaatctcttgaagccaaacaatctcagaatccatga

SEQ ID NO: 49 - DNA, 1311 bp, Artificial Sequence
  GsHPPD-02 Nucleotide Sequence
atggttcaaacaaatcaatctggttctgggaatgatttcaagctggttggtttctcaaattttgtgcgtagcaatcccaaatcagaccgcttcacggtcaagagattccaccacattgaattttggtgcactgatgccactaatgtggcgaggaggttttcatggggtttagggatgcagttcgtcgccaagagtgacctctccacaggaaatttgacgcatgcaagctacctgctgcggagccgcgacttgaatttcctgtttacagcaccatattcacccagtattgcagttgctcaaaacctttcgccacaaagcactgcttccataccttcatttgatcactcgctttgtcggtcctttgctgcaacacatggacttggcgtcagagcaattgccatcgaggtggacgacgccgaaactgccttcaccacgagcgtgacacatggcgcgctccctttttgtccaccaacaccactaggagatgtggctacaattgctgaagttaaattatatggtgatgttgtgctcagatatgtttcttacaccacaaccatcaactccgaccatgattttctgcctggttttgagaagattgaagatactctatcgtatcctttggattatggcctgcgtcggctcgatcatgctgttggcaacgtacctgaattaggtcctgctgtatcttatgtgaaatcttttactgggttccatgagtttgcagagttcaccgctgaggatgtaggaacaagtgaatctgggctgaactcagttgttttggccaacaatgaggaaatggtcctcttaccaatgaacgagccggtgttcggcactaagcgcaaatctcaaatacagacctacttggagcacaatgaaggagctggtgtgcagcacctcgccctcgtctcggaggacatcttcaaaactttaagggagatgaggaaacgatcctttgtgggaggatttgaattcatgccttctccgccgccgacatactacaagaagctcaagcagcgcgcgggggacattttgtctgatgagcagatcaaggagtgtgaagagcttgggattcttgttgatagagatgatcaaggaacgcttctgcagatatttaccaagcccgtcggcgaccggcctactatattcattgagatcatccagagaattggttgcatggtgaaggatgaagaagggaaacagtaccagaagggcggctgcggcgggtttggaaaaggaaacttcagtgagctgtttaaaagtatagaggagtatgaaaagagcttggaagcaaaacaatcacaaaatccatga

SEQ ID NO: 50 - protein, 436 aa, Artificial Sequence
  GsHPPDm-F372A Amino Acid Sequence
MVQTNQSGSGNDFKLVGFSNFVRSNPKSDRFTVKRFHHIEFWCTDATNVARRFSWGLGMQFVAKSDLSTGNLTHASYLLRSRDLNFLFTAPYSPSIAVAQNLSPQSTASIPSFDHSLCRSFAATHGLGVRAIAIEVDDAETAFTTSVTHGALPFCPPTPLGDVATIAEVKLYGDVVLRYVSYTTTINSDHDFLPGFEKIEDTLSYPLDYGLRRLDHAVGNVPELGPAVSYVKSFTGFHEFAEFTAEDVGTSESGLNSVVLANNEEMVLLPMNEPVFGTKRKSQIQTYLEHNEGAGVQHLALVSEDIFKTLREMRKRSFVGGFEFMPSPPPTYYKKLKQRAGDILSDEQIKECEELGILVDRDDQGTLLQIATKPVGDRPTIFIEIIQRIGCMVKDEEGKQYQKGGCGGFGKGNFSELFKSIEEYEKSLEAKQSQNP

SEQ ID NO: 51 - DNA, 1311 bp, Artificial Sequence
  GsHPPDm-F372A-01 Nucleotide Sequence
atggtccagacaaaccagtctggttccggcaatgatttcaagctcgtcggattctcgaatttcgtccggtcaaatccaaaatccgatcggttcaccgtcaaacgtttccaccacatcgagttttggtgtaccgacgccactaacgtcgctcgccgtttttcatggggtctcggtatgcaatttgtagctaaatcggatttatccaccggaaatttgacccatgcttcttatctcctccgttcccgtgacctgaacttccttttcactgccccctattccccttctattgccgttgctcaaaacctctcccctcaatccaccgcttcgatcccttcttttgatcattcactctgccgctccttcgctgccacccacggcttaggcgttcgcgccatcgccatcgaagttgacgatgccgaaaccgctttcaccaccagtgtcacacatggcgcgttacccttttgccctcctaccccactcggcgacgtcgccactatcgccgaagtcaaactctacggcgacgtcgttttgcgttacgtcagttacaccaccaccataaactccgaccatgatttcttgccgggattcgagaaaatagaagacaccctttcttaccctttagattacggactccgacgactcgaccacgccgtcggcaacgtcccagaactcggtcccgctgtttcgtacgttaaatccttcaccggcttccacgaattcgctgaattcacagctgaagacgtcggaactagcgaaagtggactaaactccgtcgttttagctaacaacgaagaaatggtattacttccgatgaacgaaccggtgttcggaacaaaaaggaaaagccaaatccaaacgtatttagaacacaacgaaggtgccggagttcaacatttggcattggtgagtgaagatatattcaagacgttaagagaaatgaggaagagaagcttcgtcggcggttttgagttcatgccgtcgccgccgccgacttattataaaaaattgaagcaaagggcaggggatattttgagtgatgaacagattaaagagtgtgaagaactggggattctggttgatagagatgatcaagggactttgctgcaaattgctactaagccagttggtgataggccaaccatcttcatagagataatacaaagaattgggtgcatggtgaaggatgaagaaggaaagcaataccaaaaaggtggatgtggtggttttgggaaaggcaacttttctgagctcttcaaatccattgaagaatatgagaaatctcttgaagccaaacaatctcagaatccatga

SEQ ID NO: 52 - DNA, 1311 bp, Artificial Sequence
  GsHPPDm-F372A-02 Nucleotide Sequence
atggttcaaacaaatcaatctggttctgggaatgatttcaagctggttggtttctcaaattttgtgcgtagcaatcccaaatcagaccgcttcacggtcaagagattccaccacattgaattttggtgcactgatgccactaatgtggcgaggaggttttcatggggtttagggatgcagttcgtcgccaagagtgacctctccacaggaaatttgacgcatgcaagctacctgctgcggagccgcgacttgaatttcctgtttacagcaccatattcacccagtattgcagttgctcaaaacctttcgccacaaagcactgcttccataccttcatttgatcactcgctttgtcggtcctttgctgcaacacatggacttggcgtcagagcaattgccatcgaggtggacgacgccgaaactgccttcaccacgagcgtgacacatggcgcgctccctttttgtccaccaacaccactaggagatgtggctacaattgctgaagttaaattatatggtgatgttgtgctcagatatgtttcttacaccacaaccatcaactccgaccatgattttctgcctggttttgagaagattgaagatactctatcgtatcctttggattatggcctgcgtcggctcgatcatgctgttggcaacgtacctgaattaggtcctgctgtatcttatgtgaaatcttttactgggttccatgagtttgcagagttcaccgctgaggatgtaggaacaagtgaatctgggctgaactcagttgttttggccaacaatgaggaaatggtcctcttaccaatgaacgagccggtgttcggcactaagcgcaaatctcaaatacagacctacttggagcacaatgaaggagctggtgtgcagcacctcgccctcgtctcggaggacatcttcaaaactttaagggagatgaggaaacgatcctttgtgggaggatttgaattcatgccttctccgccgccgacatactacaagaagctcaagcagcgcgcgggggacattttgtctgatgagcagatcaaggagtgtgaagagcttgggattcttgttgatagagatgatcaaggaacgcttctgcagatagccaccaagcccgtcggcgaccggcctactatattcattgagatcatccagagaattggttgcatggtgaaggatgaagaagggaaacagtaccagaagggcggctgcggcgggtttggaaaaggaaacttcagtgagctgtttaaaagtatagaggagtatgaaaagagcttggaagcaaaacaatcacaaaatccatga

SEQ ID NO: 53 - protein, 436 aa, Artificial Sequence
  GsHPPDm-F383W Amino Acid Sequence
MVQTNQSGSGNDFKLVGFSNFVRSNPKSDRFTVKRFHHIEFWCTDATNVARRFSWGLGMQFVAKSDLSTGNLTHASYLLRSRDLNFLFTAPYSPSIAVAQNLSPQSTASIPSFDHSLCRSFAATHGLGVRAIAIEVDDAETAFTTSVTHGALPFCPPTPLGDVATIAEVKLYGDVVLRYVSYTTTINSDHDFLPGFEKIEDTLSYPLDYGLRRLDHAVGNVPELGPAVSYVKSFTGFHEFAEFTAEDVGTSESGLNSVVLANNEEMVLLPMNEPVFGTKRKSQIQTYLEHNEGAGVQHLALVSEDIFKTLREMRKRSFVGGFEFMPSPPPTYYKKLKQRAGDILSDEQIKECEELGILVDRDDQGTLLQIFTKPVGDRPTIWIEIIQRIGCMVKDEEGKQYQKGGCGGFGKGNFSELFKSIEEYEKSLEAKQSQNP

SEQ ID NO: 54 - DNA, 1311 bp, Artificial Sequence
  GsHPPDm-F383W-01 Nucleotide Sequence
atggtccagacaaaccagtctggttccggcaatgatttcaagctcgtcggattctcgaatttcgtccggtcaaatccaaaatccgatcggttcaccgtcaaacgtttccaccacatcgagttttggtgtaccgacgccactaacgtcgctcgccgtttttcatggggtctcggtatgcaatttgtagctaaatcggatttatccaccggaaatttgacccatgcttcttatctcctccgttcccgtgacctgaacttccttttcactgccccctattccccttctattgccgttgctcaaaacctctcccctcaatccaccgcttcgatcccttcttttgatcattcactctgccgctccttcgctgccacccacggcttaggcgttcgcgccatcgccatcgaagttgacgatgccgaaaccgctttcaccaccagtgtcacacatggcgcgttacccttttgccctcctaccccactcggcgacgtcgccactatcgccgaagtcaaactctacggcgacgtcgttttgcgttacgtcagttacaccaccaccataaactccgaccatgatttcttgccgggattcgagaaaatagaagacaccctttcttaccctttagattacggactccgacgactcgaccacgccgtcggcaacgtcccagaactcggtcccgctgtttcgtacgttaaatccttcaccggcttccacgaattcgctgaattcacagctgaagacgtcggaactagcgaaagtggactaaactccgtcgttttagctaacaacgaagaaatggtattacttccgatgaacgaaccggtgttcggaacaaaaaggaaaagccaaatccaaacgtatttagaacacaacgaaggtgccggagttcaacatttggcattggtgagtgaagatatattcaagacgttaagagaaatgaggaagagaagcttcgtcggcggttttgagttcatgccgtcgccgccgccgacttattataaaaaattgaagcaaagggcaggggatattttgagtgatgaacagattaaagagtgtgaagaactggggattctggttgatagagatgatcaagggactttgctgcaaattttcactaagccagttggtgataggccaaccatctggatagagataatacaaagaattgggtgcatggtgaaggatgaagaaggaaagcaataccaaaaaggtggatgtggtggttttgggaaaggcaacttttctgagctcttcaaatccattgaagaatatgagaaatctcttgaagccaaacaatctcagaatccatga

SEQ ID NO: 55 - DNA, 1311 bp, Artificial Sequence
  GsHPPDm-F383W-02 Nucleotide Sequence
atggttcaaacaaatcaatctggttctgggaatgatttcaagctggttggtttctcaaattttgtgcgtagcaatcccaaatcagaccgcttcacggtcaagagattccaccacattgaattttggtgcactgatgccactaatgtggcgaggaggttttcatggggtttagggatgcagttcgtcgccaagagtgacctctccacaggaaatttgacgcatgcaagctacctgctgcggagccgcgacttgaatttcctgtttacagcaccatattcacccagtattgcagttgctcaaaacctttcgccacaaagcactgcttccataccttcatttgatcactcgctttgtcggtcctttgctgcaacacatggacttggcgtcagagcaattgccatcgaggtggacgacgccgaaactgccttcaccacgagcgtgacacatggcgcgctccctttttgtccaccaacaccactaggagatgtggctacaattgctgaagttaaattatatggtgatgttgtgctcagatatgtttcttacaccacaaccatcaactccgaccatgattttctgcctggttttgagaagattgaagatactctatcgtatcctttggattatggcctgcgtcggctcgatcatgctgttggcaacgtacctgaattaggtcctgctgtatcttatgtgaaatcttttactgggttccatgagtttgcagagttcaccgctgaggatgtaggaacaagtgaatctgggctgaactcagttgttttggccaacaatgaggaaatggtcctcttaccaatgaacgagccggtgttcggcactaagcgcaaatctcaaatacagacctacttggagcacaatgaaggagctggtgtgcagcacctcgccctcgtctcggaggacatcttcaaaactttaagggagatgaggaaacgatcctttgtgggaggatttgaattcatgccttctccgccgccgacatactacaagaagctcaagcagcgcgcgggggacattttgtctgatgagcagatcaaggagtgtgaagagcttgggattcttgttgatagagatgatcaaggaacgcttctgcagatatttaccaagcccgtcggcgaccggcctactatatggattgagatcatccagagaattggttgcatggtgaaggatgaagaagggaaacagtaccagaagggcggctgcggcgggtttggaaaaggaaacttcagtgagctgtttaaaagtatagaggagtatgaaaagagcttggaagcaaaacaatcacaaaatccatga

SEQ ID NO: 56 - protein, 436 aa, Artificial Sequence
  GsHPPDm-F372A-F383W Amino Acid Sequence
MVQTNQSGSGNDFKLVGFSNFVRSNPKSDRFTVKRFHHIEFWCTDATNVARRFSWGLGMQFVAKSDLSTGNLTHASYLLRSRDLNFLFTAPYSPSIAVAQNLSPQSTASIPSFDHSLCRSFAATHGLGVRAIAIEVDDAETAFTTSVTHGALPFCPPTPLGDVATIAEVKLYGDVVLRYVSYTTTINSDHDFLPGFEKIEDTLSYPLDYGLRRLDHAVGNVPELGPAVSYVKSFTGFHEFAEFTAEDVGTSESGLNSVVLANNEEMVLLPMNEPVFGTKRKSQIQTYLEHNEGAGVQHLALVSEDIFKTLREMRKRSFVGGFEFMPSPPPTYYKKLKQRAGDILSDEQIKECEELGILVDRDDQGTLLQIATKPVGDRPTIWIEIIQRIGCMVKDEEGKQYQKGGCGGFGKGNFSELFKSIEEYEKSLEAKQSQNP

SEQ ID NO: 57 - DNA, 1311 bp, Artificial Sequence
  GsHPPDm-F372A-F383W-01 Nucleotide Sequence
atggtccagacaaaccagtctggttccggcaatgatttcaagctcgtcggattctcgaatttcgtccggtcaaatccaaaatccgatcggttcaccgtcaaacgtttccaccacatcgagttttggtgtaccgacgccactaacgtcgctcgccgtttttcatggggtctcggtatgcaatttgtagctaaatcggatttatccaccggaaatttgacccatgcttcttatctcctccgttcccgtgacctgaacttccttttcactgccccctattccccttctattgccgttgctcaaaacctctcccctcaatccaccgcttcgatcccttcttttgatcattcactctgccgctccttcgctgccacccacggcttaggcgttcgcgccatcgccatcgaagttgacgatgccgaaaccgctttcaccaccagtgtcacacatggcgcgttacccttttgccctcctaccccactcggcgacgtcgccactatcgccgaagtcaaactctacggcgacgtcgttttgcgttacgtcagttacaccaccaccataaactccgaccatgatttcttgccgggattcgagaaaatagaagacaccctttcttaccctttagattacggactccgacgactcgaccacgccgtcggcaacgtcccagaactcggtcccgctgtttcgtacgttaaatccttcaccggcttccacgaattcgctgaattcacagctgaagacgtcggaactagcgaaagtggactaaactccgtcgttttagctaacaacgaagaaatggtattacttccgatgaacgaaccggtgttcggaacaaaaaggaaaagccaaatccaaacgtatttagaacacaacgaaggtgccggagttcaacatttggcattggtgagtgaagatatattcaagacgttaagagaaatgaggaagagaagcttcgtcggcggttttgagttcatgccgtcgccgccgccgacttattataaaaaattgaagcaaagggcaggggatattttgagtgatgaacagattaaagagtgtgaagaactggggattctggttgatagagatgatcaagggactttgctgcaaattgctactaagccagttggtgataggccaaccatctggatagagataatacaaagaattgggtgcatggtgaaggatgaagaaggaaagcaataccaaaaaggtggatgtggtggttttgggaaaggcaacttttctgagctcttcaaatccattgaagaatatgagaaatctcttgaagccaaacaatctcagaatccatga

SEQ ID NO: 58 - DNA, 1311 bp, Artificial Sequence
  GsHPPDm-F372A-F383W-02 Nucleotide Sequence
atggttcaaacaaatcaatctggttctgggaatgatttcaagctggttggtttctcaaattttgtgcgtagcaatcccaaatcagaccgcttcacggtcaagagattccaccacattgaattttggtgcactgatgccactaatgtggcgaggaggttttcatggggtttagggatgcagttcgtcgccaagagtgacctctccacaggaaatttgacgcatgcaagctacctgctgcggagccgcgacttgaatttcctgtttacagcaccatattcacccagtattgcagttgctcaaaacctttcgccacaaagcactgcttccataccttcatttgatcactcgctttgtcggtcctttgctgcaacacatggacttggcgtcagagcaattgccatcgaggtggacgacgccgaaactgccttcaccacgagcgtgacacatggcgcgctccctttttgtccaccaacaccactaggagatgtggctacaattgctgaagttaaattatatggtgatgttgtgctcagatatgtttcttacaccacaaccatcaactccgaccatgattttctgcctggttttgagaagattgaagatactctatcgtatcctttggattatggcctgcgtcggctcgatcatgctgttggcaacgtacctgaattaggtcctgctgtatcttatgtgaaatcttttactgggttccatgagtttgcagagttcaccgctgaggatgtaggaacaagtgaatctgggctgaactcagttgttttggccaacaatgaggaaatggtcctcttaccaatgaacgagccggtgttcggcactaagcgcaaatctcaaatacagacctacttggagcacaatgaaggagctggtgtgcagcacctcgccctcgtctcggaggacatcttcaaaactttaagggagatgaggaaacgatcctttgtgggaggatttgaattcatgccttctccgccgccgacatactacaagaagctcaagcagcgcgcgggggacattttgtctgatgagcagatcaaggagtgtgaagagcttgggattcttgttgatagagatgatcaaggaacgcttctgcagatagccaccaagcccgtcggcgaccggcctactatatggattgagatcatccagagaattggttgcatggtgaaggatgaagaagggaaacagtaccagaagggcggctgcggcgggtttggaaaaggaaacttcagtgagctgtttaaaagtatagaggagtatgaaaagagcttggaagcaaaacaatcacaaaatccatga

SEQ ID NO: 59 - protein, 440 aa, Brassica napus
  The amino acid sequence of Brassica napus wild-type HPPD (BnHPPD)
MGHENAAVCETQQHDDAASPGFKLVGFSKFVRKNPKSDKFKVKRFHHIEFWCGDATNVSRRFSWGLGMRFSAKSDLSTGNMVHASYLLTSGDLRFLFTAPYSPSLSAGEAQPSATASIPSFDHASCRSFFSSHGLGVRAVAIEVEDAESAFSISVANGAVPSSPPNVLNGAVTIAEVKLYGDVVLRYVSYYNGTVSFLPGFESVDDTSSFPLDYGIRRLDHAVGNVPELGPALTYLAGFTGFHQFAEFTADDVGTAESGLNSAVLANNDEMVLLPINEPVHGTKRKSQIQTFLEHNEGAGLQHLALMSEDIFRTLREMRKRSGVGGFDFMPSPPPTYYKNLKKRVGDVLSEEQIEECEELGILVDRDDQGTLLQIFTKPLGDRPTIFIEIIQRVGCMKRDEEGKVYQSGGCGGFGKGNFSELFKSIEEYEKTLEAKQLVG

SEQ ID NO: 60 - DNA, 1323 bp, Brassica napus
  BnHPPD-01 Nucleotide Sequence
atggggcacgaaaacgccgccgtttgcgaaactcagcagcacgacgacgctgcgtcgcctggattcaagctcgtcggattctccaagttcgtgaggaagaatccaaagtccgacaagttcaaggtaaagcgcttccaccacatcgagttctggtgcggggacgccaccaacgtctcccgccgcttctcgtggggactaggcatgcgattctccgccaaatccgatctctccaccggaaacatggttcacgcctcctacctactcacctccggcgacctccgattcctcttcaccgctccctactctccctctctctccgccggcgaagctcaaccgtccgctacagcctcaatcccatcgttcgatcacgcttcttgccgctccttcttctcttcgcacggactcggcgtgagagccgtagcgatcgaagtcgaagacgctgagtcagcattctcaatcagcgtagcaaacggcgccgttccttcctcccctcctaacgtcctcaacggagccgttacgatcgcggaagttaaactatacggagacgtcgtcctccgttacgttagttattataacggaaccgttagtttcctccccggatttgaatctgttgacgatacgtcgtcgtttccgctagattacggtatacgccgtctcgaccacgcggtgggaaacgtccccgagctcggcccagctttaacttacctcgcggggttcaccggcttccaccagttcgcggagttcactgcagacgacgtgggaacagccgagagcggattgaactcggctgtgctagccaacaacgacgagatggttctgttgccgataaacgagccggttcacgggacgaagaggaagagccagatccagacgtttcttgagcacaacgaaggagccgggctgcagcatttggctctgatgagcgaagatatattcaggacgctgagggagatgaggaagaggagcggcgttggagggttcgacttcatgccttctcctccgcctacttattacaagaatctcaagaaaagggttggagatgtgcttagtgaggagcagattgaggagtgtgaggagttggggattcttgtggatagagatgatcaggggacgttgcttcagatctttacgaaaccacttggtgacaggccgacgatatttatagagataatacagagagtgggatgcatgaagagagatgaggaagggaaggtttaccagagtggaggatgtggtgggtttggtaaaggtaacttctctgagctctttaagtctattgaagagtatgagaagacacttgaagccaaacagcttgtgggttga

SEQ ID NO: 61 - DNA, 1323 bp, Artificial Sequence
  BnHPPD-02 Nucleotide Sequence
atgggacatgaaaacgcggcagtgtgtgaaactcaacaacatgatgacgccgcctccccggggtttaaacttgtcgggttctcaaaatttgttaggaagaatccaaagtctgacaagttcaaggtgaaacgcttccaccacatcgagttctggtgcggggatgcaacaaatgtttcacgccgcttttcatggggactaggaatgaggtttagcgcaaagagtgatctctccactggtaatatggttcatgcgagctacttgctcacatctggagacctgagattcctcttcaccgcaccatattctccctccctgtcagctggtgaagctcagccttcagcaactgcaagtatcccttcgtttgatcatgcatcgtgcaggtctttcttcagttcacatggactcggcgtcagagcagtagcgatcgaagtagaggatgctgaatcagctttctccatatctgtcgccaacggcgcggtgccttcttctccaccaaacgtcttgaatggtgctgttaccattgctgaggtgaagctgtacggagatgttgttttaagatatgtttcatattacaatgggaccgtttcttttcttcccggctttgaatctgttgatgatacttcttccttccctcttgattatgggatcaggcggctggaccacgccgtcggcaacgtgccggagttaggtcctgctttgacatatcttgccggcttcactggattccatcaatttgcagagtttacggctgacgacgtggggaccgcggagagtgggctgaactcagcagtcttggccaacaatgatgaaatggtgctcctccccatcaatgaacctgtgcatggaacaaagagaaagtcgcagattcaaacatttttagagcacaatgagggagctgggctacagcacctcgcattgatgtcagaagatatttttcgaacgttgagggagatgcggaaacgatctggtgtaggcggctttgacttcatgccatcccctccgccaacctactacaagaacctgaagaagagggttggagacgtcctttccgaggagcaaattgaagaatgtgaggagcttggaattctggtggacagagatgatcaaggaacactacttcagatcttcacaaaaccattgggcgacaggccaacgatattcattgagatcattcagcgcgttggatgcatgaagcgtgatgaggaagggaaggtctaccagagtggcggttgtggtggatttggaaaaggaaatttttctgagctgttcaaaagcatagaagagtatgagaaaacattggaggccaagcagcttgttggttga

SEQ ID NO: 62 - protein, 440 aa, Artificial Sequence
  BnHPPDm-F372A Amino Acid Sequence
MGHENAAVCETQQHDDAASPGFKLVGFSKFVRKNPKSDKFKVKRFHHIEFWCGDATNVSRRFSWGLGMRFSAKSDLSTGNMVHASYLLTSGDLRFLFTAPYSPSLSAGEAQPSATASIPSFDHASCRSFFSSHGLGVRAVAIEVEDAESAFSISVANGAVPSSPPNVLNGAVTIAEVKLYGDVVLRYVSYYNGTVSFLPGFESVDDTSSFPLDYGIRRLDHAVGNVPELGPALTYLAGFTGFHQFAEFTADDVGTAESGLNSAVLANNDEMVLLPINEPVHGTKRKSQIQTFLEHNEGAGLQHLALMSEDIFRTLREMRKRSGVGGFDFMPSPPPTYYKNLKKRVGDVLSEEQIEECEELGILVDRDDQGTLLQIATKPLGDRPTIFIEIIQRVGCMKRDEEGKVYQSGGCGGFGKGNFSELFKSIEEYEKTLEAKQLVG

SEQ ID NO: 63 - DNA, 1323 bp, Artificial Sequence
  BnHPPDm-F372A-01 Nucleotide Sequence
atggggcacgaaaacgccgccgtttgcgaaactcagcagcacgacgacgctgcgtcgcctggattcaagctcgtcggattctccaagttcgtgaggaagaatccaaagtccgacaagttcaaggtaaagcgcttccaccacatcgagttctggtgcggggacgccaccaacgtctcccgccgcttctcgtggggactaggcatgcgattctccgccaaatccgatctctccaccggaaacatggttcacgcctcctacctactcacctccggcgacctccgattcctcttcaccgctccctactctccctctctctccgccggcgaagctcaaccgtccgctacagcctcaatcccatcgttcgatcacgcttcttgccgctccttcttctcttcgcacggactcggcgtgagagccgtagcgatcgaagtcgaagacgctgagtcagcattctcaatcagcgtagcaaacggcgccgttccttcctcccctcctaacgtcctcaacggagccgttacgatcgcggaagttaaactatacggagacgtcgtcctccgttacgttagttattataacggaaccgttagtttcctccccggatttgaatctgttgacgatacgtcgtcgtttccgctagattacggtatacgccgtctcgaccacgcggtgggaaacgtccccgagctcggcccagctttaacttacctcgcggggttcaccggcttccaccagttcgcggagttcactgcagacgacgtgggaacagccgagagcggattgaactcggctgtgctagccaacaacgacgagatggttctgttgccgataaacgagccggttcacgggacgaagaggaagagccagatccagacgtttcttgagcacaacgaaggagccgggctgcagcatttggctctgatgagcgaagatatattcaggacgctgagggagatgaggaagaggagcggcgttggagggttcgacttcatgccttctcctccgcctacttattacaagaatctcaagaaaagggttggagatgtgcttagtgaggagcagattgaggagtgtgaggagttggggattcttgtggatagagatgatcaggggacgttgcttcagatcgctacgaaaccacttggtgacaggccgacgatatttatagagataatacagagagtgggatgcatgaagagagatgaggaagggaaggtttaccagagtggaggatgtggtgggtttggtaaaggtaacttctctgagctctttaagtctattgaagagtatgagaagacacttgaagccaaacagcttgtgggttga

SEQ ID NO: 64 - DNA, 1323 bp, Artificial Sequence
  BnHPPDm-F372A-02 Nucleotide Sequence
atgggacatgaaaacgcggcagtgtgtgaaactcaacaacatgatgacgccgcctccccggggtttaaacttgtcgggttctcaaaatttgttaggaagaatccaaagtctgacaagttcaaggtgaaacgcttccaccacatcgagttctggtgcggggatgcaacaaatgtttcacgccgcttttcatggggactaggaatgaggtttagcgcaaagagtgatctctccactggtaatatggttcatgcgagctacttgctcacatctggagacctgagattcctcttcaccgcaccatattctccctccctgtcagctggtgaagctcagccttcagcaactgcaagtatcccttcgtttgatcatgcatcgtgcaggtctttcttcagttcacatggactcggcgtcagagcagtagcgatcgaagtagaggatgctgaatcagctttctccatatctgtcgccaacggcgcggtgccttcttctccaccaaacgtcttgaatggtgctgttaccattgctgaggtgaagctgtacggagatgttgttttaagatatgtttcatattacaatgggaccgtttcttttcttcccggctttgaatctgttgatgatacttcttccttccctcttgattatgggatcaggcggctggaccacgccgtcggcaacgtgccggagttaggtcctgctttgacatatcttgccggcttcactggattccatcaatttgcagagtttacggctgacgacgtggggaccgcggagagtgggctgaactcagcagtcttggccaacaatgatgaaatggtgctcctccccatcaatgaacctgtgcatggaacaaagagaaagtcgcagattcaaacatttttagagcacaatgagggagctgggctacagcacctcgcattgatgtcagaagatatttttcgaacgttgagggagatgcggaaacgatctggtgtaggcggctttgacttcatgccatcccctccgccaacctactacaagaacctgaagaagagggttggagacgtcctttccgaggagcaaattgaagaatgtgaggagcttggaattctggtggacagagatgatcaaggaacactacttcagatcgccacaaaaccattgggcgacaggccaacgatattcattgagatcattcagcgcgttggatgcatgaagcgtgatgaggaagggaaggtctaccagagtggcggttgtggtggatttggaaaaggaaatttttctgagctgttcaaaagcatagaagagtatgagaaaacattggaggccaagcagcttgttggttga

SEQ ID NO: 65 - protein, 440 aa, Artificial Sequence
  BnHPPDm-F383W Amino Acid Sequence
MGHENAAVCETQQHDDAASPGFKLVGFSKFVRKNPKSDKFKVKRFHHIEFWCGDATNVSRRFSWGLGMRFSAKSDLSTGNMVHASYLLTSGDLRFLFTAPYSPSLSAGEAQPSATASIPSFDHASCRSFFSSHGLGVRAVAIEVEDAESAFSISVANGAVPSSPPNVLNGAVTIAEVKLYGDVVLRYVSYYNGTVSFLPGFESVDDTSSFPLDYGIRRLDHAVGNVPELGPALTYLAGFTGFHQFAEFTADDVGTAESGLNSAVLANNDEMVLLPINEPVHGTKRKSQIQTFLEHNEGAGLQHLALMSEDIFRTLREMRKRSGVGGFDFMPSPPPTYYKNLKKRVGDVLSEEQIEECEELGILVDRDDQGTLLQIFTKPLGDRPTIWIEIIQRVGCMKRDEEGKVYQSGGCGGFGKGNFSELFKSIEEYEKTLEAKQLVG

SEQ ID NO: 66 - DNA, 1323 bp, Artificial Sequence
  BnHPPDm-F383W-01 Nucleotide Sequence
atggggcacgaaaacgccgccgtttgcgaaactcagcagcacgacgacgctgcgtcgcctggattcaagctcgtcggattctccaagttcgtgaggaagaatccaaagtccgacaagttcaaggtaaagcgcttccaccacatcgagttctggtgcggggacgccaccaacgtctcccgccgcttctcgtggggactaggcatgcgattctccgccaaatccgatctctccaccggaaacatggttcacgcctcctacctactcacctccggcgacctccgattcctcttcaccgctccctactctccctctctctccgccggcgaagctcaaccgtccgctacagcctcaatcccatcgttcgatcacgcttcttgccgctccttcttctcttcgcacggactcggcgtgagagccgtagcgatcgaagtcgaagacgctgagtcagcattctcaatcagcgtagcaaacggcgccgttccttcctcccctcctaacgtcctcaacggagccgttacgatcgcggaagttaaactatacggagacgtcgtcctccgttacgttagttattataacggaaccgttagtttcctccccggatttgaatctgttgacgatacgtcgtcgtttccgctagattacggtatacgccgtctcgaccacgcggtgggaaacgtccccgagctcggcccagctttaacttacctcgcggggttcaccggcttccaccagttcgcggagttcactgcagacgacgtgggaacagccgagagcggattgaactcggctgtgctagccaacaacgacgagatggttctgttgccgataaacgagccggttcacgggacgaagaggaagagccagatccagacgtttcttgagcacaacgaaggagccgggctgcagcatttggctctgatgagcgaagatatattcaggacgctgagggagatgaggaagaggagcggcgttggagggttcgacttcatgccttctcctccgcctacttattacaagaatctcaagaaaagggttggagatgtgcttagtgaggagcagattgaggagtgtgaggagttggggattcttgtggatagagatgatcaggggacgttgcttcagatctttacgaaaccacttggtgacaggccgacgatatggatagagataatacagagagtgggatgcatgaagagagatgaggaagggaaggtttaccagagtggaggatgtggtgggtttggtaaaggtaacttctctgagctctttaagtctattgaagagtatgagaagacacttgaagccaaacagcttgtgggttga

SEQ ID NO: 67 - DNA, 1323 bp, Artificial Sequence
  BnHPPDm-F383W-02 Nucleotide Sequence
atgggacatgaaaacgcggcagtgtgtgaaactcaacaacatgatgacgccgcctccccggggtttaaacttgtcgggttctcaaaatttgttaggaagaatccaaagtctgacaagttcaaggtgaaacgcttccaccacatcgagttctggtgcggggatgcaacaaatgtttcacgccgcttttcatggggactaggaatgaggtttagcgcaaagagtgatctctccactggtaatatggttcatgcgagctacttgctcacatctggagacctgagattcctcttcaccgcaccatattctccctccctgtcagctggtgaagctcagccttcagcaactgcaagtatcccttcgtttgatcatgcatcgtgcaggtctttcttcagttcacatggactcggcgtcagagcagtagcgatcgaagtagaggatgctgaatcagctttctccatatctgtcgccaacggcgcggtgccttcttctccaccaaacgtcttgaatggtgctgttaccattgctgaggtgaagctgtacggagatgttgttttaagatatgtttcatattacaatgggaccgtttcttttcttcccggctttgaatctgttgatgatacttcttccttccctcttgattatgggatcaggcggctggaccacgccgtcggcaacgtgccggagttaggtcctgctttgacatatcttgccggcttcactggattccatcaatttgcagagtttacggctgacgacgtggggaccgcggagagtgggctgaactcagcagtcttggccaacaatgatgaaatggtgctcctccccatcaatgaacctgtgcatggaacaaagagaaagtcgcagattcaaacatttttagagcacaatgagggagctgggctacagcacctcgcattgatgtcagaagatatttttcgaacgttgagggagatgcggaaacgatctggtgtaggcggctttgacttcatgccatcccctccgccaacctactacaagaacctgaagaagagggttggagacgtcctttccgaggagcaaattgaagaatgtgaggagcttggaattctggtggacagagatgatcaaggaacactacttcagatcttcacaaaaccattgggcgacaggccaacgatatggattgagatcattcagcgcgttggatgcatgaagcgtgatgaggaagggaaggtctaccagagtggcggttgtggtggatttggaaaaggaaatttttctgagctgttcaaaagcatagaagagtatgagaaaacattggaggccaagcagcttgttggttga

SEQ ID NO: 68 - protein, 440 aa, Artificial Sequence
  BnHPPDm-F372A-F383W Amino Acid Sequence
MGHENAAVCETQQHDDAASPGFKLVGFSKFVRKNPKSDKFKVKRFHHIEFWCGDATNVSRRFSWGLGMRFSAKSDLSTGNMVHASYLLTSGDLRFLFTAPYSPSLSAGEAQPSATASIPSFDHASCRSFFSSHGLGVRAVAIEVEDAESAFSISVANGAVPSSPPNVLNGAVTIAEVKLYGDVVLRYVSYYNGTVSFLPGFESVDDTSSFPLDYGIRRLDHAVGNVPELGPALTYLAGFTGFHQFAEFTADDVGTAESGLNSAVLANNDEMVLLPINEPVHGTKRKSQIQTFLEHNEGAGLQHLALMSEDIFRTLREMRKRSGVGGFDFMPSPPPTYYKNLKKRVGDVLSEEQIEECEELGILVDRDDQGTLLQIATKPLGDRPTIWIEIIQRVGCMKRDEEGKVYQSGGCGGFGKGNFSELFKSIEEYEKTLEAKQLVG

SEQ ID NO: 69 - DNA, 1323 bp, Artificial Sequence
  BnHPPDm-F372A-F383W-01 Nucleotide Sequence
atggggcacgaaaacgccgccgtttgcgaaactcagcagcacgacgacgctgcgtcgcctggattcaagctcgtcggattctccaagttcgtgaggaagaatccaaagtccgacaagttcaaggtaaagcgcttccaccacatcgagttctggtgcggggacgccaccaacgtctcccgccgcttctcgtggggactaggcatgcgattctccgccaaatccgatctctccaccggaaacatggttcacgcctcctacctactcacctccggcgacctccgattcctcttcaccgctccctactctccctctctctccgccggcgaagctcaaccgtccgctacagcctcaatcccatcgttcgatcacgcttcttgccgctccttcttctcttcgcacggactcggcgtgagagccgtagcgatcgaagtcgaagacgctgagtcagcattctcaatcagcgtagcaaacggcgccgttccttcctcccctcctaacgtcctcaacggagccgttacgatcgcggaagttaaactatacggagacgtcgtcctccgttacgttagttattataacggaaccgttagtttcctccccggatttgaatctgttgacgatacgtcgtcgtttccgctagattacggtatacgccgtctcgaccacgcggtgggaaacgtccccgagctcggcccagctttaacttacctcgcggggttcaccggcttccaccagttcgcggagttcactgcagacgacgtgggaacagccgagagcggattgaactcggctgtgctagccaacaacgacgagatggttctgttgccgataaacgagccggttcacgggacgaagaggaagagccagatccagacgtttcttgagcacaacgaaggagccgggctgcagcatttggctctgatgagcgaagatatattcaggacgctgagggagatgaggaagaggagcggcgttggagggttcgacttcatgccttctcctccgcctacttattacaagaatctcaagaaaagggttggagatgtgcttagtgaggagcagattgaggagtgtgaggagttggggattcttgtggatagagatgatcaggggacgttgcttcagatcgctacgaaaccacttggtgacaggccgacgatatggatagagataatacagagagtgggatgcatgaagagagatgaggaagggaaggtttaccagagtggaggatgtggtgggtttggtaaaggtaacttctctgagctctttaagtctattgaagagtatgagaagacacttgaagccaaacagcttgtgggttga

SEQ ID NO: 70 - DNA, 1323 bp, Artificial Sequence
  BnHPPDm-F372A-F383W-02 Nucleotide Sequence
atgggacatgaaaacgcggcagtgtgtgaaactcaacaacatgatgacgccgcctccccggggtttaaacttgtcgggttctcaaaatttgttaggaagaatccaaagtctgacaagttcaaggtgaaacgcttccaccacatcgagttctggtgcggggatgcaacaaatgtttcacgccgcttttcatggggactaggaatgaggtttagcgcaaagagtgatctctccactggtaatatggttcatgcgagctacttgctcacatctggagacctgagattcctcttcaccgcaccatattctccctccctgtcagctggtgaagctcagccttcagcaactgcaagtatcccttcgtttgatcatgcatcgtgcaggtctttcttcagttcacatggactcggcgtcagagcagtagcgatcgaagtagaggatgctgaatcagctttctccatatctgtcgccaacggcgcggtgccttcttctccaccaaacgtcttgaatggtgctgttaccattgctgaggtgaagctgtacggagatgttgttttaagatatgtttcatattacaatgggaccgtttcttttcttcccggctttgaatctgttgatgatacttcttccttccctcttgattatgggatcaggcggctggaccacgccgtcggcaacgtgccggagttaggtcctgctttgacatatcttgccggcttcactggattccatcaatttgcagagtttacggctgacgacgtggggaccgcggagagtgggctgaactcagcagtcttggccaacaatgatgaaatggtgctcctccccatcaatgaacctgtgcatggaacaaagagaaagtcgcagattcaaacatttttagagcacaatgagggagctgggctacagcacctcgcattgatgtcagaagatatttttcgaacgttgagggagatgcggaaacgatctggtgtaggcggctttgacttcatgccatcccctccgccaacctactacaagaacctgaagaagagggttggagacgtcctttccgaggagcaaattgaagaatgtgaggagcttggaattctggtggacagagatgatcaaggaacactacttcagatcgccacaaaaccattgggcgacaggccaacgatatggattgagatcattcagcgcgttggatgcatgaagcgtgatgaggaagggaaggtctaccagagtggcggttgtggtggatttggaaaaggaaatttttctgagctgttcaaaagcatagaagagtatgagaaaacattggaggccaagcagcttgttggttga

SEQ ID NO: 71 - protein, 488 aa, Glycine max
  The amino acid sequence of Glycine max wild-type HPPD (GmHPPD)
MPMYTPSLSAPSSNHIQPSVTLPLYITTTKLNLKQQHHTTPMPIPMCNEIQAQAQAQAQPGFKLVGFKNFVRTNPKSDRFQVNRFHHIEFWCTDATNASRRFSWGLGMPIVAKSDLSTGNQIHASYLLRSGDLSFLFSAPYSPSLSAGSSAASSASIPSFDAATCLAFAAKHGFGVRAIALEVADAEAAFSASVAKGAEPASPPVLVDDRTGFAEVRLYGDVVLRYVSYKDAAPQAPHADPSRWFLPGFEAAASSSSFPELDYGIRRLDHAVGNVPELAPAVRYLKGFSGFHEFAEFTAEDVGTSESGLNSVVLANNSETVLLPLNEPVYGTKRKSQIETYLEHNEGAGVQHLALVTHDIFTTLREMRKRSFLGGFEFMPSPPPTYYANLHNRAADVLTVDQIKQCEELGILVDRDDQGTLLQIFTKPVGDRPTIFIEIIQRIGCMVEDEEGKVYQKGACGGFGKGNFSELFKSIEEYEKTLEAKRTA

SEQ ID NO: 72 - DNA, 1467 bp, Glycine max
  GmHPPD-01 Nucleotide Sequence
atgcccatgtacactccatcactctccgcaccctcctccaatcacattcaaccaagtgtcacactccccttatatatcacaaccaccaagctcaatctcaagcagcagcatcacaccacaccaatgccaatacccatgtgcaacgaaattcaagcccaagcccaagcccaagcccaacctgggtttaagctcgtcggtttcaaaaacttcgtccgaaccaatcctaagtcggaccgctttcaagtcaaccgcttccaccacatcgagttctggtgcaccgatgccaccaacgcctctcgccgattctcttggggacttggaatgcctattgtggcaaaatctgatctctccaccggaaaccaaatccacgcctcctacctcctccgctccggcgacctctccttcctcttctccgctccttactctccctctctctccgccggctcctccgctgcctcctccgcctccattcccagtttcgacgccgccacctgccttgccttcgctgccaaacacggcttcggcgtccgcgccatcgccttggaagtcgccgacgcggaagccgctttcagcgccagcgtcgcgaaaggagccgagccggcgtcgccgccggttctcgtcgacgatcgcaccggcttcgcggaggtgcgcctctacggcgacgtggtgctccgctacgtcagctacaaggacgccgcgccgcaggcgccacacgcagatccgtcgcggtggttcctgccgggattcgaggccgcggcgtcgtcgtcttcgtttccggagctggactacgggatccggcggctggaccacgccgtcgggaacgttccggagctggcgccggcggtgaggtacctgaaaggcttcagcggattccacgagttcgcggagttcaccgcggaggacgtgggaacgagcgagagcgggttgaactcggtggttctggcgaacaactcggagacggtgttgctgccgctgaacgagccggtttacggaacgaagaggaagagccagattgagacgtatttggaacacaacgaaggtgctggtgtgcagcaccttgcgcttgttactcacgacatcttcaccacactgagagagatgagaaagcgaagtttccttggtggatttgagttcatgccttctcctcctcccacctattacgccaacctccacaaccgtgccgctgatgtgttgaccgttgaccagattaagcagtgtgaggagcttgggattcttgttgacagagatgatcagggcactctgcttcagattttcacyaagcctgttggggacaggccaacgatattcatagagataattcagaggatcgggtgcatggtggaggatgaggaagggaaggtgtaccagaagggtgcatgtgggggttttgggaaaggcaatttttctgagcttttcaaatccattgaagaatatgagaagactttggaagctaaaagaaccgcgtaa

SEQ ID NO: 73 - DNA, 1467 bp, Artificial Sequence
  GmHPPD-02 Nucleotide Sequence
atgccaatgtacacaccatcgctctccgccccttcttccaaccatattcagccatccgtgactctgcctctctacatcacaaccaccaagttgaacctgaagcagcagcaccatacgactcctatgcctatacccatgtgcaatgagatccaagcacaggctcaggcacaagctcaacccggattcaaactcgtgggattcaagaacttcgtccgtaccaatccaaaatctgaccgcttccaggtgaacagattccaccacatagagttttggtgtactgatgcaacgaatgcttcgaggaggttttcatggggcttaggcatgccgattgtagcaaagtcagacctttctacagggaaccaaattcatgcaagctatctgctccgctcaggtgatttgtctttcttgttctcagctccatattctccatcattatctgctgggtcatcagcagcatctagtgcgtcgatccctagctttgatgccgccacctgcctcgccttcgccgccaaacatggatttggtgttcgcgccattgctcttgaggttgccgatgccgaggctgcttttagcgcctccgtcgccaagggagctgagcctgcgtcacctcctgttcttgttgatgatcgaactggttttgctgaagtgcgtctttacggcgacgtggtgctcagatatgttagttacaaggatgctgctcctcaagcgccgcacgctgatccttcaagatggtttcttccggggtttgaggccgctgctagttcatcttccttcccggagttggattacggcatacggcggcttgaccatgctgtcggcaatgttcctgagcttgctccggcggtacggtacttgaaaggtttctccgggttccatgaatttgcagagttcacggcggaagatgttggaacaagtgaaagcggattgaattctgttgttttggccaacaacagtgaaactgttctgctccccctcaatgaaccagtttatggcacaaagcgcaagagccagattgaaacatatctcgagcacaatgaaggcgccggcgtccagcatcttgctttggtgactcatgatatcttcacaacacttagggagatgaggaagaggagtttcctcggcgggtttgaattcatgcccagtcccccgccgacctactatgcaaatctgcacaacagggctgcagatgtgctgactgtagaccagatcaagcaatgtgaagaacttggaattttagtggatagagacgaccaaggtacactacttcaaatattcaccaaaccagtcggtgacagaccaacaattttcatcgagattatacaaagaattggatgcatggtcgaggatgaagaagggaaggtgtaccagaagggagcatgtggtggttttgggaaaggaaatttttctgagctgtttaaatccatcgaggaatatgagaaaaccttagaagctaaaagaactgcatga

SEQ ID NO: 74 - protein, 488 aa, Artificial Sequence
  GmHPPDm-F372A Amino Acid Sequence
MPMYTPSLSAPSSNHIQPSVTLPLYITTTKLNLKQQHHTTPMPIPMCNEIQAQAQAQAQPGFKLVGFKNFVRTNPKSDRFQVNRFHHIEFWCTDATNASRRFSWGLGMPIVAKSDLSTGNQIHASYLLRSGDLSFLFSAPYSPSLSAGSSAASSASIPSFDAATCLAFAAKHGFGVRAIALEVADAEAAFSASVAKGAEPASPPVLVDDRTGFAEVRLYGDVVLRYVSYKDAAPQAPHADPSRWFLPGFEAAASSSSFPELDYGIRRLDHAVGNVPELAPAVRYLKGFSGFHEFAEFTAEDVGTSESGLNSVVLANNSETVLLPLNEPVYGTKRKSQIETYLEHNEGAGVQHLALVTHDIFTTLREMRKRSFLGGFEFMPSPPPTYYANLHNRAADVLTVDQIKQCEELGILVDRDDQGTLLQIATKPVGDRPTIFIEIIQRIGCMVEDEEGKVYQKGACGGFGKGNFSELFKSIEEYEKTLEAKRTA

SEQ ID NO: 75 - DNA, 1467 bp, Artificial Sequence
  GmHPPDm-F372A-01 Nucleotide Sequence
atgcccatgtacactccatcactctccgcaccctcctccaatcacattcaaccaagtgtcacactccccttatatatcacaaccaccaagctcaatctcaagcagcagcatcacaccacaccaatgccaatacccatgtgcaacgaaattcaagcccaagcccaagcccaagcccaacctgggtttaagctcgtcggtttcaaaaacttcgtccgaaccaatcctaagtcggaccgctttcaagtcaaccgcttccaccacatcgagttctggtgcaccgatgccaccaacgcctctcgccgattctcttggggacttggaatgcctattgtggcaaaatctgatctctccaccggaaaccaaatccacgcctcctacctcctccgctccggcgacctctccttcctcttctccgctccttactctccctctctctccgccggctcctccgctgcctcctccgcctccattcccagtttcgacgccgccacctgccttgccttcgctgccaaacacggcttcggcgtccgcgccatcgccttggaagtcgccgacgcggaagccgctttcagcgccagcgtcgcgaaaggagccgagccggcgtcgccgccggttctcgtcgacgatcgcaccggcttcgcggaggtgcgcctctacggcgacgtggtgctccgctacgtcagctacaaggacgccgcgccgcaggcgccacacgcagatccgtcgcggtggttcctgccgggattcgaggccgcggcgtcgtcgtcttcgtttccggagctggactacgggatccggcggctggaccacgccgtcgggaacgttccggagctggcgccggcggtgaggtacctgaaaggcttcagcggattccacgagttcgcggagttcaccgcggaggacgtgggaacgagcgagagcgggttgaactcggtggttctggcgaacaactcggagacggtgttgctgccgctgaacgagccggtttacggaacgaagaggaagagccagattgagacgtatttggaacacaacgaaggtgctggtgtgcagcaccttgcgcttgttactcacgacatcttcaccacactgagagagatgagaaagcgaagtttccttggtggatttgagttcatgccttctcctcctcccacctattacgccaacctccacaaccgtgccgctgatgtgttgaccgttgaccagattaagcagtgtgaggagcttgggattcttgttgacagagatgatcagggcactctgcttcagattgctacyaagcctgttggggacaggccaacgatattcatagagataattcagaggatcgggtgcatggtggaggatgaggaagggaaggtgtaccagaagggtgcatgtgggggttttgggaaaggcaatttttctgagcttttcaaatccattgaagaatatgagaagactttggaagctaaaagaaccgcgtaa

SEQ ID NO: 76 - DNA, 1467 bp, Artificial Sequence
  GmHPPDm-F372A-02 Nucleotide Sequence
atgccaatgtacacaccatcgctctccgccccttcttccaaccatattcagccatccgtgactctgcctctctacatcacaaccaccaagttgaacctgaagcagcagcaccatacgactcctatgcctatacccatgtgcaatgagatccaagcacaggctcaggcacaagctcaacccggattcaaactcgtgggattcaagaacttcgtccgtaccaatccaaaatctgaccgcttccaggtgaacagattccaccacatagagttttggtgtactgatgcaacgaatgcttcgaggaggttttcatggggcttaggcatgccgattgtagcaaagtcagacctttctacagggaaccaaattcatgcaagctatctgctccgctcaggtgatttgtctttcttgttctcagctccatattctccatcattatctgctgggtcatcagcagcatctagtgcgtcgatccctagctttgatgccgccacctgcctcgccttcgccgccaaacatggatttggtgttcgcgccattgctcttgaggttgccgatgccgaggctgcttttagcgcctccgtcgccaagggagctgagcctgcgtcacctcctgttcttgttgatgatcgaactggttttgctgaagtgcgtctttacggcgacgtggtgctcagatatgttagttacaaggatgctgctcctcaagcgccgcacgctgatccttcaagatggtttcttccggggtttgaggccgctgctagttcatcttccttcccggagttggattacggcatacggcggcttgaccatgctgtcggcaatgttcctgagcttgctccggcggtacggtacttgaaaggtttctccgggttccatgaatttgcagagttcacggcggaagatgttggaacaagtgaaagcggattgaattctgttgttttggccaacaacagtgaaactgttctgctccccctcaatgaaccagtttatggcacaaagcgcaagagccagattgaaacatatctcgagcacaatgaaggcgccggcgtccagcatcttgctttggtgactcatgatatcttcacaacacttagggagatgaggaagaggagtttcctcggcgggtttgaattcatgcccagtcccccgccgacctactatgcaaatctgcacaacagggctgcagatgtgctgactgtagaccagatcaagcaatgtgaagaacttggaattttagtggatagagacgaccaaggtacactacttcaaatagccaccaaaccagtcggtgacagaccaacaattttcatcgagattatacaaagaattggatgcatggtcgaggatgaagaagggaaggtgtaccagaagggagcatgtggtggttttgggaaaggaaatttttctgagctgtttaaatccatcgaggaatatgagaaaaccttagaagctaaaagaactgcatga

SEQ ID NO: 77 - protein, 488 aa, Artificial Sequence
  GmHPPDm-F383W Amino Acid Sequence
MPMYTPSLSAPSSNHIQPSVTLPLYITTTKLNLKQQHHTTPMPIPMCNEIQAQAQAQAQPGFKLVGFKNFVRTNPKSDRFQVNRFHHIEFWCTDATNASRRFSWGLGMPIVAKSDLSTGNQIHASYLLRSGDLSFLFSAPYSPSLSAGSSAASSASIPSFDAATCLAFAAKHGFGVRAIALEVADAEAAFSASVAKGAEPASPPVLVDDRTGFAEVRLYGDVVLRYVSYKDAAPQAPHADPSRWFLPGFEAAASSSSFPELDYGIRRLDHAVGNVPELAPAVRYLKGFSGFHEFAEFTAEDVGTSESGLNSVVLANNSETVLLPLNEPVYGTKRKSQIETYLEHNEGAGVQHLALVTHDIFTTLREMRKRSFLGGFEFMPSPPPTYYANLHNRAADVLTVDQIKQCEELGILVDRDDQGTLLQIFTKPVGDRPTIWIEIIQRIGCMVEDEEGKVYQKGACGGFGKGNFSELFKSIEEYEKTLEAKRTA

SEQ ID NO: 78 - DNA, 1467 bp, Artificial Sequence
  GmHPPDm-F383W-01 Nucleotide Sequence
atgcccatgtacactccatcactctccgcaccctcctccaatcacattcaaccaagtgtcacactccccttatatatcacaaccaccaagctcaatctcaagcagcagcatcacaccacaccaatgccaatacccatgtgcaacgaaattcaagcccaagcccaagcccaagcccaacctgggtttaagctcgtcggtttcaaaaacttcgtccgaaccaatcctaagtcggaccgctttcaagtcaaccgcttccaccacatcgagttctggtgcaccgatgccaccaacgcctctcgccgattctcttggggacttggaatgcctattgtggcaaaatctgatctctccaccggaaaccaaatccacgcctcctacctcctccgctccggcgacctctccttcctcttctccgctccttactctccctctctctccgccggctcctccgctgcctcctccgcctccattcccagtttcgacgccgccacctgccttgccttcgctgccaaacacggcttcggcgtccgcgccatcgccttggaagtcgccgacgcggaagccgctttcagcgccagcgtcgcgaaaggagccgagccggcgtcgccgccggttctcgtcgacgatcgcaccggcttcgcggaggtgcgcctctacggcgacgtggtgctccgctacgtcagctacaaggacgccgcgccgcaggcgccacacgcagatccgtcgcggtggttcctgccgggattcgaggccgcggcgtcgtcgtcttcgtttccggagctggactacgggatccggcggctggaccacgccgtcgggaacgttccggagctggcgccggcggtgaggtacctgaaaggcttcagcggattccacgagttcgcggagttcaccgcggaggacgtgggaacgagcgagagcgggttgaactcggtggttctggcgaacaactcggagacggtgttgctgccgctgaacgagccggtttacggaacgaagaggaagagccagattgagacgtatttggaacacaacgaaggtgctggtgtgcagcaccttgcgcttgttactcacgacatcttcaccacactgagagagatgagaaagcgaagtttccttggtggatttgagttcatgccttctcctcctcccacctattacgccaacctccacaaccgtgccgctgatgtgttgaccgttgaccagattaagcagtgtgaggagcttgggattcttgttgacagagatgatcagggcactctgcttcagattttcacyaagcctgttggggacaggccaacgatatggatagagataattcagaggatcgggtgcatggtggaggatgaggaagggaaggtgtaccagaagggtgcatgtgggggttttgggaaaggcaatttttctgagcttttcaaatccattgaagaatatgagaagactttggaagctaaaagaaccgcgtaa

SEQ ID NO: 79 - DNA, 1467 bp, Artificial Sequence
  GmHPPDm-F383W-02 Nucleotide Sequence
atgccaatgtacacaccatcgctctccgccccttcttccaaccatattcagccatccgtgactctgcctctctacatcacaaccaccaagttgaacctgaagcagcagcaccatacgactcctatgcctatacccatgtgcaatgagatccaagcacaggctcaggcacaagctcaacccggattcaaactcgtgggattcaagaacttcgtccgtaccaatccaaaatctgaccgcttccaggtgaacagattccaccacatagagttttggtgtactgatgcaacgaatgcttcgaggaggttttcatggggcttaggcatgccgattgtagcaaagtcagacctttctacagggaaccaaattcatgcaagctatctgctccgctcaggtgatttgtctttcttgttctcagctccatattctccatcattatctgctgggtcatcagcagcatctagtgcgtcgatccctagctttgatgccgccacctgcctcgccttcgccgccaaacatggatttggtgttcgcgccattgctcttgaggttgccgatgccgaggctgcttttagcgcctccgtcgccaagggagctgagcctgcgtcacctcctgttcttgttgatgatcgaactggttttgctgaagtgcgtctttacggcgacgtggtgctcagatatgttagttacaaggatgctgctcctcaagcgccgcacgctgatccttcaagatggtttcttccggggtttgaggccgctgctagttcatcttccttcccggagttggattacggcatacggcggcttgaccatgctgtcggcaatgttcctgagcttgctccggcggtacggtacttgaaaggtttctccgggttccatgaatttgcagagttcacggcggaagatgttggaacaagtgaaagcggattgaattctgttgttttggccaacaacagtgaaactgttctgctccccctcaatgaaccagtttatggcacaaagcgcaagagccagattgaaacatatctcgagcacaatgaaggcgccggcgtccagcatcttgctttggtgactcatgatatcttcacaacacttagggagatgaggaagaggagtttcctcggcgggtttgaattcatgcccagtcccccgccgacctactatgcaaatctgcacaacagggctgcagatgtgctgactgtagaccagatcaagcaatgtgaagaacttggaattttagtggatagagacgaccaaggtacactacttcaaatattcaccaaaccagtcggtgacagaccaacaatttggatcgagattatacaaagaattggatgcatggtcgaggatgaagaagggaaggtgtaccagaagggagcatgtggtggttttgggaaaggaaatttttctgagctgtttaaatccatcgaggaatatgagaaaaccttagaagctaaaagaactgcatga

SEQ ID NO: 80 - protein, 488 aa, Artificial Sequence
  GmHPPDm-F372A-F383W Amino Acid Sequence
MPMYTPSLSAPSSNHIQPSVTLPLYITTTKLNLKQQHHTTPMPIPMCNEIQAQAQAQAQPGFKLVGFKNFVRTNPKSDRFQVNRFHHIEFWCTDATNASRRFSWGLGMPIVAKSDLSTGNQIHASYLLRSGDLSFLFSAPYSPSLSAGSSAASSASIPSFDAATCLAFAAKHGFGVRAIALEVADAEAAFSASVAKGAEPASPPVLVDDRTGFAEVRLYGDVVLRYVSYKDAAPQAPHADPSRWFLPGFEAAASSSSFPELDYGIRRLDHAVGNVPELAPAVRYLKGFSGFHEFAEFTAEDVGTSESGLNSVVLANNSETVLLPLNEPVYGTKRKSQIETYLEHNEGAGVQHLALVTHDIFTTLREMRKRSFLGGFEFMPSPPPTYYANLHNRAADVLTVDQIKQCEELGILVDRDDQGTLLQIATKPVGDRPTIWIEIIQRIGCMVEDEEGKVYQKGACGGFGKGNFSELFKSIEEYEKTLEAKRTA

SEQ ID NO: 81 - DNA, 1467 bp, Artificial Sequence
  GmHPPDm-F372A-F383W-01 Nucleotide Sequence
atgcccatgtacactccatcactctccgcaccctcctccaatcacattcaaccaagtgtcacactccccttatatatcacaaccaccaagctcaatctcaagcagcagcatcacaccacaccaatgccaatacccatgtgcaacgaaattcaagcccaagcccaagcccaagcccaacctgggtttaagctcgtcggtttcaaaaacttcgtccgaaccaatcctaagtcggaccgctttcaagtcaaccgcttccaccacatcgagttctggtgcaccgatgccaccaacgcctctcgccgattctcttggggacttggaatgcctattgtggcaaaatctgatctctccaccggaaaccaaatccacgcctcctacctcctccgctccggcgacctctccttcctcttctccgctccttactctccctctctctccgccggctcctccgctgcctcctccgcctccattcccagtttcgacgccgccacctgccttgccttcgctgccaaacacggcttcggcgtccgcgccatcgccttggaagtcgccgacgcggaagccgctttcagcgccagcgtcgcgaaaggagccgagccggcgtcgccgccggttctcgtcgacgatcgcaccggcttcgcggaggtgcgcctctacggcgacgtggtgctccgctacgtcagctacaaggacgccgcgccgcaggcgccacacgcagatccgtcgcggtggttcctgccgggattcgaggccgcggcgtcgtcgtcttcgtttccggagctggactacgggatccggcggctggaccacgccgtcgggaacgttccggagctggcgccggcggtgaggtacctgaaaggcttcagcggattccacgagttcgcggagttcaccgcggaggacgtgggaacgagcgagagcgggttgaactcggtggttctggcgaacaactcggagacggtgttgctgccgctgaacgagccggtttacggaacgaagaggaagagccagattgagacgtatttggaacacaacgaaggtgctggtgtgcagcaccttgcgcttgttactcacgacatcttcaccacactgagagagatgagaaagcgaagtttccttggtggatttgagttcatgccttctcctcctcccacctattacgccaacctccacaaccgtgccgctgatgtgttgaccgttgaccagattaagcagtgtgaggagcttgggattcttgttgacagagatgatcagggcactctgcttcagattgctacyaagcctgttggggacaggccaacgatatggatagagataattcagaggatcgggtgcatggtggaggatgaggaagggaaggtgtaccagaagggtgcatgtgggggttttgggaaaggcaatttttctgagcttttcaaatccattgaagaatatgagaagactttggaagctaaaagaaccgcgtaa

SEQ ID NO: 82 - DNA, 1467 bp, Artificial Sequence
  GmHPPDm-F372A-F383W-02 Nucleotide Sequence
atgccaatgtacacaccatcgctctccgccccttcttccaaccatattcagccatccgtgactctgcctctctacatcacaaccaccaagttgaacctgaagcagcagcaccatacgactcctatgcctatacccatgtgcaatgagatccaagcacaggctcaggcacaagctcaacccggattcaaactcgtgggattcaagaacttcgtccgtaccaatccaaaatctgaccgcttccaggtgaacagattccaccacatagagttttggtgtactgatgcaacgaatgcttcgaggaggttttcatggggcttaggcatgccgattgtagcaaagtcagacctttctacagggaaccaaattcatgcaagctatctgctccgctcaggtgatttgtctttcttgttctcagctccatattctccatcattatctgctgggtcatcagcagcatctagtgcgtcgatccctagctttgatgccgccacctgcctcgccttcgccgccaaacatggatttggtgttcgcgccattgctcttgaggttgccgatgccgaggctgcttttagcgcctccgtcgccaagggagctgagcctgcgtcacctcctgttcttgttgatgatcgaactggttttgctgaagtgcgtctttacggcgacgtggtgctcagatatgttagttacaaggatgctgctcctcaagcgccgcacgctgatccttcaagatggtttcttccggggtttgaggccgctgctagttcatcttccttcccggagttggattacggcatacggcggcttgaccatgctgtcggcaatgttcctgagcttgctccggcggtacggtacttgaaaggtttctccgggttccatgaatttgcagagttcacggcggaagatgttggaacaagtgaaagcggattgaattctgttgttttggccaacaacagtgaaactgttctgctccccctcaatgaaccagtttatggcacaaagcgcaagagccagattgaaacatatctcgagcacaatgaaggcgccggcgtccagcatcttgctttggtgactcatgatatcttcacaacacttagggagatgaggaagaggagtttcctcggcgggtttgaattcatgcccagtcccccgccgacctactatgcaaatctgcacaacagggctgcagatgtgctgactgtagaccagatcaagcaatgtgaagaacttggaattttagtggatagagacgaccaaggtacactacttcaaatagccaccaaaccagtcggtgacagaccaacaatttggatcgagattatacaaagaattggatgcatggtcgaggatgaagaagggaaggtgtaccagaagggagcatgtggtggttttgggaaaggaaatttttctgagctgtttaaatccatcgaggaatatgagaaaaccttagaagctaaaagaactgcatga

SEQ ID NO: 83 - protein, 447 aa, Nicotiana tabacum
  The amino acid sequence of Nicotiana tabacum wild-type HPPD (NtHPPD)
MGKLETVTTTSAAAADDSSELTTNFKLVGFKNFIRTNPRSDFFSVKSFHHIEFWCGDATNTARRFSWSLGMPIAAKSDLSTGNSVHASYLLRPVSGSLQFLFTAPYSPSISTPSSAAIPSFSTSTHRSFTTTHGLGVRAVALEVENAYTAFSASVSRGAKPMFEPVTIDEQVAMAEVHLYGDVVLRFVSYLKDADNLVFLPGFEAMDETASYKELDYGIRRLDHAVGNVPELGPVVDYIKRFTGFHEFAEFTAEDVGTAESGLNSMVLANNDETVLLPLNEPVYGTKRKSQIQTYLEHNEGAGVQHLALVTEDIFKTLTEMRKRSGVGGFEFMPSPPPTYYKNLKNRAGDVLSDEQILACEELGILVDRDDQGTLLQIFTKPVGDRPTIFIEIIQRIGCMLKDGKGQVYQKGGCGGFGKGNFSELFRSIEEYEKTLEAKQANQVAAA

SEQ ID NO: 84 - DNA, 1344 bp, Nicotiana tabacum
  NtHPPD-01 Nucleotide Sequence
atgggcaaattagaaactgtcaccaccacctctgctgccgctgccgatgactcatcggagctgaccaccaatttcaagctagtgggtttcaagaattttattcgaaccaatccccgttccgattttttctccgttaaaagcttccatcacatagaattttggtgcggcgatgctaccaatacggctcgccgtttctcttggtctctcgggatgccaattgcagctaaatccgacctctccactggaaactccgttcacgcttcgtacctcctccgtcccgtttcaggttcgcttcagttcctcttcactgctccttattcgccgtctatttcgacgccgtcatctgcagccatccccagtttctctacttccacacaccgctcttttacgacaactcacgggctcggcgtccgtgccgttgctttggaagtggagaatgcttacacggcgttctctgcgagtgtttcacgtggggcgaaacccatgtttgaacctgtgactattgatgaacaagtcgctatggctgaagttcacttatacggcgacgtcgttttgcggtttgtgagctatctgaaagatgcggacaacctcgttttcctcccaggtttcgaggccatggatgaaacagcatcatacaaagaactagattatgggattcgccggctggaccatgctgttgggaatgtgccggagctgggtcctgtagtggattatatcaagcgctttacggggtttcatgaattcgccgagttcacagctgaagatgttgggactgctgagagcgggctgaactctatggtcctggcaaacaatgacgaaacagtgctgcttccgttgaatgagccggtttatggaaccaaaaggaagagtcaaattcaaacgtatttagagcacaatgaaggggcaggagtgcaacatttagctttggttacagaggatatatttaaaacattgacggaaatgaggaaaaggagtggagttgggggttttgaattcatgccttcacctccgcctacttattataagaatttgaagaatagggcaggggatgtactgagtgatgaacagattctggcttgcgaagaattgggaatattagtggatagggatgatcaggggaccctgctacagatattcaccaagcctgtgggggacaggccaacaatatttatagaaataattcagagaatcggttgcatgctcaaagacggaaaaggtcaggtgtatcagaagggcggctgtggaggcttcggaaagggaaacttttcagagctctttagatccatcgaagaatatgagaagacgcttgaagccaaacaagctaatcaagttgctgctgcttga

SEQ ID NO: 85 - DNA, 1344 bp, Artificial Sequence
  NtHPPD-02 Nucleotide Sequence
atggggaagctggaaaccgtcactaccacctcggcggcggctgctgatgattcatcggaattaacaaccaacttcaagttggttggtttcaaaaatttcatcagaacaaacccaaggtctgatttcttctccgtcaagagcttccaccacattgaattctggtgcggtgacgcaactaacacagcgcgccgcttctcatggagcctagggatgccaattgcagctaagagtgatctttcaacaggaaacagcgtgcacgcctcctacctcctccggcccgtaagcggttctttacagttcctgtttacagcaccatattcaccttctatttcgactcctagttcagctgcaatcccatctttttccacatctacacataggtctttcactacaacacatggactgggtgttcgtgccgtcgccctcgaggtggagaatgcttatactgccttcagtgcttctgtctccagaggcgccaagccaatgtttgaacctgtgacaattgatgaacaagtagcaatggctgaggttcatttgtacggcgatgttgtgctgcgatttgtttcttatctcaaggacgccgacaacctggtcttcctgccggggtttgaggccatggatgaaactgctagttacaaagaacttgattatggaatacggcgtttggatcatgctgtgggcaatgttccagaactcggcccggtagttgattacatcaagaggtttactggatttcatgaatttgcagagtttaccgctgaagatgtgggaactgcggaaagtgggctaaactccatggttcttgcgaacaatgatgagactgtgctcctccctctgaatgagcctgtttatggcaccaaaagaaaatctcagatacaaacatatcttgagcataatgaaggagctggggtgcagcaccttgctcttgttactgaagacatctttaagactttgacagagatgaggaagagaagtggagttggaggttttgagttcatgccttcccccccgccgacctactacaagaatttgaagaacagggctggtgacgtcctctcagacgagcagattttggcttgtgaggagcttggcatcttggtagaccgggacgaccaggggacgcttctccaaattttcacaaaacccgtcggggaccgccccaccatatttattgagatcatccagaggataggctgcatgcttaaagatggaaaaggtcaagtgtaccagaagggtggttgtggtgggtttggcaaaggaaatttttctgagctgttcagaagcatagaagaatatgagaagacactggaagcaaaacaagcaaatcaagttgcggccgcgtga

SEQ ID NO: 86 - protein, 447 aa, Artificial Sequence
  NtHPPDm-F372A Amino Acid Sequence
MGKLETVTTTSAAAADDSSELTTNFKLVGFKNFIRTNPRSDFFSVKSFHHIEFWCGDATNTARRFSWSLGMPIAAKSDLSTGNSVHASYLLRPVSGSLQFLFTAPYSPSISTPSSAAIPSFSTSTHRSFTTTHGLGVRAVALEVENAYTAFSASVSRGAKPMFEPVTIDEQVAMAEVHLYGDVVLRFVSYLKDADNLVFLPGFEAMDETASYKELDYGIRRLDHAVGNVPELGPVVDYIKRFTGFHEFAEFTAEDVGTAESGLNSMVLANNDETVLLPLNEPVYGTKRKSQIQTYLEHNEGAGVQHLALVTEDIFKTLTEMRKRSGVGGFEFMPSPPPTYYKNLKNRAGDVLSDEQILACEELGILVDRDDQGTLLQIATKPVGDRPTIFIEIIQRIGCMLKDGKGQVYQKGGCGGFGKGNFSELFRSIEEYEKTLEAKQANQVAAA

SEQ ID NO: 87 - DNA, 1344 bp, Artificial Sequence
  NtHPPDm-F372A-01 Nucleotide Sequence
atgggcaaattagaaactgtcaccaccacctctgctgccgctgccgatgactcatcggagctgaccaccaatttcaagctagtgggtttcaagaattttattcgaaccaatccccgttccgattttttctccgttaaaagcttccatcacatagaattttggtgcggcgatgctaccaatacggctcgccgtttctcttggtctctcgggatgccaattgcagctaaatccgacctctccactggaaactccgttcacgcttcgtacctcctccgtcccgtttcaggttcgcttcagttcctcttcactgctccttattcgccgtctatttcgacgccgtcatctgcagccatccccagtttctctacttccacacaccgctcttttacgacaactcacgggctcggcgtccgtgccgttgctttggaagtggagaatgcttacacggcgttctctgcgagtgtttcacgtggggcgaaacccatgtttgaacctgtgactattgatgaacaagtcgctatggctgaagttcacttatacggcgacgtcgttttgcggtttgtgagctatctgaaagatgcggacaacctcgttttcctcccaggtttcgaggccatggatgaaacagcatcatacaaagaactagattatgggattcgccggctggaccatgctgttgggaatgtgccggagctgggtcctgtagtggattatatcaagcgctttacggggtttcatgaattcgccgagttcacagctgaagatgttgggactgctgagagcgggctgaactctatggtcctggcaaacaatgacgaaacagtgctgcttccgttgaatgagccggtttatggaaccaaaaggaagagtcaaattcaaacgtatttagagcacaatgaaggggcaggagtgcaacatttagctttggttacagaggatatatttaaaacattgacggaaatgaggaaaaggagtggagttgggggttttgaattcatgccttcacctccgcctacttattataagaatttgaagaatagggcaggggatgtactgagtgatgaacagattctggcttgcgaagaattgggaatattagtggatagggatgatcaggggaccctgctacagatagctaccaagcctgtgggggacaggccaacaatatttatagaaataattcagagaatcggttgcatgctcaaagacggaaaaggtcaggtgtatcagaagggcggctgtggaggcttcggaaagggaaacttttcagagctctttagatccatcgaagaatatgagaagacgcttgaagccaaacaagctaatcaagttgctgctgcttga

SEQ ID NO: 88 - DNA, 1344 bp, Artificial Sequence
  NtHPPDm-F372A-02 Nucleotide Sequence
atggggaagctggaaaccgtcactaccacctcggcggcggctgctgatgattcatcggaattaacaaccaacttcaagttggttggtttcaaaaatttcatcagaacaaacccaaggtctgatttcttctccgtcaagagcttccaccacattgaattctggtgcggtgacgcaactaacacagcgcgccgcttctcatggagcctagggatgccaattgcagctaagagtgatctttcaacaggaaacagcgtgcacgcctcctacctcctccggcccgtaagcggttctttacagttcctgtttacagcaccatattcaccttctatttcgactcctagttcagctgcaatcccatctttttccacatctacacataggtctttcactacaacacatggactgggtgttcgtgccgtcgccctcgaggtggagaatgcttatactgccttcagtgcttctgtctccagaggcgccaagccaatgtttgaacctgtgacaattgatgaacaagtagcaatggctgaggttcatttgtacggcgatgttgtgctgcgatttgtttcttatctcaaggacgccgacaacctggtcttcctgccggggtttgaggccatggatgaaactgctagttacaaagaacttgattatggaatacggcgtttggatcatgctgtgggcaatgttccagaactcggcccggtagttgattacatcaagaggtttactggatttcatgaatttgcagagtttaccgctgaagatgtgggaactgcggaaagtgggctaaactccatggttcttgcgaacaatgatgagactgtgctcctccctctgaatgagcctgtttatggcaccaaaagaaaatctcagatacaaacatatcttgagcataatgaaggagctggggtgcagcaccttgctcttgttactgaagacatctttaagactttgacagagatgaggaagagaagtggagttggaggttttgagttcatgccttcccccccgccgacctactacaagaatttgaagaacagggctggtgacgtcctctcagacgagcagattttggcttgtgaggagcttggcatcttggtagaccgggacgaccaggggacgcttctccaaattgccacaaaacccgtcggggaccgccccaccatatttattgagatcatccagaggataggctgcatgcttaaagatggaaaaggtcaagtgtaccagaagggtggttgtggtgggtttggcaaaggaaatttttctgagctgttcagaagcatagaagaatatgagaagacactggaagcaaaacaagcaaatcaagttgcggccgcgtga

SEQ ID NO: 89 - protein, 447 aa, Artificial Sequence
  NtHPPDm-F383W Amino Acid Sequence
MGKLETVTTTSAAAADDSSELTTNFKLVGFKNFIRTNPRSDFFSVKSFHHIEFWCGDATNTARRFSWSLGMPIAAKSDLSTGNSVHASYLLRPVSGSLQFLFTAPYSPSISTPSSAAIPSFSTSTHRSFTTTHGLGVRAVALEVENAYTAFSASVSRGAKPMFEPVTIDEQVAMAEVHLYGDVVLRFVSYLKDADNLVFLPGFEAMDETASYKELDYGIRRLDHAVGNVPELGPVVDYIKRFTGFHEFAEFTAEDVGTAESGLNSMVLANNDETVLLPLNEPVYGTKRKSQIQTYLEHNEGAGVQHLALVTEDIFKTLTEMRKRSGVGGFEFMPSPPPTYYKNLKNRAGDVLSDEQILACEELGILVDRDDQGTLLQIFTKPVGDRPTIWIEIIQRIGCMLKDGKGQVYQKGGCGGFGKGNFSELFRSIEEYEKTLEAKQANQVAAA

SEQ ID NO: 90 - DNA, 1344 bp, Artificial Sequence
  NtHPPDm-F383W-01 Nucleotide Sequence
atgggcaaattagaaactgtcaccaccacctctgctgccgctgccgatgactcatcggagctgaccaccaatttcaagctagtgggtttcaagaattttattcgaaccaatccccgttccgattttttctccgttaaaagcttccatcacatagaattttggtgcggcgatgctaccaatacggctcgccgtttctcttggtctctcgggatgccaattgcagctaaatccgacctctccactggaaactccgttcacgcttcgtacctcctccgtcccgtttcaggttcgcttcagttcctcttcactgctccttattcgccgtctatttcgacgccgtcatctgcagccatccccagtttctctacttccacacaccgctcttttacgacaactcacgggctcggcgtccgtgccgttgctttggaagtggagaatgcttacacggcgttctctgcgagtgtttcacgtggggcgaaacccatgtttgaacctgtgactattgatgaacaagtcgctatggctgaagttcacttatacggcgacgtcgttttgcggtttgtgagctatctgaaagatgcggacaacctcgttttcctcccaggtttcgaggccatggatgaaacagcatcatacaaagaactagattatgggattcgccggctggaccatgctgttgggaatgtgccggagctgggtcctgtagtggattatatcaagcgctttacggggtttcatgaattcgccgagttcacagctgaagatgttgggactgctgagagcgggctgaactctatggtcctggcaaacaatgacgaaacagtgctgcttccgttgaatgagccggtttatggaaccaaaaggaagagtcaaattcaaacgtatttagagcacaatgaaggggcaggagtgcaacatttagctttggttacagaggatatatttaaaacattgacggaaatgaggaaaaggagtggagttgggggttttgaattcatgccttcacctccgcctacttattataagaatttgaagaatagggcaggggatgtactgagtgatgaacagattctggcttgcgaagaattgggaatattagtggatagggatgatcaggggaccctgctacagatattcaccaagcctgtgggggacaggccaacaatatggatagaaataattcagagaatcggttgcatgctcaaagacggaaaaggtcaggtgtatcagaagggcggctgtggaggcttcggaaagggaaacttttcagagctctttagatccatcgaagaatatgagaagacgcttgaagccaaacaagctaatcaagttgctgctgcttga

SEQ ID NO: 91 - DNA, 1344 bp, Artificial Sequence
  NtHPPDm-F383W-02 Nucleotide Sequence
atggggaagctggaaaccgtcactaccacctcggcggcggctgctgatgattcatcggaattaacaaccaacttcaagttggttggtttcaaaaatttcatcagaacaaacccaaggtctgatttcttctccgtcaagagcttccaccacattgaattctggtgcggtgacgcaactaacacagcgcgccgcttctcatggagcctagggatgccaattgcagctaagagtgatctttcaacaggaaacagcgtgcacgcctcctacctcctccggcccgtaagcggttctttacagttcctgtttacagcaccatattcaccttctatttcgactcctagttcagctgcaatcccatctttttccacatctacacataggtctttcactacaacacatggactgggtgttcgtgccgtcgccctcgaggtggagaatgcttatactgccttcagtgcttctgtctccagaggcgccaagccaatgtttgaacctgtgacaattgatgaacaagtagcaatggctgaggttcatttgtacggcgatgttgtgctgcgatttgtttcttatctcaaggacgccgacaacctggtcttcctgccggggtttgaggccatggatgaaactgctagttacaaagaacttgattatggaatacggcgtttggatcatgctgtgggcaatgttccagaactcggcccggtagttgattacatcaagaggtttactggatttcatgaatttgcagagtttaccgctgaagatgtgggaactgcggaaagtgggctaaactccatggttcttgcgaacaatgatgagactgtgctcctccctctgaatgagcctgtttatggcaccaaaagaaaatctcagatacaaacatatcttgagcataatgaaggagctggggtgcagcaccttgctcttgttactgaagacatctttaagactttgacagagatgaggaagagaagtggagttggaggttttgagttcatgccttcccccccgccgacctactacaagaatttgaagaacagggctggtgacgtcctctcagacgagcagattttggcttgtgaggagcttggcatcttggtagaccgggacgaccaggggacgcttctccaaattttcacaaaacccgtcggggaccgccccaccatatggattgagatcatccagaggataggctgcatgcttaaagatggaaaaggtcaagtgtaccagaagggtggttgtggtgggtttggcaaaggaaatttttctgagctgttcagaagcatagaagaatatgagaagacactggaagcaaaacaagcaaatcaagttgcggccgcgtga

SEQ ID NO: 92 - protein, 447 aa, Artificial Sequence
  NtHPPDm-F372A-F383W Amino Acid Sequence
MGKLETVTTTSAAAADDSSELTTNFKLVGFKNFIRTNPRSDFFSVKSFHHIEFWCGDATNTARRFSWSLGMPIAAKSDLSTGNSVHASYLLRPVSGSLQFLFTAPYSPSISTPSSAAIPSFSTSTHRSFTTTHGLGVRAVALEVENAYTAFSASVSRGAKPMFEPVTIDEQVAMAEVHLYGDVVLRFVSYLKDADNLVFLPGFEAMDETASYKELDYGIRRLDHAVGNVPELGPVVDYIKRFTGFHEFAEFTAEDVGTAESGLNSMVLANNDETVLLPLNEPVYGTKRKSQIQTYLEHNEGAGVQHLALVTEDIFKTLTEMRKRSGVGGFEFMPSPPPTYYKNLKNRAGDVLSDEQILACEELGILVDRDDQGTLLQIATKPVGDRPTIWIEIIQRIGCMLKDGKGQVYQKGGCGGFGKGNFSELFRSIEEYEKTLEAKQANQVAAA

SEQ ID NO: 93 - DNA, 1344 bp, Artificial Sequence
  NtHPPDm-F372A-F383W-01 Nucleotide Sequence
atgggcaaattagaaactgtcaccaccacctctgctgccgctgccgatgactcatcggagctgaccaccaatttcaagctagtgggtttcaagaattttattcgaaccaatccccgttccgattttttctccgttaaaagcttccatcacatagaattttggtgcggcgatgctaccaatacggctcgccgtttctcttggtctctcgggatgccaattgcagctaaatccgacctctccactggaaactccgttcacgcttcgtacctcctccgtcccgtttcaggttcgcttcagttcctcttcactgctccttattcgccgtctatttcgacgccgtcatctgcagccatccccagtttctctacttccacacaccgctcttttacgacaactcacgggctcggcgtccgtgccgttgctttggaagtggagaatgcttacacggcgttctctgcgagtgtttcacgtggggcgaaacccatgtttgaacctgtgactattgatgaacaagtcgctatggctgaagttcacttatacggcgacgtcgttttgcggtttgtgagctatctgaaagatgcggacaacctcgttttcctcccaggtttcgaggccatggatgaaacagcatcatacaaagaactagattatgggattcgccggctggaccatgctgttgggaatgtgccggagctgggtcctgtagtggattatatcaagcgctttacggggtttcatgaattcgccgagttcacagctgaagatgttgggactgctgagagcgggctgaactctatggtcctggcaaacaatgacgaaacagtgctgcttccgttgaatgagccggtttatggaaccaaaaggaagagtcaaattcaaacgtatttagagcacaatgaaggggcaggagtgcaacatttagctttggttacagaggatatatttaaaacattgacggaaatgaggaaaaggagtggagttgggggttttgaattcatgccttcacctccgcctacttattataagaatttgaagaatagggcaggggatgtactgagtgatgaacagattctggcttgcgaagaattgggaatattagtggatagggatgatcaggggaccctgctacagatagctaccaagcctgtgggggacaggccaacaatatggatagaaataattcagagaatcggttgcatgctcaaagacggaaaaggtcaggtgtatcagaagggcggctgtggaggcttcggaaagggaaacttttcagagctctttagatccatcgaagaatatgagaagacgcttgaagccaaacaagctaatcaagttgctgctgcttga

SEQ ID NO: 94 - DNA, 1344 bp, Artificial Sequence
  NtHPPDm-F372A-F383W-02 Nucleotide Sequence
atggggaagctggaaaccgtcactaccacctcggcggcggctgctgatgattcatcggaattaacaaccaacttcaagttggttggtttcaaaaatttcatcagaacaaacccaaggtctgatttcttctccgtcaagagcttccaccacattgaattctggtgcggtgacgcaactaacacagcgcgccgcttctcatggagcctagggatgccaattgcagctaagagtgatctttcaacaggaaacagcgtgcacgcctcctacctcctccggcccgtaagcggttctttacagttcctgtttacagcaccatattcaccttctatttcgactcctagttcagctgcaatcccatctttttccacatctacacataggtctttcactacaacacatggactgggtgttcgtgccgtcgccctcgaggtggagaatgcttatactgccttcagtgcttctgtctccagaggcgccaagccaatgtttgaacctgtgacaattgatgaacaagtagcaatggctgaggttcatttgtacggcgatgttgtgctgcgatttgtttcttatctcaaggacgccgacaacctggtcttcctgccggggtttgaggccatggatgaaactgctagttacaaagaacttgattatggaatacggcgtttggatcatgctgtgggcaatgttccagaactcggcccggtagttgattacatcaagaggtttactggatttcatgaatttgcagagtttaccgctgaagatgtgggaactgcggaaagtgggctaaactccatggttcttgcgaacaatgatgagactgtgctcctccctctgaatgagcctgtttatggcaccaaaagaaaatctcagatacaaacatatcttgagcataatgaaggagctggggtgcagcaccttgctcttgttactgaagacatctttaagactttgacagagatgaggaagagaagtggagttggaggttttgagttcatgccttcccccccgccgacctactacaagaatttgaagaacagggctggtgacgtcctctcagacgagcagattttggcttgtgaggagcttggcatcttggtagaccgggacgaccaggggacgcttctccaaattgccacaaaacccgtcggggaccgccccaccatatggattgagatcatccagaggataggctgcatgcttaaagatggaaaaggtcaagtgtaccagaagggtggttgtggtgggtttggcaaaggaaatttttctgagctgttcagaagcatagaagaatatgagaagacactggaagcaaaacaagcaaatcaagttgcggccgcgtga

SEQ ID NO: 95 - protein, 446 aa, Oryza sativa
  The amino acid sequence of Oryza sativa wild-type HPPD (OsHPPD)
MPPTPTPTATTGAVSAAAAAGENAGFRLVGHRRFVRANPRSDRFQALAFHHVELWCADAASAAGRFAFALGAPLAARSDLSTGNSAHASLLLRSASVAFLFTAPYGGDHGVGADAATTASIPSFSPGAARRFAADHGLAVHAVALRVADAADAFRASVAAGARPAFQPADLGGGFGLAEVELYGDVVLRFVSHPDGADAPFLPGFEGVSNPGAVDYGLRRFDHVVGNVPELAPVAAYISGFTGFHEFAEFTAEDVGTAESGLNSVVLANNAETVLLPLNEPVHGTKRRSQIQTYLDHHGGPGVQHIALASDDVLGTLREMRARSAMGGFEFLAPPPPNYYDGVRRRAGDVLSEEQINECQELGVLVDRDDQGVLLQIFTKPVGDRPTFFLEMIQRIGCMEKDESGQEYQKGGCGGFGKGNFSELFKSIEEYEKSLEAKQAPTVQGS

SEQ ID NO: 96 - DNA, 1341 bp, Oryza sativa
  OsHPPD-01 Nucleotide Sequence
atgcctcccactcccacccccaccgccaccaccggcgccgtctcggccgctgcggcggcgggggagaacgcggggttccgcctcgtcgggcaccgccgcttcgtccgcgccaacccgcggagcgaccggttccaggcgctcgcgttccaccacgtcgagctctggtgcgccgacgccgcgtccgccgcgggccggttcgccttcgccctgggcgcgccgctcgccgccaggtccgacctctccacggggaactccgcgcacgcctccctcctcctccgctccgcctccgtcgcgttcctcttcaccgccccctacggcggcgaccacggcgtcggcgcggacgcggccaccaccgcctccatcccttccttctccccaggcgccgcgcggaggttcgccgcggaccacggcctcgcggtgcacgccgtggcgctgcgcgtcgccgacgcggccgacgccttccgcgccagcgtcgcggccggtgcgcgcccggcgttccagcccgccgacctcggcggtggcttcggcctcgcggaggtggagctctacggcgacgtcgtgctccgcttcgtcagccacccggacggcgccgacgcgcccttcctcccgggtttcgagggcgtcagcaacccgggcgccgtggactacggcctccgccggttcgaccacgtcgtcggcaacgtgccggagctcgctccggtagccgcgtacatctccgggttcaccgggttccacgagttcgccgagttcaccgccgaggacgtgggcaccgccgagagcggcctcaactcggtggtgctcgccaacaacgcggagaccgtgctgctgccgctcaacgagccggtgcacggcaccaagcggcggagccagatacagacgtacctggaccaccacggcggcccgggggtgcagcacatcgcgctggccagcgacgacgtgctcgggacgctgagggagatgcgggcgcgctccgccatgggcggcttcgagttcttggcgccgccgccgcccaactactacgacggcgtgcggcggcgcgccggggacgtgctctcggaggagcagatcaacgagtgccaggagctcggggtgctcgtggacagggatgaccagggggtgttgctccagatcttcaccaagccagtaggagacaggccaacctttttcttggagatgatacaaaggattgggtgcatggagaaggatgagagtgggcaggagtaccagaagggcggctgcggcgggtttgggaagggcaacttctcggagctgttcaagtccattgaggagtatgagaaatcccttgaagccaagcaagcccctacagttcaaggatcctag

SEQ ID NO: 97 - DNA, 1341 bp, Artificial Sequence
  OsHPPD-02 Nucleotide Sequence
atgccacccacgccaacaccaacggccaccactggtgccgtctcggccgcggcagcggccggtgagaatgctggtttcaggctagtcggccaccgccgcttcgtgagggcaaatccaagatctgatcggttccaagcacttgctttccaccatgttgagctgtggtgcgctgacgccgcttcagctgccgggaggtttgcttttgctttaggggcgccgctcgccgcaaggagtgatctttccaccggaaattctgctcatgcttctcttctacttagatcagcaagtgttgcatttctgttcactgcaccttatggcggagaccatggtgtcggggccgatgctgcaacaacagctagcataccatcattttctcccggcgccgcaagaagatttgcagccgatcatggcctggcagttcatgctgtggcattgagggtcgccgacgcggctgatgcgttccgcgccagcgtggctgctggagctaggccggcgttccagcctgctgaccttgggggtggatttggattggcggaggttgaattatatggtgatgttgtgctccgttttgtttcccatccagatggtgctgatgctccatttctacctggatttgaaggggtgtcaaaccccggcgcggtggattatggactgcgtcgatttgatcacgtggtaggtaatgttcctgagttggctcccgtggcggcctacatttcaggctttactggcttccatgaatttgccgagttcaccgcggaagatgtgggaactgctgaaagtggattgaactctgttgtcctggcgaacaatgcagagactgtattgctccccttgaatgagcctgtgcacggcaccaaacggcgatctcaaattcagacatacctcgaccaccacgggggccctggtgttcagcatattgctctagccagcgacgacgtactgggaacactgagggagatgagagcccgttccgccatgggtggctttgagtttctggcccctccgccgccaaactactacgacggcgtcagacggcgggcgggtgacgtcttgagtgaggagcagatcaatgaatgtcaagaacttggggttcttgttgatagagatgatcaaggagtgctcctccaaatattcacaaaacctgttggcgaccgcccgaccttcttccttgaaatgatccaaaggatcggctgcatggagaaggatgaatcgggccaggagtaccagaagggtgggtgtggtggctttgggaagggcaacttcagcgagctgttcaagtcaattgaagaatatgaaaaatcattggaggcaaagcaagctccgacggtgcagggaagctga

SEQ ID NO: 98 - protein, 446 aa, Artificial Sequence
  OsHPPDm-F372A Amino Acid Sequence
MPPTPTPTATTGAVSAAAAAGENAGFRLVGHRRFVRANPRSDRFQALAFHHVELWCADAASAAGRFAFALGAPLAARSDLSTGNSAHASLLLRSASVAFLFTAPYGGDHGVGADAATTASIPSFSPGAARRFAADHGLAVHAVALRVADAADAFRASVAAGARPAFQPADLGGGFGLAEVELYGDVVLRFVSHPDGADAPFLPGFEGVSNPGAVDYGLRRFDHVVGNVPELAPVAAYISGFTGFHEFAEFTAEDVGTAESGLNSVVLANNAETVLLPLNEPVHGTKRRSQIQTYLDHHGGPGVQHIALASDDVLGTLREMRARSAMGGFEFLAPPPPNYYDGVRRRAGDVLSEEQINECQELGVLVDRDDQGVLLQIATKPVGDRPTFFLEMIQRIGCMEKDESGQEYQKGGCGGFGKGNFSELFKSIEEYEKSLEAKQAPTVQGS

SEQ ID NO: 99 - DNA, 1341 bp, Artificial Sequence
  OsHPPDm-F372A-01 Nucleotide Sequence
atgcctcccactcccacccccaccgccaccaccggcgccgtctcggccgctgcggcggcgggggagaacgcggggttccgcctcgtcgggcaccgccgcttcgtccgcgccaacccgcggagcgaccggttccaggcgctcgcgttccaccacgtcgagctctggtgcgccgacgccgcgtccgccgcgggccggttcgccttcgccctgggcgcgccgctcgccgccaggtccgacctctccacggggaactccgcgcacgcctccctcctcctccgctccgcctccgtcgcgttcctcttcaccgccccctacggcggcgaccacggcgtcggcgcggacgcggccaccaccgcctccatcccttccttctccccaggcgccgcgcggaggttcgccgcggaccacggcctcgcggtgcacgccgtggcgctgcgcgtcgccgacgcggccgacgccttccgcgccagcgtcgcggccggtgcgcgcccggcgttccagcccgccgacctcggcggtggcttcggcctcgcggaggtggagctctacggcgacgtcgtgctccgcttcgtcagccacccggacggcgccgacgcgcccttcctcccgggtttcgagggcgtcagcaacccgggcgccgtggactacggcctccgccggttcgaccacgtcgtcggcaacgtgccggagctcgctccggtagccgcgtacatctccgggttcaccgggttccacgagttcgccgagttcaccgccgaggacgtgggcaccgccgagagcggcctcaactcggtggtgctcgccaacaacgcggagaccgtgctgctgccgctcaacgagccggtgcacggcaccaagcggcggagccagatacagacgtacctggaccaccacggcggcccgggggtgcagcacatcgcgctggccagcgacgacgtgctcgggacgctgagggagatgcgggcgcgctccgccatgggcggcttcgagttcttggcgccgccgccgcccaactactacgacggcgtgcggcggcgcgccggggacgtgctctcggaggagcagatcaacgagtgccaggagctcggggtgctcgtggacagggatgaccagggggtgttgctccagatcgctaccaagccagtaggagacaggccaacctttttcttggagatgatacaaaggattgggtgcatggagaaggatgagagtgggcaggagtaccagaagggcggctgcggcgggtttgggaagggcaacttctcggagctgttcaagtccattgaggagtatgagaaatcccttgaagccaagcaagcccctacagttcaaggatcctag

SEQ ID NO: 100 - DNA, 1341 bp, Artificial Sequence
  OsHPPDm-F372A-02 Nucleotide Sequence
atgccacccacgccaacaccaacggccaccactggtgccgtctcggccgcggcagcggccggtgagaatgctggtttcaggctagtcggccaccgccgcttcgtgagggcaaatccaagatctgatcggttccaagcacttgctttccaccatgttgagctgtggtgcgctgacgccgcttcagctgccgggaggtttgcttttgctttaggggcgccgctcgccgcaaggagtgatctttccaccggaaattctgctcatgcttctcttctacttagatcagcaagtgttgcatttctgttcactgcaccttatggcggagaccatggtgtcggggccgatgctgcaacaacagctagcataccatcattttctcccggcgccgcaagaagatttgcagccgatcatggcctggcagttcatgctgtggcattgagggtcgccgacgcggctgatgcgttccgcgccagcgtggctgctggagctaggccggcgttccagcctgctgaccttgggggtggatttggattggcggaggttgaattatatggtgatgttgtgctccgttttgtttcccatccagatggtgctgatgctccatttctacctggatttgaaggggtgtcaaaccccggcgcggtggattatggactgcgtcgatttgatcacgtggtaggtaatgttcctgagttggctcccgtggcggcctacatttcaggctttactggcttccatgaatttgccgagttcaccgcggaagatgtgggaactgctgaaagtggattgaactctgttgtcctggcgaacaatgcagagactgtattgctccccttgaatgagcctgtgcacggcaccaaacggcgatctcaaattcagacatacctcgaccaccacgggggccctggtgttcagcatattgctctagccagcgacgacgtactgggaacactgagggagatgagagcccgttccgccatgggtggctttgagtttctggcccctccgccgccaaactactacgacggcgtcagacggcgggcgggtgacgtcttgagtgaggagcagatcaatgaatgtcaagaacttggggttcttgttgatagagatgatcaaggagtgctcctccaaatagccacaaaacctgttggcgaccgcccgaccttcttccttgaaatgatccaaaggatcggctgcatggagaaggatgaatcgggccaggagtaccagaagggtgggtgtggtggctttgggaagggcaacttcagcgagctgttcaagtcaattgaagaatatgaaaaatcattggaggcaaagcaagctccgacggtgcagggaagctga

SEQ ID NO: 101 - protein, 446 aa, Artificial Sequence
  OsHPPDm-F383W Amino Acid Sequence
MPPTPTPTATTGAVSAAAAAGENAGFRLVGHRRFVRANPRSDRFQALAFHHVELWCADAASAAGRFAFALGAPLAARSDLSTGNSAHASLLLRSASVAFLFTAPYGGDHGVGADAATTASIPSFSPGAARRFAADHGLAVHAVALRVADAADAFRASVAAGARPAFQPADLGGGFGLAEVELYGDVVLRFVSHPDGADAPFLPGFEGVSNPGAVDYGLRRFDHVVGNVPELAPVAAYISGFTGFHEFAEFTAEDVGTAESGLNSVVLANNAETVLLPLNEPVHGTKRRSQIQTYLDHHGGPGVQHIALASDDVLGTLREMRARSAMGGFEFLAPPPPNYYDGVRRRAGDVLSEEQINECQELGVLVDRDDQGVLLQIFTKPVGDRPTFWLEMIQRIGCMEKDESGQEYQKGGCGGFGKGNFSELFKSIEEYEKSLEAKQAPTVQGS

SEQ ID NO: 102 - DNA, 1341 bp, Artificial Sequence
  OsHPPDm-F383W-01 Nucleotide Sequence
atgcctcccactcccacccccaccgccaccaccggcgccgtctcggccgctgcggcggcgggggagaacgcggggttccgcctcgtcgggcaccgccgcttcgtccgcgccaacccgcggagcgaccggttccaggcgctcgcgttccaccacgtcgagctctggtgcgccgacgccgcgtccgccgcgggccggttcgccttcgccctgggcgcgccgctcgccgccaggtccgacctctccacggggaactccgcgcacgcctccctcctcctccgctccgcctccgtcgcgttcctcttcaccgccccctacggcggcgaccacggcgtcggcgcggacgcggccaccaccgcctccatcccttccttctccccaggcgccgcgcggaggttcgccgcggaccacggcctcgcggtgcacgccgtggcgctgcgcgtcgccgacgcggccgacgccttccgcgccagcgtcgcggccggtgcgcgcccggcgttccagcccgccgacctcggcggtggcttcggcctcgcggaggtggagctctacggcgacgtcgtgctccgcttcgtcagccacccggacggcgccgacgcgcccttcctcccgggtttcgagggcgtcagcaacccgggcgccgtggactacggcctccgccggttcgaccacgtcgtcggcaacgtgccggagctcgctccggtagccgcgtacatctccgggttcaccgggttccacgagttcgccgagttcaccgccgaggacgtgggcaccgccgagagcggcctcaactcggtggtgctcgccaacaacgcggagaccgtgctgctgccgctcaacgagccggtgcacggcaccaagcggcggagccagatacagacgtacctggaccaccacggcggcccgggggtgcagcacatcgcgctggccagcgacgacgtgctcgggacgctgagggagatgcgggcgcgctccgccatgggcggcttcgagttcttggcgccgccgccgcccaactactacgacggcgtgcggcggcgcgccggggacgtgctctcggaggagcagatcaacgagtgccaggagctcggggtgctcgtggacagggatgaccagggggtgttgctccagatcttcaccaagccagtaggagacaggccaaccttttggttggagatgatacaaaggattgggtgcatggagaaggatgagagtgggcaggagtaccagaagggcggctgcggcgggtttgggaagggcaacttctcggagctgttcaagtccattgaggagtatgagaaatcccttgaagccaagcaagcccctacagttcaaggatcctag

SEQ ID NO: 103 - DNA, 1341 bp, Artificial Sequence
  OsHPPDm-F383W-02 Nucleotide Sequence
atgccacccacgccaacaccaacggccaccactggtgccgtctcggccgcggcagcggccggtgagaatgctggtttcaggctagtcggccaccgccgcttcgtgagggcaaatccaagatctgatcggttccaagcacttgctttccaccatgttgagctgtggtgcgctgacgccgcttcagctgccgggaggtttgcttttgctttaggggcgccgctcgccgcaaggagtgatctttccaccggaaattctgctcatgcttctcttctacttagatcagcaagtgttgcatttctgttcactgcaccttatggcggagaccatggtgtcggggccgatgctgcaacaacagctagcataccatcattttctcccggcgccgcaagaagatttgcagccgatcatggcctggcagttcatgctgtggcattgagggtcgccgacgcggctgatgcgttccgcgccagcgtggctgctggagctaggccggcgttccagcctgctgaccttgggggtggatttggattggcggaggttgaattatatggtgatgttgtgctccgttttgtttcccatccagatggtgctgatgctccatttctacctggatttgaaggggtgtcaaaccccggcgcggtggattatggactgcgtcgatttgatcacgtggtaggtaatgttcctgagttggctcccgtggcggcctacatttcaggctttactggcttccatgaatttgccgagttcaccgcggaagatgtgggaactgctgaaagtggattgaactctgttgtcctggcgaacaatgcagagactgtattgctccccttgaatgagcctgtgcacggcaccaaacggcgatctcaaattcagacatacctcgaccaccacgggggccctggtgttcagcatattgctctagccagcgacgacgtactgggaacactgagggagatgagagcccgttccgccatgggtggctttgagtttctggcccctccgccgccaaactactacgacggcgtcagacggcgggcgggtgacgtcttgagtgaggagcagatcaatgaatgtcaagaacttggggttcttgttgatagagatgatcaaggagtgctcctccaaatattcacaaaacctgttggcgaccgcccgaccttctggcttgaaatgatccaaaggatcggctgcatggagaaggatgaatcgggccaggagtaccagaagggtgggtgtggtggctttgggaagggcaacttcagcgagctgttcaagtcaattgaagaatatgaaaaatcattggaggcaaagcaagctccgacggtgcagggaagctga

SEQ ID NO: 104 - protein, 446 aa, Artificial Sequence
  OsHPPDm-F372A-F383W Amino Acid Sequence
MPPTPTPTATTGAVSAAAAAGENAGFRLVGHRRFVRANPRSDRFQALAFHHVELWCADAASAAGRFAFALGAPLAARSDLSTGNSAHASLLLRSASVAFLFTAPYGGDHGVGADAATTASIPSFSPGAARRFAADHGLAVHAVALRVADAADAFRASVAAGARPAFQPADLGGGFGLAEVELYGDVVLRFVSHPDGADAPFLPGFEGVSNPGAVDYGLRRFDHVVGNVPELAPVAAYISGFTGFHEFAEFTAEDVGTAESGLNSVVLANNAETVLLPLNEPVHGTKRRSQIQTYLDHHGGPGVQHIALASDDVLGTLREMRARSAMGGFEFLAPPPPNYYDGVRRRAGDVLSEEQINECQELGVLVDRDDQGVLLQIATKPVGDRPTFWLEMIQRIGCMEKDESGQEYQKGGCGGFGKGNFSELFKSIEEYEKSLEAKQAPTVQGS

SEQ ID NO: 105 - DNA, 1341 bp, Artificial Sequence
  OsHPPDm-F372A-F383W-01 Nucleotide Sequence
atgcctcccactcccacccccaccgccaccaccggcgccgtctcggccgctgcggcggcgggggagaacgcggggttccgcctcgtcgggcaccgccgcttcgtccgcgccaacccgcggagcgaccggttccaggcgctcgcgttccaccacgtcgagctctggtgcgccgacgccgcgtccgccgcgggccggttcgccttcgccctgggcgcgccgctcgccgccaggtccgacctctccacggggaactccgcgcacgcctccctcctcctccgctccgcctccgtcgcgttcctcttcaccgccccctacggcggcgaccacggcgtcggcgcggacgcggccaccaccgcctccatcccttccttctccccaggcgccgcgcggaggttcgccgcggaccacggcctcgcggtgcacgccgtggcgctgcgcgtcgccgacgcggccgacgccttccgcgccagcgtcgcggccggtgcgcgcccggcgttccagcccgccgacctcggcggtggcttcggcctcgcggaggtggagctctacggcgacgtcgtgctccgcttcgtcagccacccggacggcgccgacgcgcccttcctcccgggtttcgagggcgtcagcaacccgggcgccgtggactacggcctccgccggttcgaccacgtcgtcggcaacgtgccggagctcgctccggtagccgcgtacatctccgggttcaccgggttccacgagttcgccgagttcaccgccgaggacgtgggcaccgccgagagcggcctcaactcggtggtgctcgccaacaacgcggagaccgtgctgctgccgctcaacgagccggtgcacggcaccaagcggcggagccagatacagacgtacctggaccaccacggcggcccgggggtgcagcacatcgcgctggccagcgacgacgtgctcgggacgctgagggagatgcgggcgcgctccgccatgggcggcttcgagttcttggcgccgccgccgcccaactactacgacggcgtgcggcggcgcgccggggacgtgctctcggaggagcagatcaacgagtgccaggagctcggggtgctcgtggacagggatgaccagggggtgttgctccagatcgctaccaagccagtaggagacaggccaaccttttggttggagatgatacaaaggattgggtgcatggagaaggatgagagtgggcaggagtaccagaagggcggctgcggcgggtttgggaagggcaacttctcggagctgttcaagtccattgaggagtatgagaaatcccttgaagccaagcaagcccctacagttcaaggatcctag

SEQ ID NO: 106 - DNA, 1341 bp, Artificial Sequence
  OsHPPDm-F372A-F383W-02 Nucleotide Sequence
atgccacccacgccaacaccaacggccaccactggtgccgtctcggccgcggcagcggccggtgagaatgctggtttcaggctagtcggccaccgccgcttcgtgagggcaaatccaagatctgatcggttccaagcacttgctttccaccatgttgagctgtggtgcgctgacgccgcttcagctgccgggaggtttgcttttgctttaggggcgccgctcgccgcaaggagtgatctttccaccggaaattctgctcatgcttctcttctacttagatcagcaagtgttgcatttctgttcactgcaccttatggcggagaccatggtgtcggggccgatgctgcaacaacagctagcataccatcattttctcccggcgccgcaagaagatttgcagccgatcatggcctggcagttcatgctgtggcattgagggtcgccgacgcggctgatgcgttccgcgccagcgtggctgctggagctaggccggcgttccagcctgctgaccttgggggtggatttggattggcggaggttgaattatatggtgatgttgtgctccgttttgtttcccatccagatggtgctgatgctccatttctacctggatttgaaggggtgtcaaaccccggcgcggtggattatggactgcgtcgatttgatcacgtggtaggtaatgttcctgagttggctcccgtggcggcctacatttcaggctttactggcttccatgaatttgccgagttcaccgcggaagatgtgggaactgctgaaagtggattgaactctgttgtcctggcgaacaatgcagagactgtattgctccccttgaatgagcctgtgcacggcaccaaacggcgatctcaaattcagacatacctcgaccaccacgggggccctggtgttcagcatattgctctagccagcgacgacgtactgggaacactgagggagatgagagcccgttccgccatgggtggctttgagtttctggcccctccgccgccaaactactacgacggcgtcagacggcgggcgggtgacgtcttgagtgaggagcagatcaatgaatgtcaagaacttggggttcttgttgatagagatgatcaaggagtgctcctccaaatagccacaaaacctgttggcgaccgcccgaccttctggcttgaaatgatccaaaggatcggctgcatggagaaggatgaatcgggccaggagtaccagaagggtgggtgtggtggctttgggaagggcaacttcagcgagctgttcaagtcaattgaagaatatgaaaaatcattggaggcaaagcaagctccgacggtgcagggaagctga

SEQ ID NO: 107 - protein, 440 aa, Sorghum bicolor
  The amino acid sequence of Sorghum bicolor wild-type HPPD (SbHPPD)
MPPTPTTAAATGAAVAAASAEQAAFRLVGHRNFVRVNPRSDRFHTLAFHHVELWCADAASAAGRFSFGLGAPLAARSDLSTGNTAHASLLLRSGALAFLFTAPYAHGADAATASLPSFSAAEARRFAADHGLAVRAVALRVADAEDAFRASVAAGARPAFEPVELGLGFRLAEVELYGDVVLRYVSYPDDADASFLPGFVGVTSPGAADYGLRRFDHIVGNVPELAPAAAYFAGFTGFHEFAEFTAEDVGTTESGLNSMVLANNAENVLLPLNEPVHGTKRRSQIQTYLDHHGGPGVQHMALASDDVLRTLREMQARSAMGGFEFMAPPAPEYYDGVRRRAGDVLTEAQIKECQELGVLVDRDDQGVLLQIFTKPVGDRPTLFLEIIQRIGCMEKDEKGQEYQKGGCGGFGKGNFSQLFKSIEDYEKSLEAKQAAAAQGS

SEQ ID NO: 108 - DNA, 1323 bp, Sorghum bicolor
  SbHPPD-01 Nucleotide Sequence
atgcccccgacccccaccacagccgccgcaaccggcgccgccgtggcggcggcatcagcggagcaggcggcgttccgcctcgtgggccaccgcaacttcgtccgcgtgaacccgcgctccgaccgcttccacacgctcgcgttccaccacgtggagctctggtgcgccgacgcggcctccgccgcgggccgcttctccttcgggctcggcgcgccgctcgccgcgcggtccgacctctccacggggaacaccgcgcacgcgtccctgctgctccgctcgggcgccctcgcgttcctcttcacggcgccctacgcgcacggcgccgacgccgccacggcctcgctgccctccttctccgccgccgaggcgcggcgcttcgcggccgaccacggcctcgcggtgcgcgccgtcgcgctccgcgtggccgacgcggaggacgccttccgcgccagcgtcgcggccggcgcgcgcccggcgttcgagcccgtcgagctcggcctcggcttccgcctcgccgaagtcgagctctacggcgacgtcgtgctccggtacgtgagctacccggacgacgcggacgcgtccttcctgccggggttcgtgggcgtgaccagccccggcgcggcggactacgggctgaggaggttcgaccacatcgtcggcaacgtgccggagctggcgccggcggccgcctacttcgctggcttcacggggttccacgagttcgccgagttcacggcggaggacgtgggcaccacggagagcgggctcaactcgatggtgctcgccaacaacgcggagaacgtgctgctcccactcaacgagccggtgcacggcaccaagcgccgcagccagatacagacgtacttggaccaccacggcggccccggcgtgcagcacatggcgctggccagcgacgacgtgctcaggacgctgagggagatgcaagcgcgctcggccatgggcggcttcgagttcatggcgcctccggcgcccgaatactatgacggcgtgaggcggcgcgccggggacgtgctcacggaggcacagattaaggagtgtcaggaactaggggtgctggtggacagagatgaccagggcgtgctgctccagatcttcaccaagccagtgggggacaggccaacgttgttcttggagatcattcaaaggatcgggtgcatggagaaggatgagaaggggcaagaataccagaagggtggctgtggcgggtttggcaagggaaacttctcccagctgttcaaatccattgaggattatgagaagtcccttgaagctaagcaagctgcagcagctcagggatcctag

SEQ ID NO: 109 - DNA, 1323 bp, Artificial Sequence
  SbHPPD-02 Nucleotide Sequence
atgccgcccactccaacaactgctgctgcgacgggagcagctgtcgccgctgcttctgctgagcaggctgccttcaggctcgtcgggcacagaaattttgttcgtgtaaatccaaggagtgataggttccacaccttggcttttcaccacgtggagttgtggtgtgctgatgcagcctcggcagcggggcgcttctcgtttggtctcggtgctccgctcgccgcaagatctgatcttagcactggaaacacagcgcatgcctccctgctcctgcgctctggcgcgctggcgttcctcttcacggcgccatatgctcacggcgccgacgccgccaccgcgtcattgccgtcttttagtgcagccgaagcaagaagatttgcagcagaccacggcctcgccgtaagggccgtggccttacgtgtcgccgatgccgaagatgctttccgcgcctctgtagcagctggagcaaggccagcatttgaacctgttgaattggggttaggattccgtcttgcagaagttgagctttatggcgacgttgttttgagatacgtttcatatcctgatgacgctgacgctagcttcttgcctggttttgtgggggtgacatcacctggggcagcagattatggtctcaggcggtttgatcatattgttggaaacgttcctgaactcgcgccggcggcagcctacttcgccggtttcactgggtttcatgaatttgctgaattcacagccgaggatgtcggcaccaccgagagtggactgaactccatggtgctggccaacaatgcagagaatgtccttcttcccttgaatgaaccagttcatggaacaaaaaggcgttcccaaatacaaacatacctcgaccatcatggtggaccaggcgttcagcatatggctctcgctagtgacgatgttctacgaaccctgcgagagatgcaggcgcggtctgcaatgggaggatttgagttcatggcacctcctgcccctgaatattatgatggtgttcggagaagggcaggtgatgtgctaactgaagctcaaatcaaggagtgccaggagcttggcgtgctggtcgatcgggatgatcaaggtgtgcttctgcagatttttactaaaccagtgggtgaccgccccacgctgttcctagagatcatccagagaatagggtgcatggagaaggacgaaaaaggacaagagtaccagaagggaggttgtggcggctttggaaaagggaacttctcccaattattcaagtcaattgaagactatgaaaagagtttggaggctaagcaagctgcagccgcccagggcagctga

SEQ ID NO: 110 - protein, 440 aa, Artificial Sequence
  SbHPPDm-F372A Amino Acid Sequence
MPPTPTTAAATGAAVAAASAEQAAFRLVGHRNFVRVNPRSDRFHTLAFHHVELWCADAASAAGRFSFGLGAPLAARSDLSTGNTAHASLLLRSGALAFLFTAPYAHGADAATASLPSFSAAEARRFAADHGLAVRAVALRVADAEDAFRASVAAGARPAFEPVELGLGFRLAEVELYGDVVLRYVSYPDDADASFLPGFVGVTSPGAADYGLRRFDHIVGNVPELAPAAAYFAGFTGFHEFAEFTAEDVGTTESGLNSMVLANNAENVLLPLNEPVHGTKRRSQIQTYLDHHGGPGVQHMALASDDVLRTLREMQARSAMGGFEFMAPPAPEYYDGVRRRAGDVLTEAQIKECQELGVLVDRDDQGVLLQIATKPVGDRPTLFLEIIQRIGCMEKDEKGQEYQKGGCGGFGKGNFSQLFKSIEDYEKSLEAKQAAAAQGS

SEQ ID NO: 111 - DNA, 1323 bp, Artificial Sequence
  SbHPPDm-F372A-01 Nucleotide Sequence
atgcccccgacccccaccacagccgccgcaaccggcgccgccgtggcggcggcatcagcggagcaggcggcgttccgcctcgtgggccaccgcaacttcgtccgcgtgaacccgcgctccgaccgcttccacacgctcgcgttccaccacgtggagctctggtgcgccgacgcggcctccgccgcgggccgcttctccttcgggctcggcgcgccgctcgccgcgcggtccgacctctccacggggaacaccgcgcacgcgtccctgctgctccgctcgggcgccctcgcgttcctcttcacggcgccctacgcgcacggcgccgacgccgccacggcctcgctgccctccttctccgccgccgaggcgcggcgcttcgcggccgaccacggcctcgcggtgcgcgccgtcgcgctccgcgtggccgacgcggaggacgccttccgcgccagcgtcgcggccggcgcgcgcccggcgttcgagcccgtcgagctcggcctcggcttccgcctcgccgaagtcgagctctacggcgacgtcgtgctccggtacgtgagctacccggacgacgcggacgcgtccttcctgccggggttcgtgggcgtgaccagccccggcgcggcggactacgggctgaggaggttcgaccacatcgtcggcaacgtgccggagctggcgccggcggccgcctacttcgctggcttcacggggttccacgagttcgccgagttcacggcggaggacgtgggcaccacggagagcgggctcaactcgatggtgctcgccaacaacgcggagaacgtgctgctcccactcaacgagccggtgcacggcaccaagcgccgcagccagatacagacgtacttggaccaccacggcggccccggcgtgcagcacatggcgctggccagcgacgacgtgctcaggacgctgagggagatgcaagcgcgctcggccatgggcggcttcgagttcatggcgcctccggcgcccgaatactatgacggcgtgaggcggcgcgccggggacgtgctcacggaggcacagattaaggagtgtcaggaactaggggtgctggtggacagagatgaccagggcgtgctgctccagatcgctaccaagccagtgggggacaggccaacgttgttcttggagatcattcaaaggatcgggtgcatggagaaggatgagaaggggcaagaataccagaagggtggctgtggcgggtttggcaagggaaacttctcccagctgttcaaatccattgaggattatgagaagtcccttgaagctaagcaagctgcagcagctcagggatcctag

SEQ ID NO: 112 - DNA, 1323 bp, Artificial Sequence
  SbHPPDm-F372A-02 Nucleotide Sequence
atgccgcccactccaacaactgctgctgcgacgggagcagctgtcgccgctgcttctgctgagcaggctgccttcaggctcgtcgggcacagaaattttgttcgtgtaaatccaaggagtgataggttccacaccttggcttttcaccacgtggagttgtggtgtgctgatgcagcctcggcagcggggcgcttctcgtttggtctcggtgctccgctcgccgcaagatctgatcttagcactggaaacacagcgcatgcctccctgctcctgcgctctggcgcgctggcgttcctcttcacggcgccatatgctcacggcgccgacgccgccaccgcgtcattgccgtcttttagtgcagccgaagcaagaagatttgcagcagaccacggcctcgccgtaagggccgtggccttacgtgtcgccgatgccgaagatgctttccgcgcctctgtagcagctggagcaaggccagcatttgaacctgttgaattggggttaggattccgtcttgcagaagttgagctttatggcgacgttgttttgagatacgtttcatatcctgatgacgctgacgctagcttcttgcctggttttgtgggggtgacatcacctggggcagcagattatggtctcaggcggtttgatcatattgttggaaacgttcctgaactcgcgccggcggcagcctacttcgccggtttcactgggtttcatgaatttgctgaattcacagccgaggatgtcggcaccaccgagagtggactgaactccatggtgctggccaacaatgcagagaatgtccttcttcccttgaatgaaccagttcatggaacaaaaaggcgttcccaaatacaaacatacctcgaccatcatggtggaccaggcgttcagcatatggctctcgctagtgacgatgttctacgaaccctgcgagagatgcaggcgcggtctgcaatgggaggatttgagttcatggcacctcctgcccctgaatattatgatggtgttcggagaagggcaggtgatgtgctaactgaagctcaaatcaaggagtgccaggagcttggcgtgctggtcgatcgggatgatcaaggtgtgcttctgcagattgccactaaaccagtgggtgaccgccccacgctgttcctagagatcatccagagaatagggtgcatggagaaggacgaaaaaggacaagagtaccagaagggaggttgtggcggctttggaaaagggaacttctcccaattattcaagtcaattgaagactatgaaaagagtttggaggctaagcaagctgcagccgcccagggcagctga

SEQ ID NO: 113 - protein, 440 aa, Artificial Sequence
  SbHPPDm-F383W Amino Acid Sequence
MPPTPTTAAATGAAVAAASAEQAAFRLVGHRNFVRVNPRSDRFHTLAFHHVELWCADAASAAGRFSFGLGAPLAARSDLSTGNTAHASLLLRSGALAFLFTAPYAHGADAATASLPSFSAAEARRFAADHGLAVRAVALRVADAEDAFRASVAAGARPAFEPVELGLGFRLAEVELYGDVVLRYVSYPDDADASFLPGFVGVTSPGAADYGLRRFDHIVGNVPELAPAAAYFAGFTGFHEFAEFTAEDVGTTESGLNSMVLANNAENVLLPLNEPVHGTKRRSQIQTYLDHHGGPGVQHMALASDDVLRTLREMQARSAMGGFEFMAPPAPEYYDGVRRRAGDVLTEAQIKECQELGVLVDRDDQGVLLQIFTKPVGDRPTLWLEIIQRIGCMEKDEKGQEYQKGGCGGFGKGNFSQLFKSIEDYEKSLEAKQAAAAQGS

SEQ ID NO: 114 - DNA, 1323 bp, Artificial Sequence
  SbHPPDm-F383W-01 Nucleotide Sequence
atgcccccgacccccaccacagccgccgcaaccggcgccgccgtggcggcggcatcagcggagcaggcggcgttccgcctcgtgggccaccgcaacttcgtccgcgtgaacccgcgctccgaccgcttccacacgctcgcgttccaccacgtggagctctggtgcgccgacgcggcctccgccgcgggccgcttctccttcgggctcggcgcgccgctcgccgcgcggtccgacctctccacggggaacaccgcgcacgcgtccctgctgctccgctcgggcgccctcgcgttcctcttcacggcgccctacgcgcacggcgccgacgccgccacggcctcgctgccctccttctccgccgccgaggcgcggcgcttcgcggccgaccacggcctcgcggtgcgcgccgtcgcgctccgcgtggccgacgcggaggacgccttccgcgccagcgtcgcggccggcgcgcgcccggcgttcgagcccgtcgagctcggcctcggcttccgcctcgccgaagtcgagctctacggcgacgtcgtgctccggtacgtgagctacccggacgacgcggacgcgtccttcctgccggggttcgtgggcgtgaccagccccggcgcggcggactacgggctgaggaggttcgaccacatcgtcggcaacgtgccggagctggcgccggcggccgcctacttcgctggcttcacggggttccacgagttcgccgagttcacggcggaggacgtgggcaccacggagagcgggctcaactcgatggtgctcgccaacaacgcggagaacgtgctgctcccactcaacgagccggtgcacggcaccaagcgccgcagccagatacagacgtacttggaccaccacggcggccccggcgtgcagcacatggcgctggccagcgacgacgtgctcaggacgctgagggagatgcaagcgcgctcggccatgggcggcttcgagttcatggcgcctccggcgcccgaatactatgacggcgtgaggcggcgcgccggggacgtgctcacggaggcacagattaaggagtgtcaggaactaggggtgctggtggacagagatgaccagggcgtgctgctccagatcttcaccaagccagtgggggacaggccaacgttgtggttggagatcattcaaaggatcgggtgcatggagaaggatgagaaggggcaagaataccagaagggtggctgtggcgggtttggcaagggaaacttctcccagctgttcaaatccattgaggattatgagaagtcccttgaagctaagcaagctgcagcagctcagggatcctag

SEQ ID NO: 115 - DNA, 1323 bp, Artificial Sequence
  SbHPPDm-F383W-02 Nucleotide Sequence
atgccgcccactccaacaactgctgctgcgacgggagcagctgtcgccgctgcttctgctgagcaggctgccttcaggctcgtcgggcacagaaattttgttcgtgtaaatccaaggagtgataggttccacaccttggcttttcaccacgtggagttgtggtgtgctgatgcagcctcggcagcggggcgcttctcgtttggtctcggtgctccgctcgccgcaagatctgatcttagcactggaaacacagcgcatgcctccctgctcctgcgctctggcgcgctggcgttcctcttcacggcgccatatgctcacggcgccgacgccgccaccgcgtcattgccgtcttttagtgcagccgaagcaagaagatttgcagcagaccacggcctcgccgtaagggccgtggccttacgtgtcgccgatgccgaagatgctttccgcgcctctgtagcagctggagcaaggccagcatttgaacctgttgaattggggttaggattccgtcttgcagaagttgagctttatggcgacgttgttttgagatacgtttcatatcctgatgacgctgacgctagcttcttgcctggttttgtgggggtgacatcacctggggcagcagattatggtctcaggcggtttgatcatattgttggaaacgttcctgaactcgcgccggcggcagcctacttcgccggtttcactgggtttcatgaatttgctgaattcacagccgaggatgtcggcaccaccgagagtggactgaactccatggtgctggccaacaatgcagagaatgtccttcttcccttgaatgaaccagttcatggaacaaaaaggcgttcccaaatacaaacatacctcgaccatcatggtggaccaggcgttcagcatatggctctcgctagtgacgatgttctacgaaccctgcgagagatgcaggcgcggtctgcaatgggaggatttgagttcatggcacctcctgcccctgaatattatgatggtgttcggagaagggcaggtgatgtgctaactgaagctcaaatcaaggagtgccaggagcttggcgtgctggtcgatcgggatgatcaaggtgtgcttctgcagatttttactaaaccagtgggtgaccgccccacgctgtggctagagatcatccagagaatagggtgcatggagaaggacgaaaaaggacaagagtaccagaagggaggttgtggcggctttggaaaagggaacttctcccaattattcaagtcaattgaagactatgaaaagagtttggaggctaagcaagctgcagccgcccagggcagctga

SEQ ID NO: 116 - protein, 440 aa, Artificial Sequence
  SbHPPDm-F372A-F383W Amino Acid Sequence
MPPTPTTAAATGAAVAAASAEQAAFRLVGHRNFVRVNPRSDRFHTLAFHHVELWCADAASAAGRFSFGLGAPLAARSDLSTGNTAHASLLLRSGALAFLFTAPYAHGADAATASLPSFSAAEARRFAADHGLAVRAVALRVADAEDAFRASVAAGARPAFEPVELGLGFRLAEVELYGDVVLRYVSYPDDADASFLPGFVGVTSPGAADYGLRRFDHIVGNVPELAPAAAYFAGFTGFHEFAEFTAEDVGTTESGLNSMVLANNAENVLLPLNEPVHGTKRRSQIQTYLDHHGGPGVQHMALASDDVLRTLREMQARSAMGGFEFMAPPAPEYYDGVRRRAGDVLTEAQIKECQELGVLVDRDDQGVLLQIATKPVGDRPTLWLEIIQRIGCMEKDEKGQEYQKGGCGGFGKGNFSQLFKSIEDYEKSLEAKQAAAAQGS

SEQ ID NO: 117 - DNA, 1323 bp, Artificial Sequence
  SbHPPDm-F372A-F383W-01 Nucleotide Sequence
atgcccccgacccccaccacagccgccgcaaccggcgccgccgtggcggcggcatcagcggagcaggcggcgttccgcctcgtgggccaccgcaacttcgtccgcgtgaacccgcgctccgaccgcttccacacgctcgcgttccaccacgtggagctctggtgcgccgacgcggcctccgccgcgggccgcttctccttcgggctcggcgcgccgctcgccgcgcggtccgacctctccacggggaacaccgcgcacgcgtccctgctgctccgctcgggcgccctcgcgttcctcttcacggcgccctacgcgcacggcgccgacgccgccacggcctcgctgccctccttctccgccgccgaggcgcggcgcttcgcggccgaccacggcctcgcggtgcgcgccgtcgcgctccgcgtggccgacgcggaggacgccttccgcgccagcgtcgcggccggcgcgcgcccggcgttcgagcccgtcgagctcggcctcggcttccgcctcgccgaagtcgagctctacggcgacgtcgtgctccggtacgtgagctacccggacgacgcggacgcgtccttcctgccggggttcgtgggcgtgaccagccccggcgcggcggactacgggctgaggaggttcgaccacatcgtcggcaacgtgccggagctggcgccggcggccgcctacttcgctggcttcacggggttccacgagttcgccgagttcacggcggaggacgtgggcaccacggagagcgggctcaactcgatggtgctcgccaacaacgcggagaacgtgctgctcccactcaacgagccggtgcacggcaccaagcgccgcagccagatacagacgtacttggaccaccacggcggccccggcgtgcagcacatggcgctggccagcgacgacgtgctcaggacgctgagggagatgcaagcgcgctcggccatgggcggcttcgagttcatggcgcctccggcgcccgaatactatgacggcgtgaggcggcgcgccggggacgtgctcacggaggcacagattaaggagtgtcaggaactaggggtgctggtggacagagatgaccagggcgtgctgctccagatcgctaccaagccagtgggggacaggccaacgttgtggttggagatcattcaaaggatcgggtgcatggagaaggatgagaaggggcaagaataccagaagggtggctgtggcgggtttggcaagggaaacttctcccagctgttcaaatccattgaggattatgagaagtcccttgaagctaagcaagctgcagcagctcagggatcctag

SEQ ID NO: 118 - DNA, 1323 bp, Artificial Sequence
  SbHPPDm-F372A-F383W-02 Nucleotide Sequence
atgccgcccactccaacaactgctgctgcgacgggagcagctgtcgccgctgcttctgctgagcaggctgccttcaggctcgtcgggcacagaaattttgttcgtgtaaatccaaggagtgataggttccacaccttggcttttcaccacgtggagttgtggtgtgctgatgcagcctcggcagcggggcgcttctcgtttggtctcggtgctccgctcgccgcaagatctgatcttagcactggaaacacagcgcatgcctccctgctcctgcgctctggcgcgctggcgttcctcttcacggcgccatatgctcacggcgccgacgccgccaccgcgtcattgccgtcttttagtgcagccgaagcaagaagatttgcagcagaccacggcctcgccgtaagggccgtggccttacgtgtcgccgatgccgaagatgctttccgcgcctctgtagcagctggagcaaggccagcatttgaacctgttgaattggggttaggattccgtcttgcagaagttgagctttatggcgacgttgttttgagatacgtttcatatcctgatgacgctgacgctagcttcttgcctggttttgtgggggtgacatcacctggggcagcagattatggtctcaggcggtttgatcatattgttggaaacgttcctgaactcgcgccggcggcagcctacttcgccggtttcactgggtttcatgaatttgctgaattcacagccgaggatgtcggcaccaccgagagtggactgaactccatggtgctggccaacaatgcagagaatgtccttcttcccttgaatgaaccagttcatggaacaaaaaggcgttcccaaatacaaacatacctcgaccatcatggtggaccaggcgttcagcatatggctctcgctagtgacgatgttctacgaaccctgcgagagatgcaggcgcggtctgcaatgggaggatttgagttcatggcacctcctgcccctgaatattatgatggtgttcggagaagggcaggtgatgtgctaactgaagctcaaatcaaggagtgccaggagcttggcgtgctggtcgatcgggatgatcaaggtgtgcttctgcagattgccactaaaccagtgggtgaccgccccacgctgtggctagagatcatccagagaatagggtgcatggagaaggacgaaaaaggacaagagtaccagaagggaggttgtggcggctttggaaaagggaacttctcccaattattcaagtcaattgaagactatgaaaagagtttggaggctaagcaagctgcagccgcccagggcagctga

SEQ ID NO: 119 - protein, 434 aa, Hordeum vulgare
  The amino acid sequence of Hordeum vulgare wild-type HPPD (HvHPPD)
MPPTPTTPAATGAAAAVTPEHARPHRMVRFNPRSDRFHTLSFHHVEFWCADAASAAGRFAFALGAPLAARSDLSTGNSAHASQLLRSGSLAFLFTAPYANGCDAATASLPSFSADAARRFSADHGIAVRSVALRVADAAEAFRASRRRGARPAFAPVDLGRGFAFAEVELYGDVVLRFVSHPDGTDVPFLPGFEGVTNPDAVDYGLTRFDHVVGNVPELAPAAAYIAGFTGFHEFAEFTAEDVGTTESGLNSVVLANNSEGVLLPLNEPVHGTKRRSQIQTFLEHHGGPGVQHIAVASSDVLRTLRKMRARSAMGGFDFLPPPLPKYYEGVRRLAGDVLSEAQIKECQELGVLVDRDDQGVLLQIFTKPVGDRPTLFLEMIQRIGCMEKDERGEEYQKGGCGGFGKGNFSELFKSIEDYEKSLEAKQSAAVQGS

SEQ ID NO: 120 - DNA, 1305 bp, Hordeum vulgare
  HvHPPD-01 Nucleotide Sequence
atgccgcccacccccaccacccccgcggctaccggcgccgccgccgcggtgacgccggagcacgcgcgaccgcaccgaatggtccgcttcaacccgcgcagcgaccgcttccacacgctctccttccaccacgtcgagttctggtgcgcggacgccgcctccgccgccggccgcttcgcgttcgcgctcggcgcgccgctcgccgccaggtccgacctctccacggggaactccgcgcacgcctcccagctgctccgctcgggctccctcgccttcctcttcaccgcgccctacgccaacggctgcgacgccgccaccgcctccctgccctccttctccgccgacgccgcgcgccggttctccgccgaccacgggatcgcggtgcgctccgtagcgctgcgcgtcgcagacgccgccgaggccttccgcgccagtcgtcgacggggcgcgcgcccggccttcgcccccgtggacctcggccgcggcttcgcgttcgcggaggtcgagctctacggcgacgtcgtgctccgcttcgtcagccacccggacggcacggacgtgcccttcttgccggggttcgagggcgtaaccaacccggacgccgtggactacggcctgacgcggttcgaccacgtcgtcggcaacgtcccggagcttgcccccgccgcagcctacatcgccgggttcacggggttccacgagttcgccgagttcacggcggaggacgtgggcacgaccgagagcgggctcaactcggtggtgctcgccaacaactcggagggcgtgctgctgccgctcaacgagccggtgcacggcaccaagcgccggagccagatacagacgttcctggaacaccacggcggcccgggcgtgcagcacatcgcggtggccagcagtgacgtgctcaggacgctcaggaagatgcgtgcgcgctccgccatgggcggcttcgacttcctgccacccccgctgccgaagtactacgaaggcgtgcgacgccttgccggggatgtcctctcggaggcgcagatcaaggaatgccaggagctgggtgtgctcgtcgatagggacgaccaaggggtgttgctccaaatcttcaccaagccagtaggggacaggccgaccttgttcctggagatgatccagaggatcgggtgcatggagaaggacgagagaggggaagagtaccagaagggtggctgcggcgggttcggcaaaggcaacttctccgagctgttcaagtccattgaagattacgagaagtcccttgaagccaagcaatctgctgcagttcagggatcatag

SEQ ID NO: 121 - DNA, 1305 bp, Artificial Sequence
  HvHPPD-02 Nucleotide Sequence
atgccgccgacgcccaccaccccagcagctaccggagctgcggctgcagtaacccctgagcatgctcggccccacaggatggtgaggtttaatccaagatcagatcgttttcatacactctcgttccaccatgttgagttctggtgcgccgacgcggcttcagcggccgggaggttcgccttcgcgctgggggcccctcttgccgcgcgtagtgatttgtctactgggaattcagcgcacgcgtcccagcttctccgaagcggcagtctcgcctttctcttcactgcaccatatgcaaatggatgtgatgcagcaactgcttccctgccgagcttttctgcggatgccgcgaggcgattcagtgctgaccatgggatcgccgtccggtcagttgctcttagagtggctgatgctgctgaggcattcagggcttcaaggcgtcgtggtgcacgcccggcgtttgccccggttgatcttgggcgggggtttgcttttgcagaggtggagctgtacggcgacgtggtgctccgatttgtttctcacccggacggcactgatgtgcccttcttgccaggatttgaaggtgtgaccaaccctgatgccgtggattatggactcacaagatttgatcatgtggttggcaatgttcctgaattggcacctgctgccgcttacatcgcaggttttactggcttccatgaatttgctgaattcacggcggaggatgttggtacaactgagtcagggctgaacagtgttgttttagccaacaactcagaaggagttctccttcccttgaatgaacctgttcatggaaccaagcgccgctcccaaattcaaacatttcttgagcaccacggcggccctggtgttcaacatattgctgtcgcctctagcgacgtcctgcgtacattacgcaagatgagggctcggtccgcaatgggtggtttcgacttcctccctccaccattgccaaaatattatgaaggcgtcagaagacttgcaggagatgtcctctctgaagctcagatcaaggagtgccaagaacttggcgtcttggttgatagagatgaccaaggagtacttctgcagatatttacaaaacccgttggtgacaggccaactcttttcctggagatgattcagagaattggctgcatggagaaagatgaaagaggcgaggagtaccagaagggtggttgtggaggctttggaaaaggaaacttctcagagctgttcaagtccatagaagattacgagaaaagtctagaagccaagcagtctgctgcagtgcaaggttcctga

SEQ ID NO: 122 - protein, 434 aa, Artificial Sequence
  HvHPPDm-F372A Amino Acid Sequence
MPPTPTTPAATGAAAAVTPEHARPHRMVRFNPRSDRFHTLSFHHVEFWCADAASAAGRFAFALGAPLAARSDLSTGNSAHASQLLRSGSLAFLFTAPYANGCDAATASLPSFSADAARRFSADHGIAVRSVALRVADAAEAFRASRRRGARPAFAPVDLGRGFAFAEVELYGDVVLRFVSHPDGTDVPFLPGFEGVTNPDAVDYGLTRFDHVVGNVPELAPAAAYIAGFTGFHEFAEFTAEDVGTTESGLNSVVLANNSEGVLLPLNEPVHGTKRRSQIQTFLEHHGGPGVQHIAVASSDVLRTLRKMRARSAMGGFDFLPPPLPKYYEGVRRLAGDVLSEAQIKECQELGVLVDRDDQGVLLQIATKPVGDRPTLFLEMIQRIGCMEKDERGEEYQKGGCGGFGKGNFSELFKSIEDYEKSLEAKQSAAVQGS

SEQ ID NO: 123 - DNA, 1305 bp, Artificial Sequence
  HvHPPDm-F372A-01 Nucleotide Sequence
atgccgcccacccccaccacccccgcggctaccggcgccgccgccgcggtgacgccggagcacgcgcgaccgcaccgaatggtccgcttcaacccgcgcagcgaccgcttccacacgctctccttccaccacgtcgagttctggtgcgcggacgccgcctccgccgccggccgcttcgcgttcgcgctcggcgcgccgctcgccgccaggtccgacctctccacggggaactccgcgcacgcctcccagctgctccgctcgggctccctcgccttcctcttcaccgcgccctacgccaacggctgcgacgccgccaccgcctccctgccctccttctccgccgacgccgcgcgccggttctccgccgaccacgggatcgcggtgcgctccgtagcgctgcgcgtcgcagacgccgccgaggccttccgcgccagtcgtcgacggggcgcgcgcccggccttcgcccccgtggacctcggccgcggcttcgcgttcgcggaggtcgagctctacggcgacgtcgtgctccgcttcgtcagccacccggacggcacggacgtgcccttcttgccggggttcgagggcgtaaccaacccggacgccgtggactacggcctgacgcggttcgaccacgtcgtcggcaacgtcccggagcttgcccccgccgcagcctacatcgccgggttcacggggttccacgagttcgccgagttcacggcggaggacgtgggcacgaccgagagcgggctcaactcggtggtgctcgccaacaactcggagggcgtgctgctgccgctcaacgagccggtgcacggcaccaagcgccggagccagatacagacgttcctggaacaccacggcggcccgggcgtgcagcacatcgcggtggccagcagtgacgtgctcaggacgctcaggaagatgcgtgcgcgctccgccatgggcggcttcgacttcctgccacccccgctgccgaagtactacgaaggcgtgcgacgccttgccggggatgtcctctcggaggcgcagatcaaggaatgccaggagctgggtgtgctcgtcgatagggacgaccaaggggtgttgctccaaatcgctaccaagccagtaggggacaggccgaccttgttcctggagatgatccagaggatcgggtgcatggagaaggacgagagaggggaagagtaccagaagggtggctgcggcgggttcggcaaaggcaacttctccgagctgttcaagtccattgaagattacgagaagtcccttgaagccaagcaatctgctgcagttcagggatcatag

SEQ ID NO: 124 - DNA, 1305 bp, Artificial Sequence
  HvHPPDm-F372A-02 Nucleotide Sequence
atgccgccgacgcccaccaccccagcagctaccggagctgcggctgcagtaacccctgagcatgctcggccccacaggatggtgaggtttaatccaagatcagatcgttttcatacactctcgttccaccatgttgagttctggtgcgccgacgcggcttcagcggccgggaggttcgccttcgcgctgggggcccctcttgccgcgcgtagtgatttgtctactgggaattcagcgcacgcgtcccagcttctccgaagcggcagtctcgcctttctcttcactgcaccatatgcaaatggatgtgatgcagcaactgcttccctgccgagcttttctgcggatgccgcgaggcgattcagtgctgaccatgggatcgccgtccggtcagttgctcttagagtggctgatgctgctgaggcattcagggcttcaaggcgtcgtggtgcacgcccggcgtttgccccggttgatcttgggcgggggtttgcttttgcagaggtggagctgtacggcgacgtggtgctccgatttgtttctcacccggacggcactgatgtgcccttcttgccaggatttgaaggtgtgaccaaccctgatgccgtggattatggactcacaagatttgatcatgtggttggcaatgttcctgaattggcacctgctgccgcttacatcgcaggttttactggcttccatgaatttgctgaattcacggcggaggatgttggtacaactgagtcagggctgaacagtgttgttttagccaacaactcagaaggagttctccttcccttgaatgaacctgttcatggaaccaagcgccgctcccaaattcaaacatttcttgagcaccacggcggccctggtgttcaacatattgctgtcgcctctagcgacgtcctgcgtacattacgcaagatgagggctcggtccgcaatgggtggtttcgacttcctccctccaccattgccaaaatattatgaaggcgtcagaagacttgcaggagatgtcctctctgaagctcagatcaaggagtgccaagaacttggcgtcttggttgatagagatgaccaaggagtacttctgcagatagccacaaaacccgttggtgacaggccaactcttttcctggagatgattcagagaattggctgcatggagaaagatgaaagaggcgaggagtaccagaagggtggttgtggaggctttggaaaaggaaacttctcagagctgttcaagtccatagaagattacgagaaaagtctagaagccaagcagtctgctgcagtgcaaggttcctga

SEQ ID NO: 125 - protein, 434 aa, Artificial Sequence
  HvHPPDm-F383W Amino Acid Sequence
MPPTPTTPAATGAAAAVTPEHARPHRMVRFNPRSDRFHTLSFHHVEFWCADAASAAGRFAFALGAPLAARSDLSTGNSAHASQLLRSGSLAFLFTAPYANGCDAATASLPSFSADAARRFSADHGIAVRSVALRVADAAEAFRASRRRGARPAFAPVDLGRGFAFAEVELYGDVVLRFVSHPDGTDVPFLPGFEGVTNPDAVDYGLTRFDHVVGNVPELAPAAAYIAGFTGFHEFAEFTAEDVGTTESGLNSVVLANNSEGVLLPLNEPVHGTKRRSQIQTFLEHHGGPGVQHIAVASSDVLRTLRKMRARSAMGGFDFLPPPLPKYYEGVRRLAGDVLSEAQIKECQELGVLVDRDDQGVLLQIFTKPVGDRPTLWLEMIQRIGCMEKDERGEEYQKGGCGGFGKGNFSELFKSIEDYEKSLEAKQSAAVQGS

SEQ ID NO: 126 - DNA, 1305 bp, Artificial Sequence
  HvHPPDm-F383W-01 Nucleotide Sequence
atgccgcccacccccaccacccccgcggctaccggcgccgccgccgcggtgacgccggagcacgcgcgaccgcaccgaatggtccgcttcaacccgcgcagcgaccgcttccacacgctctccttccaccacgtcgagttctggtgcgcggacgccgcctccgccgccggccgcttcgcgttcgcgctcggcgcgccgctcgccgccaggtccgacctctccacggggaactccgcgcacgcctcccagctgctccgctcgggctccctcgccttcctcttcaccgcgccctacgccaacggctgcgacgccgccaccgcctccctgccctccttctccgccgacgccgcgcgccggttctccgccgaccacgggatcgcggtgcgctccgtagcgctgcgcgtcgcagacgccgccgaggccttccgcgccagtcgtcgacggggcgcgcgcccggccttcgcccccgtggacctcggccgcggcttcgcgttcgcggaggtcgagctctacggcgacgtcgtgctccgcttcgtcagccacccggacggcacggacgtgcccttcttgccggggttcgagggcgtaaccaacccggacgccgtggactacggcctgacgcggttcgaccacgtcgtcggcaacgtcccggagcttgcccccgccgcagcctacatcgccgggttcacggggttccacgagttcgccgagttcacggcggaggacgtgggcacgaccgagagcgggctcaactcggtggtgctcgccaacaactcggagggcgtgctgctgccgctcaacgagccggtgcacggcaccaagcgccggagccagatacagacgttcctggaacaccacggcggcccgggcgtgcagcacatcgcggtggccagcagtgacgtgctcaggacgctcaggaagatgcgtgcgcgctccgccatgggcggcttcgacttcctgccacccccgctgccgaagtactacgaaggcgtgcgacgccttgccggggatgtcctctcggaggcgcagatcaaggaatgccaggagctgggtgtgctcgtcgatagggacgaccaaggggtgttgctccaaatcttcaccaagccagtaggggacaggccgaccttgtggctggagatgatccagaggatcgggtgcatggagaaggacgagagaggggaagagtaccagaagggtggctgcggcgggttcggcaaaggcaacttctccgagctgttcaagtccattgaagattacgagaagtcccttgaagccaagcaatctgctgcagttcagggatcatag

SEQ ID NO: 127 - DNA, 1305 bp, Artificial Sequence
  HvHPPDm-F383W-02 Nucleotide Sequence
atgccgccgacgcccaccaccccagcagctaccggagctgcggctgcagtaacccctgagcatgctcggccccacaggatggtgaggtttaatccaagatcagatcgttttcatacactctcgttccaccatgttgagttctggtgcgccgacgcggcttcagcggccgggaggttcgccttcgcgctgggggcccctcttgccgcgcgtagtgatttgtctactgggaattcagcgcacgcgtcccagcttctccgaagcggcagtctcgcctttctcttcactgcaccatatgcaaatggatgtgatgcagcaactgcttccctgccgagcttttctgcggatgccgcgaggcgattcagtgctgaccatgggatcgccgtccggtcagttgctcttagagtggctgatgctgctgaggcattcagggcttcaaggcgtcgtggtgcacgcccggcgtttgccccggttgatcttgggcgggggtttgcttttgcagaggtggagctgtacggcgacgtggtgctccgatttgtttctcacccggacggcactgatgtgcccttcttgccaggatttgaaggtgtgaccaaccctgatgccgtggattatggactcacaagatttgatcatgtggttggcaatgttcctgaattggcacctgctgccgcttacatcgcaggttttactggcttccatgaatttgctgaattcacggcggaggatgttggtacaactgagtcagggctgaacagtgttgttttagccaacaactcagaaggagttctccttcccttgaatgaacctgttcatggaaccaagcgccgctcccaaattcaaacatttcttgagcaccacggcggccctggtgttcaacatattgctgtcgcctctagcgacgtcctgcgtacattacgcaagatgagggctcggtccgcaatgggtggtttcgacttcctccctccaccattgccaaaatattatgaaggcgtcagaagacttgcaggagatgtcctctctgaagctcagatcaaggagtgccaagaacttggcgtcttggttgatagagatgaccaaggagtacttctgcagatatttacaaaacccgttggtgacaggccaactctttggctggagatgattcagagaattggctgcatggagaaagatgaaagaggcgaggagtaccagaagggtggttgtggaggctttggaaaaggaaacttctcagagctgttcaagtccatagaagattacgagaaaagtctagaagccaagcagtctgctgcagtgcaaggttcctga

SEQ ID NO: 128 - protein, 434 aa, Artificial Sequence
  HvHPPDm-F372A-F383W Amino Acid Sequence
MPPTPTTPAATGAAAAVTPEHARPHRMVRFNPRSDRFHTLSFHHVEFWCADAASAAGRFAFALGAPLAARSDLSTGNSAHASQLLRSGSLAFLFTAPYANGCDAATASLPSFSADAARRFSADHGIAVRSVALRVADAAEAFRASRRRGARPAFAPVDLGRGFAFAEVELYGDVVLRFVSHPDGTDVPFLPGFEGVTNPDAVDYGLTRFDHVVGNVPELAPAAAYIAGFTGFHEFAEFTAEDVGTTESGLNSVVLANNSEGVLLPLNEPVHGTKRRSQIQTFLEHHGGPGVQHIAVASSDVLRTLRKMRARSAMGGFDFLPPPLPKYYEGVRRLAGDVLSEAQIKECQELGVLVDRDDQGVLLQIATKPVGDRPTLWLEMIQRIGCMEKDERGEEYQKGGCGGFGKGNFSELFKSIEDYEKSLEAKQSAAVQGS

SEQ ID NO: 129 - DNA, 1305 bp, Artificial Sequence
  HvHPPDm-F372A-F383W-01 Nucleotide Sequence
atgccgcccacccccaccacccccgcggctaccggcgccgccgccgcggtgacgccggagcacgcgcgaccgcaccgaatggtccgcttcaacccgcgcagcgaccgcttccacacgctctccttccaccacgtcgagttctggtgcgcggacgccgcctccgccgccggccgcttcgcgttcgcgctcggcgcgccgctcgccgccaggtccgacctctccacggggaactccgcgcacgcctcccagctgctccgctcgggctccctcgccttcctcttcaccgcgccctacgccaacggctgcgacgccgccaccgcctccctgccctccttctccgccgacgccgcgcgccggttctccgccgaccacgggatcgcggtgcgctccgtagcgctgcgcgtcgcagacgccgccgaggccttccgcgccagtcgtcgacggggcgcgcgcccggccttcgcccccgtggacctcggccgcggcttcgcgttcgcggaggtcgagctctacggcgacgtcgtgctccgcttcgtcagccacccggacggcacggacgtgcccttcttgccggggttcgagggcgtaaccaacccggacgccgtggactacggcctgacgcggttcgaccacgtcgtcggcaacgtcccggagcttgcccccgccgcagcctacatcgccgggttcacggggttccacgagttcgccgagttcacggcggaggacgtgggcacgaccgagagcgggctcaactcggtggtgctcgccaacaactcggagggcgtgctgctgccgctcaacgagccggtgcacggcaccaagcgccggagccagatacagacgttcctggaacaccacggcggcccgggcgtgcagcacatcgcggtggccagcagtgacgtgctcaggacgctcaggaagatgcgtgcgcgctccgccatgggcggcttcgacttcctgccacccccgctgccgaagtactacgaaggcgtgcgacgccttgccggggatgtcctctcggaggcgcagatcaaggaatgccaggagctgggtgtgctcgtcgatagggacgaccaaggggtgttgctccaaatcgctaccaagccagtaggggacaggccgaccttgtggctggagatgatccagaggatcgggtgcatggagaaggacgagagaggggaagagtaccagaagggtggctgcggcgggttcggcaaaggcaacttctccgagctgttcaagtccattgaagattacgagaagtcccttgaagccaagcaatctgctgcagttcagggatcatag

SEQ ID NO: 130 - DNA, 1305 bp, Artificial Sequence
  HvHPPDm-F372A-F383W-02 Nucleotide Sequence
atgccgccgacgcccaccaccccagcagctaccggagctgcggctgcagtaacccctgagcatgctcggccccacaggatggtgaggtttaatccaagatcagatcgttttcatacactctcgttccaccatgttgagttctggtgcgccgacgcggcttcagcggccgggaggttcgccttcgcgctgggggcccctcttgccgcgcgtagtgatttgtctactgggaattcagcgcacgcgtcccagcttctccgaagcggcagtctcgcctttctcttcactgcaccatatgcaaatggatgtgatgcagcaactgcttccctgccgagcttttctgcggatgccgcgaggcgattcagtgctgaccatgggatcgccgtccggtcagttgctcttagagtggctgatgctgctgaggcattcagggcttcaaggcgtcgtggtgcacgcccggcgtttgccccggttgatcttgggcgggggtttgcttttgcagaggtggagctgtacggcgacgtggtgctccgatttgtttctcacccggacggcactgatgtgcccttcttgccaggatttgaaggtgtgaccaaccctgatgccgtggattatggactcacaagatttgatcatgtggttggcaatgttcctgaattggcacctgctgccgcttacatcgcaggttttactggcttccatgaatttgctgaattcacggcggaggatgttggtacaactgagtcagggctgaacagtgttgttttagccaacaactcagaaggagttctccttcccttgaatgaacctgttcatggaaccaagcgccgctcccaaattcaaacatttcttgagcaccacggcggccctggtgttcaacatattgctgtcgcctctagcgacgtcctgcgtacattacgcaagatgagggctcggtccgcaatgggtggtttcgacttcctccctccaccattgccaaaatattatgaaggcgtcagaagacttgcaggagatgtcctctctgaagctcagatcaaggagtgccaagaacttggcgtcttggttgatagagatgaccaaggagtacttctgcagatagccacaaaacccgttggtgacaggccaactctttggctggagatgattcagagaattggctgcatggagaaagatgaaagaggcgaggagtaccagaagggtggttgtggaggctttggaaaaggaaacttctcagagctgttcaagtccatagaagattacgagaaaagtctagaagccaagcagtctgctgcagtgcaaggttcctga

SEQ ID NO: 131 - protein, 444 aa, Zea mays
  The amino acid sequence of Zea mays wild-type HPPD (ZmHPPD)
MPPTPTAAAAGAAVAAASAAEQAAFRLVGHRNFVRFNPRSDRFHTLAFHHVELWCADAASAAGRFSFGLGAPLAARSDLSTGNSAHASLLLRSGSLSFLFTAPYAHGADAATAALPSFSAAAARRFAADHGLAVRAVALRVADAEEAFRTSVAAGARPAFGPVDLGRGFRLAEVELYGDVVLRYVSYPDGAAGEPFLPGFEGVASPGAADYGLSRFDHIVGNVPELAPAAAYFAGFTGFHEFAEFTTEDVGTAESGLNSMVLANNSENVLLPLNEPVHGTKRRSQIQTFLDHHGGPGVQHMALASDDVLRTLREMQARSAMGGFEFMAPPTSDYYDGVRRRAGDVLTEAQIKECQELGVLVDRDDQGVLLQIFPKPVGDRPTLFLEIIQRIGCMERDEKGQEYQKGGCGGFGKGNFSQLFKSIEDYEKSLEAMQAAAAATAQGS

SEQ ID NO: 132 - DNA, 1335 bp, Zea mays
  ZmHPPD-01 Nucleotide Sequence
atgcccccgacccccacagccgccgcagccggcgccgccgtggcggcggcatcagcagcggagcaggcggcgttccgcctcgtgggccaccgcaacttcgtccgcttcaacccgcgctccgaccgcttccacacgctcgcgttccaccacgtggagctctggtgcgccgacgcggcctccgccgcgggccgcttctccttcggcctgggcgcgccgctcgccgcgcgctccgacctctccacgggcaactccgcgcacgcgtccctgctgctccgctccggctccctctccttcctcttcacggcgccctacgcgcacggcgccgacgccgccaccgctgcgctgccctccttctccgccgccgccgcgcggcgcttcgcggccgaccacggcctcgcggtgcgcgccgtcgcgctccgcgtcgccgacgccgaggaggccttccgcaccagcgtcgcggccggggcgcgcccggctttcggccccgtcgacctcggccgcggcttccgcctcgccgaggtcgagctctacggcgacgtcgtgctccggtacgtgagctacccggacggcgcggcgggcgagcccttcctgccggggttcgagggcgtggccagccccggggcggccgactacgggctgagcaggttcgaccacatcgtcggcaacgtgccggagctggcgcccgccgccgcctacttcgccggcttcacggggttccacgagttcgccgagttcacgacggaggacgtgggcaccgcggagagcggcctcaactccatggtgctcgccaacaactcggagaacgtgctgctcccgctcaacgagccggtgcacggcaccaagcgccgcagccagatacagacgttcctggaccaccacggcggccccggcgtgcagcacatggcgctggccagcgacgacgtgctcaggacgctgagggagatgcaggcgcgctcggccatgggcggcttcgagttcatggcgcctcccacatccgactactatgacggcgtgaggcggcgcgccggggacgtgctcacggaagcacagattaaggagtgccaggagctaggggtgctggtggatagggatgaccagggcgtgctgctccaaatcttccccaagccagtgggggacaggccaacgctgttcttggagatcatccaaaggatcgggtgcatggagagggatgagaaggggcaagaataccagaagggtggctgcggcgggttcggcaagggaaacttctcgcagctgttcaaatccatcgaggattatgagaagtcccttgaagccatgcaagctgctgcagcagctacagctcagggatcctag

SEQ ID NO: 133 - DNA, 1335 bp, Artificial Sequence
  ZmHPPD-02 Nucleotide Sequence
atgccacccacacccacagcagcagcggcgggcgcagcggtcgcagcggcgtcagcggcggagcaagcggcgttcagattggttggtcaccgcaacttcgtgagattcaatcctcgctcagatagattccatactctggccttccaccatgttgagctttggtgcgctgatgctgcttctgctgctggaaggttcagcttcggtttgggtgctcccctcgctgctagatctgatttgagcactggtaactcagcacatgcttccctcctgcttagatctggctctctgagcttccttttcactgctccatatgctcatggtgctgatgctgctacagctgctctcccttcattctccgctgctgctgctaggagattcgctgctgatcacggattggctgtgagggctgttgcacttagagttgctgatgctgaggaggccttccgcacctctgttgctgctggagccagaccagctttcggacctgttgatctcggaaggggtttccgcctggctgaggtggagctttacggcgatgtggttctgcgctacgttagctatcctgatggtgctgctggtgaacctttccttccaggattcgagggtgtggcctcaccaggtgccgctgattacggcctgtccagattcgaccacattgttggaaatgttcctgagcttgctccagctgctgcctacttcgctggcttcaccggattccatgagttcgccgagttcaccactgaggatgtgggaactgctgagtctggtttgaatagcatggtgctcgccaacaattcagagaacgttttgctccctctgaatgagcccgtgcacggaacaaagagaaggtcccagattcaaaccttcttggatcaccacggcggcccaggtgttcagcatatggctctcgcctccgatgacgtgttgagaaccctcagggagatgcaagccaggtctgctatgggtggcttcgagttcatggccccacctacaagcgattactatgatggtgtgcgcagaagggctggcgacgttcttaccgaggctcagatcaaggagtgccaagagctgggcgtgcttgttgatagagatgaccagggagttctgcttcaaattttccccaagccagtgggcgacaggcctactttgttcctcgagattatccagagaatcggatgcatggagagggatgagaagggtcaggagtaccaaaagggaggttgcggcggattcggcaagggaaatttctcacaactcttcaagtccatcgaggactatgaaaagagtctggaagcgatgcaggcagcagcagcagcaaccgcacaggggtcgtga

SEQ ID NO: 134 - protein, 444 aa, Artificial Sequence
  ZmHPPDm-F372A Amino Acid Sequence
MPPTPTAAAAGAAVAAASAAEQAAFRLVGHRNFVRFNPRSDRFHTLAFHHVELWCADAASAAGRFSFGLGAPLAARSDLSTGNSAHASLLLRSGSLSFLFTAPYAHGADAATAALPSFSAAAARRFAADHGLAVRAVALRVADAEEAFRTSVAAGARPAFGPVDLGRGFRLAEVELYGDVVLRYVSYPDGAAGEPFLPGFEGVASPGAADYGLSRFDHIVGNVPELAPAAAYFAGFTGFHEFAEFTTEDVGTAESGLNSMVLANNSENVLLPLNEPVHGTKRRSQIQTFLDHHGGPGVQHMALASDDVLRTLREMQARSAMGGFEFMAPPTSDYYDGVRRRAGDVLTEAQIKECQELGVLVDRDDQGVLLQIAPKPVGDRPTLFLEIIQRIGCMERDEKGQEYQKGGCGGFGKGNFSQLFKSIEDYEKSLEAMQAAAAATAQGS

SEQ ID NO: 135 - DNA, 1335 bp, Artificial Sequence
  ZmHPPDm-F372A-01 Nucleotide Sequence
atgcccccgacccccacagccgccgcagccggcgccgccgtggcggcggcatcagcagcggagcaggcggcgttccgcctcgtgggccaccgcaacttcgtccgcttcaacccgcgctccgaccgcttccacacgctcgcgttccaccacgtggagctctggtgcgccgacgcggcctccgccgcgggccgcttctccttcggcctgggcgcgccgctcgccgcgcgctccgacctctccacgggcaactccgcgcacgcgtccctgctgctccgctccggctccctctccttcctcttcacggcgccctacgcgcacggcgccgacgccgccaccgctgcgctgccctccttctccgccgccgccgcgcggcgcttcgcggccgaccacggcctcgcggtgcgcgccgtcgcgctccgcgtcgccgacgccgaggaggccttccgcaccagcgtcgcggccggggcgcgcccggctttcggccccgtcgacctcggccgcggcttccgcctcgccgaggtcgagctctacggcgacgtcgtgctccggtacgtgagctacccggacggcgcggcgggcgagcccttcctgccggggttcgagggcgtggccagccccggggcggccgactacgggctgagcaggttcgaccacatcgtcggcaacgtgccggagctggcgcccgccgccgcctacttcgccggcttcacggggttccacgagttcgccgagttcacgacggaggacgtgggcaccgcggagagcggcctcaactccatggtgctcgccaacaactcggagaacgtgctgctcccgctcaacgagccggtgcacggcaccaagcgccgcagccagatacagacgttcctggaccaccacggcggccccggcgtgcagcacatggcgctggccagcgacgacgtgctcaggacgctgagggagatgcaggcgcgctcggccatgggcggcttcgagttcatggcgcctcccacatccgactactatgacggcgtgaggcggcgcgccggggacgtgctcacggaagcacagattaaggagtgccaggagctaggggtgctggtggatagggatgaccagggcgtgctgctccaaatcgctcccaagccagtgggggacaggccaacgctgttcttggagatcatccaaaggatcgggtgcatggagagggatgagaaggggcaagaataccagaagggtggctgcggcgggttcggcaagggaaacttctcgcagctgttcaaatccatcgaggattatgagaagtcccttgaagccatgcaagctgctgcagcagctacagctcagggatcctag

SEQ ID NO: 136 - DNA, 1335 bp, Artificial Sequence
  ZmHPPDm-F372A-02 Nucleotide Sequence
atgccacccacacccacagcagcagcggcgggcgcagcggtcgcagcggcgtcagcggcggagcaagcggcgttcagattggttggtcaccgcaacttcgtgagattcaatcctcgctcagatagattccatactctggccttccaccatgttgagctttggtgcgctgatgctgcttctgctgctggaaggttcagcttcggtttgggtgctcccctcgctgctagatctgatttgagcactggtaactcagcacatgcttccctcctgcttagatctggctctctgagcttccttttcactgctccatatgctcatggtgctgatgctgctacagctgctctcccttcattctccgctgctgctgctaggagattcgctgctgatcacggattggctgtgagggctgttgcacttagagttgctgatgctgaggaggccttccgcacctctgttgctgctggagccagaccagctttcggacctgttgatctcggaaggggtttccgcctggctgaggtggagctttacggcgatgtggttctgcgctacgttagctatcctgatggtgctgctggtgaacctttccttccaggattcgagggtgtggcctcaccaggtgccgctgattacggcctgtccagattcgaccacattgttggaaatgttcctgagcttgctccagctgctgcctacttcgctggcttcaccggattccatgagttcgccgagttcaccactgaggatgtgggaactgctgagtctggtttgaatagcatggtgctcgccaacaattcagagaacgttttgctccctctgaatgagcccgtgcacggaacaaagagaaggtcccagattcaaaccttcttggatcaccacggcggcccaggtgttcagcatatggctctcgcctccgatgacgtgttgagaaccctcagggagatgcaagccaggtctgctatgggtggcttcgagttcatggccccacctacaagcgattactatgatggtgtgcgcagaagggctggcgacgttcttaccgaggctcagatcaaggagtgccaagagctgggcgtgcttgttgatagagatgaccagggagttctgcttcaaattgctcccaagccagtgggcgacaggcctactttgttcctcgagattatccagagaatcggatgcatggagagggatgagaagggtcaggagtaccaaaagggaggttgcggcggattcggcaagggaaatttctcacaactcttcaagtccatcgaggactatgaaaagagtctggaagcgatgcaggcagcagcagcagcaaccgcacaggggtcgtga

SEQ ID NO: 137 - protein, 444 aa, Artificial Sequence
  ZmHPPDm-F383W Amino Acid Sequence
MPPTPTAAAAGAAVAAASAAEQAAFRLVGHRNFVRFNPRSDRFHTLAFHHVELWCADAASAAGRFSFGLGAPLAARSDLSTGNSAHASLLLRSGSLSFLFTAPYAHGADAATAALPSFSAAAARRFAADHGLAVRAVALRVADAEEAFRTSVAAGARPAFGPVDLGRGFRLAEVELYGDVVLRYVSYPDGAAGEPFLPGFEGVASPGAADYGLSRFDHIVGNVPELAPAAAYFAGFTGFHEFAEFTTEDVGTAESGLNSMVLANNSENVLLPLNEPVHGTKRRSQIQTFLDHHGGPGVQHMALASDDVLRTLREMQARSAMGGFEFMAPPTSDYYDGVRRRAGDVLTEAQIKECQELGVLVDRDDQGVLLQIFPKPVGDRPTLWLEIIQRIGCMERDEKGQEYQKGGCGGFGKGNFSQLFKSIEDYEKSLEAMQAAAAATAQGS

SEQ ID NO: 138 - DNA, 1335 bp, Artificial Sequence
  ZmHPPDm-F383W-01 Nucleotide Sequence
atgcccccgacccccacagccgccgcagccggcgccgccgtggcggcggcatcagcagcggagcaggcggcgttccgcctcgtgggccaccgcaacttcgtccgcttcaacccgcgctccgaccgcttccacacgctcgcgttccaccacgtggagctctggtgcgccgacgcggcctccgccgcgggccgcttctccttcggcctgggcgcgccgctcgccgcgcgctccgacctctccacgggcaactccgcgcacgcgtccctgctgctccgctccggctccctctccttcctcttcacggcgccctacgcgcacggcgccgacgccgccaccgctgcgctgccctccttctccgccgccgccgcgcggcgcttcgcggccgaccacggcctcgcggtgcgcgccgtcgcgctccgcgtcgccgacgccgaggaggccttccgcaccagcgtcgcggccggggcgcgcccggctttcggccccgtcgacctcggccgcggcttccgcctcgccgaggtcgagctctacggcgacgtcgtgctccggtacgtgagctacccggacggcgcggcgggcgagcccttcctgccggggttcgagggcgtggccagccccggggcggccgactacgggctgagcaggttcgaccacatcgtcggcaacgtgccggagctggcgcccgccgccgcctacttcgccggcttcacggggttccacgagttcgccgagttcacgacggaggacgtgggcaccgcggagagcggcctcaactccatggtgctcgccaacaactcggagaacgtgctgctcccgctcaacgagccggtgcacggcaccaagcgccgcagccagatacagacgttcctggaccaccacggcggccccggcgtgcagcacatggcgctggccagcgacgacgtgctcaggacgctgagggagatgcaggcgcgctcggccatgggcggcttcgagttcatggcgcctcccacatccgactactatgacggcgtgaggcggcgcgccggggacgtgctcacggaagcacagattaaggagtgccaggagctaggggtgctggtggatagggatgaccagggcgtgctgctccaaatcttccccaagccagtgggggacaggccaacgctgtggttggagatcatccaaaggatcgggtgcatggagagggatgagaaggggcaagaataccagaagggtggctgcggcgggttcggcaagggaaacttctcgcagctgttcaaatccatcgaggattatgagaagtcccttgaagccatgcaagctgctgcagcagctacagctcagggatcctag

SEQ ID NO: 139 - DNA, 1335 bp, Artificial Sequence
  ZmHPPDm-F383W-02 Nucleotide Sequence
atgccacccacacccacagcagcagcggcgggcgcagcggtcgcagcggcgtcagcggcggagcaagcggcgttcagattggttggtcaccgcaacttcgtgagattcaatcctcgctcagatagattccatactctggccttccaccatgttgagctttggtgcgctgatgctgcttctgctgctggaaggttcagcttcggtttgggtgctcccctcgctgctagatctgatttgagcactggtaactcagcacatgcttccctcctgcttagatctggctctctgagcttccttttcactgctccatatgctcatggtgctgatgctgctacagctgctctcccttcattctccgctgctgctgctaggagattcgctgctgatcacggattggctgtgagggctgttgcacttagagttgctgatgctgaggaggccttccgcacctctgttgctgctggagccagaccagctttcggacctgttgatctcggaaggggtttccgcctggctgaggtggagctttacggcgatgtggttctgcgctacgttagctatcctgatggtgctgctggtgaacctttccttccaggattcgagggtgtggcctcaccaggtgccgctgattacggcctgtccagattcgaccacattgttggaaatgttcctgagcttgctccagctgctgcctacttcgctggcttcaccggattccatgagttcgccgagttcaccactgaggatgtgggaactgctgagtctggtttgaatagcatggtgctcgccaacaattcagagaacgttttgctccctctgaatgagcccgtgcacggaacaaagagaaggtcccagattcaaaccttcttggatcaccacggcggcccaggtgttcagcatatggctctcgcctccgatgacgtgttgagaaccctcagggagatgcaagccaggtctgctatgggtggcttcgagttcatggccccacctacaagcgattactatgatggtgtgcgcagaagggctggcgacgttcttaccgaggctcagatcaaggagtgccaagagctgggcgtgcttgttgatagagatgaccagggagttctgcttcaaattttccccaagccagtgggcgacaggcctactttgtggctcgagattatccagagaatcggatgcatggagagggatgagaagggtcaggagtaccaaaagggaggttgcggcggattcggcaagggaaatttctcacaactcttcaagtccatcgaggactatgaaaagagtctggaagcgatgcaggcagcagcagcagcaaccgcacaggggtcgtga

SEQ ID NO: 140 - protein, 444 aa, Artificial Sequence
  ZmHPPDm-F372A-F383W Amino Acid Sequence
MPPTPTAAAAGAAVAAASAAEQAAFRLVGHRNFVRFNPRSDRFHTLAFHHVELWCADAASAAGRFSFGLGAPLAARSDLSTGNSAHASLLLRSGSLSFLFTAPYAHGADAATAALPSFSAAAARRFAADHGLAVRAVALRVADAEEAFRTSVAAGARPAFGPVDLGRGFRLAEVELYGDVVLRYVSYPDGAAGEPFLPGFEGVASPGAADYGLSRFDHIVGNVPELAPAAAYFAGFTGFHEFAEFTTEDVGTAESGLNSMVLANNSENVLLPLNEPVHGTKRRSQIQTFLDHHGGPGVQHMALASDDVLRTLREMQARSAMGGFEFMAPPTSDYYDGVRRRAGDVLTEAQIKECQELGVLVDRDDQGVLLQIAPKPVGDRPTLWLEIIQRIGCMERDEKGQEYQKGGCGGFGKGNFSQLFKSIEDYEKSLEAMQAAAAATAQGS

SEQ ID NO: 141 - DNA, 1335 bp, Artificial Sequence
  ZmHPPDm-F372A-F383W-01 Nucleotide Sequence
atgcccccgacccccacagccgccgcagccggcgccgccgtggcggcggcatcagcagcggagcaggcggcgttccgcctcgtgggccaccgcaacttcgtccgcttcaacccgcgctccgaccgcttccacacgctcgcgttccaccacgtggagctctggtgcgccgacgcggcctccgccgcgggccgcttctccttcggcctgggcgcgccgctcgccgcgcgctccgacctctccacgggcaactccgcgcacgcgtccctgctgctccgctccggctccctctccttcctcttcacggcgccctacgcgcacggcgccgacgccgccaccgctgcgctgccctccttctccgccgccgccgcgcggcgcttcgcggccgaccacggcctcgcggtgcgcgccgtcgcgctccgcgtcgccgacgccgaggaggccttccgcaccagcgtcgcggccggggcgcgcccggctttcggccccgtcgacctcggccgcggcttccgcctcgccgaggtcgagctctacggcgacgtcgtgctccggtacgtgagctacccggacggcgcggcgggcgagcccttcctgccggggttcgagggcgtggccagccccggggcggccgactacgggctgagcaggttcgaccacatcgtcggcaacgtgccggagctggcgcccgccgccgcctacttcgccggcttcacggggttccacgagttcgccgagttcacgacggaggacgtgggcaccgcggagagcggcctcaactccatggtgctcgccaacaactcggagaacgtgctgctcccgctcaacgagccggtgcacggcaccaagcgccgcagccagatacagacgttcctggaccaccacggcggccccggcgtgcagcacatggcgctggccagcgacgacgtgctcaggacgctgagggagatgcaggcgcgctcggccatgggcggcttcgagttcatggcgcctcccacatccgactactatgacggcgtgaggcggcgcgccggggacgtgctcacggaagcacagattaaggagtgccaggagctaggggtgctggtggatagggatgaccagggcgtgctgctccaaatcgctcccaagccagtgggggacaggccaacgctgtggttggagatcatccaaaggatcgggtgcatggagagggatgagaaggggcaagaataccagaagggtggctgcggcgggttcggcaagggaaacttctcgcagctgttcaaatccatcgaggattatgagaagtcccttgaagccatgcaagctgctgcagcagctacagctcagggatcctag

SEQ ID NO: 142 - DNA, 1335 bp, Artificial Sequence
  ZmHPPDm-F372A-F383W-02 Nucleotide Sequence
atgccacccacacccacagcagcagcggcgggcgcagcggtcgcagcggcgtcagcggcggagcaagcggcgttcagattggttggtcaccgcaacttcgtgagattcaatcctcgctcagatagattccatactctggccttccaccatgttgagctttggtgcgctgatgctgcttctgctgctggaaggttcagcttcggtttgggtgctcccctcgctgctagatctgatttgagcactggtaactcagcacatgcttccctcctgcttagatctggctctctgagcttccttttcactgctccatatgctcatggtgctgatgctgctacagctgctctcccttcattctccgctgctgctgctaggagattcgctgctgatcacggattggctgtgagggctgttgcacttagagttgctgatgctgaggaggccttccgcacctctgttgctgctggagccagaccagctttcggacctgttgatctcggaaggggtttccgcctggctgaggtggagctttacggcgatgtggttctgcgctacgttagctatcctgatggtgctgctggtgaacctttccttccaggattcgagggtgtggcctcaccaggtgccgctgattacggcctgtccagattcgaccacattgttggaaatgttcctgagcttgctccagctgctgcctacttcgctggcttcaccggattccatgagttcgccgagttcaccactgaggatgtgggaactgctgagtctggtttgaatagcatggtgctcgccaacaattcagagaacgttttgctccctctgaatgagcccgtgcacggaacaaagagaaggtcccagattcaaaccttcttggatcaccacggcggcccaggtgttcagcatatggctctcgcctccgatgacgtgttgagaaccctcagggagatgcaagccaggtctgctatgggtggcttcgagttcatggccccacctacaagcgattactatgatggtgtgcgcagaagggctggcgacgttcttaccgaggctcagatcaaggagtgccaagagctgggcgtgcttgttgatagagatgaccagggagttctgcttcaaattgctcccaagccagtgggcgacaggcctactttgtggctcgagattatccagagaatcggatgcatggagagggatgagaagggtcaggagtaccaaaagggaggttgcggcggattcggcaagggaaatttctcacaactcttcaagtccatcgaggactatgaaaagagtctggaagcgatgcaggcagcagcagcagcaaccgcacaggggtcgtga

SEQ ID NO: 143 - protein, 358 aa, Pseudomonas fluorescens
  The amino acid sequence of Pseudomonas fluorescens wild-type HPPD
MADLYENPMGLMGFEFIEFASPTPGTLEPIFEIMGFTKVATHRSKNVHLYRQGEINLILNNEPNSIASYFAAEHGPSVCGMAFRVKDSQKAYNRALELGAQPIHIDTGPMELNLPAIKGIGGAPLYLIDRFGEGSSIYDIDFVYLEGVERNPVGAGLKVIDHLTHNVYRGRMVYWANFYEKLFNFREARYFDIKGEYTGLTSKAMSAPDGMIRIPLNEESSKGAGQIEEFLMQFNGEGIQHVAFLTDDLVKTWDALKKIGMRFMTAPPDTYYEMLEGRLPDHGEPVDQLQARGILLDGSSVEGDKRLLLQIFSETLMGPVFFEFIQRKGDDGFGEGNFKALFESIERDQVRRGVLTAD

SEQ ID NO: 144 - DNA, 1077 bp, Pseudomonas fluorescens
  PfHPPD-01 Nucleotide Sequence
atggcagatctatacgaaaacccaatgggcctgatgggctttgaattcatcgaattcgcgtcgccgacgccgggcaccctggagccgatcttcgagatcatgggcttcaccaaagtcgcgacccaccgttccaagaacgtgcacctgtaccgccagggcgagatcaacctgatcctcaacaacgagcccaacagcatcgcctcctactttgcggccgaacacggcccgtcggtgtgcggcatggcgttccgcgtgaaggactcgcaaaaggcctacaaccgcgccctggaactcggcgcccagccgatccatattgacaccgggccgatggaattgaacctgccggcgatcaagggcatcggcggcgcgccgttgtacctgatcgaccgtttcggcgaaggcagctcgatctacgacatcgacttcgtgtacctcgaaggtgtggagcgcaatccggtcggtgcaggtctcaaagtcatcgaccacctgacccacaacgtctatcgcggccgcatggtctactgggccaacttctacgagaaattgttcaacttccgtgaagcgcgttacttcgatatcaagggcgagtacaccggcctgacttccaaggccatgagtgcgccggacggcatgatccgcatcccgctgaacgaagagtcgtccaagggcgcggggcagatcgaagagttcctgatgcagttcaacggcgaaggcatccagcacgtggcgttcctcaccgacgacctggtcaagacctgggacgcgttgaagaaaatcggcatgcgcttcatgaccgcgccgccagacacttattacgaaatgctcgaaggccgcctgcctgaccacggcgagccggtggatcaactgcaggcacgcggtatcctgctggacggatcttccgtggaaggcgacaaacgcctgctgctgcagatcttctcggaaaccctgatgggcccggtgttcttcgaattcatccagcgcaagggcgacgatgggtttggcgagggcaacttcaaggcgctgttcgagtccatcgaacgtgaccaggtgcgtcgtggtgtattgaccgccgattaa

SEQ ID NO: 145 - DNA, 1077 bp, Artificial Sequence
  PfHPPD-02 Nucleotide Sequence
atggccgatttgtacgagaacccaatgggactcatgggtttcgagttcattgagttcgcttcccccaccccaggtactttggagcctattttcgagatcatgggcttcactaaggttgccacacacaggtctaagaatgtgcatctctaccgccaaggagagattaacctgatccttaacaatgagcctaatagcatcgcctcatacttcgctgctgagcatggtccatctgtttgcggcatggctttcagagtgaaggattcacaaaaggcctacaacagggctttggagctcggcgcccagcccattcatatcgacaccggacctatggagctgaatcttcctgccattaagggcatcggcggagctccattgtacctcattgatcgcttcggcgagggctcctctatctacgatatcgacttcgtgtacctggagggcgttgagagaaaccctgtgggagctggtctgaaggttatcgaccaccttactcataatgtttacagaggaaggatggtgtactgggccaacttctacgagaagctgttcaatttccgcgaggctagatacttcgatattaagggcgagtacacaggacttacctccaaggccatgtctgctcccgacggtatgattaggatcccattgaacgaggagagctcaaagggcgccggacagattgaggagttcctcatgcaattcaatggtgaaggcatccagcacgttgctttcctgacagatgaccttgtgaagacctgggatgccctcaagaagattggcatgaggttcatgaccgctccacctgacacttactacgagatgttggagggacgcctccctgatcatggcgagcccgttgaccagctgcaagctagaggaatcctcctggatggttcctctgtggagggcgacaagaggcttttgctccaaattttcagcgagactcttatgggacccgtgttcttcgagttcatccagaggaagggcgatgacggattcggcgagggcaacttcaaggccctgttcgagtctattgagagagatcaggtgaggcgcggcgttcttacagctgactga

SEQ ID NO: 146 - protein, 358 aa, Artificial Sequence
  PfHPPDm-F372A Amino Acid Sequence
MADLYENPMGLMGFEFIEFASPTPGTLEPIFEIMGFTKVATHRSKNVHLYRQGEINLILNNEPNSIASYFAAEHGPSVCGMAFRVKDSQKAYNRALELGAQPIHIDTGPMELNLPAIKGIGGAPLYLIDRFGEGSSIYDIDFVYLEGVERNPVGAGLKVIDHLTHNVYRGRMVYWANFYEKLFNFREARYFDIKGEYTGLTSKAMSAPDGMIRIPLNEESSKGAGQIEEFLMQFNGEGIQHVAFLTDDLVKTWDALKKIGMRFMTAPPDTYYEMLEGRLPDHGEPVDQLQARGILLDGSSVEGDKRLLLQIASETLMGPVFFEFIQRKGDDGFGEGNFKALFESIERDQVRRGVLTAD

SEQ ID NO: 147 - DNA, 1077 bp, Artificial Sequence
  PfHPPDm-F372A-01 Nucleotide Sequence
atggcagatctatacgaaaacccaatgggcctgatgggctttgaattcatcgaattcgcgtcgccgacgccgggcaccctggagccgatcttcgagatcatgggcttcaccaaagtcgcgacccaccgttccaagaacgtgcacctgtaccgccagggcgagatcaacctgatcctcaacaacgagcccaacagcatcgcctcctactttgcggccgaacacggcccgtcggtgtgcggcatggcgttccgcgtgaaggactcgcaaaaggcctacaaccgcgccctggaactcggcgcccagccgatccatattgacaccgggccgatggaattgaacctgccggcgatcaagggcatcggcggcgcgccgttgtacctgatcgaccgtttcggcgaaggcagctcgatctacgacatcgacttcgtgtacctcgaaggtgtggagcgcaatccggtcggtgcaggtctcaaagtcatcgaccacctgacccacaacgtctatcgcggccgcatggtctactgggccaacttctacgagaaattgttcaacttccgtgaagcgcgttacttcgatatcaagggcgagtacaccggcctgacttccaaggccatgagtgcgccggacggcatgatccgcatcccgctgaacgaagagtcgtccaagggcgcggggcagatcgaagagttcctgatgcagttcaacggcgaaggcatccagcacgtggcgttcctcaccgacgacctggtcaagacctgggacgcgttgaagaaaatcggcatgcgcttcatgaccgcgccgccagacacttattacgaaatgctcgaaggccgcctgcctgaccacggcgagccggtggatcaactgcaggcacgcggtatcctgctggacggatcttccgtggaaggcgacaaacgcctgctgctgcagatcgcttcggaaaccctgatgggcccggtgttcttcgaattcatccagcgcaagggcgacgatgggtttggcgagggcaacttcaaggcgctgttcgagtccatcgaacgtgaccaggtgcgtcgtggtgtattgaccgccgattaa

SEQ ID NO: 148 - DNA, 1077 bp, Artificial Sequence
  PfHPPDm-F372A-02 Nucleotide Sequence
atggccgatttgtacgagaacccaatgggactcatgggtttcgagttcattgagttcgcttcccccaccccaggtactttggagcctattttcgagatcatgggcttcactaaggttgccacacacaggtctaagaatgtgcatctctaccgccaaggagagattaacctgatccttaacaatgagcctaatagcatcgcctcatacttcgctgctgagcatggtccatctgtttgcggcatggctttcagagtgaaggattcacaaaaggcctacaacagggctttggagctcggcgcccagcccattcatatcgacaccggacctatggagctgaatcttcctgccattaagggcatcggcggagctccattgtacctcattgatcgcttcggcgagggctcctctatctacgatatcgacttcgtgtacctggagggcgttgagagaaaccctgtgggagctggtctgaaggttatcgaccaccttactcataatgtttacagaggaaggatggtgtactgggccaacttctacgagaagctgttcaatttccgcgaggctagatacttcgatattaagggcgagtacacaggacttacctccaaggccatgtctgctcccgacggtatgattaggatcccattgaacgaggagagctcaaagggcgccggacagattgaggagttcctcatgcaattcaatggtgaaggcatccagcacgttgctttcctgacagatgaccttgtgaagacctgggatgccctcaagaagattggcatgaggttcatgaccgctccacctgacacttactacgagatgttggagggacgcctccctgatcatggcgagcccgttgaccagctgcaagctagaggaatcctcctggatggttcctctgtggagggcgacaagaggcttttgctccaaattgctagcgagactcttatgggacccgtgttcttcgagttcatccagaggaagggcgatgacggattcggcgagggcaacttcaaggccctgttcgagtctattgagagagatcaggtgaggcgcggcgttcttacagctgactga

SEQ ID NO: 149 - protein, 358 aa, Artificial Sequence
  PfHPPDm-F383W Amino Acid Sequence
MADLYENPMGLMGFEFIEFASPTPGTLEPIFEIMGFTKVATHRSKNVHLYRQGEINLILNNEPNSIASYFAAEHGPSVCGMAFRVKDSQKAYNRALELGAQPIHIDTGPMELNLPAIKGIGGAPLYLIDRFGEGSSIYDIDFVYLEGVERNPVGAGLKVIDHLTHNVYRGRMVYWANFYEKLFNFREARYFDIKGEYTGLTSKAMSAPDGMIRIPLNEESSKGAGQIEEFLMQFNGEGIQHVAFLTDDLVKTWDALKKIGMRFMTAPPDTYYEMLEGRLPDHGEPVDQLQARGILLDGSSVEGDKRLLLQIFSETLMGPVWFEFIQRKGDDGFGEGNFKALFESIERDQVRRGVLTAD

SEQ ID NO: 150 - DNA, 1077 bp, Artificial Sequence
  PfHPPDm-F383W-01 Nucleotide Sequence
atggcagatctatacgaaaacccaatgggcctgatgggctttgaattcatcgaattcgcgtcgccgacgccgggcaccctggagccgatcttcgagatcatgggcttcaccaaagtcgcgacccaccgttccaagaacgtgcacctgtaccgccagggcgagatcaacctgatcctcaacaacgagcccaacagcatcgcctcctactttgcggccgaacacggcccgtcggtgtgcggcatggcgttccgcgtgaaggactcgcaaaaggcctacaaccgcgccctggaactcggcgcccagccgatccatattgacaccgggccgatggaattgaacctgccggcgatcaagggcatcggcggcgcgccgttgtacctgatcgaccgtttcggcgaaggcagctcgatctacgacatcgacttcgtgtacctcgaaggtgtggagcgcaatccggtcggtgcaggtctcaaagtcatcgaccacctgacccacaacgtctatcgcggccgcatggtctactgggccaacttctacgagaaattgttcaacttccgtgaagcgcgttacttcgatatcaagggcgagtacaccggcctgacttccaaggccatgagtgcgccggacggcatgatccgcatcccgctgaacgaagagtcgtccaagggcgcggggcagatcgaagagttcctgatgcagttcaacggcgaaggcatccagcacgtggcgttcctcaccgacgacctggtcaagacctgggacgcgttgaagaaaatcggcatgcgcttcatgaccgcgccgccagacacttattacgaaatgctcgaaggccgcctgcctgaccacggcgagccggtggatcaactgcaggcacgcggtatcctgctggacggatcttccgtggaaggcgacaaacgcctgctgctgcagatcttctcggaaaccctgatgggcccggtgtggttcgaattcatccagcgcaagggcgacgatgggtttggcgagggcaacttcaaggcgctgttcgagtccatcgaacgtgaccaggtgcgtcgtggtgtattgaccgccgattaa

SEQ ID NO: 151 - DNA, 1077 bp, Artificial Sequence
  PfHPPDm-F383W-02 Nucleotide Sequence
atggccgatttgtacgagaacccaatgggactcatgggtttcgagttcattgagttcgcttcccccaccccaggtactttggagcctattttcgagatcatgggcttcactaaggttgccacacacaggtctaagaatgtgcatctctaccgccaaggagagattaacctgatccttaacaatgagcctaatagcatcgcctcatacttcgctgctgagcatggtccatctgtttgcggcatggctttcagagtgaaggattcacaaaaggcctacaacagggctttggagctcggcgcccagcccattcatatcgacaccggacctatggagctgaatcttcctgccattaagggcatcggcggagctccattgtacctcattgatcgcttcggcgagggctcctctatctacgatatcgacttcgtgtacctggagggcgttgagagaaaccctgtgggagctggtctgaaggttatcgaccaccttactcataatgtttacagaggaaggatggtgtactgggccaacttctacgagaagctgttcaatttccgcgaggctagatacttcgatattaagggcgagtacacaggacttacctccaaggccatgtctgctcccgacggtatgattaggatcccattgaacgaggagagctcaaagggcgccggacagattgaggagttcctcatgcaattcaatggtgaaggcatccagcacgttgctttcctgacagatgaccttgtgaagacctgggatgccctcaagaagattggcatgaggttcatgaccgctccacctgacacttactacgagatgttggagggacgcctccctgatcatggcgagcccgttgaccagctgcaagctagaggaatcctcctggatggttcctctgtggagggcgacaagaggcttttgctccaaattttcagcgagactcttatgggacccgtgtggttcgagttcatccagaggaagggcgatgacggattcggcgagggcaacttcaaggccctgttcgagtctattgagagagatcaggtgaggcgcggcgttcttacagctgactga

SEQ ID NO: 152 - protein, 358 aa, Artificial Sequence
  PfHPPDm-F372A-F383W Amino Acid Sequence
MADLYENPMGLMGFEFIEFASPTPGTLEPIFEIMGFTKVATHRSKNVHLYRQGEINLILNNEPNSIASYFAAEHGPSVCGMAFRVKDSQKAYNRALELGAQPIHIDTGPMELNLPAIKGIGGAPLYLIDRFGEGSSIYDIDFVYLEGVERNPVGAGLKVIDHLTHNVYRGRMVYWANFYEKLFNFREARYFDIKGEYTGLTSKAMSAPDGMIRIPLNEESSKGAGQIEEFLMQFNGEGIQHVAFLTDDLVKTWDALKKIGMRFMTAPPDTYYEMLEGRLPDHGEPVDQLQARGILLDGSSVEGDKRLLLQIASETLMGPVWFEFIQRKGDDGFGEGNFKALFESIERDQVRRGVLTAD

SEQ ID NO: 153 - DNA, 1077 bp, Artificial Sequence
  PfHPPDm-F372A-F383W-01 Nucleotide Sequence
atggcagatctatacgaaaacccaatgggcctgatgggctttgaattcatcgaattcgcgtcgccgacgccgggcaccctggagccgatcttcgagatcatgggcttcaccaaagtcgcgacccaccgttccaagaacgtgcacctgtaccgccagggcgagatcaacctgatcctcaacaacgagcccaacagcatcgcctcctactttgcggccgaacacggcccgtcggtgtgcggcatggcgttccgcgtgaaggactcgcaaaaggcctacaaccgcgccctggaactcggcgcccagccgatccatattgacaccgggccgatggaattgaacctgccggcgatcaagggcatcggcggcgcgccgttgtacctgatcgaccgtttcggcgaaggcagctcgatctacgacatcgacttcgtgtacctcgaaggtgtggagcgcaatccggtcggtgcaggtctcaaagtcatcgaccacctgacccacaacgtctatcgcggccgcatggtctactgggccaacttctacgagaaattgttcaacttccgtgaagcgcgttacttcgatatcaagggcgagtacaccggcctgacttccaaggccatgagtgcgccggacggcatgatccgcatcccgctgaacgaagagtcgtccaagggcgcggggcagatcgaagagttcctgatgcagttcaacggcgaaggcatccagcacgtggcgttcctcaccgacgacctggtcaagacctgggacgcgttgaagaaaatcggcatgcgcttcatgaccgcgccgccagacacttattacgaaatgctcgaaggccgcctgcctgaccacggcgagccggtggatcaactgcaggcacgcggtatcctgctggacggatcttccgtggaaggcgacaaacgcctgctgctgcagatcgcttcggaaaccctgatgggcccggtgtggttcgaattcatccagcgcaagggcgacgatgggtttggcgagggcaacttcaaggcgctgttcgagtccatcgaacgtgaccaggtgcgtcgtggtgtattgaccgccgattaa

SEQ ID NO: 154 - DNA, 1077 bp, Artificial Sequence
  PfHPPDm-F372A-F383W-02 Nucleotide Sequence
atggccgatttgtacgagaacccaatgggactcatgggtttcgagttcattgagttcgcttcccccaccccaggtactttggagcctattttcgagatcatgggcttcactaaggttgccacacacaggtctaagaatgtgcatctctaccgccaaggagagattaacctgatccttaacaatgagcctaatagcatcgcctcatacttcgctgctgagcatggtccatctgtttgcggcatggctttcagagtgaaggattcacaaaaggcctacaacagggctttggagctcggcgcccagcccattcatatcgacaccggacctatggagctgaatcttcctgccattaagggcatcggcggagctccattgtacctcattgatcgcttcggcgagggctcctctatctacgatatcgacttcgtgtacctggagggcgttgagagaaaccctgtgggagctggtctgaaggttatcgaccaccttactcataatgtttacagaggaaggatggtgtactgggccaacttctacgagaagctgttcaatttccgcgaggctagatacttcgatattaagggcgagtacacaggacttacctccaaggccatgtctgctcccgacggtatgattaggatcccattgaacgaggagagctcaaagggcgccggacagattgaggagttcctcatgcaattcaatggtgaaggcatccagcacgttgctttcctgacagatgaccttgtgaagacctgggatgccctcaagaagattggcatgaggttcatgaccgctccacctgacacttactacgagatgttggagggacgcctccctgatcatggcgagcccgttgaccagctgcaagctagaggaatcctcctggatggttcctctgtggagggcgacaagaggcttttgctccaaattgctagcgagactcttatgggacccgtgtggttcgagttcatccagaggaagggcgatgacggattcggcgagggcaacttcaaggccctgttcgagtctattgagagagatcaggtgaggcgcggcgttcttacagctgactga

SEQ ID NO: 155 - protein, 440 aa, Artificial Sequence
  AsHPPDm-F372G Amino Acid Sequence
MPPTPATATGAAAAAVTPEHAARSFPRVVRVNPRSDRFPVLSFHHVELWCADAASAAGRFSFALGAPLAARSDLSTGNSAHASLLLRSGALAFLFTAPYAPPPQEAATAAATASIPSFSADAARTFAAAHGLAVRSVGVRVADAAEAFRVSVAGGARPAFAPADLGHGFGLAEVELYGDVVLRFVSYPDETDLPFLPGFERVSSPGAVDYGLTRFDHVVGNVPEMAPVIDYMKGFLGFHEFAEFTAEDVGTTESGLNSVVLANNSEAVLLPLNEPVHGTKRRSQIQTYLEYHGGPGVQHIALASNDVLRTLREMRARTPMGGFEFMAPPQAKYYEGVRRIAGDVLSEEQIKECQELGVLVDRDDQGVLLQIGTKPVGDRPTFFLEMIQRIGCMEKDEVGQEYQKGGCGGFGKGNFSELFKSIEDYEKSLEVKQSVVAQKS

SEQ ID NO: 156 - DNA, 1323 bp, Artificial Sequence
  AsHPPDm-F372G-01 Nucleotide Sequence
atgccgcccacccccgccaccgccaccggcgccgccgcggccgccgtgactccagagcacgcggcccggagctttccccgagtggtccgcgtcaacccgcgcagcgaccgcttccccgtgctctccttccaccacgtcgagctctggtgcgccgacgccgcctcagcggccggacgcttctccttcgcgctcggcgcgccgctcgccgcccggtccgacctctccacggggaactccgcgcacgcctccctcctgctccgctcgggcgccctcgccttcctcttcacggcgccctacgcgccgccgccgcaggaggccgccacggccgcagccaccgcctccatcccctccttctccgccgacgccgcgcggacgttcgccgccgcccacggcctcgcggtgcgctccgtcggggtccgcgtcgctgacgccgccgaggccttccgcgtcagcgtagccggcggcgctcgcccggccttcgccccagccgacctcggccatggcttcggcctcgccgaggtcgagctctacggcgacgtcgtgctacgcttcgtcagctacccggacgagacagacctgccattcctgccagggttcgagcgcgtgagcagccccggcgccgtggactacggcctcacgcggttcgaccacgtcgtgggcaacgtcccggagatggccccggtcatagactacatgaaaggcttcttggggttccacgagttcgccgagttcaccgccgaggacgtgggcacgaccgagagcgggctcaactcggtggtgctcgccaacaactccgaggccgtgctgctgccgctcaacgagcccgtgcacggcacaaagcgacggagccagatacagacgtacctggagtatcacggcgggcccggcgtgcagcacatcgcgctcgccagcaacgacgtgctcaggacgctcagggagatgcgggcgcgcacgcccatgggcggcttcgagttcatggcgccaccgcaggcgaaatactatgaaggcgtgcggcgcatcgcaggtgacgtgctctcggaagagcagatcaaggaatgccaggagctgggggtgctagtcgacagggatgatcaaggggtgttgctccaaatcggtaccaagccagtaggggacaggccaacgtttttcctggagatgatccaaagaatcgggtgcatggagaaggacgaggtcgggcaagagtaccagaagggtggctgcggcgggtttggcaagggcaatttctccgagctgttcaagtccattgaggactatgagaaatcccttgaggtcaagcaatctgttgtagctcagaaatcctag

SEQ ID NO: 157 - DNA, 1323 bp, Artificial Sequence
  AsHPPDm-F372G-02 Nucleotide Sequence
atgccacctactccagctacagctactggtgctgctgctgctgccgttactcctgagcacgctgccaggtcattccccagggtggttcgcgtgaaccccagatctgataggttcccagttctgagcttccaccatgttgagctgtggtgcgctgatgctgcttctgctgctggcaggttctctttcgctcttggtgctccactcgctgctagatctgatctgtctacaggaaatagcgctcatgcctcactcctgcttcgctcaggtgctttggccttcctcttcaccgctccatatgctcccccacctcaggaggctgctactgctgctgctacagcctccattccaagcttctcagctgatgccgctagaaccttcgctgctgctcatggacttgccgtgaggtctgttggtgttcgcgtggctgatgctgctgaggctttcagagtttccgttgccggcggagctaggccagctttcgctcctgctgatttgggacatggtttcggcctggctgaggttgagctttacggtgacgtggttctccgcttcgtgtcttacccagatgagactgacctgcctttccttcccggcttcgagagagtttcctctcctggtgccgtggattacggcctgacaaggttcgaccacgtggttggaaacgttcccgagatggctccagtgatcgattacatgaagggcttccttggattccatgagttcgccgagttcactgctgaggacgtgggaaccactgagtccggtttgaactctgtggttctcgccaacaattctgaggctgttttgctccctctgaatgagcctgtgcatggaaccaagaggagaagccagattcaaacttacctggagtaccacggtggccctggagttcagcatatcgcccttgcttctaatgatgtgttgcgcacactcagagagatgcgcgccagaacccccatgggaggtttcgagttcatggccccaccacaggctaagtactacgagggcgttagaaggattgctggagacgtgttgagcgaggagcagatcaaggagtgccaagagctgggtgttcttgtggatagggatgaccagggcgttctgcttcaaattggtactaagccagtgggcgaccgccctacattcttccttgagatgattcaaagaatcggctgcatggagaaggatgaggttggacaggagtaccaaaagggcggatgcggtggcttcggaaagggtaacttcagcgagttgttcaagtcaatcgaggactacgagaagagcctcgaggtgaagcagtcagtggttgcccaaaagtcctga

SEQ ID NO: 158 - protein, 440 aa, Artificial Sequence
  AsHPPDm-F372G-F383W Amino Acid Sequence
MPPTPATATGAAAAAVTPEHAARSFPRVVRVNPRSDRFPVLSFHHVELWCADAASAAGRFSFALGAPLAARSDLSTGNSAHASLLLRSGALAFLFTAPYAPPPQEAATAAATASIPSFSADAARTFAAAHGLAVRSVGVRVADAAEAFRVSVAGGARPAFAPADLGHGFGLAEVELYGDVVLRFVSYPDETDLPFLPGFERVSSPGAVDYGLTRFDHVVGNVPEMAPVIDYMKGFLGFHEFAEFTAEDVGTTESGLNSVVLANNSEAVLLPLNEPVHGTKRRSQIQTYLEYHGGPGVQHIALASNDVLRTLREMRARTPMGGFEFMAPPQAKYYEGVRRIAGDVLSEEQIKECQELGVLVDRDDQGVLLQIGTKPVGDRPTFWLEMIQRIGCMEKDEVGQEYQKGGCGGFGKGNFSELFKSIEDYEKSLEVKQSVVAQKS

SEQ ID NO: 159 - DNA, 1323 bp, Artificial Sequence
  AsHPPDm-F372G-F383W-01 Nucleotide Sequence
atgccgcccacccccgccaccgccaccggcgccgccgcggccgccgtgactccagagcacgcggcccggagctttccccgagtggtccgcgtcaacccgcgcagcgaccgcttccccgtgctctccttccaccacgtcgagctctggtgcgccgacgccgcctcagcggccggacgcttctccttcgcgctcggcgcgccgctcgccgcccggtccgacctctccacggggaactccgcgcacgcctccctcctgctccgctcgggcgccctcgccttcctcttcacggcgccctacgcgccgccgccgcaggaggccgccacggccgcagccaccgcctccatcccctccttctccgccgacgccgcgcggacgttcgccgccgcccacggcctcgcggtgcgctccgtcggggtccgcgtcgctgacgccgccgaggccttccgcgtcagcgtagccggcggcgctcgcccggccttcgccccagccgacctcggccatggcttcggcctcgccgaggtcgagctctacggcgacgtcgtgctacgcttcgtcagctacccggacgagacagacctgccattcctgccagggttcgagcgcgtgagcagccccggcgccgtggactacggcctcacgcggttcgaccacgtcgtgggcaacgtcccggagatggccccggtcatagactacatgaaaggcttcttggggttccacgagttcgccgagttcaccgccgaggacgtgggcacgaccgagagcgggctcaactcggtggtgctcgccaacaactccgaggccgtgctgctgccgctcaacgagcccgtgcacggcacaaagcgacggagccagatacagacgtacctggagtatcacggcgggcccggcgtgcagcacatcgcgctcgccagcaacgacgtgctcaggacgctcagggagatgcgggcgcgcacgcccatgggcggcttcgagttcatggcgccaccgcaggcgaaatactatgaaggcgtgcggcgcatcgcaggtgacgtgctctcggaagagcagatcaaggaatgccaggagctgggggtgctagtcgacagggatgatcaaggggtgttgctccaaatcggtaccaagccagtaggggacaggccaacgttttggctggagatgatccaaagaatcgggtgcatggagaaggacgaggtcgggcaagagtaccagaagggtggctgcggcgggtttggcaagggcaatttctccgagctgttcaagtccattgaggactatgagaaatcccttgaggtcaagcaatctgttgtagctcagaaatcctag

SEQ ID NO: 160 - DNA, 1323 bp, Artificial Sequence
  AsHPPDm-F372G-F383W-02 Nucleotide Sequence
atgccacctactccagctacagctactggtgctgctgctgctgccgttactcctgagcacgctgccaggtcattccccagggtggttcgcgtgaaccccagatctgataggttcccagttctgagcttccaccatgttgagctgtggtgcgctgatgctgcttctgctgctggcaggttctctttcgctcttggtgctccactcgctgctagatctgatctgtctacaggaaatagcgctcatgcctcactcctgcttcgctcaggtgctttggccttcctcttcaccgctccatatgctcccccacctcaggaggctgctactgctgctgctacagcctccattccaagcttctcagctgatgccgctagaaccttcgctgctgctcatggacttgccgtgaggtctgttggtgttcgcgtggctgatgctgctgaggctttcagagtttccgttgccggcggagctaggccagctttcgctcctgctgatttgggacatggtttcggcctggctgaggttgagctttacggtgacgtggttctccgcttcgtgtcttacccagatgagactgacctgcctttccttcccggcttcgagagagtttcctctcctggtgccgtggattacggcctgacaaggttcgaccacgtggttggaaacgttcccgagatggctccagtgatcgattacatgaagggcttccttggattccatgagttcgccgagttcactgctgaggacgtgggaaccactgagtccggtttgaactctgtggttctcgccaacaattctgaggctgttttgctccctctgaatgagcctgtgcatggaaccaagaggagaagccagattcaaacttacctggagtaccacggtggccctggagttcagcatatcgcccttgcttctaatgatgtgttgcgcacactcagagagatgcgcgccagaacccccatgggaggtttcgagttcatggccccaccacaggctaagtactacgagggcgttagaaggattgctggagacgtgttgagcgaggagcagatcaaggagtgccaagagctgggtgttcttgtggatagggatgaccagggcgttctgcttcaaattggtactaagccagtgggcgaccgccctacattctggcttgagatgattcaaagaatcggctgcatggagaaggatgaggttggacaggagtaccaaaagggcggatgcggtggcttcggaaagggtaacttcagcgagttgttcaagtcaatcgaggactacgagaagagcctcgaggtgaagcagtcagtggttgcccaaaagtcctga

SEQ ID NO: 161 - protein, 440 aa, Artificial Sequence
  AsHPPDm-F372V Amino Acid Sequence
MPPTPATATGAAAAAVTPEHAARSFPRVVRVNPRSDRFPVLSFHHVELWCADAASAAGRFSFALGAPLAARSDLSTGNSAHASLLLRSGALAFLFTAPYAPPPQEAATAAATASIPSFSADAARTFAAAHGLAVRSVGVRVADAAEAFRVSVAGGARPAFAPADLGHGFGLAEVELYGDVVLRFVSYPDETDLPFLPGFERVSSPGAVDYGLTRFDHVVGNVPEMAPVIDYMKGFLGFHEFAEFTAEDVGTTESGLNSVVLANNSEAVLLPLNEPVHGTKRRSQIQTYLEYHGGPGVQHIALASNDVLRTLREMRARTPMGGFEFMAPPQAKYYEGVRRIAGDVLSEEQIKECQELGVLVDRDDQGVLLQIVTKPVGDRPTFFLEMIQRIGCMEKDEVGQEYQKGGCGGFGKGNFSELFKSIEDYEKSLEVKQSVVAQKS

SEQ ID NO: 162 - DNA, 1323 bp, Artificial Sequence
  AsHPPDm-F372V-01 Nucleotide Sequence
atgccgcccacccccgccaccgccaccggcgccgccgcggccgccgtgactccagagcacgcggcccggagctttccccgagtggtccgcgtcaacccgcgcagcgaccgcttccccgtgctctccttccaccacgtcgagctctggtgcgccgacgccgcctcagcggccggacgcttctccttcgcgctcggcgcgccgctcgccgcccggtccgacctctccacggggaactccgcgcacgcctccctcctgctccgctcgggcgccctcgccttcctcttcacggcgccctacgcgccgccgccgcaggaggccgccacggccgcagccaccgcctccatcccctccttctccgccgacgccgcgcggacgttcgccgccgcccacggcctcgcggtgcgctccgtcggggtccgcgtcgctgacgccgccgaggccttccgcgtcagcgtagccggcggcgctcgcccggccttcgccccagccgacctcggccatggcttcggcctcgccgaggtcgagctctacggcgacgtcgtgctacgcttcgtcagctacccggacgagacagacctgccattcctgccagggttcgagcgcgtgagcagccccggcgccgtggactacggcctcacgcggttcgaccacgtcgtgggcaacgtcccggagatggccccggtcatagactacatgaaaggcttcttggggttccacgagttcgccgagttcaccgccgaggacgtgggcacgaccgagagcgggctcaactcggtggtgctcgccaacaactccgaggccgtgctgctgccgctcaacgagcccgtgcacggcacaaagcgacggagccagatacagacgtacctggagtatcacggcgggcccggcgtgcagcacatcgcgctcgccagcaacgacgtgctcaggacgctcagggagatgcgggcgcgcacgcccatgggcggcttcgagttcatggcgccaccgcaggcgaaatactatgaaggcgtgcggcgcatcgcaggtgacgtgctctcggaagagcagatcaaggaatgccaggagctgggggtgctagtcgacagggatgatcaaggggtgttgctccaaatcgtcaccaagccagtaggggacaggccaacgtttttcctggagatgatccaaagaatcgggtgcatggagaaggacgaggtcgggcaagagtaccagaagggtggctgcggcgggtttggcaagggcaatttctccgagctgttcaagtccattgaggactatgagaaatcccttgaggtcaagcaatctgttgtagctcagaaatcctag

SEQ ID NO: 163 - DNA, 1323 bp, Artificial Sequence
  AsHPPDm-F372V-02 Nucleotide Sequence
atgccacctactccagctacagctactggtgctgctgctgctgccgttactcctgagcacgctgccaggtcattccccagggtggttcgcgtgaaccccagatctgataggttcccagttctgagcttccaccatgttgagctgtggtgcgctgatgctgcttctgctgctggcaggttctctttcgctcttggtgctccactcgctgctagatctgatctgtctacaggaaatagcgctcatgcctcactcctgcttcgctcaggtgctttggccttcctcttcaccgctccatatgctcccccacctcaggaggctgctactgctgctgctacagcctccattccaagcttctcagctgatgccgctagaaccttcgctgctgctcatggacttgccgtgaggtctgttggtgttcgcgtggctgatgctgctgaggctttcagagtttccgttgccggcggagctaggccagctttcgctcctgctgatttgggacatggtttcggcctggctgaggttgagctttacggtgacgtggttctccgcttcgtgtcttacccagatgagactgacctgcctttccttcccggcttcgagagagtttcctctcctggtgccgtggattacggcctgacaaggttcgaccacgtggttggaaacgttcccgagatggctccagtgatcgattacatgaagggcttccttggattccatgagttcgccgagttcactgctgaggacgtgggaaccactgagtccggtttgaactctgtggttctcgccaacaattctgaggctgttttgctccctctgaatgagcctgtgcatggaaccaagaggagaagccagattcaaacttacctggagtaccacggtggccctggagttcagcatatcgcccttgcttctaatgatgtgttgcgcacactcagagagatgcgcgccagaacccccatgggaggtttcgagttcatggccccaccacaggctaagtactacgagggcgttagaaggattgctggagacgtgttgagcgaggagcagatcaaggagtgccaagagctgggtgttcttgtggatagggatgaccagggcgttctgcttcaaattgtcactaagccagtgggcgaccgccctacattcttccttgagatgattcaaagaatcggctgcatggagaaggatgaggttggacaggagtaccaaaagggcggatgcggtggcttcggaaagggtaacttcagcgagttgttcaagtcaatcgaggactacgagaagagcctcgaggtgaagcagtcagtggttgcccaaaagtcctga

SEQ ID NO: 164 - protein, 440 aa, Artificial Sequence
  AsHPPDm-F372V-F383W Amino Acid Sequence
MPPTPATATGAAAAAVTPEHAARSFPRVVRVNPRSDRFPVLSFHHVELWCADAASAAGRFSFALGAPLAARSDLSTGNSAHASLLLRSGALAFLFTAPYAPPPQEAATAAATASIPSFSADAARTFAAAHGLAVRSVGVRVADAAEAFRVSVAGGARPAFAPADLGHGFGLAEVELYGDVVLRFVSYPDETDLPFLPGFERVSSPGAVDYGLTRFDHVVGNVPEMAPVIDYMKGFLGFHEFAEFTAEDVGTTESGLNSVVLANNSEAVLLPLNEPVHGTKRRSQIQTYLEYHGGPGVQHIALASNDVLRTLREMRARTPMGGFEFMAPPQAKYYEGVRRIAGDVLSEEQIKECQELGVLVDRDDQGVLLQIVTKPVGDRPTFWLEMIQRIGCMEKDEVGQEYQKGGCGGFGKGNFSELFKSIEDYEKSLEVKQSVVAQKS

SEQ ID NO: 165 - DNA, 1323 bp, Artificial Sequence
  AsHPPDm-F372V-F383W-01 Nucleotide Sequence
atgccgcccacccccgccaccgccaccggcgccgccgcggccgccgtgactccagagcacgcggcccggagctttccccgagtggtccgcgtcaacccgcgcagcgaccgcttccccgtgctctccttccaccacgtcgagctctggtgcgccgacgccgcctcagcggccggacgcttctccttcgcgctcggcgcgccgctcgccgcccggtccgacctctccacggggaactccgcgcacgcctccctcctgctccgctcgggcgccctcgccttcctcttcacggcgccctacgcgccgccgccgcaggaggccgccacggccgcagccaccgcctccatcccctccttctccgccgacgccgcgcggacgttcgccgccgcccacggcctcgcggtgcgctccgtcggggtccgcgtcgctgacgccgccgaggccttccgcgtcagcgtagccggcggcgctcgcccggccttcgccccagccgacctcggccatggcttcggcctcgccgaggtcgagctctacggcgacgtcgtgctacgcttcgtcagctacccggacgagacagacctgccattcctgccagggttcgagcgcgtgagcagccccggcgccgtggactacggcctcacgcggttcgaccacgtcgtgggcaacgtcccggagatggccccggtcatagactacatgaaaggcttcttggggttccacgagttcgccgagttcaccgccgaggacgtgggcacgaccgagagcgggctcaactcggtggtgctcgccaacaactccgaggccgtgctgctgccgctcaacgagcccgtgcacggcacaaagcgacggagccagatacagacgtacctggagtatcacggcgggcccggcgtgcagcacatcgcgctcgccagcaacgacgtgctcaggacgctcagggagatgcgggcgcgcacgcccatgggcggcttcgagttcatggcgccaccgcaggcgaaatactatgaaggcgtgcggcgcatcgcaggtgacgtgctctcggaagagcagatcaaggaatgccaggagctgggggtgctagtcgacagggatgatcaaggggtgttgctccaaatcgtcaccaagccagtaggggacaggccaacgttttggctggagatgatccaaagaatcgggtgcatggagaaggacgaggtcgggcaagagtaccagaagggtggctgcggcgggtttggcaagggcaatttctccgagctgttcaagtccattgaggactatgagaaatcccttgaggtcaagcaatctgttgtagctcagaaatcctag

SEQ ID NO: 166 - DNA, 1323 bp, Artificial Sequence
  AsHPPDm-F372V-F383W-02 Nucleotide Sequence
atgccacctactccagctacagctactggtgctgctgctgctgccgttactcctgagcacgctgccaggtcattccccagggtggttcgcgtgaaccccagatctgataggttcccagttctgagcttccaccatgttgagctgtggtgcgctgatgctgcttctgctgctggcaggttctctttcgctcttggtgctccactcgctgctagatctgatctgtctacaggaaatagcgctcatgcctcactcctgcttcgctcaggtgctttggccttcctcttcaccgctccatatgctcccccacctcaggaggctgctactgctgctgctacagcctccattccaagcttctcagctgatgccgctagaaccttcgctgctgctcatggacttgccgtgaggtctgttggtgttcgcgtggctgatgctgctgaggctttcagagtttccgttgccggcggagctaggccagctttcgctcctgctgatttgggacatggtttcggcctggctgaggttgagctttacggtgacgtggttctccgcttcgtgtcttacccagatgagactgacctgcctttccttcccggcttcgagagagtttcctctcctggtgccgtggattacggcctgacaaggttcgaccacgtggttggaaacgttcccgagatggctccagtgatcgattacatgaagggcttccttggattccatgagttcgccgagttcactgctgaggacgtgggaaccactgagtccggtttgaactctgtggttctcgccaacaattctgaggctgttttgctccctctgaatgagcctgtgcatggaaccaagaggagaagccagattcaaacttacctggagtaccacggtggccctggagttcagcatatcgcccttgcttctaatgatgtgttgcgcacactcagagagatgcgcgccagaacccccatgggaggtttcgagttcatggccccaccacaggctaagtactacgagggcgttagaaggattgctggagacgtgttgagcgaggagcagatcaaggagtgccaagagctgggtgttcttgtggatagggatgaccagggcgttctgcttcaaattgtcactaagccagtgggcgaccgccctacattctggcttgagatgattcaaagaatcggctgcatggagaaggatgaggttggacaggagtaccaaaagggcggatgcggtggcttcggaaagggtaacttcagcgagttgttcaagtcaatcgaggactacgagaagagcctcgaggtgaagcagtcagtggttgcccaaaagtcctga

SEQ ID NO: 167 - protein, 439 aa, Artificial Sequence
  AsHPPDm-A107-F372A Amino Acid Sequence
MPPTPATATGAAAAAVTPEHAARSFPRVVRVNPRSDRFPVLSFHHVELWCADAASAAGRFSFALGAPLAARSDLSTGNSAHASLLLRSGALAFLFTAPYAPPPQEATAAATASIPSFSADAARTFAAAHGLAVRSVGVRVADAAEAFRVSVAGGARPAFAPADLGHGFGLAEVELYGDVVLRFVSYPDETDLPFLPGFERVSSPGAVDYGLTRFDHVVGNVPEMAPVIDYMKGFLGFHEFAEFTAEDVGTTESGLNSVVLANNSEAVLLPLNEPVHGTKRRSQIQTYLEYHGGPGVQHIALASNDVLRTLREMRARTPMGGFEFMAPPQAKYYEGVRRIAGDVLSEEQIKECQELGVLVDRDDQGVLLQIATKPVGDRPTFFLEMIQRIGCMEKDEVGQEYQKGGCGGFGKGNFSELFKSIEDYEKSLEVKQSVVAQKS

SEQ ID NO: 168 - DNA, 1320 bp, Artificial Sequence
  AsHPPDm-A107-F372A-01 Nucleotide Sequence
atgccgcccacccccgccaccgccaccggcgccgccgcggccgccgtgactccagagcacgcggcccggagctttccccgagtggtccgcgtcaacccgcgcagcgaccgcttccccgtgctctccttccaccacgtcgagctctggtgcgccgacgccgcctcagcggccggacgcttctccttcgcgctcggcgcgccgctcgccgcccggtccgacctctccacggggaactccgcgcacgcctccctcctgctccgctcgggcgccctcgccttcctcttcacggcgccctacgcgccgccgccgcaggaggccacggccgcagccaccgcctccatcccctccttctccgccgacgccgcgcggacgttcgccgccgcccacggcctcgcggtgcgctccgtcggggtccgcgtcgctgacgccgccgaggccttccgcgtcagcgtagccggcggcgctcgcccggccttcgccccagccgacctcggccatggcttcggcctcgccgaggtcgagctctacggcgacgtcgtgctacgcttcgtcagctacccggacgagacagacctgccattcctgccagggttcgagcgcgtgagcagccccggcgccgtggactacggcctcacgcggttcgaccacgtcgtgggcaacgtcccggagatggccccggtcatagactacatgaaaggcttcttggggttccacgagttcgccgagttcaccgccgaggacgtgggcacgaccgagagcgggctcaactcggtggtgctcgccaacaactccgaggccgtgctgctgccgctcaacgagcccgtgcacggcacaaagcgacggagccagatacagacgtacctggagtatcacggcgggcccggcgtgcagcacatcgcgctcgccagcaacgacgtgctcaggacgctcagggagatgcgggcgcgcacgcccatgggcggcttcgagttcatggcgccaccgcaggcgaaatactatgaaggcgtgcggcgcatcgcaggtgacgtgctctcggaagagcagatcaaggaatgccaggagctgggggtgctagtcgacagggatgatcaaggggtgttgctccaaatcgctaccaagccagtaggggacaggccaacgtttttcctggagatgatccaaagaatcgggtgcatggagaaggacgaggtcgggcaagagtaccagaagggtggctgcggcgggtttggcaagggcaatttctccgagctgttcaagtccattgaggactatgagaaatcccttgaggtcaagcaatctgttgtagctcagaaatcctag

SEQ ID NO: 169 - DNA, 1320 bp, Artificial Sequence
  AsHPPDm-A107-F372A-02 Nucleotide Sequence
atgccacctactccagctacagctactggtgctgctgctgctgccgttactcctgagcacgctgccaggtcattccccagggtggttcgcgtgaaccccagatctgataggttcccagttctgagcttccaccatgttgagctgtggtgcgctgatgctgcttctgctgctggcaggttctctttcgctcttggtgctccactcgctgctagatctgatctgtctacaggaaatagcgctcatgcctcactcctgcttcgctcaggtgctttggccttcctcttcaccgctccatatgctcccccacctcaggaggctactgctgctgctacagcctccattccaagcttctcagctgatgccgctagaaccttcgctgctgctcatggacttgccgtgaggtctgttggtgttcgcgtggctgatgctgctgaggctttcagagtttccgttgccggcggagctaggccagctttcgctcctgctgatttgggacatggtttcggcctggctgaggttgagctttacggtgacgtggttctccgcttcgtgtcttacccagatgagactgacctgcctttccttcccggcttcgagagagtttcctctcctggtgccgtggattacggcctgacaaggttcgaccacgtggttggaaacgttcccgagatggctccagtgatcgattacatgaagggcttccttggattccatgagttcgccgagttcactgctgaggacgtgggaaccactgagtccggtttgaactctgtggttctcgccaacaattctgaggctgttttgctccctctgaatgagcctgtgcatggaaccaagaggagaagccagattcaaacttacctggagtaccacggtggccctggagttcagcatatcgcccttgcttctaatgatgtgttgcgcacactcagagagatgcgcgccagaacccccatgggaggtttcgagttcatggccccaccacaggctaagtactacgagggcgttagaaggattgctggagacgtgttgagcgaggagcagatcaaggagtgccaagagctgggtgttcttgtggatagggatgaccagggcgttctgcttcaaattgccactaagccagtgggcgaccgccctacattcttccttgagatgattcaaagaatcggctgcatggagaaggatgaggttggacaggagtaccaaaagggcggatgcggtggcttcggaaagggtaacttcagcgagttgttcaagtcaatcgaggactacgagaagagcctcgaggtgaagcagtcagtggttgcccaaaagtcctga

SEQ ID NO: 170 - protein, 439 aa, Artificial Sequence
  AsHPPDm-A107-F383W Amino Acid Sequence
MPPTPATATGAAAAAVTPEHAARSFPRVVRVNPRSDRFPVLSFHHVELWCADAASAAGRFSFALGAPLAARSDLSTGNSAHASLLLRSGALAFLFTAPYAPPPQEATAAATASIPSFSADAARTFAAAHGLAVRSVGVRVADAAEAFRVSVAGGARPAFAPADLGHGFGLAEVELYGDVVLRFVSYPDETDLPFLPGFERVSSPGAVDYGLTRFDHVVGNVPEMAPVIDYMKGFLGFHEFAEFTAEDVGTTESGLNSVVLANNSEAVLLPLNEPVHGTKRRSQIQTYLEYHGGPGVQHIALASNDVLRTLREMRARTPMGGFEFMAPPQAKYYEGVRRIAGDVLSEEQIKECQELGVLVDRDDQGVLLQIFTKPVGDRPTFWLEMIQRIGCMEKDEVGQEYQKGGCGGFGKGNFSELFKSIEDYEKSLEVKQSVVAQKS

SEQ ID NO: 171 - DNA, 1320 bp, Artificial Sequence
  AsHPPDm-A107-F383W-01 Nucleotide Sequence
atgccgcccacccccgccaccgccaccggcgccgccgcggccgccgtgactccagagcacgcggcccggagctttccccgagtggtccgcgtcaacccgcgcagcgaccgcttccccgtgctctccttccaccacgtcgagctctggtgcgccgacgccgcctcagcggccggacgcttctccttcgcgctcggcgcgccgctcgccgcccggtccgacctctccacggggaactccgcgcacgcctccctcctgctccgctcgggcgccctcgccttcctcttcacggcgccctacgcgccgccgccgcaggaggccacggccgcagccaccgcctccatcccctccttctccgccgacgccgcgcggacgttcgccgccgcccacggcctcgcggtgcgctccgtcggggtccgcgtcgctgacgccgccgaggccttccgcgtcagcgtagccggcggcgctcgcccggccttcgccccagccgacctcggccatggcttcggcctcgccgaggtcgagctctacggcgacgtcgtgctacgcttcgtcagctacccggacgagacagacctgccattcctgccagggttcgagcgcgtgagcagccccggcgccgtggactacggcctcacgcggttcgaccacgtcgtgggcaacgtcccggagatggccccggtcatagactacatgaaaggcttcttggggttccacgagttcgccgagttcaccgccgaggacgtgggcacgaccgagagcgggctcaactcggtggtgctcgccaacaactccgaggccgtgctgctgccgctcaacgagcccgtgcacggcacaaagcgacggagccagatacagacgtacctggagtatcacggcgggcccggcgtgcagcacatcgcgctcgccagcaacgacgtgctcaggacgctcagggagatgcgggcgcgcacgcccatgggcggcttcgagttcatggcgccaccgcaggcgaaatactatgaaggcgtgcggcgcatcgcaggtgacgtgctctcggaagagcagatcaaggaatgccaggagctgggggtgctagtcgacagggatgatcaaggggtgttgctccaaatcttcaccaagccagtaggggacaggccaacgttttggctggagatgatccaaagaatcgggtgcatggagaaggacgaggtcgggcaagagtaccagaagggtggctgcggcgggtttggcaagggcaatttctccgagctgttcaagtccattgaggactatgagaaatcccttgaggtcaagcaatctgttgtagctcagaaatcctag

SEQ ID NO: 172 - DNA, 1320 bp, Artificial Sequence
  AsHPPDm-A107-F383W-02 Nucleotide Sequence
atgccacctactccagctacagctactggtgctgctgctgctgccgttactcctgagcacgctgccaggtcattccccagggtggttcgcgtgaaccccagatctgataggttcccagttctgagcttccaccatgttgagctgtggtgcgctgatgctgcttctgctgctggcaggttctctttcgctcttggtgctccactcgctgctagatctgatctgtctacaggaaatagcgctcatgcctcactcctgcttcgctcaggtgctttggccttcctcttcaccgctccatatgctcccccacctcaggaggctactgctgctgctacagcctccattccaagcttctcagctgatgccgctagaaccttcgctgctgctcatggacttgccgtgaggtctgttggtgttcgcgtggctgatgctgctgaggctttcagagtttccgttgccggcggagctaggccagctttcgctcctgctgatttgggacatggtttcggcctggctgaggttgagctttacggtgacgtggttctccgcttcgtgtcttacccagatgagactgacctgcctttccttcccggcttcgagagagtttcctctcctggtgccgtggattacggcctgacaaggttcgaccacgtggttggaaacgttcccgagatggctccagtgatcgattacatgaagggcttccttggattccatgagttcgccgagttcactgctgaggacgtgggaaccactgagtccggtttgaactctgtggttctcgccaacaattctgaggctgttttgctccctctgaatgagcctgtgcatggaaccaagaggagaagccagattcaaacttacctggagtaccacggtggccctggagttcagcatatcgcccttgcttctaatgatgtgttgcgcacactcagagagatgcgcgccagaacccccatgggaggtttcgagttcatggccccaccacaggctaagtactacgagggcgttagaaggattgctggagacgtgttgagcgaggagcagatcaaggagtgccaagagctgggtgttcttgtggatagggatgaccagggcgttctgcttcaaattttcactaagccagtgggcgaccgccctacattctggcttgagatgattcaaagaatcggctgcatggagaaggatgaggttggacaggagtaccaaaagggcggatgcggtggcttcggaaagggtaacttcagcgagttgttcaagtcaatcgaggactacgagaagagcctcgaggtgaagcagtcagtggttgcccaaaagtcctga

SEQ ID NO: 173 - protein, 439 aa, Artificial Sequence
  HPPDm-1 Amino Acid Sequence
MPPTPATATGAAAAAVTPEHAARSFPRVVRVNPRSDRFPVLSFHHVELWCADAASAAGRFSFALGAPLAARSDLSTGNSAHASLLLRSGALAFLFTAPYAPPPQEATAAATASIPSFSADAARTFAAAHGLAVRSVGVRVADAAEAFRVSVAGGARPAFAPADLGHGFGLAEVELYGDVVLRFVSYPDETDLPFLPGFERVSSPGAVDYGLTRFDHVVGNVPEMAPVIDYMKGFLGFHEFAEFTAEDVGTTESGLNSVVLANNSEAVLLPLNEPVHGTKRRSQIQTYLEYHGGPGVQHIALASNDVLRTLREMRARTPMGGFEFMAPPQAKYYEGVRRIAGDVLSEEQIKECQELGVLVDRDDQGVLLQIATKPVGDRPTFWLEMIQRIGCMEKDEVGQEYQKGGCGGFGKGNFSELFKSIEDYEKSLEVKQSVVAQKS

SEQ ID NO: 174 - DNA, 1320 bp, Artificial Sequence
  HPPDm-1-01 Nucleotide Sequence
atgccgcccacccccgccaccgccaccggcgccgccgcggccgccgtgactccagagcacgcggcccggagctttccccgagtggtccgcgtcaacccgcgcagcgaccgcttccccgtgctctccttccaccacgtcgagctctggtgcgccgacgccgcctcagcggccggacgcttctccttcgcgctcggcgcgccgctcgccgcccggtccgacctctccacggggaactccgcgcacgcctccctcctgctccgctcgggcgccctcgccttcctcttcacggcgccctacgcgccgccgccgcaggaggccacggccgcagccaccgcctccatcccctccttctccgccgacgccgcgcggacgttcgccgccgcccacggcctcgcggtgcgctccgtcggggtccgcgtcgctgacgccgccgaggccttccgcgtcagcgtagccggcggcgctcgcccggccttcgccccagccgacctcggccatggcttcggcctcgccgaggtcgagctctacggcgacgtcgtgctacgcttcgtcagctacccggacgagacagacctgccattcctgccagggttcgagcgcgtgagcagccccggcgccgtggactacggcctcacgcggttcgaccacgtcgtgggcaacgtcccggagatggccccggtcatagactacatgaaaggcttcttggggttccacgagttcgccgagttcaccgccgaggacgtgggcacgaccgagagcgggctcaactcggtggtgctcgccaacaactccgaggccgtgctgctgccgctcaacgagcccgtgcacggcacaaagcgacggagccagatacagacgtacctggagtatcacggcgggcccggcgtgcagcacatcgcgctcgccagcaacgacgtgctcaggacgctcagggagatgcgggcgcgcacgcccatgggcggcttcgagttcatggcgccaccgcaggcgaaatactatgaaggcgtgcggcgcatcgcaggtgacgtgctctcggaagagcagatcaaggaatgccaggagctgggggtgctagtcgacagggatgatcaaggggtgttgctccaaatcgctaccaagccagtaggggacaggccaacgttttggctggagatgatccaaagaatcgggtgcatggagaaggacgaggtcgggcaagagtaccagaagggtggctgcggcgggtttggcaagggcaatttctccgagctgttcaagtccattgaggactatgagaaatcccttgaggtcaagcaatctgttgtagctcagaaatcctag

SEQ ID NO: 175 - DNA, 1320 bp, Artificial Sequence
  HPPDm-1-02 Nucleotide Sequence
atgccacctactccagctacagctactggtgctgctgctgctgccgttactcctgagcacgctgccaggtcattccccagggtggttcgcgtgaaccccagatctgataggttcccagttctgagcttccaccatgttgagctgtggtgcgctgatgctgcttctgctgctggcaggttctctttcgctcttggtgctccactcgctgctagatctgatctgtctacaggaaatagcgctcatgcctcactcctgcttcgctcaggtgctttggccttcctcttcaccgctccatatgctcccccacctcaggaggctactgctgctgctacagcctccattccaagcttctcagctgatgccgctagaaccttcgctgctgctcatggacttgccgtgaggtctgttggtgttcgcgtggctgatgctgctgaggctttcagagtttccgttgccggcggagctaggccagctttcgctcctgctgatttgggacatggtttcggcctggctgaggttgagctttacggtgacgtggttctccgcttcgtgtcttacccagatgagactgacctgcctttccttcccggcttcgagagagtttcctctcctggtgccgtggattacggcctgacaaggttcgaccacgtggttggaaacgttcccgagatggctccagtgatcgattacatgaagggcttccttggattccatgagttcgccgagttcactgctgaggacgtgggaaccactgagtccggtttgaactctgtggttctcgccaacaattctgaggctgttttgctccctctgaatgagcctgtgcatggaaccaagaggagaagccagattcaaacttacctggagtaccacggtggccctggagttcagcatatcgcccttgcttctaatgatgtgttgcgcacactcagagagatgcgcgccagaacccccatgggaggtttcgagttcatggccccaccacaggctaagtactacgagggcgttagaaggattgctggagacgtgttgagcgaggagcagatcaaggagtgccaagagctgggtgttcttgtggatagggatgaccagggcgttctgcttcaaattgccactaagccagtgggcgaccgccctacattctggcttgagatgattcaaagaatcggctgcatggagaaggatgaggttggacaggagtaccaaaagggcggatgcggtggcttcggaaagggtaacttcagcgagttgttcaagtcaatcgaggactacgagaagagcctcgaggtgaagcagtcagtggttgcccaaaagtcctga

SEQ ID NO: 176 - protein, 440 aa, Artificial Sequence
  AsHPPDm-A111T-F372A Amino Acid Sequence
MPPTPATATGAAAAAVTPEHAARSFPRVVRVNPRSDRFPVLSFHHVELWCADAASAAGRFSFALGAPLAARSDLSTGNSAHASLLLRSGALAFLFTAPYAPPPQEAATAATTASIPSFSADAARTFAAAHGLAVRSVGVRVADAAEAFRVSVAGGARPAFAPADLGHGFGLAEVELYGDVVLRFVSYPDETDLPFLPGFERVSSPGAVDYGLTRFDHVVGNVPEMAPVIDYMKGFLGFHEFAEFTAEDVGTTESGLNSVVLANNSEAVLLPLNEPVHGTKRRSQIQTYLEYHGGPGVQHIALASNDVLRTLREMRARTPMGGFEFMAPPQAKYYEGVRRIAGDVLSEEQIKECQELGVLVDRDDQGVLLQIATKPVGDRPTFFLEMIQRIGCMEKDEVGQEYQKGGCGGFGKGNFSELFKSIEDYEKSLEVKQSVVAQKS

SEQ ID NO: 177 - DNA, 1323 bp, Artificial Sequence
  AsHPPDm-A111T-F372A-01 Nucleotide Sequence
atgccgcccacccccgccaccgccaccggcgccgccgcggccgccgtgactccagagcacgcggcccggagctttccccgagtggtccgcgtcaacccgcgcagcgaccgcttccccgtgctctccttccaccacgtcgagctctggtgcgccgacgccgcctcagcggccggacgcttctccttcgcgctcggcgcgccgctcgccgcccggtccgacctctccacggggaactccgcgcacgcctccctcctgctccgctcgggcgccctcgccttcctcttcacggcgccctacgcgccgccgccgcaggaggccgccacggccgcaaccaccgcctccatcccctccttctccgccgacgccgcgcggacgttcgccgccgcccacggcctcgcggtgcgctccgtcggggtccgcgtcgctgacgccgccgaggccttccgcgtcagcgtagccggcggcgctcgcccggccttcgccccagccgacctcggccatggcttcggcctcgccgaggtcgagctctacggcgacgtcgtgctacgcttcgtcagctacccggacgagacagacctgccattcctgccagggttcgagcgcgtgagcagccccggcgccgtggactacggcctcacgcggttcgaccacgtcgtgggcaacgtcccggagatggccccggtcatagactacatgaaaggcttcttggggttccacgagttcgccgagttcaccgccgaggacgtgggcacgaccgagagcgggctcaactcggtggtgctcgccaacaactccgaggccgtgctgctgccgctcaacgagcccgtgcacggcacaaagcgacggagccagatacagacgtacctggagtatcacggcgggcccggcgtgcagcacatcgcgctcgccagcaacgacgtgctcaggacgctcagggagatgcgggcgcgcacgcccatgggcggcttcgagttcatggcgccaccgcaggcgaaatactatgaaggcgtgcggcgcatcgcaggtgacgtgctctcggaagagcagatcaaggaatgccaggagctgggggtgctagtcgacagggatgatcaaggggtgttgctccaaatcgctaccaagccagtaggggacaggccaacgtttttcctggagatgatccaaagaatcgggtgcatggagaaggacgaggtcgggcaagagtaccagaagggtggctgcggcgggtttggcaagggcaatttctccgagctgttcaagtccattgaggactatgagaaatcccttgaggtcaagcaatctgttgtagctcagaaatcctag

SEQ ID NO: 178 - DNA, 1323 bp, Artificial Sequence
  AsHPPDm-A111T-F372A-02 Nucleotide Sequence
atgccacctactccagctacagctactggtgctgctgctgctgccgttactcctgagcacgctgccaggtcattccccagggtggttcgcgtgaaccccagatctgataggttcccagttctgagcttccaccatgttgagctgtggtgcgctgatgctgcttctgctgctggcaggttctctttcgctcttggtgctccactcgctgctagatctgatctgtctacaggaaatagcgctcatgcctcactcctgcttcgctcaggtgctttggccttcctcttcaccgctccatatgctcccccacctcaggaggctgctactgctgctactacagcctccattccaagcttctcagctgatgccgctagaaccttcgctgctgctcatggacttgccgtgaggtctgttggtgttcgcgtggctgatgctgctgaggctttcagagtttccgttgccggcggagctaggccagctttcgctcctgctgatttgggacatggtttcggcctggctgaggttgagctttacggtgacgtggttctccgcttcgtgtcttacccagatgagactgacctgcctttccttcccggcttcgagagagtttcctctcctggtgccgtggattacggcctgacaaggttcgaccacgtggttggaaacgttcccgagatggctccagtgatcgattacatgaagggcttccttggattccatgagttcgccgagttcactgctgaggacgtgggaaccactgagtccggtttgaactctgtggttctcgccaacaattctgaggctgttttgctccctctgaatgagcctgtgcatggaaccaagaggagaagccagattcaaacttacctggagtaccacggtggccctggagttcagcatatcgcccttgcttctaatgatgtgttgcgcacactcagagagatgcgcgccagaacccccatgggaggtttcgagttcatggccccaccacaggctaagtactacgagggcgttagaaggattgctggagacgtgttgagcgaggagcagatcaaggagtgccaagagctgggtgttcttgtggatagggatgaccagggcgttctgcttcaaattgccactaagccagtgggcgaccgccctacattcttccttgagatgattcaaagaatcggctgcatggagaaggatgaggttggacaggagtaccaaaagggcggatgcggtggcttcggaaagggtaacttcagcgagttgttcaagtcaatcgaggactacgagaagagcctcgaggtgaagcagtcagtggttgcccaaaagtcctga

SEQ ID NO: 179 - protein, 440 aa, Artificial Sequence
  AsHPPDm-A111T-F383W Amino Acid Sequence
MPPTPATATGAAAAAVTPEHAARSFPRVVRVNPRSDRFPVLSFHHVELWCADAASAAGRFSFALGAPLAARSDLSTGNSAHASLLLRSGALAFLFTAPYAPPPQEAATAATTASIPSFSADAARTFAAAHGLAVRSVGVRVADAAEAFRVSVAGGARPAFAPADLGHGFGLAEVELYGDVVLRFVSYPDETDLPFLPGFERVSSPGAVDYGLTRFDHVVGNVPEMAPVIDYMKGFLGFHEFAEFTAEDVGTTESGLNSVVLANNSEAVLLPLNEPVHGTKRRSQIQTYLEYHGGPGVQHIALASNDVLRTLREMRARTPMGGFEFMAPPQAKYYEGVRRIAGDVLSEEQIKECQELGVLVDRDDQGVLLQIFTKPVGDRPTFWLEMIQRIGCMEKDEVGQEYQKGGCGGFGKGNFSELFKSIEDYEKSLEVKQSVVAQKS

SEQ ID NO: 180 - DNA, 1323 bp, Artificial Sequence
  AsHPPDm-A111T-F383W-01 Nucleotide Sequence
atgccgcccacccccgccaccgccaccggcgccgccgcggccgccgtgactccagagcacgcggcccggagctttccccgagtggtccgcgtcaacccgcgcagcgaccgcttccccgtgctctccttccaccacgtcgagctctggtgcgccgacgccgcctcagcggccggacgcttctccttcgcgctcggcgcgccgctcgccgcccggtccgacctctccacggggaactccgcgcacgcctccctcctgctccgctcgggcgccctcgccttcctcttcacggcgccctacgcgccgccgccgcaggaggccgccacggccgcaaccaccgcctccatcccctccttctccgccgacgccgcgcggacgttcgccgccgcccacggcctcgcggtgcgctccgtcggggtccgcgtcgctgacgccgccgaggccttccgcgtcagcgtagccggcggcgctcgcccggccttcgccccagccgacctcggccatggcttcggcctcgccgaggtcgagctctacggcgacgtcgtgctacgcttcgtcagctacccggacgagacagacctgccattcctgccagggttcgagcgcgtgagcagccccggcgccgtggactacggcctcacgcggttcgaccacgtcgtgggcaacgtcccggagatggccccggtcatagactacatgaaaggcttcttggggttccacgagttcgccgagttcaccgccgaggacgtgggcacgaccgagagcgggctcaactcggtggtgctcgccaacaactccgaggccgtgctgctgccgctcaacgagcccgtgcacggcacaaagcgacggagccagatacagacgtacctggagtatcacggcgggcccggcgtgcagcacatcgcgctcgccagcaacgacgtgctcaggacgctcagggagatgcgggcgcgcacgcccatgggcggcttcgagttcatggcgccaccgcaggcgaaatactatgaaggcgtgcggcgcatcgcaggtgacgtgctctcggaagagcagatcaaggaatgccaggagctgggggtgctagtcgacagggatgatcaaggggtgttgctccaaatcttcaccaagccagtaggggacaggccaacgttttggctggagatgatccaaagaatcgggtgcatggagaaggacgaggtcgggcaagagtaccagaagggtggctgcggcgggtttggcaagggcaatttctccgagctgttcaagtccattgaggactatgagaaatcccttgaggtcaagcaatctgttgtagctcagaaatcctag

SEQ ID NO: 181 - DNA, 1323 bp, Artificial Sequence
  AsHPPDm-A111T-F383W-02 Nucleotide Sequence
atgccacctactccagctacagctactggtgctgctgctgctgccgttactcctgagcacgctgccaggtcattccccagggtggttcgcgtgaaccccagatctgataggttcccagttctgagcttccaccatgttgagctgtggtgcgctgatgctgcttctgctgctggcaggttctctttcgctcttggtgctccactcgctgctagatctgatctgtctacaggaaatagcgctcatgcctcactcctgcttcgctcaggtgctttggccttcctcttcaccgctccatatgctcccccacctcaggaggctgctactgctgctactacagcctccattccaagcttctcagctgatgccgctagaaccttcgctgctgctcatggacttgccgtgaggtctgttggtgttcgcgtggctgatgctgctgaggctttcagagtttccgttgccggcggagctaggccagctttcgctcctgctgatttgggacatggtttcggcctggctgaggttgagctttacggtgacgtggttctccgcttcgtgtcttacccagatgagactgacctgcctttccttcccggcttcgagagagtttcctctcctggtgccgtggattacggcctgacaaggttcgaccacgtggttggaaacgttcccgagatggctccagtgatcgattacatgaagggcttccttggattccatgagttcgccgagttcactgctgaggacgtgggaaccactgagtccggtttgaactctgtggttctcgccaacaattctgaggctgttttgctccctctgaatgagcctgtgcatggaaccaagaggagaagccagattcaaacttacctggagtaccacggtggccctggagttcagcatatcgcccttgcttctaatgatgtgttgcgcacactcagagagatgcgcgccagaacccccatgggaggtttcgagttcatggccccaccacaggctaagtactacgagggcgttagaaggattgctggagacgtgttgagcgaggagcagatcaaggagtgccaagagctgggtgttcttgtggatagggatgaccagggcgttctgcttcaaattttcactaagccagtgggcgaccgccctacattctggcttgagatgattcaaagaatcggctgcatggagaaggatgaggttggacaggagtaccaaaagggcggatgcggtggcttcggaaagggtaacttcagcgagttgttcaagtcaatcgaggactacgagaagagcctcgaggtgaagcagtcagtggttgcccaaaagtcctga

SEQ ID NO: 182 - protein, 440 aa, Artificial Sequence
  HPPDm-2 Amino Acid Sequence
MPPTPATATGAAAAAVTPEHAARSFPRVVRVNPRSDRFPVLSFHHVELWCADAASAAGRFSFALGAPLAARSDLSTGNSAHASLLLRSGALAFLFTAPYAPPPQEAATAATTASIPSFSADAARTFAAAHGLAVRSVGVRVADAAEAFRVSVAGGARPAFAPADLGHGFGLAEVELYGDVVLRFVSYPDETDLPFLPGFERVSSPGAVDYGLTRFDHVVGNVPEMAPVIDYMKGFLGFHEFAEFTAEDVGTTESGLNSVVLANNSEAVLLPLNEPVHGTKRRSQIQTYLEYHGGPGVQHIALASNDVLRTLREMRARTPMGGFEFMAPPQAKYYEGVRRIAGDVLSEEQIKECQELGVLVDRDDQGVLLQIATKPVGDRPTFWLEMIQRIGCMEKDEVGQEYQKGGCGGFGKGNFSELFKSIEDYEKSLEVKQSVVAQKS

SEQ ID NO: 183 - DNA, 1323 bp, Artificial Sequence
  HPPDm-2-01 Nucleotide Sequence
atgccgcccacccccgccaccgccaccggcgccgccgcggccgccgtgactccagagcacgcggcccggagctttccccgagtggtccgcgtcaacccgcgcagcgaccgcttccccgtgctctccttccaccacgtcgagctctggtgcgccgacgccgcctcagcggccggacgcttctccttcgcgctcggcgcgccgctcgccgcccggtccgacctctccacggggaactccgcgcacgcctccctcctgctccgctcgggcgccctcgccttcctcttcacggcgccctacgcgccgccgccgcaggaggccgccacggccgcaaccaccgcctccatcccctccttctccgccgacgccgcgcggacgttcgccgccgcccacggcctcgcggtgcgctccgtcggggtccgcgtcgctgacgccgccgaggccttccgcgtcagcgtagccggcggcgctcgcccggccttcgccccagccgacctcggccatggcttcggcctcgccgaggtcgagctctacggcgacgtcgtgctacgcttcgtcagctacccggacgagacagacctgccattcctgccagggttcgagcgcgtgagcagccccggcgccgtggactacggcctcacgcggttcgaccacgtcgtgggcaacgtcccggagatggccccggtcatagactacatgaaaggcttcttggggttccacgagttcgccgagttcaccgccgaggacgtgggcacgaccgagagcgggctcaactcggtggtgctcgccaacaactccgaggccgtgctgctgccgctcaacgagcccgtgcacggcacaaagcgacggagccagatacagacgtacctggagtatcacggcgggcccggcgtgcagcacatcgcgctcgccagcaacgacgtgctcaggacgctcagggagatgcgggcgcgcacgcccatgggcggcttcgagttcatggcgccaccgcaggcgaaatactatgaaggcgtgcggcgcatcgcaggtgacgtgctctcggaagagcagatcaaggaatgccaggagctgggggtgctagtcgacagggatgatcaaggggtgttgctccaaatcgctaccaagccagtaggggacaggccaacgttttggctggagatgatccaaagaatcgggtgcatggagaaggacgaggtcgggcaagagtaccagaagggtggctgcggcgggtttggcaagggcaatttctccgagctgttcaagtccattgaggactatgagaaatcccttgaggtcaagcaatctgttgtagctcagaaatcctag

SEQ ID NO: 184 - DNA, 1323 bp, Artificial Sequence
  HPPDm-2-02 Nucleotide Sequence
atgccacctactccagctacagctactggtgctgctgctgctgccgttactcctgagcacgctgccaggtcattccccagggtggttcgcgtgaaccccagatctgataggttcccagttctgagcttccaccatgttgagctgtggtgcgctgatgctgcttctgctgctggcaggttctctttcgctcttggtgctccactcgctgctagatctgatctgtctacaggaaatagcgctcatgcctcactcctgcttcgctcaggtgctttggccttcctcttcaccgctccatatgctcccccacctcaggaggctgctactgctgctactacagcctccattccaagcttctcagctgatgccgctagaaccttcgctgctgctcatggacttgccgtgaggtctgttggtgttcgcgtggctgatgctgctgaggctttcagagtttccgttgccggcggagctaggccagctttcgctcctgctgatttgggacatggtttcggcctggctgaggttgagctttacggtgacgtggttctccgcttcgtgtcttacccagatgagactgacctgcctttccttcccggcttcgagagagtttcctctcctggtgccgtggattacggcctgacaaggttcgaccacgtggttggaaacgttcccgagatggctccagtgatcgattacatgaagggcttccttggattccatgagttcgccgagttcactgctgaggacgtgggaaccactgagtccggtttgaactctgtggttctcgccaacaattctgaggctgttttgctccctctgaatgagcctgtgcatggaaccaagaggagaagccagattcaaacttacctggagtaccacggtggccctggagttcagcatatcgcccttgcttctaatgatgtgttgcgcacactcagagagatgcgcgccagaacccccatgggaggtttcgagttcatggccccaccacaggctaagtactacgagggcgttagaaggattgctggagacgtgttgagcgaggagcagatcaaggagtgccaagagctgggtgttcttgtggatagggatgaccagggcgttctgcttcaaattgccactaagccagtgggcgaccgccctacattctggcttgagatgattcaaagaatcggctgcatggagaaggatgaggttggacaggagtaccaaaagggcggatgcggtggcttcggaaagggtaacttcagcgagttgttcaagtcaatcgaggactacgagaagagcctcgaggtgaagcagtcagtggttgcccaaaagtcctga

SEQ ID NO: 185 - protein, 440 aa, Artificial Sequence
  HPPDm-3 Amino Acid Sequence
MPPTPATATGAAAAAVTPEHAARSFPRVVRVNPRSDRFPVLSFHHVELWCADAASAAGRFSFALGAPLAARSDLSTGNSAHASLLLRSGALAFLFTAPYAPPPQEGATAAATASIPSFSADAARTFAAAHGLAVRSVGVRVADAAEAFRVSVAGGARPAFAPADLGHGFGLAEVELYGDVVLRFVSYPDETDLPFLPGFERVSSPGAVDYGLTRFDHVVGNVPEMAPVIDYMKGFLGFHEFAEFTAEDVGTTESGLNSVVLANNSEAVLLPLNEPVHGTKRRSQIQTYLEYHGGPGVQHIALASNDVLRTLREMRARTPMGGFEFMAPPQAKYYEGVRRIAGDVLSEEQIKECQELGVLVDRDDQGVLLQIATKPVGDRPTFWLEMIQRIGCMEKDEVGQEYQKGGCGGFGKGNFSELFKSIEDYEKSLEVKQSVVAQKS

SEQ ID NO: 186 - DNA, 1323 bp, Artificial Sequence
  HPPDm-3-01 Nucleotide Sequence
atgccgcccacccccgccaccgccaccggcgccgccgcggccgccgtgactccagagcacgcggcccggagctttccccgagtggtccgcgtcaacccgcgcagcgaccgcttccccgtgctctccttccaccacgtcgagctctggtgcgccgacgccgcctcagcggccggacgcttctccttcgcgctcggcgcgccgctcgccgcccggtccgacctctccacggggaactccgcgcacgcctccctcctgctccgctcgggcgccctcgccttcctcttcacggcgccctacgcgccgccgccgcaggagggtgccacggccgcagccaccgcctccatcccctccttctccgccgacgccgcgcggacgttcgccgccgcccacggcctcgcggtgcgctccgtcggggtccgcgtcgctgacgccgccgaggccttccgcgtcagcgtagccggcggcgctcgcccggccttcgccccagccgacctcggccatggcttcggcctcgccgaggtcgagctctacggcgacgtcgtgctacgcttcgtcagctacccggacgagacagacctgccattcctgccagggttcgagcgcgtgagcagccccggcgccgtggactacggcctcacgcggttcgaccacgtcgtgggcaacgtcccggagatggccccggtcatagactacatgaaaggcttcttggggttccacgagttcgccgagttcaccgccgaggacgtgggcacgaccgagagcgggctcaactcggtggtgctcgccaacaactccgaggccgtgctgctgccgctcaacgagcccgtgcacggcacaaagcgacggagccagatacagacgtacctggagtatcacggcgggcccggcgtgcagcacatcgcgctcgccagcaacgacgtgctcaggacgctcagggagatgcgggcgcgcacgcccatgggcggcttcgagttcatggcgccaccgcaggcgaaatactatgaaggcgtgcggcgcatcgcaggtgacgtgctctcggaagagcagatcaaggaatgccaggagctgggggtgctagtcgacagggatgatcaaggggtgttgctccaaatcgctaccaagccagtaggggacaggccaacgttttggctggagatgatccaaagaatcgggtgcatggagaaggacgaggtcgggcaagagtaccagaagggtggctgcggcgggtttggcaagggcaatttctccgagctgttcaagtccattgaggactatgagaaatcccttgaggtcaagcaatctgttgtagctcagaaatcctag

SEQ ID NO: 187 - DNA, 1323 bp, Artificial Sequence
  HPPDm-3-02 Nucleotide Sequence
atgccacctactccagctacagctactggtgctgctgctgctgccgttactcctgagcacgctgccaggtcattccccagggtggttcgcgtgaaccccagatctgataggttcccagttctgagcttccaccatgttgagctgtggtgcgctgatgctgcttctgctgctggcaggttctctttcgctcttggtgctccactcgctgctagatctgatctgtctacaggaaatagcgctcatgcctcactcctgcttcgctcaggtgctttggccttcctcttcaccgctccatatgctcccccacctcaggagggtgctactgctgctgctacagcctccattccaagcttctcagctgatgccgctagaaccttcgctgctgctcatggacttgccgtgaggtctgttggtgttcgcgtggctgatgctgctgaggctttcagagtttccgttgccggcggagctaggccagctttcgctcctgctgatttgggacatggtttcggcctggctgaggttgagctttacggtgacgtggttctccgcttcgtgtcttacccagatgagactgacctgcctttccttcccggcttcgagagagtttcctctcctggtgccgtggattacggcctgacaaggttcgaccacgtggttggaaacgttcccgagatggctccagtgatcgattacatgaagggcttccttggattccatgagttcgccgagttcactgctgaggacgtgggaaccactgagtccggtttgaactctgtggttctcgccaacaattctgaggctgttttgctccctctgaatgagcctgtgcatggaaccaagaggagaagccagattcaaacttacctggagtaccacggtggccctggagttcagcatatcgcccttgcttctaatgatgtgttgcgcacactcagagagatgcgcgccagaacccccatgggaggtttcgagttcatggccccaccacaggctaagtactacgagggcgttagaaggattgctggagacgtgttgagcgaggagcagatcaaggagtgccaagagctgggtgttcttgtggatagggatgaccagggcgttctgcttcaaattgccactaagccagtgggcgaccgccctacattctggcttgagatgattcaaagaatcggctgcatggagaaggatgaggttggacaggagtaccaaaagggcggatgcggtggcttcggaaagggtaacttcagcgagttgttcaagtcaatcgaggactacgagaagagcctcgaggtgaagcagtcagtggttgcccaaaagtcctga

SEQ ID NO: 188 - protein, 439 aa, Artificial Sequence
  HPPDm-4 Amino Acid Sequence
MPPTPATATGAAAAAVTPEHAARSFPRVVRVNPRSDRFPVLSFHHVELWCADAASAAGRFSFALGAPLAARSDLSTGNSAHASLLLRSGALAFLFTAPYAPPPQEATAAATASIPSFSADAARTFAAAHGLAVRSVGVRVADAAEAFRVSVAGGARPAFAPADLGHGFGLAEVELYGDVVLRFVSYPDETDLPFLPGFERVSSPGAVDYGLTRFDHVVGNVPEMAPVIDYMKGFLGFHEFAEFTAEDVGTTESGLNSVVLANNSEAVLLPLNEPVHGTKRRSQIQTYLEYHGGPGVQHIALASNDVLRTLREMRARTPMGGFEFMAPPQAKYYEGVRRIAGDVLSEEQINECQELGVLVDRDDQGVLLQIATKPVGDRPTFWLEMIQRIGCMEKDEVGQEYQKGGCGGFGKGNFSELFKSIEDYEKSLEVKQSVVAQKS

SEQ ID NO: 189 - DNA, 1320 bp, Artificial Sequence
  HPPDm-4-01 Nucleotide Sequence
atgccgcccacccccgccaccgccaccggcgccgccgcggccgccgtgactccagagcacgcggcccggagctttccccgagtggtccgcgtcaacccgcgcagcgaccgcttccccgtgctctccttccaccacgtcgagctctggtgcgccgacgccgcctcagcggccggacgcttctccttcgcgctcggcgcgccgctcgccgcccggtccgacctctccacggggaactccgcgcacgcctccctcctgctccgctcgggcgccctcgccttcctcttcacggcgccctacgcgccgccgccgcaggaggccacggccgcagccaccgcctccatcccctccttctccgccgacgccgcgcggacgttcgccgccgcccacggcctcgcggtgcgctccgtcggggtccgcgtcgctgacgccgccgaggccttccgcgtcagcgtagccggcggcgctcgcccggccttcgccccagccgacctcggccatggcttcggcctcgccgaggtcgagctctacggcgacgtcgtgctacgcttcgtcagctacccggacgagacagacctgccattcctgccagggttcgagcgcgtgagcagccccggcgccgtggactacggcctcacgcggttcgaccacgtcgtgggcaacgtcccggagatggccccggtcatagactacatgaaaggcttcttggggttccacgagttcgccgagttcaccgccgaggacgtgggcacgaccgagagcgggctcaactcggtggtgctcgccaacaactccgaggccgtgctgctgccgctcaacgagcccgtgcacggcacaaagcgacggagccagatacagacgtacctggagtatcacggcgggcccggcgtgcagcacatcgcgctcgccagcaacgacgtgctcaggacgctcagggagatgcgggcgcgcacgcccatgggcggcttcgagttcatggcgccaccgcaggcgaaatactatgaaggcgtgcggcgcatcgcaggtgacgtgctctcggaagagcagatcaatgaatgccaggagctgggggtgctagtcgacagggatgatcaaggggtgttgctccaaatcgctaccaagccagtaggggacaggccaacgttttggctggagatgatccaaagaatcgggtgcatggagaaggacgaggtcgggcaagagtaccagaagggtggctgcggcgggtttggcaagggcaatttctccgagctgttcaagtccattgaggactatgagaaatcccttgaggtcaagcaatctgttgtagctcagaaatcctag

SEQ ID NO: 190 - DNA, 1320 bp, Artificial Sequence
  HPPDm-4-02 Nucleotide Sequence
atgccacctactccagctacagctactggtgctgctgctgctgccgttactcctgagcacgctgccaggtcattccccagggtggttcgcgtgaaccccagatctgataggttcccagttctgagcttccaccatgttgagctgtggtgcgctgatgctgcttctgctgctggcaggttctctttcgctcttggtgctccactcgctgctagatctgatctgtctacaggaaatagcgctcatgcctcactcctgcttcgctcaggtgctttggccttcctcttcaccgctccatatgctcccccacctcaggaggctactgctgctgctacagcctccattccaagcttctcagctgatgccgctagaaccttcgctgctgctcatggacttgccgtgaggtctgttggtgttcgcgtggctgatgctgctgaggctttcagagtttccgttgccggcggagctaggccagctttcgctcctgctgatttgggacatggtttcggcctggctgaggttgagctttacggtgacgtggttctccgcttcgtgtcttacccagatgagactgacctgcctttccttcccggcttcgagagagtttcctctcctggtgccgtggattacggcctgacaaggttcgaccacgtggttggaaacgttcccgagatggctccagtgatcgattacatgaagggcttccttggattccatgagttcgccgagttcactgctgaggacgtgggaaccactgagtccggtttgaactctgtggttctcgccaacaattctgaggctgttttgctccctctgaatgagcctgtgcatggaaccaagaggagaagccagattcaaacttacctggagtaccacggtggccctggagttcagcatatcgcccttgcttctaatgatgtgttgcgcacactcagagagatgcgcgccagaacccccatgggaggtttcgagttcatggccccaccacaggctaagtactacgagggcgttagaaggattgctggagacgtgttgagcgaggagcagatcaatgagtgccaagagctgggtgttcttgtggatagggatgaccagggcgttctgcttcaaattgccactaagccagtgggcgaccgccctacattctggcttgagatgattcaaagaatcggctgcatggagaaggatgaggttggacaggagtaccaaaagggcggatgcggtggcttcggaaagggtaacttcagcgagttgttcaagtcaatcgaggactacgagaagagcctcgaggtgaagcagtcagtggttgcccaaaagtcctga

SEQ ID NO: 191 - protein, 440 aa, Artificial Sequence
  HPPDm-5 Amino Acid Sequence
MPPTPATATGAAAAAVTPEHAARSFPRVVRVNPRSDRFPVLSFHHVELWCADAASAAGRFSFALGAPLAARSDLSTGNSAHASLLLRSGALAFLFTAPYAPPPQEAATAATTASIPSFSADAARTFAAAHGLAVRSVGVRVADAAEAFRVSVAGGARPAFAPADLGHGFGLAEVELYGDVVLRFVSYPDETDLPFLPGFERVSSPGAVDYGLTRFDHVVGNVPEMAPVIDYMKGFLGFHEFAEFTAEDVGTTESGLNSVVLANNSEAVLLPLNEPVHGTKRRSQIQTYLEYHGGPGVQHIALASNDVLRTLREMRARTPMGGFEFMAPPQAKYYEGVRRIAGDVLSEEQINECQELGVLVDRDDQGVLLQIATKPVGDRPTFWLEMIQRIGCMEKDEVGQEYQKGGCGGFGKGNFSELFKSIEDYEKSLEVKQSVVAQKS

SEQ ID NO: 192 - DNA, 1323 bp, Artificial Sequence
  HPPDm-5-01 Nucleotide Sequence
atgccgcccacccccgccaccgccaccggcgccgccgcggccgccgtgactccagagcacgcggcccggagctttccccgagtggtccgcgtcaacccgcgcagcgaccgcttccccgtgctctccttccaccacgtcgagctctggtgcgccgacgccgcctcagcggccggacgcttctccttcgcgctcggcgcgccgctcgccgcccggtccgacctctccacggggaactccgcgcacgcctccctcctgctccgctcgggcgccctcgccttcctcttcacggcgccctacgcgccgccgccgcaggaggccgccacggccgcaaccaccgcctccatcccctccttctccgccgacgccgcgcggacgttcgccgccgcccacggcctcgcggtgcgctccgtcggggtccgcgtcgctgacgccgccgaggccttccgcgtcagcgtagccggcggcgctcgcccggccttcgccccagccgacctcggccatggcttcggcctcgccgaggtcgagctctacggcgacgtcgtgctacgcttcgtcagctacccggacgagacagacctgccattcctgccagggttcgagcgcgtgagcagccccggcgccgtggactacggcctcacgcggttcgaccacgtcgtgggcaacgtcccggagatggccccggtcatagactacatgaaaggcttcttggggttccacgagttcgccgagttcaccgccgaggacgtgggcacgaccgagagcgggctcaactcggtggtgctcgccaacaactccgaggccgtgctgctgccgctcaacgagcccgtgcacggcacaaagcgacggagccagatacagacgtacctggagtatcacggcgggcccggcgtgcagcacatcgcgctcgccagcaacgacgtgctcaggacgctcagggagatgcgggcgcgcacgcccatgggcggcttcgagttcatggcgccaccgcaggcgaaatactatgaaggcgtgcggcgcatcgcaggtgacgtgctctcggaagagcagatcaatgaatgccaggagctgggggtgctagtcgacagggatgatcaaggggtgttgctccaaatcgctaccaagccagtaggggacaggccaacgttttggctggagatgatccaaagaatcgggtgcatggagaaggacgaggtcgggcaagagtaccagaagggtggctgcggcgggtttggcaagggcaatttctccgagctgttcaagtccattgaggactatgagaaatcccttgaggtcaagcaatctgttgtagctcagaaatcctag

SEQ ID NO: 193 - DNA, 1323 bp, Artificial Sequence
  HPPDm-5-02 Nucleotide Sequence
atgccacctactccagctacagctactggtgctgctgctgctgccgttactcctgagcacgctgccaggtcattccccagggtggttcgcgtgaaccccagatctgataggttcccagttctgagcttccaccatgttgagctgtggtgcgctgatgctgcttctgctgctggcaggttctctttcgctcttggtgctccactcgctgctagatctgatctgtctacaggaaatagcgctcatgcctcactcctgcttcgctcaggtgctttggccttcctcttcaccgctccatatgctcccccacctcaggaggctgctactgctgctactacagcctccattccaagcttctcagctgatgccgctagaaccttcgctgctgctcatggacttgccgtgaggtctgttggtgttcgcgtggctgatgctgctgaggctttcagagtttccgttgccggcggagctaggccagctttcgctcctgctgatttgggacatggtttcggcctggctgaggttgagctttacggtgacgtggttctccgcttcgtgtcttacccagatgagactgacctgcctttccttcccggcttcgagagagtttcctctcctggtgccgtggattacggcctgacaaggttcgaccacgtggttggaaacgttcccgagatggctccagtgatcgattacatgaagggcttccttggattccatgagttcgccgagttcactgctgaggacgtgggaaccactgagtccggtttgaactctgtggttctcgccaacaattctgaggctgttttgctccctctgaatgagcctgtgcatggaaccaagaggagaagccagattcaaacttacctggagtaccacggtggccctggagttcagcatatcgcccttgcttctaatgatgtgttgcgcacactcagagagatgcgcgccagaacccccatgggaggtttcgagttcatggccccaccacaggctaagtactacgagggcgttagaaggattgctggagacgtgttgagcgaggagcagatcaatgagtgccaagagctgggtgttcttgtggatagggatgaccagggcgttctgcttcaaattgccactaagccagtgggcgaccgccctacattctggcttgagatgattcaaagaatcggctgcatggagaaggatgaggttggacaggagtaccaaaagggcggatgcggtggcttcggaaagggtaacttcagcgagttgttcaagtcaatcgaggactacgagaagagcctcgaggtgaagcagtcagtggttgcccaaaagtcctga

SEQ ID NO: 194 - protein, 440 aa, Artificial Sequence
  HPPDm-6 Amino Acid Sequence
MPPTPATATGAAAAAVTPEHAARSFPRVVRVNPRSDRFPVLSFHHVELWCADAASAAGRFSFALGAPLAARSDLSTGNSAHASLLLRSGALAFLFTAPYAPPPQEGATAAATASIPSFSADAARTFAAAHGLAVRSVGVRVADAAEAFRVSVAGGARPAFAPADLGHGFGLAEVELYGDVVLRFVSYPDETDLPFLPGFERVSSPGAVDYGLTRFDHVVGNVPEMAPVIDYMKGFLGFHEFAEFTAEDVGTTESGLNSVVLANNSEAVLLPLNEPVHGTKRRSQIQTYLEYHGGPGVQHIALASNDVLRTLREMRARTPMGGFEFMAPPQAKYYEGVRRIAGDVLSEEQINECQELGVLVDRDDQGVLLQIATKPVGDRPTFWLEMIQRIGCMEKDEVGQEYQKGGCGGFGKGNFSELFKSIEDYEKSLEVKQSVVAQKS

SEQ ID NO: 195 - DNA, 1323 bp, Artificial Sequence
  HPPDm-6-01 Nucleotide Sequence
atgccgcccacccccgccaccgccaccggcgccgccgcggccgccgtgactccagagcacgcggcccggagctttccccgagtggtccgcgtcaacccgcgcagcgaccgcttccccgtgctctccttccaccacgtcgagctctggtgcgccgacgccgcctcagcggccggacgcttctccttcgcgctcggcgcgccgctcgccgcccggtccgacctctccacggggaactccgcgcacgcctccctcctgctccgctcgggcgccctcgccttcctcttcacggcgccctacgcgccgccgccgcaggagggtgccacggccgcagccaccgcctccatcccctccttctccgccgacgccgcgcggacgttcgccgccgcccacggcctcgcggtgcgctccgtcggggtccgcgtcgctgacgccgccgaggccttccgcgtcagcgtagccggcggcgctcgcccggccttcgccccagccgacctcggccatggcttcggcctcgccgaggtcgagctctacggcgacgtcgtgctacgcttcgtcagctacccggacgagacagacctgccattcctgccagggttcgagcgcgtgagcagccccggcgccgtggactacggcctcacgcggttcgaccacgtcgtgggcaacgtcccggagatggccccggtcatagactacatgaaaggcttcttggggttccacgagttcgccgagttcaccgccgaggacgtgggcacgaccgagagcgggctcaactcggtggtgctcgccaacaactccgaggccgtgctgctgccgctcaacgagcccgtgcacggcacaaagcgacggagccagatacagacgtacctggagtatcacggcgggcccggcgtgcagcacatcgcgctcgccagcaacgacgtgctcaggacgctcagggagatgcgggcgcgcacgcccatgggcggcttcgagttcatggcgccaccgcaggcgaaatactatgaaggcgtgcggcgcatcgcaggtgacgtgctctcggaagagcagatcaatgaatgccaggagctgggggtgctagtcgacagggatgatcaaggggtgttgctccaaatcgctaccaagccagtaggggacaggccaacgttttggctggagatgatccaaagaatcgggtgcatggagaaggacgaggtcgggcaagagtaccagaagggtggctgcggcgggtttggcaagggcaatttctccgagctgttcaagtccattgaggactatgagaaatcccttgaggtcaagcaatctgttgtagctcagaaatcctag

SEQ ID NO: 196 - DNA, 1323 bp, Artificial Sequence
  HPPDm-6-02 Nucleotide Sequence
atgccacctactccagctacagctactggtgctgctgctgctgccgttactcctgagcacgctgccaggtcattccccagggtggttcgcgtgaaccccagatctgataggttcccagttctgagcttccaccatgttgagctgtggtgcgctgatgctgcttctgctgctggcaggttctctttcgctcttggtgctccactcgctgctagatctgatctgtctacaggaaatagcgctcatgcctcactcctgcttcgctcaggtgctttggccttcctcttcaccgctccatatgctcccccacctcaggagggtgctactgctgctgctacagcctccattccaagcttctcagctgatgccgctagaaccttcgctgctgctcatggacttgccgtgaggtctgttggtgttcgcgtggctgatgctgctgaggctttcagagtttccgttgccggcggagctaggccagctttcgctcctgctgatttgggacatggtttcggcctggctgaggttgagctttacggtgacgtggttctccgcttcgtgtcttacccagatgagactgacctgcctttccttcccggcttcgagagagtttcctctcctggtgccgtggattacggcctgacaaggttcgaccacgtggttggaaacgttcccgagatggctccagtgatcgattacatgaagggcttccttggattccatgagttcgccgagttcactgctgaggacgtgggaaccactgagtccggtttgaactctgtggttctcgccaacaattctgaggctgttttgctccctctgaatgagcctgtgcatggaaccaagaggagaagccagattcaaacttacctggagtaccacggtggccctggagttcagcatatcgcccttgcttctaatgatgtgttgcgcacactcagagagatgcgcgccagaacccccatgggaggtttcgagttcatggccccaccacaggctaagtactacgagggcgttagaaggattgctggagacgtgttgagcgaggagcagatcaatgagtgccaagagctgggtgttcttgtggatagggatgaccagggcgttctgcttcaaattgccactaagccagtgggcgaccgccctacattctggcttgagatgattcaaagaatcggctgcatggagaaggatgaggttggacaggagtaccaaaagggcggatgcggtggcttcggaaagggtaacttcagcgagttgttcaagtcaatcgaggactacgagaagagcctcgaggtgaagcagtcagtggttgcccaaaagtcctga

SEQ ID NO: 197 - protein, 435 aa, Artificial Sequence
  Amino Acid Sequence of HPPDm-7
MPPTPATATGAAAAAVTPEHAARSFPRVVRVNPRSDRFPVLSFHHVELWCADAASAAGRFSFALGAPLAARSDLSTGNSAHASLLLRSGALAFLFTAPYAPPPQEATAAATASIPSFSADAARTFAAAHGLAVRSVGVRVADAAEAFRVSVAGGARPAFAPADLGHGFGLAEVELYGDVVLRFVSYPDETDLPFLPGFERVSSPGAVDYGLTRFDHVVGNVPEMAPVIDYMKGFLGFHEFAEFTAEDVGTTESGLNSVVLANNSEAVLLPLNEPVHGTKRRSQIQTYLEYHGGPGVQHIALASNDVLRTLREMRARTPMGGFEFMAPPQAKYYEGVRRIAGDVLSEEQINECQELGVLVDRDDQGVLLQIATKPVGDRPTFWLEMIQRIGCMEKDEVGQEYQKGGCGGFGKGNFSELFKSIEEYEKTLEAKQLVG

SEQ ID NO: 198 - DNA, 1308 bp, Artificial Sequence
  HPPDm-7-01 Nucleotide Sequence
atgccgcccacccccgccaccgccaccggcgccgccgcggccgccgtgactccagagcacgcggcccggagctttccccgagtggtccgcgtcaacccgcgcagcgaccgcttccccgtgctctccttccaccacgtcgagctctggtgcgccgacgccgcctcagcggccggacgcttctccttcgcgctcggcgcgccgctcgccgcccggtccgacctctccacggggaactccgcgcacgcctccctcctgctccgctcgggcgccctcgccttcctcttcacggcgccctacgcgccgccgccgcaggaggccacggccgcagccaccgcctccatcccctccttctccgccgacgccgcgcggacgttcgccgccgcccacggcctcgcggtgcgctccgtcggggtccgcgtcgctgacgccgccgaggccttccgcgtcagcgtagccggcggcgctcgcccggccttcgccccagccgacctcggccatggcttcggcctcgccgaggtcgagctctacggcgacgtcgtgctacgcttcgtcagctacccggacgagacagacctgccattcctgccagggttcgagcgcgtgagcagccccggcgccgtggactacggcctcacgcggttcgaccacgtcgtgggcaacgtcccggagatggccccggtcatagactacatgaaaggcttcttggggttccacgagttcgccgagttcaccgccgaggacgtgggcacgaccgagagcgggctcaactcggtggtgctcgccaacaactccgaggccgtgctgctgccgctcaacgagcccgtgcacggcacaaagcgacggagccagatacagacgtacctggagtatcacggcgggcccggcgtgcagcacatcgcgctcgccagcaacgacgtgctcaggacgctcagggagatgcgggcgcgcacgcccatgggcggcttcgagttcatggcgccaccgcaggcgaaatactatgaaggcgtgcggcgcatcgcaggtgacgtgctctcggaagagcagatcaatgaatgccaggagctgggggtgctagtcgacagggatgatcaaggggtgttgctccaaatcgctaccaagccagtaggggacaggccaacgttttggctggagatgatccaaagaatcgggtgcatggagaaggacgaggtcgggcaagagtaccagaagggtggctgcggcgggtttggcaagggcaatttctccgagctgttcaagtccattgaggaatacgaaaagactcttgaagccaaacagttagtgggatga

SEQ ID NO: 199 - DNA, 1308 bp, Artificial Sequence
  HPPDm-7-02 Nucleotide Sequence
atgccacctactccagctacagctactggtgctgctgctgctgccgttactcctgagcacgctgccaggtcattccccagggtggttcgcgtgaaccccagatctgataggttcccagttctgagcttccaccatgttgagctgtggtgcgctgatgctgcttctgctgctggcaggttctctttcgctcttggtgctccactcgctgctagatctgatctgtctacaggaaatagcgctcatgcctcactcctgcttcgctcaggtgctttggccttcctcttcaccgctccatatgctcccccacctcaggaggctactgctgctgctacagcctccattccaagcttctcagctgatgccgctagaaccttcgctgctgctcatggacttgccgtgaggtctgttggtgttcgcgtggctgatgctgctgaggctttcagagtttccgttgccggcggagctaggccagctttcgctcctgctgatttgggacatggtttcggcctggctgaggttgagctttacggtgacgtggttctccgcttcgtgtcttacccagatgagactgacctgcctttccttcccggcttcgagagagtttcctctcctggtgccgtggattacggcctgacaaggttcgaccacgtggttggaaacgttcccgagatggctccagtgatcgattacatgaagggcttccttggattccatgagttcgccgagttcactgctgaggacgtgggaaccactgagtccggtttgaactctgtggttctcgccaacaattctgaggctgttttgctccctctgaatgagcctgtgcatggaaccaagaggagaagccagattcaaacttacctggagtaccacggtggccctggagttcagcatatcgcccttgcttctaatgatgtgttgcgcacactcagagagatgcgcgccagaacccccatgggaggtttcgagttcatggccccaccacaggctaagtactacgagggcgttagaaggattgctggagacgtgttgagcgaggagcagatcaatgagtgccaagagctgggtgttcttgtggatagggatgaccagggcgttctgcttcaaattgccactaagccagtgggcgaccgccctacattctggcttgagatgattcaaagaatcggctgcatggagaaggatgaggttggacaggagtaccaaaagggcggatgcggtggcttcggaaagggtaacttcagcgagttgttcaagtcaatcgaggagtatgagaagaccttggaggccaagcagctcgtgggttga

SEQ ID NO: 200 - protein, 436 aa, Artificial Sequence
  HPPDm-8 Amino Acid Sequence
MPPTPATATGAAAAAVTPEHAARSFPRVVRVNPRSDRFPVLSFHHVELWCADAASAAGRFSFALGAPLAARSDLSTGNSAHASLLLRSGALAFLFTAPYAPPPQEAATAATTASIPSFSADAARTFAAAHGLAVRSVGVRVADAAEAFRVSVAGGARPAFAPADLGHGFGLAEVELYGDVVLRFVSYPDETDLPFLPGFERVSSPGAVDYGLTRFDHVVGNVPEMAPVIDYMKGFLGFHEFAEFTAEDVGTTESGLNSVVLANNSEAVLLPLNEPVHGTKRRSQIQTYLEYHGGPGVQHIALASNDVLRTLREMRARTPMGGFEFMAPPQAKYYEGVRRIAGDVLSEEQINECQELGVLVDRDDQGVLLQIATKPVGDRPTFWLEMIQRIGCMEKDEVGQEYQKGGCGGFGKGNFSELFKSIEEYEKTLEAKQLVG

SEQ ID NO: 201 - DNA, 1311 bp, Artificial Sequence
  HPPDm-8-01 Nucleotide Sequence
atgccgcccacccccgccaccgccaccggcgccgccgcggccgccgtgactccagagcacgcggcccggagctttccccgagtggtccgcgtcaacccgcgcagcgaccgcttccccgtgctctccttccaccacgtcgagctctggtgcgccgacgccgcctcagcggccggacgcttctccttcgcgctcggcgcgccgctcgccgcccggtccgacctctccacggggaactccgcgcacgcctccctcctgctccgctcgggcgccctcgccttcctcttcacggcgccctacgcgccgccgccgcaggaggccgccacggccgcaaccaccgcctccatcccctccttctccgccgacgccgcgcggacgttcgccgccgcccacggcctcgcggtgcgctccgtcggggtccgcgtcgctgacgccgccgaggccttccgcgtcagcgtagccggcggcgctcgcccggccttcgccccagccgacctcggccatggcttcggcctcgccgaggtcgagctctacggcgacgtcgtgctacgcttcgtcagctacccggacgagacagacctgccattcctgccagggttcgagcgcgtgagcagccccggcgccgtggactacggcctcacgcggttcgaccacgtcgtgggcaacgtcccggagatggccccggtcatagactacatgaaaggcttcttggggttccacgagttcgccgagttcaccgccgaggacgtgggcacgaccgagagcgggctcaactcggtggtgctcgccaacaactccgaggccgtgctgctgccgctcaacgagcccgtgcacggcacaaagcgacggagccagatacagacgtacctggagtatcacggcgggcccggcgtgcagcacatcgcgctcgccagcaacgacgtgctcaggacgctcagggagatgcgggcgcgcacgcccatgggcggcttcgagttcatggcgccaccgcaggcgaaatactatgaaggcgtgcggcgcatcgcaggtgacgtgctctcggaagagcagatcaatgaatgccaggagctgggggtgctagtcgacagggatgatcaaggggtgttgctccaaatcgctaccaagccagtaggggacaggccaacgttttggctggagatgatccaaagaatcgggtgcatggagaaggacgaggtcgggcaagagtaccagaagggtggctgcggcgggtttggcaagggcaatttctccgagctgttcaagtccattgaggaatacgaaaagactcttgaagccaaacagttagtgggatga

SEQ ID NO: 202 - DNA, 1311 bp, Artificial Sequence
  HPPDm-8-02 Nucleotide Sequence
atgccacctactccagctacagctactggtgctgctgctgctgccgttactcctgagcacgctgccaggtcattccccagggtggttcgcgtgaaccccagatctgataggttcccagttctgagcttccaccatgttgagctgtggtgcgctgatgctgcttctgctgctggcaggttctctttcgctcttggtgctccactcgctgctagatctgatctgtctacaggaaatagcgctcatgcctcactcctgcttcgctcaggtgctttggccttcctcttcaccgctccatatgctcccccacctcaggaggctgctactgctgctactacagcctccattccaagcttctcagctgatgccgctagaaccttcgctgctgctcatggacttgccgtgaggtctgttggtgttcgcgtggctgatgctgctgaggctttcagagtttccgttgccggcggagctaggccagctttcgctcctgctgatttgggacatggtttcggcctggctgaggttgagctttacggtgacgtggttctccgcttcgtgtcttacccagatgagactgacctgcctttccttcccggcttcgagagagtttcctctcctggtgccgtggattacggcctgacaaggttcgaccacgtggttggaaacgttcccgagatggctccagtgatcgattacatgaagggcttccttggattccatgagttcgccgagttcactgctgaggacgtgggaaccactgagtccggtttgaactctgtggttctcgccaacaattctgaggctgttttgctccctctgaatgagcctgtgcatggaaccaagaggagaagccagattcaaacttacctggagtaccacggtggccctggagttcagcatatcgcccttgcttctaatgatgtgttgcgcacactcagagagatgcgcgccagaacccccatgggaggtttcgagttcatggccccaccacaggctaagtactacgagggcgttagaaggattgctggagacgtgttgagcgaggagcagatcaatgagtgccaagagctgggtgttcttgtggatagggatgaccagggcgttctgcttcaaattgccactaagccagtgggcgaccgccctacattctggcttgagatgattcaaagaatcggctgcatggagaaggatgaggttggacaggagtaccaaaagggcggatgcggtggcttcggaaagggtaacttcagcgagttgttcaagtcaatcgaggagtatgagaagaccttggaggccaagcagctcgtgggttga

SEQ ID NO: 203 - protein, 436 aa, Artificial Sequence
  HPPDm-9 Amino Acid Sequence
MPPTPATATGAAAAAVTPEHAARSFPRVVRVNPRSDRFPVLSFHHVELWCADAASAAGRFSFALGAPLAARSDLSTGNSAHASLLLRSGALAFLFTAPYAPPPQEGATAAATASIPSFSADAARTFAAAHGLAVRSVGVRVADAAEAFRVSVAGGARPAFAPADLGHGFGLAEVELYGDVVLRFVSYPDETDLPFLPGFERVSSPGAVDYGLTRFDHVVGNVPEMAPVIDYMKGFLGFHEFAEFTAEDVGTTESGLNSVVLANNSEAVLLPLNEPVHGTKRRSQIQTYLEYHGGPGVQHIALASNDVLRTLREMRARTPMGGFEFMAPPQAKYYEGVRRIAGDVLSEEQINECQELGVLVDRDDQGVLLQIATKPVGDRPTFWLEMIQRIGCMEKDEVGQEYQKGGCGGFGKGNFSELFKSIEEYEKTLEAKQLVG

SEQ ID NO: 204 - DNA, 1311 bp, Artificial Sequence
  HPPDm-9-01 Nucleotide Sequence
atgccgcccacccccgccaccgccaccggcgccgccgcggccgccgtgactccagagcacgcggcccggagctttccccgagtggtccgcgtcaacccgcgcagcgaccgcttccccgtgctctccttccaccacgtcgagctctggtgcgccgacgccgcctcagcggccggacgcttctccttcgcgctcggcgcgccgctcgccgcccggtccgacctctccacggggaactccgcgcacgcctccctcctgctccgctcgggcgccctcgccttcctcttcacggcgccctacgcgccgccgccgcaggagggtgccacggccgcagccaccgcctccatcccctccttctccgccgacgccgcgcggacgttcgccgccgcccacggcctcgcggtgcgctccgtcggggtccgcgtcgctgacgccgccgaggccttccgcgtcagcgtagccggcggcgctcgcccggccttcgccccagccgacctcggccatggcttcggcctcgccgaggtcgagctctacggcgacgtcgtgctacgcttcgtcagctacccggacgagacagacctgccattcctgccagggttcgagcgcgtgagcagccccggcgccgtggactacggcctcacgcggttcgaccacgtcgtgggcaacgtcccggagatggccccggtcatagactacatgaaaggcttcttggggttccacgagttcgccgagttcaccgccgaggacgtgggcacgaccgagagcgggctcaactcggtggtgctcgccaacaactccgaggccgtgctgctgccgctcaacgagcccgtgcacggcacaaagcgacggagccagatacagacgtacctggagtatcacggcgggcccggcgtgcagcacatcgcgctcgccagcaacgacgtgctcaggacgctcagggagatgcgggcgcgcacgcccatgggcggcttcgagttcatggcgccaccgcaggcgaaatactatgaaggcgtgcggcgcatcgcaggtgacgtgctctcggaagagcagatcaatgaatgccaggagctgggggtgctagtcgacagggatgatcaaggggtgttgctccaaatcgctaccaagccagtaggggacaggccaacgttttggctggagatgatccaaagaatcgggtgcatggagaaggacgaggtcgggcaagagtaccagaagggtggctgcggcgggtttggcaagggcaatttctccgagctgttcaagtccattgaggaatacgaaaagactcttgaagccaaacagttagtgggatga

SEQ ID NO: 205 - DNA, 1311 bp, Artificial Sequence
  HPPDm-9-02 Nucleotide Sequence
atgccacctactccagctacagctactggtgctgctgctgctgccgttactcctgagcacgctgccaggtcattccccagggtggttcgcgtgaaccccagatctgataggttcccagttctgagcttccaccatgttgagctgtggtgcgctgatgctgcttctgctgctggcaggttctctttcgctcttggtgctccactcgctgctagatctgatctgtctacaggaaatagcgctcatgcctcactcctgcttcgctcaggtgctttggccttcctcttcaccgctccatatgctcccccacctcaggagggtgctactgctgctgctacagcctccattccaagcttctcagctgatgccgctagaaccttcgctgctgctcatggacttgccgtgaggtctgttggtgttcgcgtggctgatgctgctgaggctttcagagtttccgttgccggcggagctaggccagctttcgctcctgctgatttgggacatggtttcggcctggctgaggttgagctttacggtgacgtggttctccgcttcgtgtcttacccagatgagactgacctgcctttccttcccggcttcgagagagtttcctctcctggtgccgtggattacggcctgacaaggttcgaccacgtggttggaaacgttcccgagatggctccagtgatcgattacatgaagggcttccttggattccatgagttcgccgagttcactgctgaggacgtgggaaccactgagtccggtttgaactctgtggttctcgccaacaattctgaggctgttttgctccctctgaatgagcctgtgcatggaaccaagaggagaagccagattcaaacttacctggagtaccacggtggccctggagttcagcatatcgcccttgcttctaatgatgtgttgcgcacactcagagagatgcgcgccagaacccccatgggaggtttcgagttcatggccccaccacaggctaagtactacgagggcgttagaaggattgctggagacgtgttgagcgaggagcagatcaatgagtgccaagagctgggtgttcttgtggatagggatgaccagggcgttctgcttcaaattgccactaagccagtgggcgaccgccctacattctggcttgagatgattcaaagaatcggctgcatggagaaggatgaggttggacaggagtaccaaaagggcggatgcggtggcttcggaaagggtaacttcagcgagttgttcaagtcaatcgaggagtatgagaagaccttggaggccaagcagctcgtgggttga

SEQ ID NO: 206 - protein, 440 aa, Artificial Sequence
  AsHPPDm-F415W Amino Acid Sequence
MPPTPATATGAAAAAVTPEHAARSFPRVVRVNPRSDRFPVLSFHHVELWCADAASAAGRFSFALGAPLAARSDLSTGNSAHASLLLRSGALAFLFTAPYAPPPQEAATAAATASIPSFSADAARTFAAAHGLAVRSVGVRVADAAEAFRVSVAGGARPAFAPADLGHGFGLAEVELYGDVVLRFVSYPDETDLPFLPGFERVSSPGAVDYGLTRFDHVVGNVPEMAPVIDYMKGFLGFHEFAEFTAEDVGTTESGLNSVVLANNSEAVLLPLNEPVHGTKRRSQIQTYLEYHGGPGVQHIALASNDVLRTLREMRARTPMGGFEFMAPPQAKYYEGVRRIAGDVLSEEQIKECQELGVLVDRDDQGVLLQIFTKPVGDRPTFFLEMIQRIGCMEKDEVGQEYQKGGCGGFGKGNWSELFKSIEDYEKSLEVKQSVVAQKS

SEQ ID NO: 207 - DNA, 1323 bp, Artificial Sequence
  AsHPPDm-F415W-01 Nucleotide Sequence
atgccgcccacccccgccaccgccaccggcgccgccgcggccgccgtgactccagagcacgcggcccggagctttccccgagtggtccgcgtcaacccgcgcagcgaccgcttccccgtgctctccttccaccacgtcgagctctggtgcgccgacgccgcctcagcggccggacgcttctccttcgcgctcggcgcgccgctcgccgcccggtccgacctctccacggggaactccgcgcacgcctccctcctgctccgctcgggcgccctcgccttcctcttcacggcgccctacgcgccgccgccgcaggaggccgccacggccgcagccaccgcctccatcccctccttctccgccgacgccgcgcggacgttcgccgccgcccacggcctcgcggtgcgctccgtcggggtccgcgtcgctgacgccgccgaggccttccgcgtcagcgtagccggcggcgctcgcccggccttcgccccagccgacctcggccatggcttcggcctcgccgaggtcgagctctacggcgacgtcgtgctacgcttcgtcagctacccggacgagacagacctgccattcctgccagggttcgagcgcgtgagcagccccggcgccgtggactacggcctcacgcggttcgaccacgtcgtgggcaacgtcccggagatggccccggtcatagactacatgaaaggcttcttggggttccacgagttcgccgagttcaccgccgaggacgtgggcacgaccgagagcgggctcaactcggtggtgctcgccaacaactccgaggccgtgctgctgccgctcaacgagcccgtgcacggcacaaagcgacggagccagatacagacgtacctggagtatcacggcgggcccggcgtgcagcacatcgcgctcgccagcaacgacgtgctcaggacgctcagggagatgcgggcgcgcacgcccatgggcggcttcgagttcatggcgccaccgcaggcgaaatactatgaaggcgtgcggcgcatcgcaggtgacgtgctctcggaagagcagatcaaggaatgccaggagctgggggtgctagtcgacagggatgatcaaggggtgttgctccaaatcttcaccaagccagtaggggacaggccaacgtttttcctggagatgatccaaagaatcgggtgcatggagaaggacgaggtcgggcaagagtaccagaagggtggctgcggcgggtttggcaagggcaattggtccgagctgttcaagtccattgaggactatgagaaatcccttgaggtcaagcaatctgttgtagctcagaaatcctag

SEQ ID NO: 208 - DNA, 1323 bp, Artificial Sequence
  AsHPPDm-F415W-02 Nucleotide Sequence
atgccacctactccagctacagctactggtgctgctgctgctgccgttactcctgagcacgctgccaggtcattccccagggtggttcgcgtgaaccccagatctgataggttcccagttctgagcttccaccatgttgagctgtggtgcgctgatgctgcttctgctgctggcaggttctctttcgctcttggtgctccactcgctgctagatctgatctgtctacaggaaatagcgctcatgcctcactcctgcttcgctcaggtgctttggccttcctcttcaccgctccatatgctcccccacctcaggaggctgctactgctgctgctacagcctccattccaagcttctcagctgatgccgctagaaccttcgctgctgctcatggacttgccgtgaggtctgttggtgttcgcgtggctgatgctgctgaggctttcagagtttccgttgccggcggagctaggccagctttcgctcctgctgatttgggacatggtttcggcctggctgaggttgagctttacggtgacgtggttctccgcttcgtgtcttacccagatgagactgacctgcctttccttcccggcttcgagagagtttcctctcctggtgccgtggattacggcctgacaaggttcgaccacgtggttggaaacgttcccgagatggctccagtgatcgattacatgaagggcttccttggattccatgagttcgccgagttcactgctgaggacgtgggaaccactgagtccggtttgaactctgtggttctcgccaacaattctgaggctgttttgctccctctgaatgagcctgtgcatggaaccaagaggagaagccagattcaaacttacctggagtaccacggtggccctggagttcagcatatcgcccttgcttctaatgatgtgttgcgcacactcagagagatgcgcgccagaacccccatgggaggtttcgagttcatggccccaccacaggctaagtactacgagggcgttagaaggattgctggagacgtgttgagcgaggagcagatcaaggagtgccaagagctgggtgttcttgtggatagggatgaccagggcgttctgcttcaaattttcactaagccagtgggcgaccgccctacattcttccttgagatgattcaaagaatcggctgcatggagaaggatgaggttggacaggagtaccaaaagggcggatgcggtggcttcggaaagggtaactggagcgagttgttcaagtcaatcgaggactacgagaagagcctcgaggtgaagcagtcagtggttgcccaaaagtcctga

SEQ ID NO: 209 - protein, 440 aa, Artificial Sequence
  AsHPPDm-F372A-F415W Amino Acid Sequence
MPPTPATATGAAAAAVTPEHAARSFPRVVRVNPRSDRFPVLSFHHVELWCADAASAAGRFSFALGAPLAARSDLSTGNSAHASLLLRSGALAFLFTAPYAPPPQEAATAAATASIPSFSADAARTFAAAHGLAVRSVGVRVADAAEAFRVSVAGGARPAFAPADLGHGFGLAEVELYGDVVLRFVSYPDETDLPFLPGFERVSSPGAVDYGLTRFDHVVGNVPEMAPVIDYMKGFLGFHEFAEFTAEDVGTTESGLNSVVLANNSEAVLLPLNEPVHGTKRRSQIQTYLEYHGGPGVQHIALASNDVLRTLREMRARTPMGGFEFMAPPQAKYYEGVRRIAGDVLSEEQIKECQELGVLVDRDDQGVLLQIATKPVGDRPTFFLEMIQRIGCMEKDEVGQEYQKGGCGGFGKGNWSELFKSIEDYEKSLEVKQSVVAQKS

SEQ ID NO: 210 - DNA, 1323 bp, Artificial Sequence
  AsHPPDm-F372A-F415W-01 Nucleotide Sequence
atgccgcccacccccgccaccgccaccggcgccgccgcggccgccgtgactccagagcacgcggcccggagctttccccgagtggtccgcgtcaacccgcgcagcgaccgcttccccgtgctctccttccaccacgtcgagctctggtgcgccgacgccgcctcagcggccggacgcttctccttcgcgctcggcgcgccgctcgccgcccggtccgacctctccacggggaactccgcgcacgcctccctcctgctccgctcgggcgccctcgccttcctcttcacggcgccctacgcgccgccgccgcaggaggccgccacggccgcagccaccgcctccatcccctccttctccgccgacgccgcgcggacgttcgccgccgcccacggcctcgcggtgcgctccgtcggggtccgcgtcgctgacgccgccgaggccttccgcgtcagcgtagccggcggcgctcgcccggccttcgccccagccgacctcggccatggcttcggcctcgccgaggtcgagctctacggcgacgtcgtgctacgcttcgtcagctacccggacgagacagacctgccattcctgccagggttcgagcgcgtgagcagccccggcgccgtggactacggcctcacgcggttcgaccacgtcgtgggcaacgtcccggagatggccccggtcatagactacatgaaaggcttcttggggttccacgagttcgccgagttcaccgccgaggacgtgggcacgaccgagagcgggctcaactcggtggtgctcgccaacaactccgaggccgtgctgctgccgctcaacgagcccgtgcacggcacaaagcgacggagccagatacagacgtacctggagtatcacggcgggcccggcgtgcagcacatcgcgctcgccagcaacgacgtgctcaggacgctcagggagatgcgggcgcgcacgcccatgggcggcttcgagttcatggcgccaccgcaggcgaaatactatgaaggcgtgcggcgcatcgcaggtgacgtgctctcggaagagcagatcaaggaatgccaggagctgggggtgctagtcgacagggatgatcaaggggtgttgctccaaatcgctaccaagccagtaggggacaggccaacgtttttcctggagatgatccaaagaatcgggtgcatggagaaggacgaggtcgggcaagagtaccagaagggtggctgcggcgggtttggcaagggcaattggtccgagctgttcaagtccattgaggactatgagaaatcccttgaggtcaagcaatctgttgtagctcagaaatcctag

SEQ ID NO: 211 - DNA, 1323 bp, Artificial Sequence
  AsHPPDm-F372A-F415W-02 Nucleotide Sequence
atgccacctactccagctacagctactggtgctgctgctgctgccgttactcctgagcacgctgccaggtcattccccagggtggttcgcgtgaaccccagatctgataggttcccagttctgagcttccaccatgttgagctgtggtgcgctgatgctgcttctgctgctggcaggttctctttcgctcttggtgctccactcgctgctagatctgatctgtctacaggaaatagcgctcatgcctcactcctgcttcgctcaggtgctttggccttcctcttcaccgctccatatgctcccccacctcaggaggctgctactgctgctgctacagcctccattccaagcttctcagctgatgccgctagaaccttcgctgctgctcatggacttgccgtgaggtctgttggtgttcgcgtggctgatgctgctgaggctttcagagtttccgttgccggcggagctaggccagctttcgctcctgctgatttgggacatggtttcggcctggctgaggttgagctttacggtgacgtggttctccgcttcgtgtcttacccagatgagactgacctgcctttccttcccggcttcgagagagtttcctctcctggtgccgtggattacggcctgacaaggttcgaccacgtggttggaaacgttcccgagatggctccagtgatcgattacatgaagggcttccttggattccatgagttcgccgagttcactgctgaggacgtgggaaccactgagtccggtttgaactctgtggttctcgccaacaattctgaggctgttttgctccctctgaatgagcctgtgcatggaaccaagaggagaagccagattcaaacttacctggagtaccacggtggccctggagttcagcatatcgcccttgcttctaatgatgtgttgcgcacactcagagagatgcgcgccagaacccccatgggaggtttcgagttcatggccccaccacaggctaagtactacgagggcgttagaaggattgctggagacgtgttgagcgaggagcagatcaaggagtgccaagagctgggtgttcttgtggatagggatgaccagggcgttctgcttcaaattgccactaagccagtgggcgaccgccctacattcttccttgagatgattcaaagaatcggctgcatggagaaggatgaggttggacaggagtaccaaaagggcggatgcggtggcttcggaaagggtaactggagcgagttgttcaagtcaatcgaggactacgagaagagcctcgaggtgaagcagtcagtggttgcccaaaagtcctga

SEQ ID NO: 212 - protein, 445 aa, Artificial Sequence
  AtHPPDm-F415W Amino Acid Sequence
MGHQNAAVSENQNHDDGAASSPGFKLVGFSKFVRKNPKSDKFKVKRFHHIEFWCGDATNVARRFSWGLGMRFSAKSDLSTGNMVHASYLLTSGDLRFLFTAPYSPSLSAGEIKPTTTASIPSFDHGSCRSFFSSHGLGVRAVAIEVEDAESAFSISVANGAIPSSPPIVLNEAVTIAEVKLYGDVVLRYVSYKAEDTEKSEFLPGFERVEDASSFPLDYGIRRLDHAVGNVPELGPALTYVAGFTGFHQFAEFTADDVGTAESGLNSAVLASNDEMVLLPINEPVHGTKRKSQIQTYLEHNEGAGLQHLALMSEDIFRTLREMRKRSSIGGFDFMPSPPPTYYQNLKKRVGDVLSDDQIKECEELGILVDRDDQGTLLQIFTKPLGDRPTIFIEIIQRVGCMMKDEEGKAYQSGGCGGFGKGNWSELFKSIEEYEKTLEAKQLVG

SEQ ID NO: 213 - DNA, 1338 bp, Artificial Sequence
  AtHPPDm-F415W-01 Nucleotide Sequence
atgggccaccaaaacgccgccgtttcagagaatcaaaaccatgatgacggcgctgcgtcgtcgccgggattcaagctcgtcggattttccaagttcgtaagaaagaatccaaagtctgataaattcaaggttaagcgcttccatcacatcgagttctggtgcggcgacgcaaccaacgtcgctcgtcgcttctcctggggtctggggatgagattctccgccaaatccgatctttccaccggaaacatggttcacgcctcttacctactcacctccggtgacctccgattccttttcactgctccttactctccgtctctctccgccggagagattaaaccgacaaccacagcttctatcccaagtttcgatcacggctcttgtcgttccttcttctcttcacatggtctcggtgttagagccgttgcgattgaagtagaagacgcagagtcagctttctccatcagtgtagctaatggcgctattccttcgtcgcctcctatcgtcctcaatgaagcagttacgatcgctgaggttaaactatacggcgatgttgttctccgatatgttagttacaaagcagaagataccgaaaaatccgaattcttgccagggttcgagcgtgtagaggatgcgtcgtcgttcccattggattatggtatccggcggcttgaccacgccgtgggaaacgttcctgagcttggtccggctttaacttatgtagcggggttcactggttttcaccaattcgcagagttcacagcagacgacgttggaaccgccgagagcggtttaaattcagcggtcctggctagcaatgatgaaatggttcttctaccgattaacgagccagtgcacggaacaaagaggaagagtcagattcagacgtatttggaacataacgaaggcgcagggctacaacatctggctctgatgagtgaagacatattcaggaccctgagagagatgaggaagaggagcagtattggaggattcgacttcatgccttctcctccgcctacttactaccagaatctcaagaaacgggtcggcgacgtgctcagcgatgatcagatcaaggagtgtgaggaattagggattcttgtagacagagatgatcaagggacgttgcttcaaatcttcacaaaaccactaggtgacaggccgacgatatttatagagataatccagagagtaggatgcatgatgaaagatgaggaagggaaggcttaccagagtggaggatgtggtggttttggcaaaggcaattggtctgagctcttcaagtccattgaagaatacgaaaagactcttgaagccaaacagttagtgggatga

SEQ ID NO: 214 - DNA, 1338 bp, Artificial Sequence
  AtHPPDm-F415W-02 Nucleotide Sequence
atgggacatcagaatgctgctgtatcagaaaatcaaaatcatgatgatggagccgcctcctcaccagggtttaagttggttgggttctccaagtttgtacggaagaacccaaaatccgacaagttcaaggttaaacgcttccaccacattgaattctggtgcggcgacgccaccaatgttgctcggcgtttttcatggggtttaggcatgagattctcagcaaagagtgacctgagcaccggcaacatggttcatgctagctatctcttaacatctggagatttgaggtttcttttcacggcgccgtactcaccatcactctccgccggcgagatcaaacccaccacgactgcaagcataccttcatttgatcatggtagttgcagatccttcttctcgtcgcacggcctaggggtgcgcgcggtcgccatcgaagttgaagatgcagaatcagcgtttagtatcagcgtggcaaatggagctattccttcctcccctccaattgtcctcaatgaggctgtaactattgccgaggtgaagttgtatggagatgttgtgctgagatatgtttcttacaaggcagaggacactgagaaatctgaatttttgcctggttttgaaagggtcgaggatgcttcaagttttcctcttgattacggcatacgacggttggatcacgcggttggaaatgtaccagaacttgggccggcgctcacttatgtggctggtttcactggattccatcaatttgctgagttcacagctgatgatgttgggactgctgaaagtgggttgaactctgcagtcctcgcctctaatgatgaaatggtgctcctcccgatcaacgagcctgtgcatggcaccaaaaggaaatcacaaatacagacatatcttgagcacaatgaaggtgcagggcttcaacatcttgcactgatgtctgaagacattttccgtacgctgagagagatgaggaagagaagtagtattggtggatttgacttcatgccttctcccccaccaacttactaccagaacttgaagaagagggttggtgatgtgctatctgatgaccagatcaaggagtgtgaagaattgggcattcttgttgatcgggacgaccaaggaacattactgcagatatttacaaaaccacttggtgaccgccccactatttttattgagatcatacaaagagtcggctgcatgatgaaggatgaggaaggaaaagcatatcaatctggtggttgtggcggctttgggaaaggaaactggtctgagctgttcaaatccatcgaggagtatgagaagaccttggaggccaagcagctcgtgggttga

SEQ ID NO: 215 - protein, 445 aa, Artificial Sequence
  AtHPPDm-F372A-F415W Amino Acid Sequence
MGHQNAAVSENQNHDDGAASSPGFKLVGFSKFVRKNPKSDKFKVKRFHHIEFWCGDATNVARRFSWGLGMRFSAKSDLSTGNMVHASYLLTSGDLRFLFTAPYSPSLSAGEIKPTTTASIPSFDHGSCRSFFSSHGLGVRAVAIEVEDAESAFSISVANGAIPSSPPIVLNEAVTIAEVKLYGDVVLRYVSYKAEDTEKSEFLPGFERVEDASSFPLDYGIRRLDHAVGNVPELGPALTYVAGFTGFHQFAEFTADDVGTAESGLNSAVLASNDEMVLLPINEPVHGTKRKSQIQTYLEHNEGAGLQHLALMSEDIFRTLREMRKRSSIGGFDFMPSPPPTYYQNLKKRVGDVLSDDQIKECEELGILVDRDDQGTLLQIATKPLGDRPTIFIEIIQRVGCMMKDEEGKAYQSGGCGGFGKGNWSELFKSIEEYEKTLEAKQLVG

SEQ ID NO: 216 - DNA, 1338 bp, Artificial Sequence
  AtHPPDm-F372A-F415W-01 Nucleotide Sequence
atgggccaccaaaacgccgccgtttcagagaatcaaaaccatgatgacggcgctgcgtcgtcgccgggattcaagctcgtcggattttccaagttcgtaagaaagaatccaaagtctgataaattcaaggttaagcgcttccatcacatcgagttctggtgcggcgacgcaaccaacgtcgctcgtcgcttctcctggggtctggggatgagattctccgccaaatccgatctttccaccggaaacatggttcacgcctcttacctactcacctccggtgacctccgattccttttcactgctccttactctccgtctctctccgccggagagattaaaccgacaaccacagcttctatcccaagtttcgatcacggctcttgtcgttccttcttctcttcacatggtctcggtgttagagccgttgcgattgaagtagaagacgcagagtcagctttctccatcagtgtagctaatggcgctattccttcgtcgcctcctatcgtcctcaatgaagcagttacgatcgctgaggttaaactatacggcgatgttgttctccgatatgttagttacaaagcagaagataccgaaaaatccgaattcttgccagggttcgagcgtgtagaggatgcgtcgtcgttcccattggattatggtatccggcggcttgaccacgccgtgggaaacgttcctgagcttggtccggctttaacttatgtagcggggttcactggttttcaccaattcgcagagttcacagcagacgacgttggaaccgccgagagcggtttaaattcagcggtcctggctagcaatgatgaaatggttcttctaccgattaacgagccagtgcacggaacaaagaggaagagtcagattcagacgtatttggaacataacgaaggcgcagggctacaacatctggctctgatgagtgaagacatattcaggaccctgagagagatgaggaagaggagcagtattggaggattcgacttcatgccttctcctccgcctacttactaccagaatctcaagaaacgggtcggcgacgtgctcagcgatgatcagatcaaggagtgtgaggaattagggattcttgtagacagagatgatcaagggacgttgcttcaaatcgctacaaaaccactaggtgacaggccgacgatatttatagagataatccagagagtaggatgcatgatgaaagatgaggaagggaaggcttaccagagtggaggatgtggtggttttggcaaaggcaattggtctgagctcttcaagtccattgaagaatacgaaaagactcttgaagccaaacagttagtgggatga

SEQ ID NO: 217 - DNA, 1338 bp, Artificial Sequence
  AtHPPDm-F372A-F415W-02 Nucleotide Sequence
atgggacatcagaatgctgctgtatcagaaaatcaaaatcatgatgatggagccgcctcctcaccagggtttaagttggttgggttctccaagtttgtacggaagaacccaaaatccgacaagttcaaggttaaacgcttccaccacattgaattctggtgcggcgacgccaccaatgttgctcggcgtttttcatggggtttaggcatgagattctcagcaaagagtgacctgagcaccggcaacatggttcatgctagctatctcttaacatctggagatttgaggtttcttttcacggcgccgtactcaccatcactctccgccggcgagatcaaacccaccacgactgcaagcataccttcatttgatcatggtagttgcagatccttcttctcgtcgcacggcctaggggtgcgcgcggtcgccatcgaagttgaagatgcagaatcagcgtttagtatcagcgtggcaaatggagctattccttcctcccctccaattgtcctcaatgaggctgtaactattgccgaggtgaagttgtatggagatgttgtgctgagatatgtttcttacaaggcagaggacactgagaaatctgaatttttgcctggttttgaaagggtcgaggatgcttcaagttttcctcttgattacggcatacgacggttggatcacgcggttggaaatgtaccagaacttgggccggcgctcacttatgtggctggtttcactggattccatcaatttgctgagttcacagctgatgatgttgggactgctgaaagtgggttgaactctgcagtcctcgcctctaatgatgaaatggtgctcctcccgatcaacgagcctgtgcatggcaccaaaaggaaatcacaaatacagacatatcttgagcacaatgaaggtgcagggcttcaacatcttgcactgatgtctgaagacattttccgtacgctgagagagatgaggaagagaagtagtattggtggatttgacttcatgccttctcccccaccaacttactaccagaacttgaagaagagggttggtgatgtgctatctgatgaccagatcaaggagtgtgaagaattgggcattcttgttgatcgggacgaccaaggaacattactgcagatagccacaaaaccacttggtgaccgccccactatttttattgagatcatacaaagagtcggctgcatgatgaaggatgaggaaggaaaagcatatcaatctggtggttgtggcggctttgggaaaggaaactggtctgagctgttcaaatccatcgaggagtatgagaagaccttggaggccaagcagctcgtgggttga

SEQ ID NO: 218 - protein, 440 aa, Artificial Sequence
  AsHPPDm-F383Y Amino Acid Sequence
MPPTPATATGAAAAAVTPEHAARSFPRVVRVNPRSDRFPVLSFHHVELWCADAASAAGRFSFALGAPLAARSDLSTGNSAHASLLLRSGALAFLFTAPYAPPPQEAATAAATASIPSFSADAARTFAAAHGLAVRSVGVRVADAAEAFRVSVAGGARPAFAPADLGHGFGLAEVELYGDVVLRFVSYPDETDLPFLPGFERVSSPGAVDYGLTRFDHVVGNVPEMAPVIDYMKGFLGFHEFAEFTAEDVGTTESGLNSVVLANNSEAVLLPLNEPVHGTKRRSQIQTYLEYHGGPGVQHIALASNDVLRTLREMRARTPMGGFEFMAPPQAKYYEGVRRIAGDVLSEEQIKECQELGVLVDRDDQGVLLQIFTKPVGDRPTFYLEMIQRIGCMEKDEVGQEYQKGGCGGFGKGNFSELFKSIEDYEKSLEVKQSVVAQKS

SEQ ID NO: 219 - DNA, 1323 bp, Artificial Sequence
  AsHPPDm-F383Y-01 Nucleotide Sequence
atgccgcccacccccgccaccgccaccggcgccgccgcggccgccgtgactccagagcacgcggcccggagctttccccgagtggtccgcgtcaacccgcgcagcgaccgcttccccgtgctctccttccaccacgtcgagctctggtgcgccgacgccgcctcagcggccggacgcttctccttcgcgctcggcgcgccgctcgccgcccggtccgacctctccacggggaactccgcgcacgcctccctcctgctccgctcgggcgccctcgccttcctcttcacggcgccctacgcgccgccgccgcaggaggccgccacggccgcagccaccgcctccatcccctccttctccgccgacgccgcgcggacgttcgccgccgcccacggcctcgcggtgcgctccgtcggggtccgcgtcgctgacgccgccgaggccttccgcgtcagcgtagccggcggcgctcgcccggccttcgccccagccgacctcggccatggcttcggcctcgccgaggtcgagctctacggcgacgtcgtgctacgcttcgtcagctacccggacgagacagacctgccattcctgccagggttcgagcgcgtgagcagccccggcgccgtggactacggcctcacgcggttcgaccacgtcgtgggcaacgtcccggagatggccccggtcatagactacatgaaaggcttcttggggttccacgagttcgccgagttcaccgccgaggacgtgggcacgaccgagagcgggctcaactcggtggtgctcgccaacaactccgaggccgtgctgctgccgctcaacgagcccgtgcacggcacaaagcgacggagccagatacagacgtacctggagtatcacggcgggcccggcgtgcagcacatcgcgctcgccagcaacgacgtgctcaggacgctcagggagatgcgggcgcgcacgcccatgggcggcttcgagttcatggcgccaccgcaggcgaaatactatgaaggcgtgcggcgcatcgcaggtgacgtgctctcggaagagcagatcaaggaatgccaggagctgggggtgctagtcgacagggatgatcaaggggtgttgctccaaatcttcaccaagccagtaggggacaggccaacgttttatctggagatgatccaaagaatcgggtgcatggagaaggacgaggtcgggcaagagtaccagaagggtggctgcggcgggtttggcaagggcaatttctccgagctgttcaagtccattgaggactatgagaaatcccttgaggtcaagcaatctgttgtagctcagaaatcctag

SEQ ID NO: 220 - DNA, 1323 bp, Artificial Sequence
  AsHPPDm-F383Y-02 Nucleotide Sequence
atgccacctactccagctacagctactggtgctgctgctgctgccgttactcctgagcacgctgccaggtcattccccagggtggttcgcgtgaaccccagatctgataggttcccagttctgagcttccaccatgttgagctgtggtgcgctgatgctgcttctgctgctggcaggttctctttcgctcttggtgctccactcgctgctagatctgatctgtctacaggaaatagcgctcatgcctcactcctgcttcgctcaggtgctttggccttcctcttcaccgctccatatgctcccccacctcaggaggctgctactgctgctgctacagcctccattccaagcttctcagctgatgccgctagaaccttcgctgctgctcatggacttgccgtgaggtctgttggtgttcgcgtggctgatgctgctgaggctttcagagtttccgttgccggcggagctaggccagctttcgctcctgctgatttgggacatggtttcggcctggctgaggttgagctttacggtgacgtggttctccgcttcgtgtcttacccagatgagactgacctgcctttccttcccggcttcgagagagtttcctctcctggtgccgtggattacggcctgacaaggttcgaccacgtggttggaaacgttcccgagatggctccagtgatcgattacatgaagggcttccttggattccatgagttcgccgagttcactgctgaggacgtgggaaccactgagtccggtttgaactctgtggttctcgccaacaattctgaggctgttttgctccctctgaatgagcctgtgcatggaaccaagaggagaagccagattcaaacttacctggagtaccacggtggccctggagttcagcatatcgcccttgcttctaatgatgtgttgcgcacactcagagagatgcgcgccagaacccccatgggaggtttcgagttcatggccccaccacaggctaagtactacgagggcgttagaaggattgctggagacgtgttgagcgaggagcagatcaaggagtgccaagagctgggtgttcttgtggatagggatgaccagggcgttctgcttcaaattttcactaagccagtgggcgaccgccctacattctatcttgagatgattcaaagaatcggctgcatggagaaggatgaggttggacaggagtaccaaaagggcggatgcggtggcttcggaaagggtaacttcagcgagttgttcaagtcaatcgaggactacgagaagagcctcgaggtgaagcagtcagtggttgcccaaaagtcctga

SEQ ID NO: 221 - protein, 440 aa, Artificial Sequence
  AsHPPDm-F372A-F383Y Amino Acid Sequence
MPPTPATATGAAAAAVTPEHAARSFPRVVRVNPRSDRFPVLSFHHVELWCADAASAAGRFSFALGAPLAARSDLSTGNSAHASLLLRSGALAFLFTAPYAPPPQEAATAAATASIPSFSADAARTFAAAHGLAVRSVGVRVADAAEAFRVSVAGGARPAFAPADLGHGFGLAEVELYGDVVLRFVSYPDETDLPFLPGFERVSSPGAVDYGLTRFDHVVGNVPEMAPVIDYMKGFLGFHEFAEFTAEDVGTTESGLNSVVLANNSEAVLLPLNEPVHGTKRRSQIQTYLEYHGGPGVQHIALASNDVLRTLREMRARTPMGGFEFMAPPQAKYYEGVRRIAGDVLSEEQIKECQELGVLVDRDDQGVLLQIATKPVGDRPTFYLEMIQRIGCMEKDEVGQEYQKGGCGGFGKGNFSELFKSIEDYEKSLEVKQSVVAQKS

SEQ ID NO: 222 - DNA, 1323 bp, Artificial Sequence
  AsHPPDm-F372A-F383Y-01 Nucleotide Sequence
atgccgcccacccccgccaccgccaccggcgccgccgcggccgccgtgactccagagcacgcggcccggagctttccccgagtggtccgcgtcaacccgcgcagcgaccgcttccccgtgctctccttccaccacgtcgagctctggtgcgccgacgccgcctcagcggccggacgcttctccttcgcgctcggcgcgccgctcgccgcccggtccgacctctccacggggaactccgcgcacgcctccctcctgctccgctcgggcgccctcgccttcctcttcacggcgccctacgcgccgccgccgcaggaggccgccacggccgcagccaccgcctccatcccctccttctccgccgacgccgcgcggacgttcgccgccgcccacggcctcgcggtgcgctccgtcggggtccgcgtcgctgacgccgccgaggccttccgcgtcagcgtagccggcggcgctcgcccggccttcgccccagccgacctcggccatggcttcggcctcgccgaggtcgagctctacggcgacgtcgtgctacgcttcgtcagctacccggacgagacagacctgccattcctgccagggttcgagcgcgtgagcagccccggcgccgtggactacggcctcacgcggttcgaccacgtcgtgggcaacgtcccggagatggccccggtcatagactacatgaaaggcttcttggggttccacgagttcgccgagttcaccgccgaggacgtgggcacgaccgagagcgggctcaactcggtggtgctcgccaacaactccgaggccgtgctgctgccgctcaacgagcccgtgcacggcacaaagcgacggagccagatacagacgtacctggagtatcacggcgggcccggcgtgcagcacatcgcgctcgccagcaacgacgtgctcaggacgctcagggagatgcgggcgcgcacgcccatgggcggcttcgagttcatggcgccaccgcaggcgaaatactatgaaggcgtgcggcgcatcgcaggtgacgtgctctcggaagagcagatcaaggaatgccaggagctgggggtgctagtcgacagggatgatcaaggggtgttgctccaaatcgctaccaagccagtaggggacaggccaacgttttatctggagatgatccaaagaatcgggtgcatggagaaggacgaggtcgggcaagagtaccagaagggtggctgcggcgggtttggcaagggcaatttctccgagctgttcaagtccattgaggactatgagaaatcccttgaggtcaagcaatctgttgtagctcagaaatcctag

SEQ ID NO: 223 - DNA, 1323 bp, Artificial Sequence
  AsHPPDm-F372A-F383Y-02 Nucleotide Sequence
atgccacctactccagctacagctactggtgctgctgctgctgccgttactcctgagcacgctgccaggtcattccccagggtggttcgcgtgaaccccagatctgataggttcccagttctgagcttccaccatgttgagctgtggtgcgctgatgctgcttctgctgctggcaggttctctttcgctcttggtgctccactcgctgctagatctgatctgtctacaggaaatagcgctcatgcctcactcctgcttcgctcaggtgctttggccttcctcttcaccgctccatatgctcccccacctcaggaggctgctactgctgctgctacagcctccattccaagcttctcagctgatgccgctagaaccttcgctgctgctcatggacttgccgtgaggtctgttggtgttcgcgtggctgatgctgctgaggctttcagagtttccgttgccggcggagctaggccagctttcgctcctgctgatttgggacatggtttcggcctggctgaggttgagctttacggtgacgtggttctccgcttcgtgtcttacccagatgagactgacctgcctttccttcccggcttcgagagagtttcctctcctggtgccgtggattacggcctgacaaggttcgaccacgtggttggaaacgttcccgagatggctccagtgatcgattacatgaagggcttccttggattccatgagttcgccgagttcactgctgaggacgtgggaaccactgagtccggtttgaactctgtggttctcgccaacaattctgaggctgttttgctccctctgaatgagcctgtgcatggaaccaagaggagaagccagattcaaacttacctggagtaccacggtggccctggagttcagcatatcgcccttgcttctaatgatgtgttgcgcacactcagagagatgcgcgccagaacccccatgggaggtttcgagttcatggccccaccacaggctaagtactacgagggcgttagaaggattgctggagacgtgttgagcgaggagcagatcaaggagtgccaagagctgggtgttcttgtggatagggatgaccagggcgttctgcttcaaattgccactaagccagtgggcgaccgccctacattctatcttgagatgattcaaagaatcggctgcatggagaaggatgaggttggacaggagtaccaaaagggcggatgcggtggcttcggaaagggtaacttcagcgagttgttcaagtcaatcgaggactacgagaagagcctcgaggtgaagcagtcagtggttgcccaaaagtcctga

SEQ ID NO: 224 - protein, 445 aa, Artificial Sequence
  AtHPPDm-F383Y Amino Acid Sequence
MGHQNAAVSENQNHDDGAASSPGFKLVGFSKFVRKNPKSDKFKVKRFHHIEFWCGDATNVARRFSWGLGMRFSAKSDLSTGNMVHASYLLTSGDLRFLFTAPYSPSLSAGEIKPTTTASIPSFDHGSCRSFFSSHGLGVRAVAIEVEDAESAFSISVANGAIPSSPPIVLNEAVTIAEVKLYGDVVLRYVSYKAEDTEKSEFLPGFERVEDASSFPLDYGIRRLDHAVGNVPELGPALTYVAGFTGFHQFAEFTADDVGTAESGLNSAVLASNDEMVLLPINEPVHGTKRKSQIQTYLEHNEGAGLQHLALMSEDIFRTLREMRKRSSIGGFDFMPSPPPTYYQNLKKRVGDVLSDDQIKECEELGILVDRDDQGTLLQIFTKPLGDRPTIYIEIIQRVGCMMKDEEGKAYQSGGCGGFGKGNFSELFKSIEEYEKTLEAKQLVG

SEQ ID NO: 225 - DNA, 1338 bp, Artificial Sequence
  AtHPPDm-F383Y-01 Nucleotide Sequence
atgggccaccaaaacgccgccgtttcagagaatcaaaaccatgatgacggcgctgcgtcgtcgccgggattcaagctcgtcggattttccaagttcgtaagaaagaatccaaagtctgataaattcaaggttaagcgcttccatcacatcgagttctggtgcggcgacgcaaccaacgtcgctcgtcgcttctcctggggtctggggatgagattctccgccaaatccgatctttccaccggaaacatggttcacgcctcttacctactcacctccggtgacctccgattccttttcactgctccttactctccgtctctctccgccggagagattaaaccgacaaccacagcttctatcccaagtttcgatcacggctcttgtcgttccttcttctcttcacatggtctcggtgttagagccgttgcgattgaagtagaagacgcagagtcagctttctccatcagtgtagctaatggcgctattccttcgtcgcctcctatcgtcctcaatgaagcagttacgatcgctgaggttaaactatacggcgatgttgttctccgatatgttagttacaaagcagaagataccgaaaaatccgaattcttgccagggttcgagcgtgtagaggatgcgtcgtcgttcccattggattatggtatccggcggcttgaccacgccgtgggaaacgttcctgagcttggtccggctttaacttatgtagcggggttcactggttttcaccaattcgcagagttcacagcagacgacgttggaaccgccgagagcggtttaaattcagcggtcctggctagcaatgatgaaatggttcttctaccgattaacgagccagtgcacggaacaaagaggaagagtcagattcagacgtatttggaacataacgaaggcgcagggctacaacatctggctctgatgagtgaagacatattcaggaccctgagagagatgaggaagaggagcagtattggaggattcgacttcatgccttctcctccgcctacttactaccagaatctcaagaaacgggtcggcgacgtgctcagcgatgatcagatcaaggagtgtgaggaattagggattcttgtagacagagatgatcaagggacgttgcttcaaatcttcacaaaaccactaggtgacaggccgacgatatatatagagataatccagagagtaggatgcatgatgaaagatgaggaagggaaggcttaccagagtggaggatgtggtggttttggcaaaggcaatttctctgagctcttcaagtccattgaagaatacgaaaagactcttgaagccaaacagttagtgggatga

SEQ ID NO: 226 - DNA, 1338 bp, Artificial Sequence
  AtHPPDm-F383Y-02 Nucleotide Sequence
atgggacatcagaatgctgctgtatcagaaaatcaaaatcatgatgatggagccgcctcctcaccagggtttaagttggttgggttctccaagtttgtacggaagaacccaaaatccgacaagttcaaggttaaacgcttccaccacattgaattctggtgcggcgacgccaccaatgttgctcggcgtttttcatggggtttaggcatgagattctcagcaaagagtgacctgagcaccggcaacatggttcatgctagctatctcttaacatctggagatttgaggtttcttttcacggcgccgtactcaccatcactctccgccggcgagatcaaacccaccacgactgcaagcataccttcatttgatcatggtagttgcagatccttcttctcgtcgcacggcctaggggtgcgcgcggtcgccatcgaagttgaagatgcagaatcagcgtttagtatcagcgtggcaaatggagctattccttcctcccctccaattgtcctcaatgaggctgtaactattgccgaggtgaagttgtatggagatgttgtgctgagatatgtttcttacaaggcagaggacactgagaaatctgaatttttgcctggttttgaaagggtcgaggatgcttcaagttttcctcttgattacggcatacgacggttggatcacgcggttggaaatgtaccagaacttgggccggcgctcacttatgtggctggtttcactggattccatcaatttgctgagttcacagctgatgatgttgggactgctgaaagtgggttgaactctgcagtcctcgcctctaatgatgaaatggtgctcctcccgatcaacgagcctgtgcatggcaccaaaaggaaatcacaaatacagacatatcttgagcacaatgaaggtgcagggcttcaacatcttgcactgatgtctgaagacattttccgtacgctgagagagatgaggaagagaagtagtattggtggatttgacttcatgccttctcccccaccaacttactaccagaacttgaagaagagggttggtgatgtgctatctgatgaccagatcaaggagtgtgaagaattgggcattcttgttgatcgggacgaccaaggaacattactgcagatatttacaaaaccacttggtgaccgccccactatttatattgagatcatacaaagagtcggctgcatgatgaaggatgaggaaggaaaagcatatcaatctggtggttgtggcggctttgggaaaggaaacttctctgagctgttcaaatccatcgaggagtatgagaagaccttggaggccaagcagctcgtgggttga

SEQ ID NO: 227 - protein, 445 aa, Artificial Sequence
  AtHPPDm-F372A-F383Y Amino Acid Sequence
MGHQNAAVSENQNHDDGAASSPGFKLVGFSKFVRKNPKSDKFKVKRFHHIEFWCGDATNVARRFSWGLGMRFSAKSDLSTGNMVHASYLLTSGDLRFLFTAPYSPSLSAGEIKPTTTASIPSFDHGSCRSFFSSHGLGVRAVAIEVEDAESAFSISVANGAIPSSPPIVLNEAVTIAEVKLYGDVVLRYVSYKAEDTEKSEFLPGFERVEDASSFPLDYGIRRLDHAVGNVPELGPALTYVAGFTGFHQFAEFTADDVGTAESGLNSAVLASNDEMVLLPINEPVHGTKRKSQIQTYLEHNEGAGLQHLALMSEDIFRTLREMRKRSSIGGFDFMPSPPPTYYQNLKKRVGDVLSDDQIKECEELGILVDRDDQGTLLQIATKPLGDRPTIYIEIIQRVGCMMKDEEGKAYQSGGCGGFGKGNFSELFKSIEEYEKTLEAKQLVG

SEQ ID NO: 228 - DNA, 1338 bp, Artificial Sequence
  AtHPPDm-F372A-F383Y-01 Nucleotide Sequence
atgggccaccaaaacgccgccgtttcagagaatcaaaaccatgatgacggcgctgcgtcgtcgccgggattcaagctcgtcggattttccaagttcgtaagaaagaatccaaagtctgataaattcaaggttaagcgcttccatcacatcgagttctggtgcggcgacgcaaccaacgtcgctcgtcgcttctcctggggtctggggatgagattctccgccaaatccgatctttccaccggaaacatggttcacgcctcttacctactcacctccggtgacctccgattccttttcactgctccttactctccgtctctctccgccggagagattaaaccgacaaccacagcttctatcccaagtttcgatcacggctcttgtcgttccttcttctcttcacatggtctcggtgttagagccgttgcgattgaagtagaagacgcagagtcagctttctccatcagtgtagctaatggcgctattccttcgtcgcctcctatcgtcctcaatgaagcagttacgatcgctgaggttaaactatacggcgatgttgttctccgatatgttagttacaaagcagaagataccgaaaaatccgaattcttgccagggttcgagcgtgtagaggatgcgtcgtcgttcccattggattatggtatccggcggcttgaccacgccgtgggaaacgttcctgagcttggtccggctttaacttatgtagcggggttcactggttttcaccaattcgcagagttcacagcagacgacgttggaaccgccgagagcggtttaaattcagcggtcctggctagcaatgatgaaatggttcttctaccgattaacgagccagtgcacggaacaaagaggaagagtcagattcagacgtatttggaacataacgaaggcgcagggctacaacatctggctctgatgagtgaagacatattcaggaccctgagagagatgaggaagaggagcagtattggaggattcgacttcatgccttctcctccgcctacttactaccagaatctcaagaaacgggtcggcgacgtgctcagcgatgatcagatcaaggagtgtgaggaattagggattcttgtagacagagatgatcaagggacgttgcttcaaatcgctacaaaaccactaggtgacaggccgacgatatatatagagataatccagagagtaggatgcatgatgaaagatgaggaagggaaggcttaccagagtggaggatgtggtggttttggcaaaggcaatttctctgagctcttcaagtccattgaagaatacgaaaagactcttgaagccaaacagttagtgggatga

SEQ ID NO: 229 - DNA, 1338 bp, Artificial Sequence
  AtHPPDm-F372A-F383Y-02 Nucleotide Sequence
atgggacatcagaatgctgctgtatcagaaaatcaaaatcatgatgatggagccgcctcctcaccagggtttaagttggttgggttctccaagtttgtacggaagaacccaaaatccgacaagttcaaggttaaacgcttccaccacattgaattctggtgcggcgacgccaccaatgttgctcggcgtttttcatggggtttaggcatgagattctcagcaaagagtgacctgagcaccggcaacatggttcatgctagctatctcttaacatctggagatttgaggtttcttttcacggcgccgtactcaccatcactctccgccggcgagatcaaacccaccacgactgcaagcataccttcatttgatcatggtagttgcagatccttcttctcgtcgcacggcctaggggtgcgcgcggtcgccatcgaagttgaagatgcagaatcagcgtttagtatcagcgtggcaaatggagctattccttcctcccctccaattgtcctcaatgaggctgtaactattgccgaggtgaagttgtatggagatgttgtgctgagatatgtttcttacaaggcagaggacactgagaaatctgaatttttgcctggttttgaaagggtcgaggatgcttcaagttttcctcttgattacggcatacgacggttggatcacgcggttggaaatgtaccagaacttgggccggcgctcacttatgtggctggtttcactggattccatcaatttgctgagttcacagctgatgatgttgggactgctgaaagtgggttgaactctgcagtcctcgcctctaatgatgaaatggtgctcctcccgatcaacgagcctgtgcatggcaccaaaaggaaatcacaaatacagacatatcttgagcacaatgaaggtgcagggcttcaacatcttgcactgatgtctgaagacattttccgtacgctgagagagatgaggaagagaagtagtattggtggatttgacttcatgccttctcccccaccaacttactaccagaacttgaagaagagggttggtgatgtgctatctgatgaccagatcaaggagtgtgaagaattgggcattcttgttgatcgggacgaccaaggaacattactgcagatagccacaaaaccacttggtgaccgccccactatttatattgagatcatacaaagagtcggctgcatgatgaaggatgaggaaggaaaagcatatcaatctggtggttgtggcggctttgggaaaggaaacttctctgagctgttcaaatccatcgaggagtatgagaagaccttggaggccaagcagctcgtgggttga

SEQ ID NO: 230 - DNA, 24 bp, Artificial Sequence
  5'end universal adapter primer 1
agtttttctgattaacagactagt

SEQ ID NO: 231 - DNA, 25 bp, Artificial Sequence
  3'end universal adapter primer 1
caaatgtttgaacgatcggcgcgcc

SEQ ID NO: 232 - DNA, 25 bp, Artificial Sequence
  primer 1
ctggaaggcgaggacgtcatcaata

SEQ ID NO: 233 - DNA, 22 bp, Artificial Sequence
  primer 2
tggcggcattgccgaaatcgag

SEQ ID NO: 234 - DNA, 28 bp, Artificial Sequence
  probe 1
atgcaggcgatgggcgcccgcatccgta